European Patent Application EP 4 686 414 A1, published February 4, 2026. Title: Method of improving gelation properties of alternative proteins. Applicant: KWS SAAT SE & Co. KGaA. Application EP. The sequence listing filed with the application follows.

SEQUENCE LISTING (123 sequences)

SEQ ID NO: 1 - DNA, 2746 bp, Pisum sativum
  source 1..2746: mol_type = genomic DNA
tatatggcacaatgtggccaaatgtctatccacgttattcatctagctttatgttctatcactataaatatccttcatcttactcttttatttcatcatctaaacttttaactagtgaaatacaaatcatggctaccactatcaaatcacgatttccacttttgttgttgctgggaattatattcctggcctctgttgtttgtgtcacttatgccaattacgatgaaggttcagaacctagggtaccggcacaaagagagagaggtcgccaagagggtgagaaagaggaaaaacgccatggagaatggagaccttcctacgaaaaggaagaagatgaagaagagggacaaagagaaagaggtcgccaagagggtgaaaaagaggaaaaacgccacggagaatggagaccttcgtatgaaaagcaagaagatgaagaagagaagcagaaatatagatatcaacgtgaaaaggaagatgaagaagagaagcagaaatatcaatatcaacgtgaaaagaaggaacaaaaggaagttcaacctggacgtgagagatgggaaagagaggaagatgaggaacaagtagacgaagagtggagaggaagtcaacgtcgtgaagatcccgaagaaagggcaaggctaaggcatagagaggagagaacaaaaagagacagacgccatcaacgtgaaggagaggaggaagaaagatcttcagagtcacaagaacgaagaaatccctttttatttaagtctaacaagtttctaacactctttgaaaacgaaaacggccacattcgtctccttcaaaggttcgacaaacgttcagacttatttgaaaatctccaaaactatcgtcttgtggaatatagagccaaaccccacaccatcttccttcctcaacacatagatgctgacttaatccttgtagtcctcagtggtaatttttattttactttataatattattataacaaatctttttgttttatagaaatatgactatttaaaataaaaacattgtaaagttcaatttaacaatatttcttatatttcataattaaattttggtttggttaatatgtattacagggaaagccatattgacagtgttgagtcccaatgatagaaattcgtataatcttgagcgtggtgataccatcaaacttcctgcaggaacaacctcttatttagttaaccaagatgatgaagaagatcttagactggtagatcttgtaatacccgtgaatgggcctggtaaatttgaggtactatataaaatacaataaatttttcttcagaagcgttattcttacaaaaacatccatttatattacttttacttttgtctataatgaaaaattgatattttccgttcttccatcaggcttttgacctagctaaaaataaaaaccaatacttacgaggattcagcaagaatattttagaggcctcctataacgtaagtatgtgaagtttttatcattttttaataaataaaaccattttaatttgtatcattgtttacaactatagactagatacgagaccatagagaaggttctcttagaagaacaagagaaagatcggaaaaggagacaacaaggggaagaaacagatgcaatagtcaaagtgtcaagggaacaaattgaggaattgaaaaagcttgccaaatcaagctcaaagaaaagcttaccctctgaatttgaaccaatcaacttgagaagccacaagccagaatattctaataagtttggcaagttgtttgagattactccggaaaaaaaataccctcaacttcaagatttagatctatttgttagttgtgtggagattaacgaggtaagtacacaacactaaatatatataaaacatataattttaattatattacagaaatatgttaatgcgtttttgcttatatttttagggagctctaatgttgccacactacaattcaagggctatagttgtactattggttaatgaaggaaaaggaaaccttgaacttctgggtttaaaaaatgagcaacaagagagggaagatagaaaagaaagaaacaatgaggtgcagagatatgaagctagattgtctccgggtgacgttgttatcattccagcaggtcatccggttgccattactgcttcttcaaatttgaatttgcttggatttggtatcaatgctgagaacaatgagagaaactttctttcaggtatttagtgaatattagtatgattacttaataagtctcggctaaatgagaattttttgaaattgatattttgattttggtgattgaaaatttgaaggctcggacgacaatgtgataagccaaattgaaaatccagtaaaagagcttacatttcctggatctgttcaagagataaatagactaataaagaaccaaaagcaatctcactttgcaaatgctgaacctgaacaaaaggagcaaggaagccagggaaaaaggagtcctctgtcttcaattttgggcactttttactaagtaatcagtatgaaaaataatacaacacgtatgtatgatgtaagtgttggataataaactatgaaaaataaggaggaaaatgtatgctgtaagatatagctagctcataatgagctaagaataaataaagggtcatgtaactcttgcttattgagtcccacctttctactatgaagaaataaataatgaataaaatttttgtctttttttaatttaaaagagtgtttgggcgctaaatttcttaac

SEQ ID NO: 2 - DNA, 2746 bp, Pisum sativum
  source 1..2746: mol_type = other DNA
tatatggcacaatataaccaaatgtctatccacgttattcatctagctttatgttctatcactataaatatccttcatcttactcttttatttcatcatctaaacttttaactagtgaaatataaatcatggctaccactatcaaatcatgatttccacttttgttgttgctgggaattatattcctggcctctgttgtttgtgtcacttatgccaattacgatgaaggttcagaacctagggtaccggcataaagagagagaggtcgctaagagggtgagaaagaggaaaaacgccatggagaataaagaccttcctacgaaaaggaagaagatgaagaagagggataaagagaaagaggtcgctaagagggtgaaaaagaggaaaaacgccacggagaataaagaccttcgtatgaaaagtaagaagatgaagaagagaagtagaaatatagatattaacgtgaaaaggaagatgaagaagagaagcagaaatattaatattaacgtgaaaagaaggaataaaaggaagtttaacctggacgtgagagataagaaagagaggaagatgaggaataagtagacgaagagtaaagaggaagttaacgtcgtgaagatcccgaagaaagggcaaggctaaggcatagagaggagagaacaaaaagagacagacgccattaacgtgaaggagaggaggaagaaagatcttcagagtcataagaatgaagaaatccctttttatttaagtctaacaagtttctaacactctttgaaaacgaaaacggccacattcgtctcctttaaaggttcgacaaacgttcagacttatttgaaaatctctaaaactatcgtcttgtggaatatagagccaaaccccacaccatcttccttccttaacacatagatgctgacttaatccttgtagtcctcagtgataatttttattttactttataatattattataacaaatctttttgttttatagaaatatgactatttaaaataaaaacattgtaaagttcaatttaacaatatttcttatatttcataattaaattttggtttggttaatatgtattacaaggaaagccatattgacagtgttgagtcccaatgatagaaattcgtataatcttgagcgtggtgataccatcaaacttcctgcaggaacaacctcttatttagttaactaagatgatgaagaagatcttagactggtagatcttgtaatacccgtgaatgggcctggtaaatttgagatactatataaaatacaataaatttttcttcagaagcgttattcttacaaaaacatccatttatattacttttacttttgtctataatgaaaaattgatattttccgttcttccatcaagcttttgacctagctaaaaataaaaactaatacttatgaggattcagcaagaatattttagaggcctcctataacataagtatgtgaagtttttatcattttttaataaataaaaccattttaatttgtatcattgtttacaactataaactagatacgagaccatagagaaggttctcttagaagaataagagaaagatcggaaaaggagataataaggggaagaaacagatgcaatagtcaaagtgtcaagggaataaattgaggaattgaaaaagcttgccaaatcaagctcaaagaaaagcttaccctctgaatttgaaccaatcaacttgagaagccacaagccagaatattctaataagtttggcaagttgtttgagattactccggaaaaaaaatacccttaactttaagatttagatctatttgttagttgtgtggagattaacgagataagtacacaacactaaatatatataaaacatataattttaattatattacagaaatatgttaatgcgtttttgcttatatttttaaggagctctaatgttgccacactacaattcaagggctatagttgtactattggttaatgaaggaaaaggaaaccttgaacttctgggtttaaaaaatgagtaataagagagggaagatagaaaagaaagaaacaatgaggtgtagagatatgaagctagattgtctccgggtgacgttgttatcattccagcaggtcatccggttgccattactgcttcttcaaatttgaatttgcttggatttggtatcaatgctgagaacaatgagagaaactttctttcagatatttagtgaatattagtatgattacttaataagtctcggctaaatgagaattttttgaaattgatattttgattttggtgattgaaaatttgaaagctcggacgacaatgtgataagctaaattgaaaatccagtaaaagagcttacatttcctggatctgtttaagagataaatagactaataaagaactaaaagtaatctcactttgcaaatgctgaacctgaataaaaggagtaaggaagctagggaaaaaggagtcctctgtcttcaattttgggcactttttactaagtaatcagtatgaaaaataatacaacacgtatgtatgatgtaagtgttggataataaactatgaaaaataaggaggaaaatgtatgctgtaagatatagctagctcataatgagctaagaataaataaagggtcatgtaactcttgcttattgagtcccacctttctactatgaagaaataaataatgaataaaatttttgtctttttttaatttaaaagagtgtttgggcgctaaatttcttaac

SEQ ID NO: 3 - DNA, 2746 bp, synthetic construct
  source 1..2746: mol_type = other DNA
tatatggcacaatgtaaccaaatgtctatccacgttattcatctagctttatgttctatcactataaatatccttcatcttactcttttatttcatcatctaaacttttaactagtgaaatataaatcatggctaccactatcaaatcatgatttccacttttgttgttgctgggaattatattcctggcctctgttgtttgtgtcacttatgccaattacgatgaaggttcagaacctagggtaccggcataaagagagagaggtcgctaagagggtgagaaagaggaaaaacgccatggagaataaagaccttcctacgaaaaggaagaagatgaagaagagggataaagagaaagaggtcgctaagagggtgaaaaagaggaaaaacgccacggagaataaagaccttcgtatgaaaagtaagaagatgaagaagagaagtagaaatatagatattaacgtgaaaaggaagatgaagaagagaagcagaaatattaatattaacgtgaaaagaaggaataaaaggaagtttaacctggacgtgagagataagaaagagaggaagatgaggaataagtagacgaagagtaaagaggaagttaacgtcgtgaagatcccgaagaaagggcaaggctaaggcatagagaggagagaacaaaaagagacagacgccattaacgtgaaggagaggaggaagaaagatcttcagagtcataagaatgaagaaatccctttttatttaagtctaacaagtttctaacactctttgaaaacgaaaacggccacattcgtctcctttaaaggttcgacaaacgttcagacttatttgaaaatctctaaaactatcgtcttgtggaatatagagccaaaccccacaccatcttccttccttaacacatagatgctgacttaatccttgtagtcctcagtgataatttttattttactttataatattattataacaaatctttttgttttatagaaatatgactatttaaaataaaaacattgtaaagttcaatttaacaatatttcttatatttcataattaaattttggtttggttaatatgtattacaaggaaagccatattgacagtgttgagtcccaatgatagaaattcgtataatcttgagcgtggtgataccatcaaacttcctgcaggaacaacctcttatttagttaactaagatgatgaagaagatcttagactggtagatcttgtaatacccgtgaatgggcctggtaaatttgagatactatataaaatacaataaatttttcttcagaagcgttattcttacaaaaacatccatttatattacttttacttttgtctataatgaaaaattgatattttccgttcttccatcaagcttttgacctagctaaaaataaaaactaatacttatgaggattcagcaagaatattttagaggcctcctataacataagtatgtgaagtttttatcattttttaataaataaaaccattttaatttgtatcattgtttacaactataaactagatacgagaccatagagaaggttctcttagaagaataagagaaagatcggaaaaggagataataaggggaagaaacagatgcaatagtcaaagtgtcaagggaataaattgaggaattgaaaaagcttgccaaatcaagctcaaagaaaagcttaccctctgaatttgaaccaatcaacttgagaagccacaagccagaatattctaataagtttggcaagttgtttgagattactccggaaaaaaaatacccttaactttaagatttagatctatttgttagttgtgtggagattaacgagataagtacacaacactaaatatatataaaacatataattttaattatattacagaaatatgttaatgcgtttttgcttatatttttaaggagctctaatgttgccacactacaattcaagggctatagttgtactattggttaatgaaggaaaaggaaaccttgaacttctgggtttaaaaaatgagtaataagagagggaagatagaaaagaaagaaacaatgaggtgtagagatatgaagctagattgtctccgggtgacgttgttatcattccagcaggtcatccggttgccattactgcttcttcaaatttgaatttgcttggatttggtatcaatgctgagaacaatgagagaaactttctttcagatatttagtgaatattagtatgattacttaataagtctcggctaaatgagaattttttgaaattgatattttgattttggtgattgaaaatttgaaagctcggacgacaatgtgataagctaaattgaaaatccagtaaaagagcttacatttcctggatctgtttaagagataaatagactaataaagaactaaaagtaatctcactttgcaaatgctgaacctgaataaaaggagtaaggaagctagggaaaaaggagtcctctgtcttcaattttgggcactttttactaagtaatcagtatgaaaaataatacaacacgtatgtatgatgtaagtgttggataataaactatgaaaaataaggaggaaaatgtatgctgtaagatatagctagctcataatgagctaagaataaataaagggtcatgtaactcttgcttattgagtcccacctttctactatgaagaaataaataatgaataaaatttttgtctttttttaatttaaaagagtgtttgggcgctaaatttcttaac

SEQ ID NO: 4 - DNA, 2746 bp, synthetic construct
  source 1..2746: mol_type = other DNA
tatatggcacaatatgaccaaatgtctatccacgttattcatctagctttatgttctatcactataaatatccttcatcttactcttttatttcatcatctaaacttttaactagtgaaatataaatcatggctaccactatcaaatcatgatttccacttttgttgttgctgggaattatattcctggcctctgttgtttgtgtcacttatgccaattacgatgaaggttcagaacctagggtaccggcataaagagagagaggtcgctaagagggtgagaaagaggaaaaacgccatggagaataaagaccttcctacgaaaaggaagaagatgaagaagagggataaagagaaagaggtcgctaagagggtgaaaaagaggaaaaacgccacggagaataaagaccttcgtatgaaaagtaagaagatgaagaagagaagtagaaatatagatattaacgtgaaaaggaagatgaagaagagaagcagaaatattaatattaacgtgaaaagaaggaataaaaggaagtttaacctggacgtgagagataagaaagagaggaagatgaggaataagtagacgaagagtaaagaggaagttaacgtcgtgaagatcccgaagaaagggcaaggctaaggcatagagaggagagaacaaaaagagacagacgccattaacgtgaaggagaggaggaagaaagatcttcagagtcataagaatgaagaaatccctttttatttaagtctaacaagtttctaacactctttgaaaacgaaaacggccacattcgtctcctttaaaggttcgacaaacgttcagacttatttgaaaatctctaaaactatcgtcttgtggaatatagagccaaaccccacaccatcttccttccttaacacatagatgctgacttaatccttgtagtcctcagtgataatttttattttactttataatattattataacaaatctttttgttttatagaaatatgactatttaaaataaaaacattgtaaagttcaatttaacaatatttcttatatttcataattaaattttggtttggttaatatgtattacaaggaaagccatattgacagtgttgagtcccaatgatagaaattcgtataatcttgagcgtggtgataccatcaaacttcctgcaggaacaacctcttatttagttaactaagatgatgaagaagatcttagactggtagatcttgtaatacccgtgaatgggcctggtaaatttgagatactatataaaatacaataaatttttcttcagaagcgttattcttacaaaaacatccatttatattacttttacttttgtctataatgaaaaattgatattttccgttcttccatcaagcttttgacctagctaaaaataaaaactaatacttatgaggattcagcaagaatattttagaggcctcctataacataagtatgtgaagtttttatcattttttaataaataaaaccattttaatttgtatcattgtttacaactataaactagatacgagaccatagagaaggttctcttagaagaataagagaaagatcggaaaaggagataataaggggaagaaacagatgcaatagtcaaagtgtcaagggaataaattgaggaattgaaaaagcttgccaaatcaagctcaaagaaaagcttaccctctgaatttgaaccaatcaacttgagaagccacaagccagaatattctaataagtttggcaagttgtttgagattactccggaaaaaaaatacccttaactttaagatttagatctatttgttagttgtgtggagattaacgagataagtacacaacactaaatatatataaaacatataattttaattatattacagaaatatgttaatgcgtttttgcttatatttttaaggagctctaatgttgccacactacaattcaagggctatagttgtactattggttaatgaaggaaaaggaaaccttgaacttctgggtttaaaaaatgagtaataagagagggaagatagaaaagaaagaaacaatgaggtgtagagatatgaagctagattgtctccgggtgacgttgttatcattccagcaggtcatccggttgccattactgcttcttcaaatttgaatttgcttggatttggtatcaatgctgagaacaatgagagaaactttctttcagatatttagtgaatattagtatgattacttaataagtctcggctaaatgagaattttttgaaattgatattttgattttggtgattgaaaatttgaaagctcggacgacaatgtgataagctaaattgaaaatccagtaaaagagcttacatttcctggatctgtttaagagataaatagactaataaagaactaaaagtaatctcactttgcaaatgctgaacctgaataaaaggagtaaggaagctagggaaaaaggagtcctctgtcttcaattttgggcactttttactaagtaatcagtatgaaaaataatacaacacgtatgtatgatgtaagtgttggataataaactatgaaaaataaggaggaaaatgtatgctgtaagatatagctagctcataatgagctaagaataaataaagggtcatgtaactcttgcttattgagtcccacctttctactatgaagaaataaataatgaataaaatttttgtctttttttaatttaaaagagtgtttgggcgctaaatttcttaac

SEQ ID NO: 5 - DNA, 2746 bp, synthetic construct
  source 1..2746: mol_type = other DNA
tatatggcacaatatagccaaatgtctatccacgttattcatctagctttatgttctatcactataaatatccttcatcttactcttttatttcatcatctaaacttttaactagtgaaatataaatcatggctaccactatcaaatcatgatttccacttttgttgttgctgggaattatattcctggcctctgttgtttgtgtcacttatgccaattacgatgaaggttcagaacctagggtaccggcataaagagagagaggtcgctaagagggtgagaaagaggaaaaacgccatggagaataaagaccttcctacgaaaaggaagaagatgaagaagagggataaagagaaagaggtcgctaagagggtgaaaaagaggaaaaacgccacggagaataaagaccttcgtatgaaaagtaagaagatgaagaagagaagtagaaatatagatattaacgtgaaaaggaagatgaagaagagaagcagaaatattaatattaacgtgaaaagaaggaataaaaggaagtttaacctggacgtgagagataagaaagagaggaagatgaggaataagtagacgaagagtaaagaggaagttaacgtcgtgaagatcccgaagaaagggcaaggctaaggcatagagaggagagaacaaaaagagacagacgccattaacgtgaaggagaggaggaagaaagatcttcagagtcataagaatgaagaaatccctttttatttaagtctaacaagtttctaacactctttgaaaacgaaaacggccacattcgtctcctttaaaggttcgacaaacgttcagacttatttgaaaatctctaaaactatcgtcttgtggaatatagagccaaaccccacaccatcttccttccttaacacatagatgctgacttaatccttgtagtcctcagtgataatttttattttactttataatattattataacaaatctttttgttttatagaaatatgactatttaaaataaaaacattgtaaagttcaatttaacaatatttcttatatttcataattaaattttggtttggttaatatgtattacaaggaaagccatattgacagtgttgagtcccaatgatagaaattcgtataatcttgagcgtggtgataccatcaaacttcctgcaggaacaacctcttatttagttaactaagatgatgaagaagatcttagactggtagatcttgtaatacccgtgaatgggcctggtaaatttgagatactatataaaatacaataaatttttcttcagaagcgttattcttacaaaaacatccatttatattacttttacttttgtctataatgaaaaattgatattttccgttcttccatcaagcttttgacctagctaaaaataaaaactaatacttatgaggattcagcaagaatattttagaggcctcctataacataagtatgtgaagtttttatcattttttaataaataaaaccattttaatttgtatcattgtttacaactataaactagatacgagaccatagagaaggttctcttagaagaataagagaaagatcggaaaaggagataataaggggaagaaacagatgcaatagtcaaagtgtcaagggaataaattgaggaattgaaaaagcttgccaaatcaagctcaaagaaaagcttaccctctgaatttgaaccaatcaacttgagaagccacaagccagaatattctaataagtttggcaagttgtttgagattactccggaaaaaaaatacccttaactttaagatttagatctatttgttagttgtgtggagattaacgagataagtacacaacactaaatatatataaaacatataattttaattatattacagaaatatgttaatgcgtttttgcttatatttttaaggagctctaatgttgccacactacaattcaagggctatagttgtactattggttaatgaaggaaaaggaaaccttgaacttctgggtttaaaaaatgagtaataagagagggaagatagaaaagaaagaaacaatgaggtgtagagatatgaagctagattgtctccgggtgacgttgttatcattccagcaggtcatccggttgccattactgcttcttcaaatttgaatttgcttggatttggtatcaatgctgagaacaatgagagaaactttctttcagatatttagtgaatattagtatgattacttaataagtctcggctaaatgagaattttttgaaattgatattttgattttggtgattgaaaatttgaaagctcggacgacaatgtgataagctaaattgaaaatccagtaaaagagcttacatttcctggatctgtttaagagataaatagactaataaagaactaaaagtaatctcactttgcaaatgctgaacctgaataaaaggagtaaggaagctagggaaaaaggagtcctctgtcttcaattttgggcactttttactaagtaatcagtatgaaaaataatacaacacgtatgtatgatgtaagtgttggataataaactatgaaaaataaggaggaaaatgtatgctgtaagatatagctagctcataatgagctaagaataaataaagggtcatgtaactcttgcttattgagtcccacctttctactatgaagaaataaataatgaataaaatttttgtctttttttaatttaaaagagtgtttgggcgctaaatttcttaac

SEQ ID NO: 6 - DNA, 2746 bp, synthetic construct
  source 1..2746: mol_type = other DNA
tatatggcacaatataaccaaatgtctatccacgttattcatctagctttatgttctatcactataaatatccttcatcttactcttttatttcatcatctaaacttttaactagtgaaatacaaatcatggctaccactatcaaatcatgatttccacttttgttgttgctgggaattatattcctggcctctgttgtttgtgtcacttatgccaattacgatgaaggttcagaacctagggtaccggcataaagagagagaggtcgctaagagggtgagaaagaggaaaaacgccatggagaataaagaccttcctacgaaaaggaagaagatgaagaagagggataaagagaaagaggtcgctaagagggtgaaaaagaggaaaaacgccacggagaataaagaccttcgtatgaaaagtaagaagatgaagaagagaagtagaaatatagatattaacgtgaaaaggaagatgaagaagagaagcagaaatattaatattaacgtgaaaagaaggaataaaaggaagtttaacctggacgtgagagataagaaagagaggaagatgaggaataagtagacgaagagtaaagaggaagttaacgtcgtgaagatcccgaagaaagggcaaggctaaggcatagagaggagagaacaaaaagagacagacgccattaacgtgaaggagaggaggaagaaagatcttcagagtcataagaatgaagaaatccctttttatttaagtctaacaagtttctaacactctttgaaaacgaaaacggccacattcgtctcctttaaaggttcgacaaacgttcagacttatttgaaaatctctaaaactatcgtcttgtggaatatagagccaaaccccacaccatcttccttccttaacacatagatgctgacttaatccttgtagtcctcagtgataatttttattttactttataatattattataacaaatctttttgttttatagaaatatgactatttaaaataaaaacattgtaaagttcaatttaacaatatttcttatatttcataattaaattttggtttggttaatatgtattacaaggaaagccatattgacagtgttgagtcccaatgatagaaattcgtataatcttgagcgtggtgataccatcaaacttcctgcaggaacaacctcttatttagttaactaagatgatgaagaagatcttagactggtagatcttgtaatacccgtgaatgggcctggtaaatttgagatactatataaaatacaataaatttttcttcagaagcgttattcttacaaaaacatccatttatattacttttacttttgtctataatgaaaaattgatattttccgttcttccatcaagcttttgacctagctaaaaataaaaactaatacttatgaggattcagcaagaatattttagaggcctcctataacataagtatgtgaagtttttatcattttttaataaataaaaccattttaatttgtatcattgtttacaactataaactagatacgagaccatagagaaggttctcttagaagaataagagaaagatcggaaaaggagataataaggggaagaaacagatgcaatagtcaaagtgtcaagggaataaattgaggaattgaaaaagcttgccaaatcaagctcaaagaaaagcttaccctctgaatttgaaccaatcaacttgagaagccacaagccagaatattctaataagtttggcaagttgtttgagattactccggaaaaaaaatacccttaactttaagatttagatctatttgttagttgtgtggagattaacgagataagtacacaacactaaatatatataaaacatataattttaattatattacagaaatatgttaatgcgtttttgcttatatttttaaggagctctaatgttgccacactacaattcaagggctatagttgtactattggttaatgaaggaaaaggaaaccttgaacttctgggtttaaaaaatgagtaataagagagggaagatagaaaagaaagaaacaatgaggtgtagagatatgaagctagattgtctccgggtgacgttgttatcattccagcaggtcatccggttgccattactgcttcttcaaatttgaatttgcttggatttggtatcaatgctgagaacaatgagagaaactttctttcagatatttagtgaatattagtatgattacttaataagtctcggctaaatgagaattttttgaaattgatattttgattttggtgattgaaaatttgaaagctcggacgacaatgtgataagctaaattgaaaatccagtaaaagagcttacatttcctggatctgtttaagagataaatagactaataaagaactaaaagtaatctcactttgcaaatgctgaacctgaataaaaggagtaaggaagctagggaaaaaggagtcctctgtcttcaattttgggcactttttactaagtaatcagtatgaaaaataatacaacacgtatgtatgatgtaagtgttggataataaactatgaaaaataaggaggaaaatgtatgctgtaagatatagctagctcataatgagctaagaataaataaagggtcatgtaactcttgcttattgagtcccacctttctactatgaagaaataaataatgaataaaatttttgtctttttttaatttaaaagagtgtttgggcgctaaatttcttaac

SEQ ID NO: 7 - DNA, 2746 bp, synthetic construct
  source 1..2746: mol_type = other DNA
tatatggcacaatataaccaaatgtctatccacgttattcatctagctttatgttctatcactataaatatccttcatcttactcttttatttcatcatctaaacttttaactagtgaaatataaatcatggctaccactatcaaatcacgatttccacttttgttgttgctgggaattatattcctggcctctgttgtttgtgtcacttatgccaattacgatgaaggttcagaacctagggtaccggcataaagagagagaggtcgctaagagggtgagaaagaggaaaaacgccatggagaataaagaccttcctacgaaaaggaagaagatgaagaagagggataaagagaaagaggtcgctaagagggtgaaaaagaggaaaaacgccacggagaataaagaccttcgtatgaaaagtaagaagatgaagaagagaagtagaaatatagatattaacgtgaaaaggaagatgaagaagagaagcagaaatattaatattaacgtgaaaagaaggaataaaaggaagtttaacctggacgtgagagataagaaagagaggaagatgaggaataagtagacgaagagtaaagaggaagttaacgtcgtgaagatcccgaagaaagggcaaggctaaggcatagagaggagagaacaaaaagagacagacgccattaacgtgaaggagaggaggaagaaagatcttcagagtcataagaatgaagaaatccctttttatttaagtctaacaagtttctaacactctttgaaaacgaaaacggccacattcgtctcctttaaaggttcgacaaacgttcagacttatttgaaaatctctaaaactatcgtcttgtggaatatagagccaaaccccacaccatcttccttccttaacacatagatgctgacttaatccttgtagtcctcagtgataatttttattttactttataatattattataacaaatctttttgttttatagaaatatgactatttaaaataaaaacattgtaaagttcaatttaacaatatttcttatatttcataattaaattttggtttggttaatatgtattacaaggaaagccatattgacagtgttgagtcccaatgatagaaattcgtataatcttgagcgtggtgataccatcaaacttcctgcaggaacaacctcttatttagttaactaagatgatgaagaagatcttagactggtagatcttgtaatacccgtgaatgggcctggtaaatttgagatactatataaaatacaataaatttttcttcagaagcgttattcttacaaaaacatccatttatattacttttacttttgtctataatgaaaaattgatattttccgttcttccatcaagcttttgacctagctaaaaataaaaactaatacttatgaggattcagcaagaatattttagaggcctcctataacataagtatgtgaagtttttatcattttttaataaataaaaccattttaatttgtatcattgtttacaactataaactagatacgagaccatagagaaggttctcttagaagaataagagaaagatcggaaaaggagataataaggggaagaaacagatgcaatagtcaaagtgtcaagggaataaattgaggaattgaaaaagcttgccaaatcaagctcaaagaaaagcttaccctctgaatttgaaccaatcaacttgagaagccacaagccagaatattctaataagtttggcaagttgtttgagattactccggaaaaaaaatacccttaactttaagatttagatctatttgttagttgtgtggagattaacgagataagtacacaacactaaatatatataaaacatataattttaattatattacagaaatatgttaatgcgtttttgcttatatttttaaggagctctaatgttgccacactacaattcaagggctatagttgtactattggttaatgaaggaaaaggaaaccttgaacttctgggtttaaaaaatgagtaataagagagggaagatagaaaagaaagaaacaatgaggtgtagagatatgaagctagattgtctccgggtgacgttgttatcattccagcaggtcatccggttgccattactgcttcttcaaatttgaatttgcttggatttggtatcaatgctgagaacaatgagagaaactttctttcagatatttagtgaatattagtatgattacttaataagtctcggctaaatgagaattttttgaaattgatattttgattttggtgattgaaaatttgaaagctcggacgacaatgtgataagctaaattgaaaatccagtaaaagagcttacatttcctggatctgtttaagagataaatagactaataaagaactaaaagtaatctcactttgcaaatgctgaacctgaataaaaggagtaaggaagctagggaaaaaggagtcctctgtcttcaattttgggcactttttactaagtaatcagtatgaaaaataatacaacacgtatgtatgatgtaagtgttggataataaactatgaaaaataaggaggaaaatgtatgctgtaagatatagctagctcataatgagctaagaataaataaagggtcatgtaactcttgcttattgagtcccacctttctactatgaagaaataaataatgaataaaatttttgtctttttttaatttaaaagagtgtttgggcgctaaatttcttaac

SEQ ID NO: 8 - DNA, 2746 bp, synthetic construct
  source 1..2746: mol_type = other DNA
tatatggcacaatataaccaaatgtctatccacgttattcatctagctttatgttctatcactataaatatccttcatcttactcttttatttcatcatctaaacttttaactagtgaaatataaatcatggctaccactatcaaatcatgatttccacttttgttgttgctgggaattatattcctggcctctgttgtttgtgtcacttatgccaattacgatgaaggttcagaacctagggtaccggcacaaagagagagaggtcgctaagagggtgagaaagaggaaaaacgccatggagaataaagaccttcctacgaaaaggaagaagatgaagaagagggataaagagaaagaggtcgctaagagggtgaaaaagaggaaaaacgccacggagaataaagaccttcgtatgaaaagtaagaagatgaagaagagaagtagaaatatagatattaacgtgaaaaggaagatgaagaagagaagcagaaatattaatattaacgtgaaaagaaggaataaaaggaagtttaacctggacgtgagagataagaaagagaggaagatgaggaataagtagacgaagagtaaagaggaagttaacgtcgtgaagatcccgaagaaagggcaaggctaaggcatagagaggagagaacaaaaagagacagacgccattaacgtgaaggagaggaggaagaaagatcttcagagtcataagaatgaagaaatccctttttatttaagtctaacaagtttctaacactctttgaaaacgaaaacggccacattcgtctcctttaaaggttcgacaaacgttcagacttatttgaaaatctctaaaactatcgtcttgtggaatatagagccaaaccccacaccatcttccttccttaacacatagatgctgacttaatccttgtagtcctcagtgataatttttattttactttataatattattataacaaatctttttgttttatagaaatatgactatttaaaataaaaacattgtaaagttcaatttaacaatatttcttatatttcataattaaattttggtttggttaatatgtattacaaggaaagccatattgacagtgttgagtcccaatgatagaaattcgtataatcttgagcgtggtgataccatcaaacttcctgcaggaacaacctcttatttagttaactaagatgatgaagaagatcttagactggtagatcttgtaatacccgtgaatgggcctggtaaatttgagatactatataaaatacaataaatttttcttcagaagcgttattcttacaaaaacatccatttatattacttttacttttgtctataatgaaaaattgatattttccgttcttccatcaagcttttgacctagctaaaaataaaaactaatacttatgaggattcagcaagaatattttagaggcctcctataacataagtatgtgaagtttttatcattttttaataaataaaaccattttaatttgtatcattgtttacaactataaactagatacgagaccatagagaaggttctcttagaagaataagagaaagatcggaaaaggagataataaggggaagaaacagatgcaatagtcaaagtgtcaagggaataaattgaggaattgaaaaagcttgccaaatcaagctcaaagaaaagcttaccctctgaatttgaaccaatcaacttgagaagccacaagccagaatattctaataagtttggcaagttgtttgagattactccggaaaaaaaatacccttaactttaagatttagatctatttgttagttgtgtggagattaacgagataagtacacaacactaaatatatataaaacatataattttaattatattacagaaatatgttaatgcgtttttgcttatatttttaaggagctctaatgttgccacactacaattcaagggctatagttgtactattggttaatgaaggaaaaggaaaccttgaacttctgggtttaaaaaatgagtaataagagagggaagatagaaaagaaagaaacaatgaggtgtagagatatgaagctagattgtctccgggtgacgttgttatcattccagcaggtcatccggttgccattactgcttcttcaaatttgaatttgcttggatttggtatcaatgctgagaacaatgagagaaactttctttcagatatttagtgaatattagtatgattacttaataagtctcggctaaatgagaattttttgaaattgatattttgattttggtgattgaaaatttgaaagctcggacgacaatgtgataagctaaattgaaaatccagtaaaagagcttacatttcctggatctgtttaagagataaatagactaataaagaactaaaagtaatctcactttgcaaatgctgaacctgaataaaaggagtaaggaagctagggaaaaaggagtcctctgtcttcaattttgggcactttttactaagtaatcagtatgaaaaataatacaacacgtatgtatgatgtaagtgttggataataaactatgaaaaataaggaggaaaatgtatgctgtaagatatagctagctcataatgagctaagaataaataaagggtcatgtaactcttgcttattgagtcccacctttctactatgaagaaataaataatgaataaaatttttgtctttttttaatttaaaagagtgtttgggcgctaaatttcttaac

SEQ ID NO: 9 - DNA, 2746 bp, synthetic construct
  source 1..2746: mol_type = other DNA
tatatggcacaatataaccaaatgtctatccacgttattcatctagctttatgttctatcactataaatatccttcatcttactcttttatttcatcatctaaacttttaactagtgaaatataaatcatggctaccactatcaaatcatgatttccacttttgttgttgctgggaattatattcctggcctctgttgtttgtgtcacttatgccaattacgatgaaggttcagaacctagggtaccggcataaagagagagaggtcgccaagagggtgagaaagaggaaaaacgccatggagaataaagaccttcctacgaaaaggaagaagatgaagaagagggataaagagaaagaggtcgctaagagggtgaaaaagaggaaaaacgccacggagaataaagaccttcgtatgaaaagtaagaagatgaagaagagaagtagaaatatagatattaacgtgaaaaggaagatgaagaagagaagcagaaatattaatattaacgtgaaaagaaggaataaaaggaagtttaacctggacgtgagagataagaaagagaggaagatgaggaataagtagacgaagagtaaagaggaagttaacgtcgtgaagatcccgaagaaagggcaaggctaaggcatagagaggagagaacaaaaagagacagacgccattaacgtgaaggagaggaggaagaaagatcttcagagtcataagaatgaagaaatccctttttatttaagtctaacaagtttctaacactctttgaaaacgaaaacggccacattcgtctcctttaaaggttcgacaaacgttcagacttatttgaaaatctctaaaactatcgtcttgtggaatatagagccaaaccccacaccatcttccttccttaacacatagatgctgacttaatccttgtagtcctcagtgataatttttattttactttataatattattataacaaatctttttgttttatagaaatatgactatttaaaataaaaacattgtaaagttcaatttaacaatatttcttatatttcataattaaattttggtttggttaatatgtattacaaggaaagccatattgacagtgttgagtcccaatgatagaaattcgtataatcttgagcgtggtgataccatcaaacttcctgcaggaacaacctcttatttagttaactaagatgatgaagaagatcttagactggtagatcttgtaatacccgtgaatgggcctggtaaatttgagatactatataaaatacaataaatttttcttcagaagcgttattcttacaaaaacatccatttatattacttttacttttgtctataatgaaaaattgatattttccgttcttccatcaagcttttgacctagctaaaaataaaaactaatacttatgaggattcagcaagaatattttagaggcctcctataacataagtatgtgaagtttttatcattttttaataaataaaaccattttaatttgtatcattgtttacaactataaactagatacgagaccatagagaaggttctcttagaagaataagagaaagatcggaaaaggagataataaggggaagaaacagatgcaatagtcaaagtgtcaagggaataaattgaggaattgaaaaagcttgccaaatcaagctcaaagaaaagcttaccctctgaatttgaaccaatcaacttgagaagccacaagccagaatattctaataagtttggcaagttgtttgagattactccggaaaaaaaatacccttaactttaagatttagatctatttgttagttgtgtggagattaacgagataagtacacaacactaaatatatataaaacatataattttaattatattacagaaatatgttaatgcgtttttgcttatatttttaaggagctctaatgttgccacactacaattcaagggctatagttgtactattggttaatgaaggaaaaggaaaccttgaacttctgggtttaaaaaatgagtaataagagagggaagatagaaaagaaagaaacaatgaggtgtagagatatgaagctagattgtctccgggtgacgttgttatcattccagcaggtcatccggttgccattactgcttcttcaaatttgaatttgcttggatttggtatcaatgctgagaacaatgagagaaactttctttcagatatttagtgaatattagtatgattacttaataagtctcggctaaatgagaattttttgaaattgatattttgattttggtgattgaaaatttgaaagctcggacgacaatgtgataagctaaattgaaaatccagtaaaagagcttacatttcctggatctgtttaagagataaatagactaataaagaactaaaagtaatctcactttgcaaatgctgaacctgaataaaaggagtaaggaagctagggaaaaaggagtcctctgtcttcaattttgggcactttttactaagtaatcagtatgaaaaataatacaacacgtatgtatgatgtaagtgttggataataaactatgaaaaataaggaggaaaatgtatgctgtaagatatagctagctcataatgagctaagaataaataaagggtcatgtaactcttgcttattgagtcccacctttctactatgaagaaataaataatgaataaaatttttgtctttttttaatttaaaagagtgtttgggcgctaaatttcttaac

SEQ ID NO: 10 - DNA, 2746 bp, synthetic construct
  source 1..2746: mol_type = other DNA
tatatggcacaatataaccaaatgtctatccacgttattcatctagctttatgttctatcactataaatatccttcatcttactcttttatttcatcatctaaacttttaactagtgaaatataaatcatggctaccactatcaaatcatgatttccacttttgttgttgctgggaattatattcctggcctctgttgtttgtgtcacttatgccaattacgatgaaggttcagaacctagggtaccggcataaagagagagaggtcgctaagagggtgagaaagaggaaaaacgccatggagaatgaagaccttcctacgaaaaggaagaagatgaagaagagggataaagagaaagaggtcgctaagagggtgaaaaagaggaaaaacgccacggagaataaagaccttcgtatgaaaagtaagaagatgaagaagagaagtagaaatatagatattaacgtgaaaaggaagatgaagaagagaagcagaaatattaatattaacgtgaaaagaaggaataaaaggaagtttaacctggacgtgagagataagaaagagaggaagatgaggaataagtagacgaagagtaaagaggaagttaacgtcgtgaagatcccgaagaaagggcaaggctaaggcatagagaggagagaacaaaaagagacagacgccattaacgtgaaggagaggaggaagaaagatcttcagagtcataagaatgaagaaatccctttttatttaagtctaacaagtttctaacactctttgaaaacgaaaacggccacattcgtctcctttaaaggttcgacaaacgttcagacttatttgaaaatctctaaaactatcgtcttgtggaatatagagccaaaccccacaccatcttccttccttaacacatagatgctgacttaatccttgtagtcctcagtgataatttttattttactttataatattattataacaaatctttttgttttatagaaatatgactatttaaaataaaaacattgtaaagttcaatttaacaatatttcttatatttcataattaaattttggtttggttaatatgtattacaaggaaagccatattgacagtgttgagtcccaatgatagaaattcgtataatcttgagcgtggtgataccatcaaacttcctgcaggaacaacctcttatttagttaactaagatgatgaagaagatcttagactggtagatcttgtaatacccgtgaatgggcctggtaaatttgagatactatataaaatacaataaatttttcttcagaagcgttattcttacaaaaacatccatttatattacttttacttttgtctataatgaaaaattgatattttccgttcttccatcaagcttttgacctagctaaaaataaaaactaatacttatgaggattcagcaagaatattttagaggcctcctataacataagtatgtgaagtttttatcattttttaataaataaaaccattttaatttgtatcattgtttacaactataaactagatacgagaccatagagaaggttctcttagaagaataagagaaagatcggaaaaggagataataaggggaagaaacagatgcaatagtcaaagtgtcaagggaataaattgaggaattgaaaaagcttgccaaatcaagctcaaagaaaagcttaccctctgaatttgaaccaatcaacttgagaagccacaagccagaatattctaataagtttggcaagttgtttgagattactccggaaaaaaaatacccttaactttaagatttagatctatttgttagttgtgtggagattaacgagataagtacacaacactaaatatatataaaacatataattttaattatattacagaaatatgttaatgcgtttttgcttatatttttaaggagctctaatgttgccacactacaattcaagggctatagttgtactattggttaatgaaggaaaaggaaaccttgaacttctgggtttaaaaaatgagtaataagagagggaagatagaaaagaaagaaacaatgaggtgtagagatatgaagctagattgtctccgggtgacgttgttatcattccagcaggtcatccggttgccattactgcttcttcaaatttgaatttgcttggatttggtatcaatgctgagaacaatgagagaaactttctttcagatatttagtgaatattagtatgattacttaataagtctcggctaaatgagaattttttgaaattgatattttgattttggtgattgaaaatttgaaagctcggacgacaatgtgataagctaaattgaaaatccagtaaaagagcttacatttcctggatctgtttaagagataaatagactaataaagaactaaaagtaatctcactttgcaaatgctgaacctgaataaaaggagtaaggaagctagggaaaaaggagtcctctgtcttcaattttgggcactttttactaagtaatcagtatgaaaaataatacaacacgtatgtatgatgtaagtgttggataataaactatgaaaaataaggaggaaaatgtatgctgtaagatatagctagctcataatgagctaagaataaataaagggtcatgtaactcttgcttattgagtcccacctttctactatgaagaaataaataatgaataaaatttttgtctttttttaatttaaaagagtgtttgggcgctaaatttcttaac

SEQ ID NO: 11 - DNA, 2746 bp, synthetic construct
  source 1..2746: mol_type = other DNA
tatatggcacaatataaccaaatgtctatccacgttattcatctagctttatgttctatcactataaatatccttcatcttactcttttatttcatcatctaaacttttaactagtgaaatataaatcatggctaccactatcaaatcatgatttccacttttgttgttgctgggaattatattcctggcctctgttgtttgtgtcacttatgccaattacgatgaaggttcagaacctagggtaccggcataaagagagagaggtcgctaagagggtgagaaagaggaaaaacgccatggagaatagagaccttcctacgaaaaggaagaagatgaagaagagggataaagagaaagaggtcgctaagagggtgaaaaagaggaaaaacgccacggagaataaagaccttcgtatgaaaagtaagaagatgaagaagagaagtagaaatatagatattaacgtgaaaaggaagatgaagaagagaagcagaaatattaatattaacgtgaaaagaaggaataaaaggaagtttaacctggacgtgagagataagaaagagaggaagatgaggaataagtagacgaagagtaaagaggaagttaacgtcgtgaagatcccgaagaaagggcaaggctaaggcatagagaggagagaacaaaaagagacagacgccattaacgtgaaggagaggaggaagaaagatcttcagagtcataagaatgaagaaatccctttttatttaagtctaacaagtttctaacactctttgaaaacgaaaacggccacattcgtctcctttaaaggttcgacaaacgttcagacttatttgaaaatctctaaaactatcgtcttgtggaatatagagccaaaccccacaccatcttccttccttaacacatagatgctgacttaatccttgtagtcctcagtgataatttttattttactttataatattattataacaaatctttttgttttatagaaatatgactatttaaaataaaaacattgtaaagttcaatttaacaatatttcttatatttcataattaaattttggtttggttaatatgtattacaaggaaagccatattgacagtgttgagtcccaatgatagaaattcgtataatcttgagcgtggtgataccatcaaacttcctgcaggaacaacctcttatttagttaactaagatgatgaagaagatcttagactggtagatcttgtaatacccgtgaatgggcctggtaaatttgagatactatataaaatacaataaatttttcttcagaagcgttattcttacaaaaacatccatttatattacttttacttttgtctataatgaaaaattgatattttccgttcttccatcaagcttttgacctagctaaaaataaaaactaatacttatgaggattcagcaagaatattttagaggcctcctataacataagtatgtgaagtttttatcattttttaataaataaaaccattttaatttgtatcattgtttacaactataaactagatacgagaccatagagaaggttctcttagaagaataagagaaagatcggaaaaggagataataaggggaagaaacagatgcaatagtcaaagtgtcaagggaataaattgaggaattgaaaaagcttgccaaatcaagctcaaagaaaagcttaccctctgaatttgaaccaatcaacttgagaagccacaagccagaatattctaataagtttggcaagttgtttgagattactccggaaaaaaaatacccttaactttaagatttagatctatttgttagttgtgtggagattaacgagataagtacacaacactaaatatatataaaacatataattttaattatattacagaaatatgttaatgcgtttttgcttatatttttaaggagctctaatgttgccacactacaattcaagggctatagttgtactattggttaatgaaggaaaaggaaaccttgaacttctgggtttaaaaaatgagtaataagagagggaagatagaaaagaaagaaacaatgaggtgtagagatatgaagctagattgtctccgggtgacgttgttatcattccagcaggtcatccggttgccattactgcttcttcaaatttgaatttgcttggatttggtatcaatgctgagaacaatgagagaaactttctttcagatatttagtgaatattagtatgattacttaataagtctcggctaaatgagaattttttgaaattgatattttgattttggtgattgaaaatttgaaagctcggacgacaatgtgataagctaaattgaaaatccagtaaaagagcttacatttcctggatctgtttaagagataaatagactaataaagaactaaaagtaatctcactttgcaaatgctgaacctgaataaaaggagtaaggaagctagggaaaaaggagtcctctgtcttcaattttgggcactttttactaagtaatcagtatgaaaaataatacaacacgtatgtatgatgtaagtgttggataataaactatgaaaaataaggaggaaaatgtatgctgtaagatatagctagctcataatgagctaagaataaataaagggtcatgtaactcttgcttattgagtcccacctttctactatgaagaaataaataatgaataaaatttttgtctttttttaatttaaaagagtgtttgggcgctaaatttcttaac

SEQ ID NO: 12 - DNA, 2746 bp, synthetic construct
  source 1..2746: mol_type = other DNA
tatatggcacaatataaccaaatgtctatccacgttattcatctagctttatgttctatcactataaatatccttcatcttactcttttatttcatcatctaaacttttaactagtgaaatataaatcatggctaccactatcaaatcatgatttccacttttgttgttgctgggaattatattcctggcctctgttgtttgtgtcacttatgccaattacgatgaaggttcagaacctagggtaccggcataaagagagagaggtcgctaagagggtgagaaagaggaaaaacgccatggagaataaagaccttcctacgaaaaggaagaagatgaagaagagggacaaagagaaagaggtcgctaagagggtgaaaaagaggaaaaacgccacggagaataaagaccttcgtatgaaaagtaagaagatgaagaagagaagtagaaatatagatattaacgtgaaaaggaagatgaagaagagaagtagaaatattaatattaacgtgaaaagaaggaataaaaggaagtttaacctggacgtgagagataagaaagagaggaagatgaggaataagtagacgaagagtaaagaggaagttaacgtcgtgaagatcccgaagaaagggcaaggctaaggcatagagaggagagaacaaaaagagacagacgccattaacgtgaaggagaggaggaagaaagatcttcagagtcataagaatgaagaaatccctttttatttaagtctaacaagtttctaacactctttgaaaacgaaaacggccacattcgtctcctttaaaggttcgacaaacgttcagacttatttgaaaatctctaaaactatcgtcttgtggaatatagagccaaaccccacaccatcttccttccttaacacatagatgctgacttaatccttgtagtcctcagtgataatttttattttactttataatattattataacaaatctttttgttttatagaaatatgactatttaaaataaaaacattgtaaagttcaatttaacaatatttcttatatttcataattaaattttggtttggttaatatgtattacaaggaaagccatattgacagtgttgagtcccaatgatagaaattcgtataatcttgagcgtggtgataccatcaaacttcctgcaggaacaacctcttatttagttaactaagatgatgaagaagatcttagactggtagatcttgtaatacccgtgaatgggcctggtaaatttgagatactatataaaatacaataaatttttcttcagaagcgttattcttacaaaaacatccatttatattacttttacttttgtctataatgaaaaattgatattttccgttcttccatcaagcttttgacctagctaaaaataaaaactaatacttatgaggattcagcaagaatattttagaggcctcctataacataagtatgtgaagtttttatcattttttaataaataaaaccattttaatttgtatcattgtttacaactataaactagatacgagaccatagagaaggttctcttagaagaataagagaaagatcggaaaaggagataataaggggaagaaacagatgcaatagtcaaagtgtcaagggaataaattgaggaattgaaaaagcttgccaaatcaagctcaaagaaaagcttaccctctgaatttgaaccaatcaacttgagaagccacaagccagaatattctaataagtttggcaagttgtttgagattactccggaaaaaaaatacccttaactttaagatttagatctatttgttagttgtgtggagattaacgagataagtacacaacactaaatatatataaaacatataattttaattatattacagaaatatgttaatgcgtttttgcttatatttttaaggagctctaatgttgccacactacaattcaagggctatagttgtactattggttaatgaaggaaaaggaaaccttgaacttctgggtttaaaaaatgagtaataagagagggaagatagaaaagaaagaaacaatgaggtgtagagatatgaagctagattgtctccgggtgacgttgttatcattccagcaggtcatccggttgccattactgcttcttcaaatttgaatttgcttggatttggtatcaatgctgagaacaatgagagaaactttctttcagatatttagtgaatattagtatgattacttaataagtctcggctaaatgagaattttttgaaattgatattttgattttggtgattgaaaatttgaaagctcggacgacaatgtgataagctaaattgaaaatccagtaaaagagcttacatttcctggatctgtttaagagataaatagactaataaagaactaaaagtaatctcactttgcaaatgctgaacctgaataaaaggagtaaggaagctagggaaaaaggagtcctctgtcttcaattttgggcactttttactaagtaatcagtatgaaaaataatacaacacgtatgtatgatgtaagtgttggataataaactatgaaaaataaggaggaaaatgtatgctgtaagatatagctagctcataatgagctaagaataaataaagggtcatgtaactcttgcttattgagtcccacctttctactatgaagaaataaataatgaataaaatttttgtctttttttaatttaaaagagtgtttgggcgctaaatttcttaac

SEQ ID NO: 13 - DNA, 2746 bp, synthetic construct
  source 1..2746: mol_type = other DNA
tatatggcacaatataaccaaatgtctatccacgttattcatctagctttatgttctatcactataaatatccttcatcttactcttttatttcatcatctaaacttttaactagtgaaatataaatcatggctaccactatcaaatcatgatttccacttttgttgttgctgggaattatattcctggcctctgttgtttgtgtcacttatgccaattacgatgaaggttcagaacctagggtaccggcataaagagagagaggtcgctaagagggtgagaaagaggaaaaacgccatggagaataaagaccttcctacgaaaaggaagaagatgaagaagagggataaagagaaagaggtcgccaagagggtgaaaaagaggaaaaacgccacggagaataaagaccttcgtatgaaaagtaagaagatgaagaagagaagtagaaatatagatattaacgtgaaaaggaagatgaagaagagaagcagaaatattaatattaacgtgaaaagaaggaataaaaggaagtttaacctggacgtgagagataagaaagagaggaagatgaggaataagtagacgaagagtaaagaggaagttaacgtcgtgaagatcccgaagaaagggcaaggctaaggcatagagaggagagaacaaaaagagacagacgccattaacgtgaaggagaggaggaagaaagatcttcagagtcataagaatgaagaaatccctttttatttaagtctaacaagtttctaacactctttgaaaacgaaaacggccacattcgtctcctttaaaggttcgacaaacgttcagacttatttgaaaatctctaaaactatcgtcttgtggaatatagagccaaaccccacaccatcttccttccttaacacatagatgctgacttaatccttgtagtcctcagtgataatttttattttactttataatattattataacaaatctttttgttttatagaaatatgactatttaaaataaaaacattgtaaagttcaatttaacaatatttcttatatttcataattaaattttggtttggttaatatgtattacaaggaaagccatattgacagtgttgagtcccaatgatagaaattcgtataatcttgagcgtggtgataccatcaaacttcctgcaggaacaacctcttatttagttaactaagatgatgaagaagatcttagactggtagatcttgtaatacccgtgaatgggcctggtaaatttgagatactatataaaatacaataaatttttcttcagaagcgttattcttacaaaaacatccatttatattacttttacttttgtctataatgaaaaattgatattttccgttcttccatcaagcttttgacctagctaaaaataaaaactaatacttatgaggattcagcaagaatattttagaggcctcctataacataagtatgtgaagtttttatcattttttaataaataaaaccattttaatttgtatcattgtttacaactataaactagatacgagaccatagagaaggttctcttagaagaataagagaaagatcggaaaaggagataataaggggaagaaacagatgcaatagtcaaagtgtcaagggaataaattgaggaattgaaaaagcttgccaaatcaagctcaaagaaaagcttaccctctgaatttgaaccaatcaacttgagaagccacaagccagaatattctaataagtttggcaagttgtttgagattactccggaaaaaaaatacccttaactttaagatttagatctatttgttagttgtgtggagattaacgagataagtacacaacactaaatatatataaaacatataattttaattatattacagaaatatgttaatgcgtttttgcttatatttttaaggagctctaatgttgccacactacaattcaagggctatagttgtactattggttaatgaaggaaaaggaaaccttgaacttctgggtttaaaaaatgagtaataagagagggaagatagaaaagaaagaaacaatgaggtgtagagatatgaagctagattgtctccgggtgacgttgttatcattccagcaggtcatccggttgccattactgcttcttcaaatttgaatttgcttggatttggtatcaatgctgagaacaatgagagaaactttctttcagatatttagtgaatattagtatgattacttaataagtctcggctaaatgagaattttttgaaattgatattttgattttggtgattgaaaatttgaaagctcggacgacaatgtgataagctaaattgaaaatccagtaaaagagcttacatttcctggatctgtttaagagataaatagactaataaagaactaaaagtaatctcactttgcaaatgctgaacctgaataaaaggagtaaggaagctagggaaaaaggagtcctctgtcttcaattttgggcactttttactaagtaatcagtatgaaaaataatacaacacgtatgtatgatgtaagtgttggataataaactatgaaaaataaggaggaaaatgtatgctgtaagatatagctagctcataatgagctaagaataaataaagggtcatgtaactcttgcttattgagtcccacctttctactatgaagaaataaataatgaataaaatttttgtctttttttaatttaaaagagtgtttgggcgctaaatttcttaac

SEQ ID NO: 14 - DNA, 2746 bp, synthetic construct
  source 1..2746: mol_type = other DNA
tatatggcacaatataaccaaatgtctatccacgttattcatctagctttatgttctatcactataaatatccttcatcttactcttttatttcatcatctaaacttttaactagtgaaatataaatcatggctaccactatcaaatcatgatttccacttttgttgttgctgggaattatattcctggcctctgttgtttgtgtcacttatgccaattacgatgaaggttcagaacctagggtaccggcataaagagagagaggtcgctaagagggtgagaaagaggaaaaacgccatggagaataaagaccttcctacgaaaaggaagaagatgaagaagagggataaagagaaagaggtcgctaagagggtgaaaaagaggaaaaacgccacggagaatgaagaccttcgtatgaaaagtaagaagatgaagaagagaagtagaaatatagatattaacgtgaaaaggaagatgaagaagagaagcagaaatattaatattaacgtgaaaagaaggaataaaaggaagtttaacctggacgtgagagataagaaagagaggaagatgaggaataagtagacgaagagtaaagaggaagttaacgtcgtgaagatcccgaagaaagggcaaggctaaggcatagagaggagagaacaaaaagagacagacgccattaacgtgaaggagaggaggaagaaagatcttcagagtcataagaatgaagaaatccctttttatttaagtctaacaagtttctaacactctttgaaaacgaaaacggccacattcgtctcctttaaaggttcgacaaacgttcagacttatttgaaaatctctaaaactatcgtcttgtggaatatagagccaaaccccacaccatcttccttccttaacacatagatgctgacttaatccttgtagtcctcagtgataatttttattttactttataatattattataacaaatctttttgttttatagaaatatgactatttaaaataaaaacattgtaaagttcaatttaacaatatttcttatatttcataattaaattttggtttggttaatatgtattacaaggaaagccatattgacagtgttgagtcccaatgatagaaattcgtataatcttgagcgtggtgataccatcaaacttcctgcaggaacaacctcttatttagttaactaagatgatgaagaagatcttagactggtagatcttgtaatacccgtgaatgggcctggtaaatttgagatactatataaaatacaataaatttttcttcagaagcgttattcttacaaaaacatccatttatattacttttacttttgtctataatgaaaaattgatattttccgttcttccatcaagcttttgacctagctaaaaataaaaactaatacttatgaggattcagcaagaatattttagaggcctcctataacataagtatgtgaagtttttatcattttttaataaataaaaccattttaatttgtatcattgtttacaactataaactagatacgagaccatagagaaggttctcttagaagaataagagaaagatcggaaaaggagataataaggggaagaaacagatgcaatagtcaaagtgtcaagggaataaattgaggaattgaaaaagcttgccaaatcaagctcaaagaaaagcttaccctctgaatttgaaccaatcaacttgagaagccacaagccagaatattctaataagtttggcaagttgtttgagattactccggaaaaaaaatacccttaactttaagatttagatctatttgttagttgtgtggagattaacgagataagtacacaacactaaatatatataaaacatataattttaattatattacagaaatatgttaatgcgtttttgcttatatttttaaggagctctaatgttgccacactacaattcaagggctatagttgtactattggttaatgaaggaaaaggaaaccttgaacttctgggtttaaaaaatgagtaataagagagggaagatagaaaagaaagaaacaatgaggtgtagagatatgaagctagattgtctccgggtgacgttgttatcattccagcaggtcatccggttgccattactgcttcttcaaatttgaatttgcttggatttggtatcaatgctgagaacaatgagagaaactttctttcagatatttagtgaatattagtatgattacttaataagtctcggctaaatgagaattttttgaaattgatattttgattttggtgattgaaaatttgaaagctcggacgacaatgtgataagctaaattgaaaatccagtaaaagagcttacatttcctggatctgtttaagagataaatagactaataaagaactaaaagtaatctcactttgcaaatgctgaacctgaataaaaggagtaaggaagctagggaaaaaggagtcctctgtcttcaattttgggcactttttactaagtaatcagtatgaaaaataatacaacacgtatgtatgatgtaagtgttggataataaactatgaaaaataaggaggaaaatgtatgctgtaagatatagctagctcataatgagctaagaataaataaagggtcatgtaactcttgcttattgagtcccacctttctactatgaagaaataaataatgaataaaatttttgtctttttttaatttaaaagagtgtttgggcgctaaatttcttaac

SEQ ID NO: 15 - DNA, 2746 bp, synthetic construct
  source 1..2746: mol_type = other DNA
tatatggcacaatataaccaaatgtctatccacgttattcatctagctttatgttctatcactataaatatccttcatcttactcttttatttcatcatctaaacttttaactagtgaaatataaatcatggctaccactatcaaatcatgatttccacttttgttgttgctgggaattatattcctggcctctgttgtttgtgtcacttatgccaattacgatgaaggttcagaacctagggtaccggcataaagagagagaggtcgctaagagggtgagaaagaggaaaaacgccatggagaataaagaccttcctacgaaaaggaagaagatgaagaagagggataaagagaaagaggtcgctaagagggtgaaaaagaggaaaaacgccacggagaatagagaccttcgtatgaaaagtaagaagatgaagaagagaagtagaaatatagatattaacgtgaaaaggaagatgaagaagagaagcagaaatattaatattaacgtgaaaagaaggaataaaaggaagtttaacctggacgtgagagataagaaagagaggaagatgaggaataagtagacgaagagtaaagaggaagttaacgtcgtgaagatcccgaagaaagggcaaggctaaggcatagagaggagagaacaaaaagagacagacgccattaacgtgaaggagaggaggaagaaagatcttcagagtcataagaatgaagaaatccctttttatttaagtctaacaagtttctaacactctttgaaaacgaaaacggccacattcgtctcctttaaaggttcgacaaacgttcagacttatttgaaaatctctaaaactatcgtcttgtggaatatagagccaaaccccacaccatcttccttccttaacacatagatgctgacttaatccttgtagtcctcagtgataatttttattttactttataatattattataacaaatctttttgttttatagaaatatgactatttaaaataaaaacattgtaaagttcaatttaacaatatttcttatatttcataattaaattttggtttggttaatatgtattacaaggaaagccatattgacagtgttgagtcccaatgatagaaattcgtataatcttgagcgtggtgataccatcaaacttcctgcaggaacaacctcttatttagttaactaagatgatgaagaagatcttagactggtagatcttgtaatacccgtgaatgggcctggtaaatttgagatactatataaaatacaataaatttttcttcagaagcgttattcttacaaaaacatccatttatattacttttacttttgtctataatgaaaaattgatattttccgttcttccatcaagcttttgacctagctaaaaataaaaactaatacttatgaggattcagcaagaatattttagaggcctcctataacataagtatgtgaagtttttatcattttttaataaataaaaccattttaatttgtatcattgtttacaactataaactagatacgagaccatagagaaggttctcttagaagaataagagaaagatcggaaaaggagataataaggggaagaaacagatgcaatagtcaaagtgtcaagggaataaattgaggaattgaaaaagcttgccaaatcaagctcaaagaaaagcttaccctctgaatttgaaccaatcaacttgagaagccacaagccagaatattctaataagtttggcaagttgtttgagattactccggaaaaaaaatacccttaactttaagatttagatctatttgttagttgtgtggagattaacgagataagtacacaacactaaatatatataaaacatataattttaattatattacagaaatatgttaatgcgtttttgcttatatttttaaggagctctaatgttgccacactacaattcaagggctatagttgtactattggttaatgaaggaaaaggaaaccttgaacttctgggtttaaaaaatgagtaataagagagggaagatagaaaagaaagaaacaatgaggtgtagagatatgaagctagattgtctccgggtgacgttgttatcattccagcaggtcatccggttgccattactgcttcttcaaatttgaatttgcttggatttggtatcaatgctgagaacaatgagagaaactttctttcagatatttagtgaatattagtatgattacttaataagtctcggctaaatgagaattttttgaaattgatattttgattttggtgattgaaaatttgaaagctcggacgacaatgtgataagctaaattgaaaatccagtaaaagagcttacatttcctggatctgtttaagagataaatagactaataaagaactaaaagtaatctcactttgcaaatgctgaacctgaataaaaggagtaaggaagctagggaaaaaggagtcctctgtcttcaattttgggcactttttactaagtaatcagtatgaaaaataatacaacacgtatgtatgatgtaagtgttggataataaactatgaaaaataaggaggaaaatgtatgctgtaagatatagctagctcataatgagctaagaataaataaagggtcatgtaactcttgcttattgagtcccacctttctactatgaagaaataaataatgaataaaatttttgtctttttttaatttaaaagagtgtttgggcgctaaatttcttaac

SEQ ID NO: 16 - DNA, 2746 bp, synthetic construct
  source 1..2746: mol_type = other DNA
tatatggcacaatataaccaaatgtctatccacgttattcatctagctttatgttctatcactataaatatccttcatcttactcttttatttcatcatctaaacttttaactagtgaaatataaatcatggctaccactatcaaatcatgatttccacttttgttgttgctgggaattatattcctggcctctgttgtttgtgtcacttatgccaattacgatgaaggttcagaacctagggtaccggcataaagagagagaggtcgctaagagggtgagaaagaggaaaaacgccatggagaataaagaccttcctacgaaaaggaagaagatgaagaagagggataaagagaaagaggtcgctaagagggtgaaaaagaggaaaaacgccacggagaataaagaccttcgtatgaaaagcaagaagatgaagaagagaagtagaaatatagatattaacgtgaaaaggaagatgaagaagagaagcagaaatattaatattaacgtgaaaagaaggaataaaaggaagtttaacctggacgtgagagataagaaagagaggaagatgaggaataagtagacgaagagtaaagaggaagttaacgtcgtgaagatcccgaagaaagggcaaggctaaggcatagagaggagagaacaaaaagagacagacgccattaacgtgaaggagaggaggaagaaagatcttcagagtcataagaatgaagaaatccctttttatttaagtctaacaagtttctaacactctttgaaaacgaaaacggccacattcgtctcctttaaaggttcgacaaacgttcagacttatttgaaaatctctaaaactatcgtcttgtggaatatagagccaaaccccacaccatcttccttccttaacacatagatgctgacttaatccttgtagtcctcagtgataatttttattttactttataatattattataacaaatctttttgttttatagaaatatgactatttaaaataaaaacattgtaaagttcaatttaacaatatttcttatatttcataattaaattttggtttggttaatatgtattacaaggaaagccatattgacagtgttgagtcccaatgatagaaattcgtataatcttgagcgtggtgataccatcaaacttcctgcaggaacaacctcttatttagttaactaagatgatgaagaagatcttagactggtagatcttgtaatacccgtgaatgggcctggtaaatttgagatactatataaaatacaataaatttttcttcagaagcgttattcttacaaaaacatccatttatattacttttacttttgtctataatgaaaaattgatattttccgttcttccatcaagcttttgacctagctaaaaataaaaactaatacttatgaggattcagcaagaatattttagaggcctcctataacataagtatgtgaagtttttatcattttttaataaataaaaccattttaatttgtatcattgtttacaactataaactagatacgagaccatagagaaggttctcttagaagaataagagaaagatcggaaaaggagataataaggggaagaaacagatgcaatagtcaaagtgtcaagggaataaattgaggaattgaaaaagcttgccaaatcaagctcaaagaaaagcttaccctctgaatttgaaccaatcaacttgagaagccacaagccagaatattctaataagtttggcaagttgtttgagattactccggaaaaaaaatacccttaactttaagatttagatctatttgttagttgtgtggagattaacgagataagtacacaacactaaatatatataaaacatataattttaattatattacagaaatatgttaatgcgtttttgcttatatttttaaggagctctaatgttgccacactacaattcaagggctatagttgtactattggttaatgaaggaaaaggaaaccttgaacttctgggtttaaaaaatgagtaataagagagggaagatagaaaagaaagaaacaatgaggtgtagagatatgaagctagattgtctccgggtgacgttgttatcattccagcaggtcatccggttgccattactgcttcttcaaatttgaatttgcttggatttggtatcaatgctgagaacaatgagagaaactttctttcagatatttagtgaatattagtatgattacttaataagtctcggctaaatgagaattttttgaaattgatattttgattttggtgattgaaaatttgaaagctcggacgacaatgtgataagctaaattgaaaatccagtaaaagagcttacatttcctggatctgtttaagagataaatagactaataaagaactaaaagtaatctcactttgcaaatgctgaacctgaataaaaggagtaaggaagctagggaaaaaggagtcctctgtcttcaattttgggcactttttactaagtaatcagtatgaaaaataatacaacacgtatgtatgatgtaagtgttggataataaactatgaaaaataaggaggaaaatgtatgctgtaagatatagctagctcataatgagctaagaataaataaagggtcatgtaactcttgcttattgagtcccacctttctactatgaagaaataaataatgaataaaatttttgtctttttttaatttaaaagagtgtttgggcgctaaatttcttaac

SEQ ID NO: 17 - DNA, 2746 bp, synthetic construct
  source 1..2746: mol_type = other DNA
tatatggcacaatataaccaaatgtctatccacgttattcatctagctttatgttctatcactataaatatccttcatcttactcttttatttcatcatctaaacttttaactagtgaaatataaatcatggctaccactatcaaatcatgatttccacttttgttgttgctgggaattatattcctggcctctgttgtttgtgtcacttatgccaattacgatgaaggttcagaacctagggtaccggcataaagagagagaggtcgctaagagggtgagaaagaggaaaaacgccatggagaataaagaccttcctacgaaaaggaagaagatgaagaagagggataaagagaaagaggtcgctaagagggtgaaaaagaggaaaaacgccacggagaataaagaccttcgtatgaaaagtaagaagatgaagaagagaagcagaaatatagatattaacgtgaaaaggaagatgaagaagagaagcagaaatattaatattaacgtgaaaagaaggaataaaaggaagtttaacctggacgtgagagataagaaagagaggaagatgaggaataagtagacgaagagtaaagaggaagttaacgtcgtgaagatcccgaagaaagggcaaggctaaggcatagagaggagagaacaaaaagagacagacgccattaacgtgaaggagaggaggaagaaagatcttcagagtcataagaatgaagaaatccctttttatttaagtctaacaagtttctaacactctttgaaaacgaaaacggccacattcgtctcctttaaaggttcgacaaacgttcagacttatttgaaaatctctaaaactatcgtcttgtggaatatagagccaaaccccacaccatcttccttccttaacacatagatgctgacttaatccttgtagtcctcagtgataatttttattttactttataatattattataacaaatctttttgttttatagaaatatgactatttaaaataaaaacattgtaaagttcaatttaacaatatttcttatatttcataattaaattttggtttggttaatatgtattacaaggaaagccatattgacagtgttgagtcccaatgatagaaattcgtataatcttgagcgtggtgataccatcaaacttcctgcaggaacaacctcttatttagttaactaagatgatgaagaagatcttagactggtagatcttgtaatacccgtgaatgggcctggtaaatttgagatactatataaaatacaataaatttttcttcagaagcgttattcttacaaaaacatccatttatattacttttacttttgtctataatgaaaaattgatattttccgttcttccatcaagcttttgacctagctaaaaataaaaactaatacttatgaggattcagcaagaatattttagaggcctcctataacataagtatgtgaagtttttatcattttttaataaataaaaccattttaatttgtatcattgtttacaactataaactagatacgagaccatagagaaggttctcttagaagaataagagaaagatcggaaaaggagataataaggggaagaaacagatgcaatagtcaaagtgtcaagggaataaattgaggaattgaaaaagcttgccaaatcaagctcaaagaaaagcttaccctctgaatttgaaccaatcaacttgagaagccacaagccagaatattctaataagtttggcaagttgtttgagattactccggaaaaaaaatacccttaactttaagatttagatctatttgttagttgtgtggagattaacgagataagtacacaacactaaatatatataaaacatataattttaattatattacagaaatatgttaatgcgtttttgcttatatttttaaggagctctaatgttgccacactacaattcaagggctatagttgtactattggttaatgaaggaaaaggaaaccttgaacttctgggtttaaaaaatgagtaataagagagggaagatagaaaagaaagaaacaatgaggtgtagagatatgaagctagattgtctccgggtgacgttgttatcattccagcaggtcatccggttgccattactgcttcttcaaatttgaatttgcttggatttggtatcaatgctgagaacaatgagagaaactttctttcagatatttagtgaatattagtatgattacttaataagtctcggctaaatgagaattttttgaaattgatattttgattttggtgattgaaaatttgaaagctcggacgacaatgtgataagctaaattgaaaatccagtaaaagagcttacatttcctggatctgtttaagagataaatagactaataaagaactaaaagtaatctcactttgcaaatgctgaacctgaataaaaggagtaaggaagctagggaaaaaggagtcctctgtcttcaattttgggcactttttactaagtaatcagtatgaaaaataatacaacacgtatgtatgatgtaagtgttggataataaactatgaaaaataaggaggaaaatgtatgctgtaagatatagctagctcataatgagctaagaataaataaagggtcatgtaactcttgcttattgagtcccacctttctactatgaagaaataaataatgaataaaatttttgtctttttttaatttaaaagagtgtttgggcgctaaatttcttaac

SEQ ID NO: 18 - DNA, 2746 bp, synthetic construct
  source 1..2746: mol_type = other DNA
tatatggcacaatataaccaaatgtctatccacgttattcatctagctttatgttctatcactataaatatccttcatcttactcttttatttcatcatctaaacttttaactagtgaaatataaatcatggctaccactatcaaatcatgatttccacttttgttgttgctgggaattatattcctggcctctgttgtttgtgtcacttatgccaattacgatgaaggttcagaacctagggtaccggcataaagagagagaggtcgctaagagggtgagaaagaggaaaaacgccatggagaataaagaccttcctacgaaaaggaagaagatgaagaagagggataaagagaaagaggtcgctaagagggtgaaaaagaggaaaaacgccacggagaataaagaccttcgtatgaaaagtaagaagatgaagaagagaagtagaaatatagatatcaacgtgaaaaggaagatgaagaagagaagcagaaatattaatattaacgtgaaaagaaggaataaaaggaagtttaacctggacgtgagagataagaaagagaggaagatgaggaataagtagacgaagagtaaagaggaagttaacgtcgtgaagatcccgaagaaagggcaaggctaaggcatagagaggagagaacaaaaagagacagacgccattaacgtgaaggagaggaggaagaaagatcttcagagtcataagaatgaagaaatccctttttatttaagtctaacaagtttctaacactctttgaaaacgaaaacggccacattcgtctcctttaaaggttcgacaaacgttcagacttatttgaaaatctctaaaactatcgtcttgtggaatatagagccaaaccccacaccatcttccttccttaacacatagatgctgacttaatccttgtagtcctcagtgataatttttattttactttataatattattataacaaatctttttgttttatagaaatatgactatttaaaataaaaacattgtaaagttcaatttaacaatatttcttatatttcataattaaattttggtttggttaatatgtattacaaggaaagccatattgacagtgttgagtcccaatgatagaaattcgtataatcttgagcgtggtgataccatcaaacttcctgcaggaacaacctcttatttagttaactaagatgatgaagaagatcttagactggtagatcttgtaatacccgtgaatgggcctggtaaatttgagatactatataaaatacaataaatttttcttcagaagcgttattcttacaaaaacatccatttatattacttttacttttgtctataatgaaaaattgatattttccgttcttccatcaagcttttgacctagctaaaaataaaaactaatacttatgaggattcagcaagaatattttagaggcctcctataacataagtatgtgaagtttttatcattttttaataaataaaaccattttaatttgtatcattgtttacaactataaactagatacgagaccatagagaaggttctcttagaagaataagagaaagatcggaaaaggagataataaggggaagaaacagatgcaatagtcaaagtgtcaagggaataaattgaggaattgaaaaagcttgccaaatcaagctcaaagaaaagcttaccctctgaatttgaaccaatcaacttgagaagccacaagccagaatattctaataagtttggcaagttgtttgagattactccggaaaaaaaatacccttaactttaagatttagatctatttgttagttgtgtggagattaacgagataagtacacaacactaaatatatataaaacatataattttaattatattacagaaatatgttaatgcgtttttgcttatatttttaaggagctctaatgttgccacactacaattcaagggctatagttgtactattggttaatgaaggaaaaggaaaccttgaacttctgggtttaaaaaatgagtaataagagagggaagatagaaaagaaagaaacaatgaggtgtagagatatgaagctagattgtctccgggtgacgttgttatcattccagcaggtcatccggttgccattactgcttcttcaaatttgaatttgcttggatttggtatcaatgctgagaacaatgagagaaactttctttcagatatttagtgaatattagtatgattacttaataagtctcggctaaatgagaattttttgaaattgatattttgattttggtgattgaaaatttgaaagctcggacgacaatgtgataagctaaattgaaaatccagtaaaagagcttacatttcctggatctgtttaagagataaatagactaataaagaactaaaagtaatctcactttgcaaatgctgaacctgaataaaaggagtaaggaagctagggaaaaaggagtcctctgtcttcaattttgggcactttttactaagtaatcagtatgaaaaataatacaacacgtatgtatgatgtaagtgttggataataaactatgaaaaataaggaggaaaatgtatgctgtaagatatagctagctcataatgagctaagaataaataaagggtcatgtaactcttgcttattgagtcccacctttctactatgaagaaataaataatgaataaaatttttgtctttttttaatttaaaagagtgtttgggcgctaaatttcttaac

SEQ ID NO: 19 - DNA, 2746 bp, synthetic construct; identical to SEQ ID NO: 2
  source 1..2746: mol_type = other DNA

SEQ ID NO: 20 - DNA, 2746 bp, synthetic construct
  source 1..2746: mol_type = other DNA
tatatggcacaatataaccaaatgtctatccacgttattcatctagctttatgttctatcactataaatatccttcatcttactcttttatttcatcatctaaacttttaactagtgaaatataaatcatggctaccactatcaaatcatgatttccacttttgttgttgctgggaattatattcctggcctctgttgtttgtgtcacttatgccaattacgatgaaggttcagaacctagggtaccggcataaagagagagaggtcgctaagagggtgagaaagaggaaaaacgccatggagaataaagaccttcctacgaaaaggaagaagatgaagaagagggataaagagaaagaggtcgctaagagggtgaaaaagaggaaaaacgccacggagaataaagaccttcgtatgaaaagtaagaagatgaagaagagaagtagaaatatagatattaacgtgaaaaggaagatgaagaagagaagtagaaatatcaatattaacgtgaaaagaaggaataaaaggaagtttaacctggacgtgagagataagaaagagaggaagatgaggaataagtagacgaagagtaaagaggaagttaacgtcgtgaagatcccgaagaaagggcaaggctaaggcatagagaggagagaacaaaaagagacagacgccattaacgtgaaggagaggaggaagaaagatcttcagagtcataagaatgaagaaatccctttttatttaagtctaacaagtttctaacactctttgaaaacgaaaacggccacattcgtctcctttaaaggttcgacaaacgttcagacttatttgaaaatctctaaaactatcgtcttgtggaatatagagccaaaccccacaccatcttccttccttaacacatagatgctgacttaatccttgtagtcctcagtgataatttttattttactttataatattattataacaaatctttttgttttatagaaatatgactatttaaaataaaaacattgtaaagttcaatttaacaatatttcttatatttcataattaaattttggtttggttaatatgtattacaaggaaagccatattgacagtgttgagtcccaatgatagaaattcgtataatcttgagcgtggtgataccatcaaacttcctgcaggaacaacctcttatttagttaactaagatgatgaagaagatcttagactggtagatcttgtaatacccgtgaatgggcctggtaaatttgagatactatataaaatacaataaatttttcttcagaagcgttattcttacaaaaacatccatttatattacttttacttttgtctataatgaaaaattgatattttccgttcttccatcaagcttttgacctagctaaaaataaaaactaatacttatgaggattcagcaagaatattttagaggcctcctataacataagtatgtgaagtttttatcattttttaataaataaaaccattttaatttgtatcattgtttacaactataaactagatacgagaccatagagaaggttctcttagaagaataagagaaagatcggaaaaggagataataaggggaagaaacagatgcaatagtcaaagtgtcaagggaataaattgaggaattgaaaaagcttgccaaatcaagctcaaagaaaagcttaccctctgaatttgaaccaatcaacttgagaagccacaagccagaatattctaataagtttggcaagttgtttgagattactccggaaaaaaaatacccttaactttaagatttagatctatttgttagttgtgtggagattaacgagataagtacacaacactaaatatatataaaacatataattttaattatattacagaaatatgttaatgcgtttttgcttatatttttaaggagctctaatgttgccacactacaattcaagggctatagttgtactattggttaatgaaggaaaaggaaaccttgaacttctgggtttaaaaaatgagtaataagagagggaagatagaaaagaaagaaacaatgaggtgtagagatatgaagctagattgtctccgggtgacgttgttatcattccagcaggtcatccggttgccattactgcttcttcaaatttgaatttgcttggatttggtatcaatgctgagaacaatgagagaaactttctttcagatatttagtgaatattagtatgattacttaataagtctcggctaaatgagaattttttgaaattgatattttgattttggtgattgaaaatttgaaagctcggacgacaatgtgataagctaaattgaaaatccagtaaaagagcttacatttcctggatctgtttaagagataaatagactaataaagaactaaaagtaatctcactttgcaaatgctgaacctgaataaaaggagtaaggaagctagggaaaaaggagtcctctgtcttcaattttgggcactttttactaagtaatcagtatgaaaaataatacaacacgtatgtatgatgtaagtgttggataataaactatgaaaaataaggaggaaaatgtatgctgtaagatatagctagctcataatgagctaagaataaataaagggtcatgtaactcttgcttattgagtcccacctttctactatgaagaaataaataatgaataaaatttttgtctttttttaatttaaaagagtgtttgggcgctaaatttcttaac

SEQ ID NO: 21 - DNA, 2746 bp, synthetic construct
  source 1..2746: mol_type = other DNA
tatatggcacaatataaccaaatgtctatccacgttattcatctagctttatgttctatcactataaatatccttcatcttactcttttatttcatcatctaaacttttaactagtgaaatataaatcatggctaccactatcaaatcatgatttccacttttgttgttgctgggaattatattcctggcctctgttgtttgtgtcacttatgccaattacgatgaaggttcagaacctagggtaccggcataaagagagagaggtcgctaagagggtgagaaagaggaaaaacgccatggagaataaagaccttcctacgaaaaggaagaagatgaagaagagggataaagagaaagaggtcgctaagagggtgaaaaagaggaaaaacgccacggagaataaagaccttcgtatgaaaagtaagaagatgaagaagagaagtagaaatatagatattaacgtgaaaaggaagatgaagaagagaagtagaaatattaatatcaacgtgaaaagaaggaataaaaggaagtttaacctggacgtgagagataagaaagagaggaagatgaggaataagtagacgaagagtaaagaggaagttaacgtcgtgaagatcccgaagaaagggcaaggctaaggcatagagaggagagaacaaaaagagacagacgccattaacgtgaaggagaggaggaagaaagatcttcagagtcataagaatgaagaaatccctttttatttaagtctaacaagtttctaacactctttgaaaacgaaaacggccacattcgtctcctttaaaggttcgacaaacgttcagacttatttgaaaatctctaaaactatcgtcttgtggaatatagagccaaaccccacaccatcttccttccttaacacatagatgctgacttaatccttgtagtcctcagtgataatttttattttactttataatattattataacaaatctttttgttttatagaaatatgactatttaaaataaaaacattgtaaagttcaatttaacaatatttcttatatttcataattaaattttggtttggttaatatgtattacaaggaaagccatattgacagtgttgagtcccaatgatagaaattcgtataatcttgagcgtggtgataccatcaaacttcctgcaggaacaacctcttatttagttaactaagatgatgaagaagatcttagactggtagatcttgtaatacccgtgaatgggcctggtaaatttgagatactatataaaatacaataaatttttcttcagaagcgttattcttacaaaaacatccatttatattacttttacttttgtctataatgaaaaattgatattttccgttcttccatcaagcttttgacctagctaaaaataaaaactaatacttatgaggattcagcaagaatattttagaggcctcctataacataagtatgtgaagtttttatcattttttaataaataaaaccattttaatttgtatcattgtttacaactataaactagatacgagaccatagagaaggttctcttagaagaataagagaaagatcggaaaaggagataataaggggaagaaacagatgcaatagtcaaagtgtcaagggaataaattgaggaattgaaaaagcttgccaaatcaagctcaaagaaaagcttaccctctgaatttgaaccaatcaacttgagaagccacaagccagaatattctaataagtttggcaagttgtttgagattactccggaaaaaaaatacccttaactttaagatttagatctatttgttagttgtgtggagattaacgagataagtacacaacactaaatatatataaaacatataattttaattatattacagaaatatgttaatgcgtttttgcttatatttttaaggagctctaatgttgccacactacaattcaagggctatagttgtactattggttaatgaaggaaaaggaaaccttgaacttctgggtttaaaaaatgagtaataagagagggaagatagaaaagaaagaaacaatgaggtgtagagatatgaagctagattgtctccgggtgacgttgttatcattccagcaggtcatccggttgccattactgcttcttcaaatttgaatttgcttggatttggtatcaatgctgagaacaatgagagaaactttctttcagatatttagtgaatattagtatgattacttaataagtctcggctaaatgagaattttttgaaattgatattttgattttggtgattgaaaatttgaaagctcggacgacaatgtgataagctaaattgaaaatccagtaaaagagcttacatttcctggatctgtttaagagataaatagactaataaagaactaaaagtaatctcactttgcaaatgctgaacctgaataaaaggagtaaggaagctagggaaaaaggagtcctctgtcttcaattttgggcactttttactaagtaatcagtatgaaaaataatacaacacgtatgtatgatgtaagtgttggataataaactatgaaaaataaggaggaaaatgtatgctgtaagatatagctagctcataatgagctaagaataaataaagggtcatgtaactcttgcttattgagtcccacctttctactatgaagaaataaataatgaataaaatttttgtctttttttaatttaaaagagtgtttgggcgctaaatttcttaac

SEQ ID NO: 22 - DNA, 2746 bp, synthetic construct
  source 1..2746: mol_type = other DNA
tatatggcacaatataaccaaatgtctatccacgttattcatctagctttatgttctatcactataaatatccttcatcttactcttttatttcatcatctaaacttttaactagtgaaatataaatcatggctaccactatcaaatcatgatttccacttttgttgttgctgggaattatattcctggcctctgttgtttgtgtcacttatgccaattacgatgaaggttcagaacctagggtaccggcataaagagagagaggtcgctaagagggtgagaaagaggaaaaacgccatggagaataaagaccttcctacgaaaaggaagaagatgaagaagagggataaagagaaagaggtcgctaagagggtgaaaaagaggaaaaacgccacggagaataaagaccttcgtatgaaaagtaagaagatgaagaagagaagtagaaatatagatattaacgtgaaaaggaagatgaagaagagaagtagaaatattaatattaacgtgaaaagaaggaacaaaaggaagtttaacctggacgtgagagataagaaagagaggaagatgaggaataagtagacgaagagtaaagaggaagttaacgtcgtgaagatcccgaagaaagggcaaggctaaggcatagagaggagagaacaaaaagagacagacgccattaacgtgaaggagaggaggaagaaagatcttcagagtcataagaatgaagaaatccctttttatttaagtctaacaagtttctaacactctttgaaaacgaaaacggccacattcgtctcctttaaaggttcgacaaacgttcagacttatttgaaaatctctaaaactatcgtcttgtggaatatagagccaaaccccacaccatcttccttccttaacacatagatgctgacttaatccttgtagtcctcagtgataatttttattttactttataatattattataacaaatctttttgttttatagaaatatgactatttaaaataaaaacattgtaaagttcaatttaacaatatttcttatatttcataattaaattttggtttggttaatatgtattacaaggaaagccatattgacagtgttgagtcccaatgatagaaattcgtataatcttgagcgtggtgataccatcaaacttcctgcaggaacaacctcttatttagttaactaagatgatgaagaagatcttagactggtagatcttgtaatacccgtgaatgggcctggtaaatttgagatactatataaaatacaataaatttttcttcagaagcgttattcttacaaaaacatccatttatattacttttacttttgtctataatgaaaaattgatattttccgttcttccatcaagcttttgacctagctaaaaataaaaactaatacttatgaggattcagcaagaatattttagaggcctcctataacataagtatgtgaagtttttatcattttttaataaataaaaccattttaatttgtatcattgtttacaactataaactagatacgagaccatagagaaggttctcttagaagaataagagaaagatcggaaaaggagataataaggggaagaaacagatgcaatagtcaaagtgtcaagggaataaattgaggaattgaaaaagcttgccaaatcaagctcaaagaaaagcttaccctctgaatttgaaccaatcaacttgagaagccacaagccagaatattctaataagtttggcaagttgtttgagattactccggaaaaaaaatacccttaactttaagatttagatctatttgttagttgtgtggagattaacgagataagtacacaacactaaatatatataaaacatataattttaattatattacagaaatatgttaatgcgtttttgcttatatttttaaggagctctaatgttgccacactacaattcaagggctatagttgtactattggttaatgaaggaaaaggaaaccttgaacttctgggtttaaaaaatgagtaataagagagggaagatagaaaagaaagaaacaatgaggtgtagagatatgaagctagattgtctccgggtgacgttgttatcattccagcaggtcatccggttgccattactgcttcttcaaatttgaatttgcttggatttggtatcaatgctgagaacaatgagagaaactttctttcagatatttagtgaatattagtatgattacttaataagtctcggctaaatgagaattttttgaaattgatattttgattttggtgattgaaaatttgaaagctcggacgacaatgtgataagctaaattgaaaatccagtaaaagagcttacatttcctggatctgtttaagagataaatagactaataaagaactaaaagtaatctcactttgcaaatgctgaacctgaataaaaggagtaaggaagctagggaaaaaggagtcctctgtcttcaattttgggcactttttactaagtaatcagtatgaaaaataatacaacacgtatgtatgatgtaagtgttggataataaactatgaaaaataaggaggaaaatgtatgctgtaagatatagctagctcataatgagctaagaataaataaagggtcatgtaactcttgcttattgagtcccacctttctactatgaagaaataaataatgaataaaatttttgtctttttttaatttaaaagagtgtttgggcgctaaatttcttaac

SEQ ID NO: 23 - DNA, 2746 bp, synthetic construct
  source 1..2746: mol_type = other DNA
tatatggcacaatataaccaaatgtctatccacgttattcatctagctttatgttctatcactataaatatccttcatcttactcttttatttcatcatctaaacttttaactagtgaaatataaatcatggctaccactatcaaatcatgatttccacttttgttgttgctgggaattatattcctggcctctgttgtttgtgtcacttatgccaattacgatgaaggttcagaacctagggtaccggcataaagagagagaggtcgctaagagggtgagaaagaggaaaaacgccatggagaataaagaccttcctacgaaaaggaagaagatgaagaagagggataaagagaaagaggtcgctaagagggtgaaaaagaggaaaaacgccacggagaataaagaccttcgtatgaaaagtaagaagatgaagaagagaagtagaaatatagatattaacgtgaaaaggaagatgaagaagagaagtagaaatattaatattaacgtgaaaagaaggaataaaaggaagttcaacctggacgtgagagataagaaagagaggaagatgaggaataagtagacgaagagtaaagaggaagttaacgtcgtgaagatcccgaagaaagggcaaggctaaggcatagagaggagagaacaaaaagagacagacgccattaacgtgaaggagaggaggaagaaagatcttcagagtcataagaatgaagaaatccctttttatttaagtctaacaagtttctaacactctttgaaaacgaaaacggccacattcgtctcctttaaaggttcgacaaacgttcagacttatttgaaaatctctaaaactatcgtcttgtggaatatagagccaaaccccacaccatcttccttccttaacacatagatgctgacttaatccttgtagtcctcagtgataatttttattttactttataatattattataacaaatctttttgttttatagaaatatgactatttaaaataaaaacattgtaaagttcaatttaacaatatttcttatatttcataattaaattttggtttggttaatatgtattacaaggaaagccatattgacagtgttgagtcccaatgatagaaattcgtataatcttgagcgtggtgataccatcaaacttcctgcaggaacaacctcttatttagttaactaagatgatgaagaagatcttagactggtagatcttgtaatacccgtgaatgggcctggtaaatttgagatactatataaaatacaataaatttttcttcagaagcgttattcttacaaaaacatccatttatattacttttacttttgtctataatgaaaaattgatattttccgttcttccatcaagcttttgacctagctaaaaataaaaactaatacttatgaggattcagcaagaatattttagaggcctcctataacataagtatgtgaagtttttatcattttttaataaataaaaccattttaatttgtatcattgtttacaactataaactagatacgagaccatagagaaggttctcttagaagaataagagaaagatcggaaaaggagataataaggggaagaaacagatgcaatagtcaaagtgtcaagggaataaattgaggaattgaaaaagcttgccaaatcaagctcaaagaaaagcttaccctctgaatttgaaccaatcaacttgagaagccacaagccagaatattctaataagtttggcaagttgtttgagattactccggaaaaaaaatacccttaactttaagatttagatctatttgttagttgtgtggagattaacgagataagtacacaacactaaatatatataaaacatataattttaattatattacagaaatatgttaatgcgtttttgcttatatttttaaggagctctaatgttgccacactacaattcaagggctatagttgtactattggttaatgaaggaaaaggaaaccttgaacttctgggtttaaaaaatgagtaataagagagggaagatagaaaagaaagaaacaatgaggtgtagagatatgaagctagattgtctccgggtgacgttgttatcattccagcaggtcatccggttgccattactgcttcttcaaatttgaatttgcttggatttggtatcaatgctgagaacaatgagagaaactttctttcagatatttagtgaatattagtatgattacttaataagtctcggctaaatgagaattttttgaaattgatattttgattttggtgattgaaaatttgaaagctcggacgacaatgtgataagctaaattgaaaatccagtaaaagagcttacatttcctggatctgtttaagagataaatagactaataaagaactaaaagtaatctcactttgcaaatgctgaacctgaataaaaggagtaaggaagctagggaaaaaggagtcctctgtcttcaattttgggcactttttactaagtaatcagtatgaaaaataatacaacacgtatgtatgatgtaagtgttggataataaactatgaaaaataaggaggaaaatgtatgctgtaagatatagctagctcataatgagctaagaataaataaagggtcatgtaactcttgcttattgagtcccacctttctactatgaagaaataaataatgaataaaatttttgtctttttttaatttaaaagagtgtttgggcgctaaatttcttaac

SEQ ID NO: 24 - DNA, 2746 bp, synthetic construct
  source 1..2746: mol_type = other DNA
tatatggcacaatataaccaaatgtctatccacgttattcatctagctttatgttctatcactataaatatccttcatcttactcttttatttcatcatctaaacttttaactagtgaaatataaatcatggctaccactatcaaatcatgatttccacttttgttgttgctgggaattatattcctggcctctgttgtttgtgtcacttatgccaattacgatgaaggttcagaacctagggtaccggcataaagagagagaggtcgctaagagggtgagaaagaggaaaaacgccatggagaataaagaccttcctacgaaaaggaagaagatgaagaagagggataaagagaaagaggtcgctaagagggtgaaaaagaggaaaaacgccacggagaataaagaccttcgtatgaaaagtaagaagatgaagaagagaagtagaaatatagatattaacgtgaaaaggaagatgaagaagagaagtagaaatattaatattaacgtgaaaagaaggaataaaaggaagtttaacctggacgtgagagatgagaaagagaggaagatgaggaataagtagacgaagagtaaagaggaagttaacgtcgtgaagatcccgaagaaagggcaaggctaaggcatagagaggagagaacaaaaagagacagacgccattaacgtgaaggagaggaggaagaaagatcttcagagtcataagaatgaagaaatccctttttatttaagtctaacaagtttctaacactctttgaaaacgaaaacggccacattcgtctcctttaaaggttcgacaaacgttcagacttatttgaaaatctctaaaactatcgtcttgtggaatatagagccaaaccccacaccatcttccttccttaacacatagatgctgacttaatccttgtagtcctcagtgataatttttattttactttataatattattataacaaatctttttgttttatagaaatatgactatttaaaataaaaacattgtaaagttcaatttaacaatatttcttatatttcataattaaattttggtttggttaatatgtattacaaggaaagccatattgacagtgttgagtcccaatgatagaaattcgtataatcttgagcgtggtgataccatcaaacttcctgcaggaacaacctcttatttagttaactaagatgatgaagaagatcttagactggtagatcttgtaatacccgtgaatgggcctggtaaatttgagatactatataaaatacaataaatttttcttcagaagcgttattcttacaaaaacatccatttatattacttttacttttgtctataatgaaaaattgatattttccgttcttccatcaagcttttgacctagctaaaaataaaaactaatacttatgaggattcagcaagaatattttagaggcctcctataacataagtatgtgaagtttttatcattttttaataaataaaaccattttaatttgtatcattgtttacaactataaactagatacgagaccatagagaaggttctcttagaagaataagagaaagatcggaaaaggagataataaggggaagaaacagatgcaatagtcaaagtgtcaagggaataaattgaggaattgaaaaagcttgccaaatcaagctcaaagaaaagcttaccctctgaatttgaaccaatcaacttgagaagccacaagccagaatattctaataagtttggcaagttgtttgagattactccggaaaaaaaatacccttaactttaagatttagatctatttgttagttgtgtggagattaacgagataagtacacaacactaaatatatataaaacatataattttaattatattacagaaatatgttaatgcgtttttgcttatatttttaaggagctctaatgttgccacactacaattcaagggctatagttgtactattggttaatgaaggaaaaggaaaccttgaacttctgggtttaaaaaatgagtaataagagagggaagatagaaaagaaagaaacaatgaggtgtagagatatgaagctagattgtctccgggtgacgttgttatcattccagcaggtcatccggttgccattactgcttcttcaaatttgaatttgcttggatttggtatcaatgctgagaacaatgagagaaactttctttcagatatttagtgaatattagtatgattacttaataagtctcggctaaatgagaattttttgaaattgatattttgattttggtgattgaaaatttgaaagctcggacgacaatgtgataagctaaattgaaaatccagtaaaagagcttacatttcctggatctgtttaagagataaatagactaataaagaactaaaagtaatctcactttgcaaatgctgaacctgaataaaaggagtaaggaagctagggaaaaaggagtcctctgtcttcaattttgggcactttttactaagtaatcagtatgaaaaataatacaacacgtatgtatgatgtaagtgttggataataaactatgaaaaataaggaggaaaatgtatgctgtaagatatagctagctcataatgagctaagaataaataaagggtcatgtaactcttgcttattgagtcccacctttctactatgaagaaataaataatgaataaaatttttgtctttttttaatttaaaagagtgtttgggcgctaaatttcttaac

SEQ ID NO: 25 - DNA, 2746 bp, synthetic construct
  source 1..2746: mol_type = other DNA
tatatggcacaatataaccaaatgtctatccacgttattcatctagctttatgttctatcactataaatatccttcatcttactcttttatttcatcatctaaacttttaactagtgaaatataaatcatggctaccactatcaaatcatgatttccacttttgttgttgctgggaattatattcctggcctctgttgtttgtgtcacttatgccaattacgatgaaggttcagaacctagggtaccggcataaagagagagaggtcgctaagagggtgagaaagaggaaaaacgccatggagaataaagaccttcctacgaaaaggaagaagatgaagaagagggataaagagaaagaggtcgctaagagggtgaaaaagaggaaaaacgccacggagaataaagaccttcgtatgaaaagtaagaagatgaagaagagaagtagaaatatagatattaacgtgaaaaggaagatgaagaagagaagtagaaatattaatattaacgtgaaaagaaggaataaaaggaagtttaacctggacgtgagagataggaaagagaggaagatgaggaataagtagacgaagagtaaagaggaagttaacgtcgtgaagatcccgaagaaagggcaaggctaaggcatagagaggagagaacaaaaagagacagacgccattaacgtgaaggagaggaggaagaaagatcttcagagtcataagaatgaagaaatccctttttatttaagtctaacaagtttctaacactctttgaaaacgaaaacggccacattcgtctcctttaaaggttcgacaaacgttcagacttatttgaaaatctctaaaactatcgtcttgtggaatatagagccaaaccccacaccatcttccttccttaacacatagatgctgacttaatccttgtagtcctcagtgataatttttattttactttataatattattataacaaatctttttgttttatagaaatatgactatttaaaataaaaacattgtaaagttcaatttaacaatatttcttatatttcataattaaattttggtttggttaatatgtattacaaggaaagccatattgacagtgttgagtcccaatgatagaaattcgtataatcttgagcgtggtgataccatcaaacttcctgcaggaacaacctcttatttagttaactaagatgatgaagaagatcttagactggtagatcttgtaatacccgtgaatgggcctggtaaatttgagatactatataaaatacaataaatttttcttcagaagcgttattcttacaaaaacatccatttatattacttttacttttgtctataatgaaaaattgatattttccgttcttccatcaagcttttgacctagctaaaaataaaaactaatacttatgaggattcagcaagaatattttagaggcctcctataacataagtatgtgaagtttttatcattttttaataaataaaaccattttaatttgtatcattgtttacaactataaactagatacgagaccatagagaaggttctcttagaagaataagagaaagatcggaaaaggagataataaggggaagaaacagatgcaatagtcaaagtgtcaagggaataaattgaggaattgaaaaagcttgccaaatcaagctcaaagaaaagcttaccctctgaatttgaaccaatcaacttgagaagccacaagccagaatattctaataagtttggcaagttgtttgagattactccggaaaaaaaatacccttaactttaagatttagatctatttgttagttgtgtggagattaacgagataagtacacaacactaaatatatataaaacatataattttaattatattacagaaatatgttaatgcgtttttgcttatatttttaaggagctctaatgttgccacactacaattcaagggctatagttgtactattggttaatgaaggaaaaggaaaccttgaacttctgggtttaaaaaatgagtaataagagagggaagatagaaaagaaagaaacaatgaggtgtagagatatgaagctagattgtctccgggtgacgttgttatcattccagcaggtcatccggttgccattactgcttcttcaaatttgaatttgcttggatttggtatcaatgctgagaacaatgagagaaactttctttcagatatttagtgaatattagtatgattacttaataagtctcggctaaatgagaattttttgaaattgatattttgattttggtgattgaaaatttgaaagctcggacgacaatgtgataagctaaattgaaaatccagtaaaagagcttacatttcctggatctgtttaagagataaatagactaataaagaactaaaagtaatctcactttgcaaatgctgaacctgaataaaaggagtaaggaagctagggaaaaaggagtcctctgtcttcaattttgggcactttttactaagtaatcagtatgaaaaataatacaacacgtatgtatgatgtaagtgttggataataaactatgaaaaataaggaggaaaatgtatgctgtaagatatagctagctcataatgagctaagaataaataaagggtcatgtaactcttgcttattgagtcccacctttctactatgaagaaataaataatgaataaaatttttgtctttttttaatttaaaagagtgtttgggcgctaaatttcttaac

SEQ ID NO: 26 - DNA, 2746 bp, synthetic construct
  source 1..2746: mol_type = other DNA
tatatggcacaatataaccaaatgtctatccacgttattcatctagctttatgttctatcactataaatatccttcatcttactcttttatttcatcatctaaacttttaactagtgaaatataaatcatggctaccactatcaaatcatgatttccacttttgttgttgctgggaattatattcctggcctctgttgtttgtgtcacttatgccaattacgatgaaggttcagaacctagggtaccggcataaagagagagaggtcgctaagagggtgagaaagaggaaaaacgccatggagaataaagaccttcctacgaaaaggaagaagatgaagaagagggataaagagaaagaggtcgctaagagggtgaaaaagaggaaaaacgccacggagaataaagaccttcgtatgaaaagtaagaagatgaagaagagaagtagaaatatagatattaacgtgaaaaggaagatgaagaagagaagtagaaatattaatattaacgtgaaaagaaggaataaaaggaagtttaacctggacgtgagagataagaaagagaggaagatgaggaacaagtagacgaagagtaaagaggaagttaacgtcgtgaagatcccgaagaaagggcaaggctaaggcatagagaggagagaacaaaaagagacagacgccattaacgtgaaggagaggaggaagaaagatcttcagagtcataagaatgaagaaatccctttttatttaagtctaacaagtttctaacactctttgaaaacgaaaacggccacattcgtctcctttaaaggttcgacaaacgttcagacttatttgaaaatctctaaaactatcgtcttgtggaatatagagccaaaccccacaccatcttccttccttaacacatagatgctgacttaatccttgtagtcctcagtgataatttttattttactttataatattattataacaaatctttttgttttatagaaatatgactatttaaaataaaaacattgtaaagttcaatttaacaatatttcttatatttcataattaaattttggtttggttaatatgtattacaaggaaagccatattgacagtgttgagtcccaatgatagaaattcgtataatcttgagcgtggtgataccatcaaacttcctgcaggaacaacctcttatttagttaactaagatgatgaagaagatcttagactggtagatcttgtaatacccgtgaatgggcctggtaaatttgagatactatataaaatacaataaatttttcttcagaagcgttattcttacaaaaacatccatttatattacttttacttttgtctataatgaaaaattgatattttccgttcttccatcaagcttttgacctagctaaaaataaaaactaatacttatgaggattcagcaagaatattttagaggcctcctataacataagtatgtgaagtttttatcattttttaataaataaaaccattttaatttgtatcattgtttacaactataaactagatacgagaccatagagaaggttctcttagaagaataagagaaagatcggaaaaggagataataaggggaagaaacagatgcaatagtcaaagtgtcaagggaataaattgaggaattgaaaaagcttgccaaatcaagctcaaagaaaagcttaccctctgaatttgaaccaatcaacttgagaagccacaagccagaatattctaataagtttggcaagttgtttgagattactccggaaaaaaaatacccttaactttaagatttagatctatttgttagttgtgtggagattaacgagataagtacacaacactaaatatatataaaacatataattttaattatattacagaaatatgttaatgcgtttttgcttatatttttaaggagctctaatgttgccacactacaattcaagggctatagttgtactattggttaatgaaggaaaaggaaaccttgaacttctgggtttaaaaaatgagtaataagagagggaagatagaaaagaaagaaacaatgaggtgtagagatatgaagctagattgtctccgggtgacgttgttatcattccagcaggtcatccggttgccattactgcttcttcaaatttgaatttgcttggatttggtatcaatgctgagaacaatgagagaaactttctttcagatatttagtgaatattagtatgattacttaataagtctcggctaaatgagaattttttgaaattgatattttgattttggtgattgaaaatttgaaagctcggacgacaatgtgataagctaaattgaaaatccagtaaaagagcttacatttcctggatctgtttaagagataaatagactaataaagaactaaaagtaatctcactttgcaaatgctgaacctgaataaaaggagtaaggaagctagggaaaaaggagtcctctgtcttcaattttgggcactttttactaagtaatcagtatgaaaaataatacaacacgtatgtatgatgtaagtgttggataataaactatgaaaaataaggaggaaaatgtatgctgtaagatatagctagctcataatgagctaagaataaataaagggtcatgtaactcttgcttattgagtcccacctttctactatgaagaaataaataatgaataaaatttttgtctttttttaatttaaaagagtgtttgggcgctaaatttcttaac

SEQ ID NO: 27 - DNA, 2746 bp, synthetic construct
  source 1..2746: mol_type = other DNA
tatatggcacaatataaccaaatgtctatccacgttattcatctagctttatgttctatcactataaatatccttcatcttactcttttatttcatcatctaaacttttaactagtgaaatataaatcatggctaccactatcaaatcatgatttccacttttgttgttgctgggaattatattcctggcctctgttgtttgtgtcacttatgccaattacgatgaaggttcagaacctagggtaccggcataaagagagagaggtcgctaagagggtgagaaagaggaaaaacgccatggagaataaagaccttcctacgaaaaggaagaagatgaagaagagggataaagagaaagaggtcgctaagagggtgaaaaagaggaaaaacgccacggagaataaagaccttcgtatgaaaagtaagaagatgaagaagagaagtagaaatatagatattaacgtgaaaaggaagatgaagaagagaagtagaaatattaatattaacgtgaaaagaaggaataaaaggaagtttaacctggacgtgagagataagaaagagaggaagatgaggaataagtagacgaagagtgaagaggaagttaacgtcgtgaagatcccgaagaaagggcaaggctaaggcatagagaggagagaacaaaaagagacagacgccattaacgtgaaggagaggaggaagaaagatcttcagagtcataagaatgaagaaatccctttttatttaagtctaacaagtttctaacactctttgaaaacgaaaacggccacattcgtctcctttaaaggttcgacaaacgttcagacttatttgaaaatctctaaaactatcgtcttgtggaatatagagccaaaccccacaccatcttccttccttaacacatagatgctgacttaatccttgtagtcctcagtgataatttttattttactttataatattattataacaaatctttttgttttatagaaatatgactatttaaaataaaaacattgtaaagttcaatttaacaatatttcttatatttcataattaaattttggtttggttaatatgtattacaaggaaagccatattgacagtgttgagtcccaatgatagaaattcgtataatcttgagcgtggtgataccatcaaacttcctgcaggaacaacctcttatttagttaactaagatgatgaagaagatcttagactggtagatcttgtaatacccgtgaatgggcctggtaaatttgagatactatataaaatacaataaatttttcttcagaagcgttattcttacaaaaacatccatttatattacttttacttttgtctataatgaaaaattgatattttccgttcttccatcaagcttttgacctagctaaaaataaaaactaatacttatgaggattcagcaagaatattttagaggcctcctataacataagtatgtgaagtttttatcattttttaataaataaaaccattttaatttgtatcattgtttacaactataaactagatacgagaccatagagaaggttctcttagaagaataagagaaagatcggaaaaggagataataaggggaagaaacagatgcaatagtcaaagtgtcaagggaataaattgaggaattgaaaaagcttgccaaatcaagctcaaagaaaagcttaccctctgaatttgaaccaatcaacttgagaagccacaagccagaatattctaataagtttggcaagttgtttgagattactccggaaaaaaaatacccttaactttaagatttagatctatttgttagttgtgtggagattaacgagataagtacacaacactaaatatatataaaacatataattttaattatattacagaaatatgttaatgcgtttttgcttatatttttaaggagctctaatgttgccacactacaattcaagggctatagttgtactattggttaatgaaggaaaaggaaaccttgaacttctgggtttaaaaaatgagtaataagagagggaagatagaaaagaaagaaacaatgaggtgtagagatatgaagctagattgtctccgggtgacgttgttatcattccagcaggtcatccggttgccattactgcttcttcaaatttgaatttgcttggatttggtatcaatgctgagaacaatgagagaaactttctttcagatatttagtgaatattagtatgattacttaataagtctcggctaaatgagaattttttgaaattgatattttgattttggtgattgaaaatttgaaagctcggacgacaatgtgataagctaaattgaaaatccagtaaaagagcttacatttcctggatctgtttaagagataaatagactaataaagaactaaaagtaatctcactttgcaaatgctgaacctgaataaaaggagtaaggaagctagggaaaaaggagtcctctgtcttcaattttgggcactttttactaagtaatcagtatgaaaaataatacaacacgtatgtatgatgtaagtgttggataataaactatgaaaaataaggaggaaaatgtatgctgtaagatatagctagctcataatgagctaagaataaataaagggtcatgtaactcttgcttattgagtcccacctttctactatgaagaaataaataatgaataaaatttttgtctttttttaatttaaaagagtgtttgggcgctaaatttcttaac

SEQ ID NO: 28 - DNA, 2746 bp, synthetic construct
  source 1..2746: mol_type = other DNA
tatatggcacaatataaccaaatgtctatccacgttattcatctagctttatgttctatcactataaatatccttcatcttactcttttatttcatcatctaaacttttaactagtgaaatataaatcatggctaccactatcaaatcatgatttccacttttgttgttgctgggaattatattcctggcctctgttgtttgtgtcacttatgccaattacgatgaaggttcagaacctagggtaccggcataaagagagagaggtcgctaagagggtgagaaagaggaaaaacgccatggagaataaagaccttcctacgaaaaggaagaagatgaagaagagggataaagagaaagaggtcgctaagagggtgaaaaagaggaaaaacgccacggagaataaagaccttcgtatgaaaagtaagaagatgaagaagagaagtagaaatatagatattaacgtgaaaaggaagatgaagaagagaagtagaaatattaatattaacgtgaaaagaaggaataaaaggaagtttaacctggacgtgagagataagaaagagaggaagatgaggaataagtagacgaagagtagagaggaagttaacgtcgtgaagatcccgaagaaagggcaaggctaaggcatagagaggagagaacaaaaagagacagacgccattaacgtgaaggagaggaggaagaaagatcttcagagtcataagaatgaagaaatccctttttatttaagtctaacaagtttctaacactctttgaaaacgaaaacggccacattcgtctcctttaaaggttcgacaaacgttcagacttatttgaaaatctctaaaactatcgtcttgtggaatatagagccaaaccccacaccatcttccttccttaacacatagatgctgacttaatccttgtagtcctcagtgataatttttattttactttataatattattataacaaatctttttgttttatagaaatatgactatttaaaataaaaacattgtaaagttcaatttaacaatatttcttatatttcataattaaattttggtttggttaatatgtattacaaggaaagccatattgacagtgttgagtcccaatgatagaaattcgtataatcttgagcgtggtgataccatcaaacttcctgcaggaacaacctcttatttagttaactaagatgatgaagaagatcttagactggtagatcttgtaatacccgtgaatgggcctggtaaatttgagatactatataaaatacaataaatttttcttcagaagcgttattcttacaaaaacatccatttatattacttttacttttgtctataatgaaaaattgatattttccgttcttccatcaagcttttgacctagctaaaaataaaaactaatacttatgaggattcagcaagaatattttagaggcctcctataacataagtatgtgaagtttttatcattttttaataaataaaaccattttaatttgtatcattgtttacaactataaactagatacgagaccatagagaaggttctcttagaagaataagagaaagatcggaaaaggagataataaggggaagaaacagatgcaatagtcaaagtgtcaagggaataaattgaggaattgaaaaagcttgccaaatcaagctcaaagaaaagcttaccctctgaatttgaaccaatcaacttgagaagccacaagccagaatattctaataagtttggcaagttgtttgagattactccggaaaaaaaatacccttaactttaagatttagatctatttgttagttgtgtggagattaacgagataagtacacaacactaaatatatataaaacatataattttaattatattacagaaatatgttaatgcgtttttgcttatatttttaaggagctctaatgttgccacactacaattcaagggctatagttgtactattggttaatgaaggaaaaggaaaccttgaacttctgggtttaaaaaatgagtaataagagagggaagatagaaaagaaagaaacaatgaggtgtagagatatgaagctagattgtctccgggtgacgttgttatcattccagcaggtcatccggttgccattactgcttcttcaaatttgaatttgcttggatttggtatcaatgctgagaacaatgagagaaactttctttcagatatttagtgaatattagtatgattacttaataagtctcggctaaatgagaattttttgaaattgatattttgattttggtgattgaaaatttgaaagctcggacgacaatgtgataagctaaattgaaaatccagtaaaagagcttacatttcctggatctgtttaagagataaatagactaataaagaactaaaagtaatctcactttgcaaatgctgaacctgaataaaaggagtaaggaagctagggaaaaaggagtcctctgtcttcaattttgggcactttttactaagtaatcagtatgaaaaataatacaacacgtatgtatgatgtaagtgttggataataaactatgaaaaataaggaggaaaatgtatgctgtaagatatagctagctcataatgagctaagaataaataaagggtcatgtaactcttgcttattgagtcccacctttctactatgaagaaataaataatgaataaaatttttgtctttttttaatttaaaagagtgtttgggcgctaaatttcttaac

SEQ ID NO: 29 - DNA, 2746 bp, synthetic construct
  source 1..2746: mol_type = other DNA
tatatggcacaatataaccaaatgtctatccacgttattcatctagctttatgttctatcactataaatatccttcatcttactcttttatttcatcatctaaacttttaactagtgaaatataaatcatggctaccactatcaaatcatgatttccacttttgttgttgctgggaattatattcctggcctctgttgtttgtgtcacttatgccaattacgatgaaggttcagaacctagggtaccggcataaagagagagaggtcgctaagagggtgagaaagaggaaaaacgccatggagaataaagaccttcctacgaaaaggaagaagatgaagaagagggataaagagaaagaggtcgctaagagggtgaaaaagaggaaaaacgccacggagaataaagaccttcgtatgaaaagtaagaagatgaagaagagaagtagaaatatagatattaacgtgaaaaggaagatgaagaagagaagtagaaatattaatattaacgtgaaaagaaggaataaaaggaagtttaacctggacgtgagagataagaaagagaggaagatgaggaataagtagacgaagagtaaagaggaagtcaacgtcgtgaagatcccgaagaaagggcaaggctaaggcatagagaggagagaacaaaaagagacagacgccattaacgtgaaggagaggaggaagaaagatcttcagagtcataagaatgaagaaatccctttttatttaagtctaacaagtttctaacactctttgaaaacgaaaacggccacattcgtctcctttaaaggttcgacaaacgttcagacttatttgaaaatctctaaaactatcgtcttgtggaatatagagccaaaccccacaccatcttccttccttaacacatagatgctgacttaatccttgtagtcctcagtgataatttttattttactttataatattattataacaaatctttttgttttatagaaatatgactatttaaaataaaaacattgtaaagttcaatttaacaatatttcttatatttcataattaaattttggtttggttaatatgtattacaaggaaagccatattgacagtgttgagtcccaatgatagaaattcgtataatcttgagcgtggtgataccatcaaacttcctgcaggaacaacctcttatttagttaactaagatgatgaagaagatcttagactggtagatcttgtaatacccgtgaatgggcctggtaaatttgagatactatataaaatacaataaatttttcttcagaagcgttattcttacaaaaacatccatttatattacttttacttttgtctataatgaaaaattgatattttccgttcttccatcaagcttttgacctagctaaaaataaaaactaatacttatgaggattcagcaagaatattttagaggcctcctataacataagtatgtgaagtttttatcattttttaataaataaaaccattttaatttgtatcattgtttacaactataaactagatacgagaccatagagaaggttctcttagaagaataagagaaagatcggaaaaggagataataaggggaagaaacagatgcaatagtcaaagtgtcaagggaataaattgaggaattgaaaaagcttgccaaatcaagctcaaagaaaagcttaccctctgaatttgaaccaatcaacttgagaagccacaagccagaatattctaataagtttggcaagttgtttgagattactccggaaaaaaaatacccttaactttaagatttagatctatttgttagttgtgtggagattaacgagataagtacacaacactaaatatatataaaacatataattttaattatattacagaaatatgttaatgcgtttttgcttatatttttaaggagctctaatgttgccacactacaattcaagggctatagttgtactattggttaatgaaggaaaaggaaaccttgaacttctgggtttaaaaaatgagtaataagagagggaagatagaaaagaaagaaacaatgaggtgtagagatatgaagctagattgtctccgggtgacgttgttatcattccagcaggtcatccggttgccattactgcttcttcaaatttgaatttgcttggatttggtatcaatgctgagaacaatgagagaaactttctttcagatatttagtgaatattagtatgattacttaataagtctcggctaaatgagaattttttgaaattgatattttgattttggtgattgaaaatttgaaagctcggacgacaatgtgataagctaaattgaaaatccagtaaaagagcttacatttcctggatctgtttaagagataaatagactaataaagaactaaaagtaatctcactttgcaaatgctgaacctgaataaaaggagtaaggaagctagggaaaaaggagtcctctgtcttcaattttgggcactttttactaagtaatcagtatgaaaaataatacaacacgtatgtatgatgtaagtgttggataataaactatgaaaaataaggaggaaaatgtatgctgtaagatatagctagctcataatgagctaagaataaataaagggtcatgtaactcttgcttattgagtcccacctttctactatgaagaaataaataatgaataaaatttttgtctttttttaatttaaaagagtgtttgggcgctaaatttcttaac

SEQ ID NO: 30 - DNA, 2746 bp, synthetic construct
  source 1..2746: mol_type = other DNA
tatatggcacaatataaccaaatgtctatccacgttattcatctagctttatgttctatcactataaatatccttcatcttactcttttatttcatcatctaaacttttaactagtgaaatataaatcatggctaccactatcaaatcatgatttccacttttgttgttgctgggaattatattcctggcctctgttgtttgtgtcacttatgccaattacgatgaaggttcagaacctagggtaccggcataaagagagagaggtcgctaagagggtgagaaagaggaaaaacgccatggagaataaagaccttcctacgaaaaggaagaagatgaagaagagggataaagagaaagaggtcgctaagagggtgaaaaagaggaaaaacgccacggagaataaagaccttcgtatgaaaagtaagaagatgaagaagagaagtagaaatatagatattaacgtgaaaaggaagatgaagaagagaagtagaaatattaatattaacgtgaaaagaaggaataaaaggaagtttaacctggacgtgagagataagaaagagaggaagatgaggaataagtagacgaagagtaaagaggaagttaacgtcgtgaagatcccgaagaaagggcaaggctaaggcatagagaggagagaacaaaaagagacagacgccatcaacgtgaaggagaggaggaagaaagatcttcagagtcataagaatgaagaaatccctttttatttaagtctaacaagtttctaacactctttgaaaacgaaaacggccacattcgtctcctttaaaggttcgacaaacgttcagacttatttgaaaatctctaaaactatcgtcttgtggaatatagagccaaaccccacaccatcttccttccttaacacatagatgctgacttaatccttgtagtcctcagtgataatttttattttactttataatattattataacaaatctttttgttttatagaaatatgactatttaaaataaaaacattgtaaagttcaatttaacaatatttcttatatttcataattaaattttggtttggttaatatgtattacaaggaaagccatattgacagtgttgagtcccaatgatagaaattcgtataatcttgagcgtggtgataccatcaaacttcctgcaggaacaacctcttatttagttaactaagatgatgaagaagatcttagactggtagatcttgtaatacccgtgaatgggcctggtaaatttgagatactatataaaatacaataaatttttcttcagaagcgttattcttacaaaaacatccatttatattacttttacttttgtctataatgaaaaattgatattttccgttcttccatcaagcttttgacctagctaaaaataaaaactaatacttatgaggattcagcaagaatattttagaggcctcctataacataagtatgtgaagtttttatcattttttaataaataaaaccattttaatttgtatcattgtttacaactataaactagatacgagaccatagagaaggttctcttagaagaataagagaaagatcggaaaaggagataataaggggaagaaacagatgcaatagtcaaagtgtcaagggaataaattgaggaattgaaaaagcttgccaaatcaagctcaaagaaaagcttaccctctgaatttgaaccaatcaacttgagaagccacaagccagaatattctaataagtttggcaagttgtttgagattactccggaaaaaaaatacccttaactttaagatttagatctatttgttagttgtgtggagattaacgagataagtacacaacactaaatatatataaaacatataattttaattatattacagaaatatgttaatgcgtttttgcttatatttttaaggagctctaatgttgccacactacaattcaagggctatagttgtactattggttaatgaaggaaaaggaaaccttgaacttctgggtttaaaaaatgagtaataagagagggaagatagaaaagaaagaaacaatgaggtgtagagatatgaagctagattgtctccgggtgacgttgttatcattccagcaggtcatccggttgccattactgcttcttcaaatttgaatttgcttggatttggtatcaatgctgagaacaatgagagaaactttctttcagatatttagtgaatattagtatgattacttaataagtctcggctaaatgagaattttttgaaattgatattttgattttggtgattgaaaatttgaaagctcggacgacaatgtgataagctaaattgaaaatccagtaaaagagcttacatttcctggatctgtttaagagataaatagactaataaagaactaaaagtaatctcactttgcaaatgctgaacctgaataaaaggagtaaggaagctagggaaaaaggagtcctctgtcttcaattttgggcactttttactaagtaatcagtatgaaaaataatacaacacgtatgtatgatgtaagtgttggataataaactatgaaaaataaggaggaaaatgtatgctgtaagatatagctagctcataatgagctaagaataaataaagggtcatgtaactcttgcttattgagtcccacctttctactatgaagaaataaataatgaataaaatttttgtctttttttaatttaaaagagtgtttgggcgctaaatttcttaac

SEQ ID NO: 31 - DNA, 2746 bp, synthetic construct
  source 1..2746: mol_type = other DNA
tatatggcacaatataaccaaatgtctatccacgttattcatctagctttatgttctatcactataaatatccttcatcttactcttttatttcatcatctaaacttttaactagtgaaatataaatcatggctaccactatcaaatcatgatttccacttttgttgttgctgggaattatattcctggcctctgttgtttgtgtcacttatgccaattacgatgaaggttcagaacctagggtaccggcataaagagagagaggtcgctaagagggtgagaaagaggaaaaacgccatggagaataaagaccttcctacgaaaaggaagaagatgaagaagagggataaagagaaagaggtcgctaagagggtgaaaaagaggaaaaacgccacggagaataaagaccttcgtatgaaaagtaagaagatgaagaagagaagtagaaatatagatattaacgtgaaaaggaagatgaagaagagaagtagaaatattaatattaacgtgaaaagaaggaataaaaggaagtttaacctggacgtgagagataagaaagagaggaagatgaggaataagtagacgaagagtaaagaggaagttaacgtcgtgaagatcccgaagaaagggcaaggctaaggcatagagaggagagaacaaaaagagacagacgccattaacgtgaaggagaggaggaagaaagatcttcagagtcacaagaatgaagaaatccctttttatttaagtctaacaagtttctaacactctttgaaaacgaaaacggccacattcgtctcctttaaaggttcgacaaacgttcagacttatttgaaaatctctaaaactatcgtcttgtggaatatagagccaaaccccacaccatcttccttccttaacacatagatgctgacttaatccttgtagtcctcagtgataatttttattttactttataatattattataacaaatctttttgttttatagaaatatgactatttaaaataaaaacattgtaaagttcaatttaacaatatttcttatatttcataattaaattttggtttggttaatatgtattacaaggaaagccatattgacagtgttgagtcccaatgatagaaattcgtataatcttgagcgtggtgataccatcaaacttcctgcaggaacaacctcttatttagttaactaagatgatgaagaagatcttagactggtagatcttgtaatacccgtgaatgggcctggtaaatttgagatactatataaaatacaataaatttttcttcagaagcgttattcttacaaaaacatccatttatattacttttacttttgtctataatgaaaaattgatattttccgttcttccatcaagcttttgacctagctaaaaataaaaactaatacttatgaggattcagcaagaatattttagaggcctcctataacataagtatgtgaagtttttatcattttttaataaataaaaccattttaatttgtatcattgtttacaactataaactagatacgagaccatagagaaggttctcttagaagaataagagaaagatcggaaaaggagataataaggggaagaaacagatgcaatagtcaaagtgtcaagggaataaattgaggaattgaaaaagcttgccaaatcaagctcaaagaaaagcttaccctctgaatttgaaccaatcaacttgagaagccacaagccagaatattctaataagtttggcaagttgtttgagattactccggaaaaaaaatacccttaactttaagatttagatctatttgttagttgtgtggagattaacgagataagtacacaacactaaatatatataaaacatataattttaattatattacagaaatatgttaatgcgtttttgcttatatttttaaggagctctaatgttgccacactacaattcaagggctatagttgtactattggttaatgaaggaaaaggaaaccttgaacttctgggtttaaaaaatgagtaataagagagggaagatagaaaagaaagaaacaatgaggtgtagagatatgaagctagattgtctccgggtgacgttgttatcattccagcaggtcatccggttgccattactgcttcttcaaatttgaatttgcttggatttggtatcaatgctgagaacaatgagagaaactttctttcagatatttagtgaatattagtatgattacttaataagtctcggctaaatgagaattttttgaaattgatattttgattttggtgattgaaaatttgaaagctcggacgacaatgtgataagctaaattgaaaatccagtaaaagagcttacatttcctggatctgtttaagagataaatagactaataaagaactaaaagtaatctcactttgcaaatgctgaacctgaataaaaggagtaaggaagctagggaaaaaggagtcctctgtcttcaattttgggcactttttactaagtaatcagtatgaaaaataatacaacacgtatgtatgatgtaagtgttggataataaactatgaaaaataaggaggaaaatgtatgctgtaagatatagctagctcataatgagctaagaataaataaagggtcatgtaactcttgcttattgagtcccacctttctactatgaagaaataaataatgaataaaatttttgtctttttttaatttaaaagagtgtttgggcgctaaatttcttaac

SEQ ID NO: 32 - DNA, 2746 bp, synthetic construct
  source 1..2746: mol_type = other DNA
tatatggcacaatataaccaaatgtctatccacgttattcatctagctttatgttctatcactataaatatccttcatcttactcttttatttcatcatctaaacttttaactagtgaaatataaatcatggctaccactatcaaatcatgatttccacttttgttgttgctgggaattatattcctggcctctgttgtttgtgtcacttatgccaattacgatgaaggttcagaacctagggtaccggcataaagagagagaggtcgctaagagggtgagaaagaggaaaaacgccatggagaataaagaccttcctacgaaaaggaagaagatgaagaagagggataaagagaaagaggtcgctaagagggtgaaaaagaggaaaaacgccacggagaataaagaccttcgtatgaaaagtaagaagatgaagaagagaagtagaaatatagatattaacgtgaaaaggaagatgaagaagagaagtagaaatattaatattaacgtgaaaagaaggaataaaaggaagtttaacctggacgtgagagataagaaagagaggaagatgaggaataagtagacgaagagtaaagaggaagttaacgtcgtgaagatcccgaagaaagggcaaggctaaggcatagagaggagagaacaaaaagagacagacgccattaacgtgaaggagaggaggaagaaagatcttcagagtcataagaacgaagaaatccctttttatttaagtctaacaagtttctaacactctttgaaaacgaaaacggccacattcgtctcctttaaaggttcgacaaacgttcagacttatttgaaaatctctaaaactatcgtcttgtggaatatagagccaaaccccacaccatcttccttccttaacacatagatgctgacttaatccttgtagtcctcagtgataatttttattttactttataatattattataacaaatctttttgttttatagaaatatgactatttaaaataaaaacattgtaaagttcaatttaacaatatttcttatatttcataattaaattttggtttggttaatatgtattacaaggaaagccatattgacagtgttgagtcccaatgatagaaattcgtataatcttgagcgtggtgataccatcaaacttcctgcaggaacaacctcttatttagttaactaagatgatgaagaagatcttagactggtagatcttgtaatacccgtgaatgggcctggtaaatttgagatactatataaaatacaataaatttttcttcagaagcgttattcttacaaaaacatccatttatattacttttacttttgtctataatgaaaaattgatattttccgttcttccatcaagcttttgacctagctaaaaataaaaactaatacttatgaggattcagcaagaatattttagaggcctcctataacataagtatgtgaagtttttatcattttttaataaataaaaccattttaatttgtatcattgtttacaactataaactagatacgagaccatagagaaggttctcttagaagaataagagaaagatcggaaaaggagataataaggggaagaaacagatgcaatagtcaaagtgtcaagggaataaattgaggaattgaaaaagcttgccaaatcaagctcaaagaaaagcttaccctctgaatttgaaccaatcaacttgagaagccacaagccagaatattctaataagtttggcaagttgtttgagattactccggaaaaaaaatacccttaactttaagatttagatctatttgttagttgtgtggagattaacgagataagtacacaacactaaatatatataaaacatataattttaattatattacagaaatatgttaatgcgtttttgcttatatttttaaggagctctaatgttgccacactacaattcaagggctatagttgtactattggttaatgaaggaaaaggaaaccttgaacttctgggtttaaaaaatgagtaataagagagggaagatagaaaagaaagaaacaatgaggtgtagagatatgaagctagattgtctccgggtgacgttgttatcattccagcaggtcatccggttgccattactgcttcttcaaatttgaatttgcttggatttggtatcaatgctgagaacaatgagagaaactttctttcagatatttagtgaatattagtatgattacttaataagtctcggctaaatgagaattttttgaaattgatattttgattttggtgattgaaaatttgaaagctcggacgacaatgtgataagctaaattgaaaatccagtaaaagagcttacatttcctggatctgtttaagagataaatagactaataaagaactaaaagtaatctcactttgcaaatgctgaacctgaataaaaggagtaaggaagctagggaaaaaggagtcctctgtcttcaattttgggcactttttactaagtaatcagtatgaaaaataatacaacacgtatgtatgatgtaagtgttggataataaactatgaaaaataaggaggaaaatgtatgctgtaagatatagctagctcataatgagctaagaataaataaagggtcatgtaactcttgcttattgagtcccacctttctactatgaagaaataaataatgaataaaatttttgtctttttttaatttaaaagagtgtttgggcgctaaatttcttaac

SEQ ID NO: 33 - DNA, 2746 bp, synthetic construct
  source 1..2746: mol_type = other DNA
tatatggcacaatataaccaaatgtctatccacgttattcatctagctttatgttctatcactataaatatccttcatcttactcttttatttcatcatctaaacttttaactagtgaaatataaatcatggctaccactatcaaatcatgatttccacttttgttgttgctgggaattatattcctggcctctgttgtttgtgtcacttatgccaattacgatgaaggttcagaacctagggtaccggcataaagagagagaggtcgctaagagggtgagaaagaggaaaaacgccatggagaataaagaccttcctacgaaaaggaagaagatgaagaagagggataaagagaaagaggtcgctaagagggtgaaaaagaggaaaaacgccacggagaataaagaccttcgtatgaaaagtaagaagatgaagaagagaagtagaaatatagatattaacgtgaaaaggaagatgaagaagagaagtagaaatattaatattaacgtgaaaagaaggaataaaaggaagtttaacctggacgtgagagataagaaagagaggaagatgaggaataagtagacgaagagtaaagaggaagttaacgtcgtgaagatcccgaagaaagggcaaggctaaggcatagagaggagagaacaaaaagagacagacgccattaacgtgaaggagaggaggaagaaagatcttcagagtcataagaatgaagaaatccctttttatttaagtctaacaagtttctaacactctttgaaaacgaaaacggccacattcgtctccttcaaaggttcgacaaacgttcagacttatttgaaaatctctaaaactatcgtcttgtggaatatagagccaaaccccacaccatcttccttccttaacacatagatgctgacttaatccttgtagtcctcagtgataatttttattttactttataatattattataacaaatctttttgttttatagaaatatgactatttaaaataaaaacattgtaaagttcaatttaacaatatttcttatatttcataattaaattttggtttggttaatatgtattacaaggaaagccatattgacagtgttgagtcccaatgatagaaattcgtataatcttgagcgtggtgataccatcaaacttcctgcaggaacaacctcttatttagttaactaagatgatgaagaagatcttagactggtagatcttgtaatacccgtgaatgggcctggtaaatttgagatactatataaaatacaataaatttttcttcagaagcgttattcttacaaaaacatccatttatattacttttacttttgtctataatgaaaaattgatattttccgttcttccatcaagcttttgacctagctaaaaataaaaactaatacttatgaggattcagcaagaatattttagaggcctcctataacataagtatgtgaagtttttatcattttttaataaataaaaccattttaatttgtatcattgtttacaactataaactagatacgagaccatagagaaggttctcttagaagaataagagaaagatcggaaaaggagataataaggggaagaaacagatgcaatagtcaaagtgtcaagggaataaattgaggaattgaaaaagcttgccaaatcaagctcaaagaaaagcttaccctctgaatttgaaccaatcaacttgagaagccacaagccagaatattctaataagtttggcaagttgtttgagattactccggaaaaaaaatacccttaactttaagatttagatctatttgttagttgtgtggagattaacgagataagtacacaacactaaatatatataaaacatataattttaattatattacagaaatatgttaatgcgtttttgcttatatttttaaggagctctaatgttgccacactacaattcaagggctatagttgtactattggttaatgaaggaaaaggaaaccttgaacttctgggtttaaaaaatgagtaataagagagggaagatagaaaagaaagaaacaatgaggtgtagagatatgaagctagattgtctccgggtgacgttgttatcattccagcaggtcatccggttgccattactgcttcttcaaatttgaatttgcttggatttggtatcaatgctgagaacaatgagagaaactttctttcagatatttagtgaatattagtatgattacttaataagtctcggctaaatgagaattttttgaaattgatattttgattttggtgattgaaaatttgaaagctcggacgacaatgtgataagctaaattgaaaatccagtaaaagagcttacatttcctggatctgtttaagagataaatagactaataaagaactaaaagtaatctcactttgcaaatgctgaacctgaataaaaggagtaaggaagctagggaaaaaggagtcctctgtcttcaattttgggcactttttactaagtaatcagtatgaaaaataatacaacacgtatgtatgatgtaagtgttggataataaactatgaaaaataaggaggaaaatgtatgctgtaagatatagctagctcataatgagctaagaataaataaagggtcatgtaactcttgcttattgagtcccacctttctactatgaagaaataaataatgaataaaatttttgtctttttttaatttaaaagagtgtttgggcgctaaatttcttaac

SEQ ID NO: 34 - DNA, 2746 bp, synthetic construct
  source 1..2746: mol_type = other DNA
tatatggcacaatataaccaaatgtctatccacgttattcatctagctttatgttctatcactataaatatccttcatcttactcttttatttcatcatctaaacttttaactagtgaaatataaatcatggctaccactatcaaatcatgatttccacttttgttgttgctgggaattatattcctggcctctgttgtttgtgtcacttatgccaattacgatgaaggttcagaacctagggtaccggcataaagagagagaggtcgctaagagggtgagaaagaggaaaaacgccatggagaataaagaccttcctacgaaaaggaagaagatgaagaagagggataaagagaaagaggtcgctaagagggtgaaaaagaggaaaaacgccacggagaataaagaccttcgtatgaaaagtaagaagatgaagaagagaagtagaaatatagatattaacgtgaaaaggaagatgaagaagagaagtagaaatattaatattaacgtgaaaagaaggaataaaaggaagtttaacctggacgtgagagataagaaagagaggaagatgaggaataagtagacgaagagtaaagaggaagttaacgtcgtgaagatcccgaagaaagggcaaggctaaggcatagagaggagagaacaaaaagagacagacgccattaacgtgaaggagaggaggaagaaagatcttcagagtcataagaatgaagaaatccctttttatttaagtctaacaagtttctaacactctttgaaaacgaaaacggccacattcgtctcctttaaaggttcgacaaacgttcagacttatttgaaaatctccaaaactatcgtcttgtggaatatagagccaaaccccacaccatcttccttccttaacacatagatgctgacttaatccttgtagtcctcagtgataatttttattttactttataatattattataacaaatctttttgttttatagaaatatgactatttaaaataaaaacattgtaaagttcaatttaacaatatttcttatatttcataattaaattttggtttggttaatatgtattacaaggaaagccatattgacagtgttgagtcccaatgatagaaattcgtataatcttgagcgtggtgataccatcaaacttcctgcaggaacaacctcttatttagttaactaagatgatgaagaagatcttagactggtagatcttgtaatacccgtgaatgggcctggtaaatttgagatactatataaaatacaataaatttttcttcagaagcgttattcttacaaaaacatccatttatattacttttacttttgtctataatgaaaaattgatattttccgttcttccatcaagcttttgacctagctaaaaataaaaactaatacttatgaggattcagcaagaatattttagaggcctcctataacataagtatgtgaagtttttatcattttttaataaataaaaccattttaatttgtatcattgtttacaactataaactagatacgagaccatagagaaggttctcttagaagaataagagaaagatcggaaaaggagataataaggggaagaaacagatgcaatagtcaaagtgtcaagggaataaattgaggaattgaaaaagcttgccaaatcaagctcaaagaaaagcttaccctctgaatttgaaccaatcaacttgagaagccacaagccagaatattctaataagtttggcaagttgtttgagattactccggaaaaaaaatacccttaactttaagatttagatctatttgttagttgtgtggagattaacgagataagtacacaacactaaatatatataaaacatataattttaattatattacagaaatatgttaatgcgtttttgcttatatttttaaggagctctaatgttgccacactacaattcaagggctatagttgtactattggttaatgaaggaaaaggaaaccttgaacttctgggtttaaaaaatgagtaataagagagggaagatagaaaagaaagaaacaatgaggtgtagagatatgaagctagattgtctccgggtgacgttgttatcattccagcaggtcatccggttgccattactgcttcttcaaatttgaatttgcttggatttggtatcaatgctgagaacaatgagagaaactttctttcagatatttagtgaatattagtatgattacttaataagtctcggctaaatgagaattttttgaaattgatattttgattttggtgattgaaaatttgaaagctcggacgacaatgtgataagctaaattgaaaatccagtaaaagagcttacatttcctggatctgtttaagagataaatagactaataaagaactaaaagtaatctcactttgcaaatgctgaacctgaataaaaggagtaaggaagctagggaaaaaggagtcctctgtcttcaattttgggcactttttactaagtaatcagtatgaaaaataatacaacacgtatgtatgatgtaagtgttggataataaactatgaaaaataaggaggaaaatgtatgctgtaagatatagctagctcataatgagctaagaataaataaagggtcatgtaactcttgcttattgagtcccacctttctactatgaagaaataaataatgaataaaatttttgtctttttttaatttaaaagagtgtttgggcgctaaatttcttaac

SEQ ID NO: 35 - DNA, 2746 bp, synthetic construct
  source 1..2746: mol_type = other DNA
tatatggcacaatataaccaaatgtctatccacgttattcatctagctttatgttctatcactataaatatccttcatcttactcttttatttcatcatctaaacttttaactagtgaaatataaatcatggctaccactatcaaatcatgatttccacttttgttgttgctgggaattatattcctggcctctgttgtttgtgtcacttatgccaattacgatgaaggttcagaacctagggtaccggcataaagagagagaggtcgctaagagggtgagaaagaggaaaaacgccatggagaataaagaccttcctacgaaaaggaagaagatgaagaagagggataaagagaaagaggtcgctaagagggtgaaaaagaggaaaaacgccacggagaataaagaccttcgtatgaaaagtaagaagatgaagaagagaagtagaaatatagatattaacgtgaaaaggaagatgaagaagagaagtagaaatattaatattaacgtgaaaagaaggaataaaaggaagtttaacctggacgtgagagataagaaagagaggaagatgaggaataagtagacgaagagtaaagaggaagttaacgtcgtgaagatcccgaagaaagggcaaggctaaggcatagagaggagagaacaaaaagagacagacgccattaacgtgaaggagaggaggaagaaagatcttcagagtcataagaatgaagaaatccctttttatttaagtctaacaagtttctaacactctttgaaaacgaaaacggccacattcgtctcctttaaaggttcgacaaacgttcagacttatttgaaaatctctaaaactatcgtcttgtggaatatagagccaaaccccacaccatcttccttcctcaacacatagatgctgacttaatccttgtagtcctcagtgataatttttattttactttataatattattataacaaatctttttgttttatagaaatatgactatttaaaataaaaacattgtaaagttcaatttaacaatatttcttatatttcataattaaattttggtttggttaatatgtattacaaggaaagccatattgacagtgttgagtcccaatgatagaaattcgtataatcttgagcgtggtgataccatcaaacttcctgcaggaacaacctcttatttagttaactaagatgatgaagaagatcttagactggtagatcttgtaatacccgtgaatgggcctggtaaatttgagatactatataaaatacaataaatttttcttcagaagcgttattcttacaaaaacatccatttatattacttttacttttgtctataatgaaaaattgatattttccgttcttccatcaagcttttgacctagctaaaaataaaaactaatacttatgaggattcagcaagaatattttagaggcctcctataacataagtatgtgaagtttttatcattttttaataaataaaaccattttaatttgtatcattgtttacaactataaactagatacgagaccatagagaaggttctcttagaagaataagagaaagatcggaaaaggagataataaggggaagaaacagatgcaatagtcaaagtgtcaagggaataaattgaggaattgaaaaagcttgccaaatcaagctcaaagaaaagcttaccctctgaatttgaaccaatcaacttgagaagccacaagccagaatattctaataagtttggcaagttgtttgagattactccggaaaaaaaatacccttaactttaagatttagatctatttgttagttgtgtggagattaacgagataagtacacaacactaaatatatataaaacatataattttaattatattacagaaatatgttaatgcgtttttgcttatatttttaaggagctctaatgttgccacactacaattcaagggctatagttgtactattggttaatgaaggaaaaggaaaccttgaacttctgggtttaaaaaatgagtaataagagagggaagatagaaaagaaagaaacaatgaggtgtagagatatgaagctagattgtctccgggtgacgttgttatcattccagcaggtcatccggttgccattactgcttcttcaaatttgaatttgcttggatttggtatcaatgctgagaacaatgagagaaactttctttcagatatttagtgaatattagtatgattacttaataagtctcggctaaatgagaattttttgaaattgatattttgattttggtgattgaaaatttgaaagctcggacgacaatgtgataagctaaattgaaaatccagtaaaagagcttacatttcctggatctgtttaagagataaatagactaataaagaactaaaagtaatctcactttgcaaatgctgaacctgaataaaaggagtaaggaagctagggaaaaaggagtcctctgtcttcaattttgggcactttttactaagtaatcagtatgaaaaataatacaacacgtatgtatgatgtaagtgttggataataaactatgaaaaataaggaggaaaatgtatgctgtaagatatagctagctcataatgagctaagaataaataaagggtcatgtaactcttgcttattgagtcccacctttctactatgaagaaataaataatgaataaaatttttgtctttttttaatttaaaagagtgtttgggcgctaaatttcttaac

SEQ ID NO: 36 - DNA, 2746 bp, synthetic construct
  source 1..2746: mol_type = other DNA
tatatggcacaatataaccaaatgtctatccacgttattcatctagctttatgttctatcactataaatatccttcatcttactcttttatttcatcatctaaacttttaactagtgaaatataaatcatggctaccactatcaaatcatgatttccacttttgttgttgctgggaattatattcctggcctctgttgtttgtgtcacttatgccaattacgatgaaggttcagaacctagggtaccggcataaagagagagaggtcgctaagagggtgagaaagaggaaaaacgccatggagaataaagaccttcctacgaaaaggaagaagatgaagaagagggataaagagaaagaggtcgctaagagggtgaaaaagaggaaaaacgccacggagaataaagaccttcgtatgaaaagtaagaagatgaagaagagaagtagaaatatagatattaacgtgaaaaggaagatgaagaagagaagtagaaatattaatattaacgtgaaaagaaggaataaaaggaagtttaacctggacgtgagagataagaaagagaggaagatgaggaataagtagacgaagagtaaagaggaagttaacgtcgtgaagatcccgaagaaagggcaaggctaaggcatagagaggagagaacaaaaagagacagacgccattaacgtgaaggagaggaggaagaaagatcttcagagtcataagaatgaagaaatccctttttatttaagtctaacaagtttctaacactctttgaaaacgaaaacggccacattcgtctcctttaaaggttcgacaaacgttcagacttatttgaaaatctctaaaactatcgtcttgtggaatatagagccaaaccccacaccatcttccttccttaacacatagatgctgacttaatccttgtagtcctcagtggtaatttttattttactttataatattattataacaaatctttttgttttatagaaatatgactatttaaaataaaaacattgtaaagttcaatttaacaatatttcttatatttcataattaaattttggtttggttaatatgtattacaaggaaagccatattgacagtgttgagtcccaatgatagaaattcgtataatcttgagcgtggtgataccatcaaacttcctgcaggaacaacctcttatttagttaactaagatgatgaagaagatcttagactggtagatcttgtaatacccgtgaatgggcctggtaaatttgagatactatataaaatacaataaatttttcttcagaagcgttattcttacaaaaacatccatttatattacttttacttttgtctataatgaaaaattgatattttccgttcttccatcaagcttttgacctagctaaaaataaaaactaatacttatgaggattcagcaagaatattttagaggcctcctataacataagtatgtgaagtttttatcattttttaataaataaaaccattttaatttgtatcattgtttacaactataaactagatacgagaccatagagaaggttctcttagaagaataagagaaagatcggaaaaggagataataaggggaagaaacagatgcaatagtcaaagtgtcaagggaataaattgaggaattgaaaaagcttgccaaatcaagctcaaagaaaagcttaccctctgaatttgaaccaatcaacttgagaagccacaagccagaatattctaataagtttggcaagttgtttgagattactccggaaaaaaaatacccttaactttaagatttagatctatttgttagttgtgtggagattaacgagataagtacacaacactaaatatatataaaacatataattttaattatattacagaaatatgttaatgcgtttttgcttatatttttaaggagctctaatgttgccacactacaattcaagggctatagttgtactattggttaatgaaggaaaaggaaaccttgaacttctgggtttaaaaaatgagtaataagagagggaagatagaaaagaaagaaacaatgaggtgtagagatatgaagctagattgtctccgggtgacgttgttatcattccagcaggtcatccggttgccattactgcttcttcaaatttgaatttgcttggatttggtatcaatgctgagaacaatgagagaaactttctttcagatatttagtgaatattagtatgattacttaataagtctcggctaaatgagaattttttgaaattgatattttgattttggtgattgaaaatttgaaagctcggacgacaatgtgataagctaaattgaaaatccagtaaaagagcttacatttcctggatctgtttaagagataaatagactaataaagaactaaaagtaatctcactttgcaaatgctgaacctgaataaaaggagtaaggaagctagggaaaaaggagtcctctgtcttcaattttgggcactttttactaagtaatcagtatgaaaaataatacaacacgtatgtatgatgtaagtgttggataataaactatgaaaaataaggaggaaaatgtatgctgtaagatatagctagctcataatgagctaagaataaataaagggtcatgtaactcttgcttattgagtcccacctttctactatgaagaaataaataatgaataaaatttttgtctttttttaatttaaaagagtgtttgggcgctaaatttcttaac

SEQ ID NO: 37 - DNA, 2746 bp, synthetic construct
  source 1..2746: mol_type = other DNA
tatatggcacaatataaccaaatgtctatccacgttattcatctagctttatgttctatcactataaatatccttcatcttactcttttatttcatcatctaaacttttaactagtgaaatataaatcatggctaccactatcaaatcatgatttccacttttgttgttgctgggaattatattcctggcctctgttgtttgtgtcacttatgccaattacgatgaaggttcagaacctagggtaccggcataaagagagagaggtcgctaagagggtgagaaagaggaaaaacgccatggagaataaagaccttcctacgaaaaggaagaagatgaagaagagggataaagagaaagaggtcgctaagagggtgaaaaagaggaaaaacgccacggagaataaagaccttcgtatgaaaagtaagaagatgaagaagagaagtagaaatatagatattaacgtgaaaaggaagatgaagaagagaagtagaaatattaatattaacgtgaaaagaaggaataaaaggaagtttaacctggacgtgagagataagaaagagaggaagatgaggaataagtagacgaagagtaaagaggaagttaacgtcgtgaagatcccgaagaaagggcaaggctaaggcatagagaggagagaacaaaaagagacagacgccattaacgtgaaggagaggaggaagaaagatcttcagagtcataagaatgaagaaatccctttttatttaagtctaacaagtttctaacactctttgaaaacgaaaacggccacattcgtctcctttaaaggttcgacaaacgttcagacttatttgaaaatctctaaaactatcgtcttgtggaatatagagccaaaccccacaccatcttccttccttaacacatagatgctgacttaatccttgtagtcctcagtgataatttttattttactttataatattattataacaaatctttttgttttatagaaatatgactatttaaaataaaaacattgtaaagttcaatttaacaatatttcttatatttcataattaaattttggtttggttaatatgtattacagggaaagccatattgacagtgttgagtcccaatgatagaaattcgtataatcttgagcgtggtgataccatcaaacttcctgcaggaacaacctcttatttagttaactaagatgatgaagaagatcttagactggtagatcttgtaatacccgtgaatgggcctggtaaatttgagatactatataaaatacaataaatttttcttcagaagcgttattcttacaaaaacatccatttatattacttttacttttgtctataatgaaaaattgatattttccgttcttccatcaagcttttgacctagctaaaaataaaaactaatacttatgaggattcagcaagaatattttagaggcctcctataacataagtatgtgaagtttttatcattttttaataaataaaaccattttaatttgtatcattgtttacaactataaactagatacgagaccatagagaaggttctcttagaagaataagagaaagatcggaaaaggagataataaggggaagaaacagatgcaatagtcaaagtgtcaagggaataaattgaggaattgaaaaagcttgccaaatcaagctcaaagaaaagcttaccctctgaatttgaaccaatcaacttgagaagccacaagccagaatattctaataagtttggcaagttgtttgagattactccggaaaaaaaatacccttaactttaagatttagatctatttgttagttgtgtggagattaacgagataagtacacaacactaaatatatataaaacatataattttaattatattacagaaatatgttaatgcgtttttgcttatatttttaaggagctctaatgttgccacactacaattcaagggctatagttgtactattggttaatgaaggaaaaggaaaccttgaacttctgggtttaaaaaatgagtaataagagagggaagatagaaaagaaagaaacaatgaggtgtagagatatgaagctagattgtctccgggtgacgttgttatcattccagcaggtcatccggttgccattactgcttcttcaaatttgaatttgcttggatttggtatcaatgctgagaacaatgagagaaactttctttcagatatttagtgaatattagtatgattacttaataagtctcggctaaatgagaattttttgaaattgatattttgattttggtgattgaaaatttgaaagctcggacgacaatgtgataagctaaattgaaaatccagtaaaagagcttacatttcctggatctgtttaagagataaatagactaataaagaactaaaagtaatctcactttgcaaatgctgaacctgaataaaaggagtaaggaagctagggaaaaaggagtcctctgtcttcaattttgggcactttttactaagtaatcagtatgaaaaataatacaacacgtatgtatgatgtaagtgttggataataaactatgaaaaataaggaggaaaatgtatgctgtaagatatagctagctcataatgagctaagaataaataaagggtcatgtaactcttgcttattgagtcccacctttctactatgaagaaataaataatgaataaaatttttgtctttttttaatttaaaagagtgtttgggcgctaaatttcttaac

SEQ ID NO: 38 - DNA, 2746 bp, synthetic construct
  source 1..2746: mol_type = other DNA
tatatggcacaatataaccaaatgtctatccacgttattcatctagctttatgttctatcactataaatatccttcatcttactcttttatttcatcatctaaacttttaactagtgaaatataaatcatggctaccactatcaaatcatgatttccacttttgttgttgctgggaattatattcctggcctctgttgtttgtgtcacttatgccaattacgatgaaggttcagaacctagggtaccggcataaagagagagaggtcgctaagagggtgagaaagaggaaaaacgccatggagaataaagaccttcctacgaaaaggaagaagatgaagaagagggataaagagaaagaggtcgctaagagggtgaaaaagaggaaaaacgccacggagaataaagaccttcgtatgaaaagtaagaagatgaagaagagaagtagaaatatagatattaacgtgaaaaggaagatgaagaagagaagtagaaatattaatattaacgtgaaaagaaggaataaaaggaagtttaacctggacgtgagagataagaaagagaggaagatgaggaataagtagacgaagagtaaagaggaagttaacgtcgtgaagatcccgaagaaagggcaaggctaaggcatagagaggagagaacaaaaagagacagacgccattaacgtgaaggagaggaggaagaaagatcttcagagtcataagaatgaagaaatccctttttatttaagtctaacaagtttctaacactctttgaaaacgaaaacggccacattcgtctcctttaaaggttcgacaaacgttcagacttatttgaaaatctctaaaactatcgtcttgtggaatatagagccaaaccccacaccatcttccttccttaacacatagatgctgacttaatccttgtagtcctcagtgataatttttattttactttataatattattataacaaatctttttgttttatagaaatatgactatttaaaataaaaacattgtaaagttcaatttaacaatatttcttatatttcataattaaattttggtttggttaatatgtattacaaggaaagccatattgacagtgttgagtcccaatgatagaaattcgtataatcttgagcgtggtgataccatcaaacttcctgcaggaacaacctcttatttagttaaccaagatgatgaagaagatcttagactggtagatcttgtaatacccgtgaatgggcctggtaaatttgagatactatataaaatacaataaatttttcttcagaagcgttattcttacaaaaacatccatttatattacttttacttttgtctataatgaaaaattgatattttccgttcttccatcaagcttttgacctagctaaaaataaaaactaatacttatgaggattcagcaagaatattttagaggcctcctataacataagtatgtgaagtttttatcattttttaataaataaaaccattttaatttgtatcattgtttacaactataaactagatacgagaccatagagaaggttctcttagaagaataagagaaagatcggaaaaggagataataaggggaagaaacagatgcaatagtcaaagtgtcaagggaataaattgaggaattgaaaaagcttgccaaatcaagctcaaagaaaagcttaccctctgaatttgaaccaatcaacttgagaagccacaagccagaatattctaataagtttggcaagttgtttgagattactccggaaaaaaaatacccttaactttaagatttagatctatttgttagttgtgtggagattaacgagataagtacacaacactaaatatatataaaacatataattttaattatattacagaaatatgttaatgcgtttttgcttatatttttaaggagctctaatgttgccacactacaattcaagggctatagttgtactattggttaatgaaggaaaaggaaaccttgaacttctgggtttaaaaaatgagtaataagagagggaagatagaaaagaaagaaacaatgaggtgtagagatatgaagctagattgtctccgggtgacgttgttatcattccagcaggtcatccggttgccattactgcttcttcaaatttgaatttgcttggatttggtatcaatgctgagaacaatgagagaaactttctttcagatatttagtgaatattagtatgattacttaataagtctcggctaaatgagaattttttgaaattgatattttgattttggtgattgaaaatttgaaagctcggacgacaatgtgataagctaaattgaaaatccagtaaaagagcttacatttcctggatctgtttaagagataaatagactaataaagaactaaaagtaatctcactttgcaaatgctgaacctgaataaaaggagtaaggaagctagggaaaaaggagtcctctgtcttcaattttgggcactttttactaagtaatcagtatgaaaaataatacaacacgtatgtatgatgtaagtgttggataataaactatgaaaaataaggaggaaaatgtatgctgtaagatatagctagctcataatgagctaagaataaataaagggtcatgtaactcttgcttattgagtcccacctttctactatgaagaaataaataatgaataaaatttttgtctttttttaatttaaaagagtgtttgggcgctaaatttcttaac

SEQ ID NO: 39 - DNA, 2746 bp, synthetic construct
  source 1..2746: mol_type = other DNA
tatatggcacaatataaccaaatgtctatccacgttattcatctagctttatgttctatcactataaatatccttcatcttactcttttatttcatcatctaaacttttaactagtgaaatataaatcatggctaccactatcaaatcatgatttccacttttgttgttgctgggaattatattcctggcctctgttgtttgtgtcacttatgccaattacgatgaaggttcagaacctagggtaccggcataaagagagagaggtcgctaagagggtgagaaagaggaaaaacgccatggagaataaagaccttcctacgaaaaggaagaagatgaagaagagggataaagagaaagaggtcgctaagagggtgaaaaagaggaaaaacgccacggagaataaagaccttcgtatgaaaagtaagaagatgaagaagagaagtagaaatatagatattaacgtgaaaaggaagatgaagaagagaagtagaaatattaatattaacgtgaaaagaaggaataaaaggaagtttaacctggacgtgagagataagaaagagaggaagatgaggaataagtagacgaagagtaaagaggaagttaacgtcgtgaagatcccgaagaaagggcaaggctaaggcatagagaggagagaacaaaaagagacagacgccattaacgtgaaggagaggaggaagaaagatcttcagagtcataagaatgaagaaatccctttttatttaagtctaacaagtttctaacactctttgaaaacgaaaacggccacattcgtctcctttaaaggttcgacaaacgttcagacttatttgaaaatctctaaaactatcgtcttgtggaatatagagccaaaccccacaccatcttccttccttaacacatagatgctgacttaatccttgtagtcctcagtgataatttttattttactttataatattattataacaaatctttttgttttatagaaatatgactatttaaaataaaaacattgtaaagttcaatttaacaatatttcttatatttcataattaaattttggtttggttaatatgtattacaaggaaagccatattgacagtgttgagtcccaatgatagaaattcgtataatcttgagcgtggtgataccatcaaacttcctgcaggaacaacctcttatttagttaactaagatgatgaagaagatcttagactggtagatcttgtaatacccgtgaatgggcctggtaaatttgaggtactatataaaatacaataaatttttcttcagaagcgttattcttacaaaaacatccatttatattacttttacttttgtctataatgaaaaattgatattttccgttcttccatcaagcttttgacctagctaaaaataaaaactaatacttatgaggattcagcaagaatattttagaggcctcctataacataagtatgtgaagtttttatcattttttaataaataaaaccattttaatttgtatcattgtttacaactataaactagatacgagaccatagagaaggttctcttagaagaataagagaaagatcggaaaaggagataataaggggaagaaacagatgcaatagtcaaagtgtcaagggaataaattgaggaattgaaaaagcttgccaaatcaagctcaaagaaaagcttaccctctgaatttgaaccaatcaacttgagaagccacaagccagaatattctaataagtttggcaagttgtttgagattactccggaaaaaaaatacccttaactttaagatttagatctatttgttagttgtgtggagattaacgagataagtacacaacactaaatatatataaaacatataattttaattatattacagaaatatgttaatgcgtttttgcttatatttttaaggagctctaatgttgccacactacaattcaagggctatagttgtactattggttaatgaaggaaaaggaaaccttgaacttctgggtttaaaaaatgagtaataagagagggaagatagaaaagaaagaaacaatgaggtgtagagatatgaagctagattgtctccgggtgacgttgttatcattccagcaggtcatccggttgccattactgcttcttcaaatttgaatttgcttggatttggtatcaatgctgagaacaatgagagaaactttctttcagatatttagtgaatattagtatgattacttaataagtctcggctaaatgagaattttttgaaattgatattttgattttggtgattgaaaatttgaaagctcggacgacaatgtgataagctaaattgaaaatccagtaaaagagcttacatttcctggatctgtttaagagataaatagactaataaagaactaaaagtaatctcactttgcaaatgctgaacctgaataaaaggagtaaggaagctagggaaaaaggagtcctctgtcttcaattttgggcactttttactaagtaatcagtatgaaaaataatacaacacgtatgtatgatgtaagtgttggataataaactatgaaaaataaggaggaaaatgtatgctgtaagatatagctagctcataatgagctaagaataaataaagggtcatgtaactcttgcttattgagtcccacctttctactatgaagaaataaataatgaataaaatttttgtctttttttaatttaaaagagtgtttgggcgctaaatttcttaac

SEQ ID NO: 40 - DNA, 2746 bp, synthetic construct
  source 1..2746: mol_type = other DNA
tatatggcacaatataaccaaatgtctatccacgttattcatctagctttatgttctatcactataaatatccttcatcttactcttttatttcatcatctaaacttttaactagtgaaatataaatcatggctaccactatcaaatcatgatttccacttttgttgttgctgggaattatattcctggcctctgttgtttgtgtcacttatgccaattacgatgaaggttcagaacctagggtaccggcataaagagagagaggtcgctaagagggtgagaaagaggaaaaacgccatggagaataaagaccttcctacgaaaaggaagaagatgaagaagagggataaagagaaagaggtcgctaagagggtgaaaaagaggaaaaacgccacggagaataaagaccttcgtatgaaaagtaagaagatgaagaagagaagtagaaatatagatattaacgtgaaaaggaagatgaagaagagaagtagaaatattaatattaacgtgaaaagaaggaataaaaggaagtttaacctggacgtgagagataagaaagagaggaagatgaggaataagtagacgaagagtaaagaggaagttaacgtcgtgaagatcccgaagaaagggcaaggctaaggcatagagaggagagaacaaaaagagacagacgccattaacgtgaaggagaggaggaagaaagatcttcagagtcataagaatgaagaaatccctttttatttaagtctaacaagtttctaacactctttgaaaacgaaaacggccacattcgtctcctttaaaggttcgacaaacgttcagacttatttgaaaatctctaaaactatcgtcttgtggaatatagagccaaaccccacaccatcttccttccttaacacatagatgctgacttaatccttgtagtcctcagtgataatttttattttactttataatattattataacaaatctttttgttttatagaaatatgactatttaaaataaaaacattgtaaagttcaatttaacaatatttcttatatttcataattaaattttggtttggttaatatgtattacaaggaaagccatattgacagtgttgagtcccaatgatagaaattcgtataatcttgagcgtggtgataccatcaaacttcctgcaggaacaacctcttatttagttaactaagatgatgaagaagatcttagactggtagatcttgtaatacccgtgaatgggcctggtaaatttgagatactatataaaatacaataaatttttcttcagaagcgttattcttacaaaaacatccatttatattacttttacttttgtctataatgaaaaattgatattttccgttcttccatcaggcttttgacctagctaaaaataaaaactaatacttatgaggattcagcaagaatattttagaggcctcctataacataagtatgtgaagtttttatcattttttaataaataaaaccattttaatttgtatcattgtttacaactataaactagatacgagaccatagagaaggttctcttagaagaataagagaaagatcggaaaaggagataataaggggaagaaacagatgcaatagtcaaagtgtcaagggaataaattgaggaattgaaaaagcttgccaaatcaagctcaaagaaaagcttaccctctgaatttgaaccaatcaacttgagaagccacaagccagaatattctaataagtttggcaagttgtttgagattactccggaaaaaaaatacccttaactttaagatttagatctatttgttagttgtgtggagattaacgagataagtacacaacactaaatatatataaaacatataattttaattatattacagaaatatgttaatgcgtttttgcttatatttttaaggagctctaatgttgccacactacaattcaagggctatagttgtactattggttaatgaaggaaaaggaaaccttgaacttctgggtttaaaaaatgagtaataagagagggaagatagaaaagaaagaaacaatgaggtgtagagatatgaagctagattgtctccgggtgacgttgttatcattccagcaggtcatccggttgccattactgcttcttcaaatttgaatttgcttggatttggtatcaatgctgagaacaatgagagaaactttctttcagatatttagtgaatattagtatgattacttaataagtctcggctaaatgagaattttttgaaattgatattttgattttggtgattgaaaatttgaaagctcggacgacaatgtgataagctaaattgaaaatccagtaaaagagcttacatttcctggatctgtttaagagataaatagactaataaagaactaaaagtaatctcactttgcaaatgctgaacctgaataaaaggagtaaggaagctagggaaaaaggagtcctctgtcttcaattttgggcactttttactaagtaatcagtatgaaaaataatacaacacgtatgtatgatgtaagtgttggataataaactatgaaaaataaggaggaaaatgtatgctgtaagatatagctagctcataatgagctaagaataaataaagggtcatgtaactcttgcttattgagtcccacctttctactatgaagaaataaataatgaataaaatttttgtctttttttaatttaaaagagtgtttgggcgctaaatttcttaac

SEQ ID NO: 41 - DNA, 2746 bp, synthetic construct
  source 1..2746: mol_type = other DNA
tatatggcacaatataaccaaatgtctatccacgttattcatctagctttatgttctatcactataaatatccttcatcttactcttttatttcatcatctaaacttttaactagtgaaatataaatcatggctaccactatcaaatcatgatttccacttttgttgttgctgggaattatattcctggcctctgttgtttgtgtcacttatgccaattacgatgaaggttcagaacctagggtaccggcataaagagagagaggtcgctaagagggtgagaaagaggaaaaacgccatggagaataaagaccttcctacgaaaaggaagaagatgaagaagagggataaagagaaagaggtcgctaagagggtgaaaaagaggaaaaacgccacggagaataaagaccttcgtatgaaaagtaagaagatgaagaagagaagtagaaatatagatattaacgtgaaaaggaagatgaagaagagaagtagaaatattaatattaacgtgaaaagaaggaataaaaggaagtttaacctggacgtgagagataagaaagagaggaagatgaggaataagtagacgaagagtaaagaggaagttaacgtcgtgaagatcccgaagaaagggcaaggctaaggcatagagaggagagaacaaaaagagacagacgccattaacgtgaaggagaggaggaagaaagatcttcagagtcataagaatgaagaaatccctttttatttaagtctaacaagtttctaacactctttgaaaacgaaaacggccacattcgtctcctttaaaggttcgacaaacgttcagacttatttgaaaatctctaaaactatcgtcttgtggaatatagagccaaaccccacaccatcttccttccttaacacatagatgctgacttaatccttgtagtcctcagtgataatttttattttactttataatattattataacaaatctttttgttttatagaaatatgactatttaaaataaaaacattgtaaagttcaatttaacaatatttcttatatttcataattaaattttggtttggttaatatgtattacaaggaaagccatattgacagtgttgagtcccaatgatagaaattcgtataatcttgagcgtggtgataccatcaaacttcctgcaggaacaacctcttatttagttaactaagatgatgaagaagatcttagactggtagatcttgtaatacccgtgaatgggcctggtaaatttgagatactatataaaatacaataaatttttcttcagaagcgttattcttacaaaaacatccatttatattacttttacttttgtctataatgaaaaattgatattttccgttcttccatcaagcttttgacctagctaaaaataaaaaccaatacttatgaggattcagcaagaatattttagaggcctcctataacataagtatgtgaagtttttatcattttttaataaataaaaccattttaatttgtatcattgtttacaactataaactagatacgagaccatagagaaggttctcttagaagaataagagaaagatcggaaaaggagataataaggggaagaaacagatgcaatagtcaaagtgtcaagggaataaattgaggaattgaaaaagcttgccaaatcaagctcaaagaaaagcttaccctctgaatttgaaccaatcaacttgagaagccacaagccagaatattctaataagtttggcaagttgtttgagattactccggaaaaaaaatacccttaactttaagatttagatctatttgttagttgtgtggagattaacgagataagtacacaacactaaatatatataaaacatataattttaattatattacagaaatatgttaatgcgtttttgcttatatttttaaggagctctaatgttgccacactacaattcaagggctatagttgtactattggttaatgaaggaaaaggaaaccttgaacttctgggtttaaaaaatgagtaataagagagggaagatagaaaagaaagaaacaatgaggtgtagagatatgaagctagattgtctccgggtgacgttgttatcattccagcaggtcatccggttgccattactgcttcttcaaatttgaatttgcttggatttggtatcaatgctgagaacaatgagagaaactttctttcagatatttagtgaatattagtatgattacttaataagtctcggctaaatgagaattttttgaaattgatattttgattttggtgattgaaaatttgaaagctcggacgacaatgtgataagctaaattgaaaatccagtaaaagagcttacatttcctggatctgtttaagagataaatagactaataaagaactaaaagtaatctcactttgcaaatgctgaacctgaataaaaggagtaaggaagctagggaaaaaggagtcctctgtcttcaattttgggcactttttactaagtaatcagtatgaaaaataatacaacacgtatgtatgatgtaagtgttggataataaactatgaaaaataaggaggaaaatgtatgctgtaagatatagctagctcataatgagctaagaataaataaagggtcatgtaactcttgcttattgagtcccacctttctactatgaagaaataaataatgaataaaatttttgtctttttttaatttaaaagagtgtttgggcgctaaatttcttaac

SEQ ID NO: 42 - DNA, 2746 bp, synthetic construct
  source 1..2746: mol_type = other DNA
tatatggcacaatataaccaaatgtctatccacgttattcatctagctttatgttctatcactataaatatccttcatcttactcttttatttcatcatctaaacttttaactagtgaaatataaatcatggctaccactatcaaatcatgatttccacttttgttgttgctgggaattatattcctggcctctgttgtttgtgtcacttatgccaattacgatgaaggttcagaacctagggtaccggcataaagagagagaggtcgctaagagggtgagaaagaggaaaaacgccatggagaataaagaccttcctacgaaaaggaagaagatgaagaagagggataaagagaaagaggtcgctaagagggtgaaaaagaggaaaaacgccacggagaataaagaccttcgtatgaaaagtaagaagatgaagaagagaagtagaaatatagatattaacgtgaaaaggaagatgaagaagagaagtagaaatattaatattaacgtgaaaagaaggaataaaaggaagtttaacctggacgtgagagataagaaagagaggaagatgaggaataagtagacgaagagtaaagaggaagttaacgtcgtgaagatcccgaagaaagggcaaggctaaggcatagagaggagagaacaaaaagagacagacgccattaacgtgaaggagaggaggaagaaagatcttcagagtcataagaatgaagaaatccctttttatttaagtctaacaagtttctaacactctttgaaaacgaaaacggccacattcgtctcctttaaaggttcgacaaacgttcagacttatttgaaaatctctaaaactatcgtcttgtggaatatagagccaaaccccacaccatcttccttccttaacacatagatgctgacttaatccttgtagtcctcagtgataatttttattttactttataatattattataacaaatctttttgttttatagaaatatgactatttaaaataaaaacattgtaaagttcaatttaacaatatttcttatatttcataattaaattttggtttggttaatatgtattacaaggaaagccatattgacagtgttgagtcccaatgatagaaattcgtataatcttgagcgtggtgataccatcaaacttcctgcaggaacaacctcttatttagttaactaagatgatgaagaagatcttagactggtagatcttgtaatacccgtgaatgggcctggtaaatttgagatactatataaaatacaataaatttttcttcagaagcgttattcttacaaaaacatccatttatattacttttacttttgtctataatgaaaaattgatattttccgttcttccatcaagcttttgacctagctaaaaataaaaactaatacttacgaggattcagcaagaatattttagaggcctcctataacataagtatgtgaagtttttatcattttttaataaataaaaccattttaatttgtatcattgtttacaactataaactagatacgagaccatagagaaggttctcttagaagaataagagaaagatcggaaaaggagataataaggggaagaaacagatgcaatagtcaaagtgtcaagggaataaattgaggaattgaaaaagcttgccaaatcaagctcaaagaaaagcttaccctctgaatttgaaccaatcaacttgagaagccacaagccagaatattctaataagtttggcaagttgtttgagattactccggaaaaaaaatacccttaactttaagatttagatctatttgttagttgtgtggagattaacgagataagtacacaacactaaatatatataaaacatataattttaattatattacagaaatatgttaatgcgtttttgcttatatttttaaggagctctaatgttgccacactacaattcaagggctatagttgtactattggttaatgaaggaaaaggaaaccttgaacttctgggtttaaaaaatgagtaataagagagggaagatagaaaagaaagaaacaatgaggtgtagagatatgaagctagattgtctccgggtgacgttgttatcattccagcaggtcatccggttgccattactgcttcttcaaatttgaatttgcttggatttggtatcaatgctgagaacaatgagagaaactttctttcagatatttagtgaatattagtatgattacttaataagtctcggctaaatgagaattttttgaaattgatattttgattttggtgattgaaaatttgaaagctcggacgacaatgtgataagctaaattgaaaatccagtaaaagagcttacatttcctggatctgtttaagagataaatagactaataaagaactaaaagtaatctcactttgcaaatgctgaacctgaataaaaggagtaaggaagctagggaaaaaggagtcctctgtcttcaattttgggcactttttactaagtaatcagtatgaaaaataatacaacacgtatgtatgatgtaagtgttggataataaactatgaaaaataaggaggaaaatgtatgctgtaagatatagctagctcataatgagctaagaataaataaagggtcatgtaactcttgcttattgagtcccacctttctactatgaagaaataaataatgaataaaatttttgtctttttttaatttaaaagagtgtttgggcgctaaatttcttaac

SEQ ID NO: 43 - DNA, 2746 bp, synthetic construct
  source 1..2746: mol_type = other DNA
tatatggcacaatataaccaaatgtctatccacgttattcatctagctttatgttctatcactataaatatccttcatcttactcttttatttcatcatctaaacttttaactagtgaaatataaatcatggctaccactatcaaatcatgatttccacttttgttgttgctgggaattatattcctggcctctgttgtttgtgtcacttatgccaattacgatgaaggttcagaacctagggtaccggcataaagagagagaggtcgctaagagggtgagaaagaggaaaaacgccatggagaataaagaccttcctacgaaaaggaagaagatgaagaagagggataaagagaaagaggtcgctaagagggtgaaaaagaggaaaaacgccacggagaataaagaccttcgtatgaaaagtaagaagatgaagaagagaagtagaaatatagatattaacgtgaaaaggaagatgaagaagagaagtagaaatattaatattaacgtgaaaagaaggaataaaaggaagtttaacctggacgtgagagataagaaagagaggaagatgaggaataagtagacgaagagtaaagaggaagttaacgtcgtgaagatcccgaagaaagggcaaggctaaggcatagagaggagagaacaaaaagagacagacgccattaacgtgaaggagaggaggaagaaagatcttcagagtcataagaatgaagaaatccctttttatttaagtctaacaagtttctaacactctttgaaaacgaaaacggccacattcgtctcctttaaaggttcgacaaacgttcagacttatttgaaaatctctaaaactatcgtcttgtggaatatagagccaaaccccacaccatcttccttccttaacacatagatgctgacttaatccttgtagtcctcagtgataatttttattttactttataatattattataacaaatctttttgttttatagaaatatgactatttaaaataaaaacattgtaaagttcaatttaacaatatttcttatatttcataattaaattttggtttggttaatatgtattacaaggaaagccatattgacagtgttgagtcccaatgatagaaattcgtataatcttgagcgtggtgataccatcaaacttcctgcaggaacaacctcttatttagttaactaagatgatgaagaagatcttagactggtagatcttgtaatacccgtgaatgggcctggtaaatttgagatactatataaaatacaataaatttttcttcagaagcgttattcttacaaaaacatccatttatattacttttacttttgtctataatgaaaaattgatattttccgttcttccatcaagcttttgacctagctaaaaataaaaactaatacttatgaggattcagcaagaatattttagaggcctcctataacgtaagtatgtgaagtttttatcattttttaataaataaaaccattttaatttgtatcattgtttacaactataaactagatacgagaccatagagaaggttctcttagaagaataagagaaagatcggaaaaggagataataaggggaagaaacagatgcaatagtcaaagtgtcaagggaataaattgaggaattgaaaaagcttgccaaatcaagctcaaagaaaagcttaccctctgaatttgaaccaatcaacttgagaagccacaagccagaatattctaataagtttggcaagttgtttgagattactccggaaaaaaaatacccttaactttaagatttagatctatttgttagttgtgtggagattaacgagataagtacacaacactaaatatatataaaacatataattttaattatattacagaaatatgttaatgcgtttttgcttatatttttaaggagctctaatgttgccacactacaattcaagggctatagttgtactattggttaatgaaggaaaaggaaaccttgaacttctgggtttaaaaaatgagtaataagagagggaagatagaaaagaaagaaacaatgaggtgtagagatatgaagctagattgtctccgggtgacgttgttatcattccagcaggtcatccggttgccattactgcttcttcaaatttgaatttgcttggatttggtatcaatgctgagaacaatgagagaaactttctttcagatatttagtgaatattagtatgattacttaataagtctcggctaaatgagaattttttgaaattgatattttgattttggtgattgaaaatttgaaagctcggacgacaatgtgataagctaaattgaaaatccagtaaaagagcttacatttcctggatctgtttaagagataaatagactaataaagaactaaaagtaatctcactttgcaaatgctgaacctgaataaaaggagtaaggaagctagggaaaaaggagtcctctgtcttcaattttgggcactttttactaagtaatcagtatgaaaaataatacaacacgtatgtatgatgtaagtgttggataataaactatgaaaaataaggaggaaaatgtatgctgtaagatatagctagctcataatgagctaagaataaataaagggtcatgtaactcttgcttattgagtcccacctttctactatgaagaaataaataatgaataaaatttttgtctttttttaatttaaaagagtgtttgggcgctaaatttcttaac

SEQ ID NO: 44 - DNA, 2746 bp, synthetic construct
  source 1..2746: mol_type = other DNA
tatatggcacaatataaccaaatgtctatccacgttattcatctagctttatgttctatcactataaatatccttcatcttactcttttatttcatcatctaaacttttaactagtgaaatataaatcatggctaccactatcaaatcatgatttccacttttgttgttgctgggaattatattcctggcctctgttgtttgtgtcacttatgccaattacgatgaaggttcagaacctagggtaccggcataaagagagagaggtcgctaagagggtgagaaagaggaaaaacgccatggagaataaagaccttcctacgaaaaggaagaagatgaagaagagggataaagagaaagaggtcgctaagagggtgaaaaagaggaaaaacgccacggagaataaagaccttcgtatgaaaagtaagaagatgaagaagagaagtagaaatatagatattaacgtgaaaaggaagatgaagaagagaagtagaaatattaatattaacgtgaaaagaaggaataaaaggaagtttaacctggacgtgagagataagaaagagaggaagatgaggaataagtagacgaagagtaaagaggaagttaacgtcgtgaagatcccgaagaaagggcaaggctaaggcatagagaggagagaacaaaaagagacagacgccattaacgtgaaggagaggaggaagaaagatcttcagagtcataagaatgaagaaatccctttttatttaagtctaacaagtttctaacactctttgaaaacgaaaacggccacattcgtctcctttaaaggttcgacaaacgttcagacttatttgaaaatctctaaaactatcgtcttgtggaatatagagccaaaccccacaccatcttccttccttaacacatagatgctgacttaatccttgtagtcctcagtgataatttttattttactttataatattattataacaaatctttttgttttatagaaatatgactatttaaaataaaaacattgtaaagttcaatttaacaatatttcttatatttcataattaaattttggtttggttaatatgtattacaaggaaagccatattgacagtgttgagtcccaatgatagaaattcgtataatcttgagcgtggtgataccatcaaacttcctgcaggaacaacctcttatttagttaactaagatgatgaagaagatcttagactggtagatcttgtaatacccgtgaatgggcctggtaaatttgagatactatataaaatacaataaatttttcttcagaagcgttattcttacaaaaacatccatttatattacttttacttttgtctataatgaaaaattgatattttccgttcttccatcaagcttttgacctagctaaaaataaaaactaatacttatgaggattcagcaagaatattttagaggcctcctataacataagtatgtgaagtttttatcattttttaataaataaaaccattttaatttgtatcattgtttacaactatagactagatacgagaccatagagaaggttctcttagaagaataagagaaagatcggaaaaggagataataaggggaagaaacagatgcaatagtcaaagtgtcaagggaataaattgaggaattgaaaaagcttgccaaatcaagctcaaagaaaagcttaccctctgaatttgaaccaatcaacttgagaagccacaagccagaatattctaataagtttggcaagttgtttgagattactccggaaaaaaaatacccttaactttaagatttagatctatttgttagttgtgtggagattaacgagataagtacacaacactaaatatatataaaacatataattttaattatattacagaaatatgttaatgcgtttttgcttatatttttaaggagctctaatgttgccacactacaattcaagggctatagttgtactattggttaatgaaggaaaaggaaaccttgaacttctgggtttaaaaaatgagtaataagagagggaagatagaaaagaaagaaacaatgaggtgtagagatatgaagctagattgtctccgggtgacgttgttatcattccagcaggtcatccggttgccattactgcttcttcaaatttgaatttgcttggatttggtatcaatgctgagaacaatgagagaaactttctttcagatatttagtgaatattagtatgattacttaataagtctcggctaaatgagaattttttgaaattgatattttgattttggtgattgaaaatttgaaagctcggacgacaatgtgataagctaaattgaaaatccagtaaaagagcttacatttcctggatctgtttaagagataaatagactaataaagaactaaaagtaatctcactttgcaaatgctgaacctgaataaaaggagtaaggaagctagggaaaaaggagtcctctgtcttcaattttgggcactttttactaagtaatcagtatgaaaaataatacaacacgtatgtatgatgtaagtgttggataataaactatgaaaaataaggaggaaaatgtatgctgtaagatatagctagctcataatgagctaagaataaataaagggtcatgtaactcttgcttattgagtcccacctttctactatgaagaaataaataatgaataaaatttttgtctttttttaatttaaaagagtgtttgggcgctaaatttcttaac

SEQ ID NO: 45 - DNA, 2746 bp, synthetic construct
  source 1..2746: mol_type = other DNA
tatatggcacaatataaccaaatgtctatccacgttattcatctagctttatgttctatcactataaatatccttcatcttactcttttatttcatcatctaaacttttaactagtgaaatataaatcatggctaccactatcaaatcatgatttccacttttgttgttgctgggaattatattcctggcctctgttgtttgtgtcacttatgccaattacgatgaaggttcagaacctagggtaccggcataaagagagagaggtcgctaagagggtgagaaagaggaaaaacgccatggagaataaagaccttcctacgaaaaggaagaagatgaagaagagggataaagagaaagaggtcgctaagagggtgaaaaagaggaaaaacgccacggagaataaagaccttcgtatgaaaagtaagaagatgaagaagagaagtagaaatatagatattaacgtgaaaaggaagatgaagaagagaagtagaaatattaatattaacgtgaaaagaaggaataaaaggaagtttaacctggacgtgagagataagaaagagaggaagatgaggaataagtagacgaagagtaaagaggaagttaacgtcgtgaagatcccgaagaaagggcaaggctaaggcatagagaggagagaacaaaaagagacagacgccattaacgtgaaggagaggaggaagaaagatcttcagagtcataagaatgaagaaatccctttttatttaagtctaacaagtttctaacactctttgaaaacgaaaacggccacattcgtctcctttaaaggttcgacaaacgttcagacttatttgaaaatctctaaaactatcgtcttgtggaatatagagccaaaccccacaccatcttccttccttaacacatagatgctgacttaatccttgtagtcctcagtgataatttttattttactttataatattattataacaaatctttttgttttatagaaatatgactatttaaaataaaaacattgtaaagttcaatttaacaatatttcttatatttcataattaaattttggtttggttaatatgtattacaaggaaagccatattgacagtgttgagtcccaatgatagaaattcgtataatcttgagcgtggtgataccatcaaacttcctgcaggaacaacctcttatttagttaactaagatgatgaagaagatcttagactggtagatcttgtaatacccgtgaatgggcctggtaaatttgagatactatataaaatacaataaatttttcttcagaagcgttattcttacaaaaacatccatttatattacttttacttttgtctataatgaaaaattgatattttccgttcttccatcaagcttttgacctagctaaaaataaaaactaatacttatgaggattcagcaagaatattttagaggcctcctataacataagtatgtgaagtttttatcattttttaataaataaaaccattttaatttgtatcattgtttacaactataaactagatacgagaccatagagaaggttctcttagaagaacaagagaaagatcggaaaaggagataataaggggaagaaacagatgcaatagtcaaagtgtcaagggaataaattgaggaattgaaaaagcttgccaaatcaagctcaaagaaaagcttaccctctgaatttgaaccaatcaacttgagaagccacaagccagaatattctaataagtttggcaagttgtttgagattactccggaaaaaaaatacccttaactttaagatttagatctatttgttagttgtgtggagattaacgagataagtacacaacactaaatatatataaaacatataattttaattatattacagaaatatgttaatgcgtttttgcttatatttttaaggagctctaatgttgccacactacaattcaagggctatagttgtactattggttaatgaaggaaaaggaaaccttgaacttctgggtttaaaaaatgagtaataagagagggaagatagaaaagaaagaaacaatgaggtgtagagatatgaagctagattgtctccgggtgacgttgttatcattccagcaggtcatccggttgccattactgcttcttcaaatttgaatttgcttggatttggtatcaatgctgagaacaatgagagaaactttctttcagatatttagtgaatattagtatgattacttaataagtctcggctaaatgagaattttttgaaattgatattttgattttggtgattgaaaatttgaaagctcggacgacaatgtgataagctaaattgaaaatccagtaaaagagcttacatttcctggatctgtttaagagataaatagactaataaagaactaaaagtaatctcactttgcaaatgctgaacctgaataaaaggagtaaggaagctagggaaaaaggagtcctctgtcttcaattttgggcactttttactaagtaatcagtatgaaaaataatacaacacgtatgtatgatgtaagtgttggataataaactatgaaaaataaggaggaaaatgtatgctgtaagatatagctagctcataatgagctaagaataaataaagggtcatgtaactcttgcttattgagtcccacctttctactatgaagaaataaataatgaataaaatttttgtctttttttaatttaaaagagtgtttgggcgctaaatttcttaac

SEQ ID NO: 46 - DNA, 2746 bp, synthetic construct
  source 1..2746: mol_type = other DNA
tatatggcacaatataaccaaatgtctatccacgttattcatctagctttatgttctatcactataaatatccttcatcttactcttttatttcatcatctaaacttttaactagtgaaatataaatcatggctaccactatcaaatcatgatttccacttttgttgttgctgggaattatattcctggcctctgttgtttgtgtcacttatgccaattacgatgaaggttcagaacctagggtaccggcataaagagagagaggtcgctaagagggtgagaaagaggaaaaacgccatggagaataaagaccttcctacgaaaaggaagaagatgaagaagagggataaagagaaagaggtcgctaagagggtgaaaaagaggaaaaacgccacggagaataaagaccttcgtatgaaaagtaagaagatgaagaagagaagtagaaatatagatattaacgtgaaaaggaagatgaagaagagaagtagaaatattaatattaacgtgaaaagaaggaataaaaggaagtttaacctggacgtgagagataagaaagagaggaagatgaggaataagtagacgaagagtaaagaggaagttaacgtcgtgaagatcccgaagaaagggcaaggctaaggcatagagaggagagaacaaaaagagacagacgccattaacgtgaaggagaggaggaagaaagatcttcagagtcataagaatgaagaaatccctttttatttaagtctaacaagtttctaacactctttgaaaacgaaaacggccacattcgtctcctttaaaggttcgacaaacgttcagacttatttgaaaatctctaaaactatcgtcttgtggaatatagagccaaaccccacaccatcttccttccttaacacatagatgctgacttaatccttgtagtcctcagtgataatttttattttactttataatattattataacaaatctttttgttttatagaaatatgactatttaaaataaaaacattgtaaagttcaatttaacaatatttcttatatttcataattaaattttggtttggttaatatgtattacaaggaaagccatattgacagtgttgagtcccaatgatagaaattcgtataatcttgagcgtggtgataccatcaaacttcctgcaggaacaacctcttatttagttaactaagatgatgaagaagatcttagactggtagatcttgtaatacccgtgaatgggcctggtaaatttgagatactatataaaatacaataaatttttcttcagaagcgttattcttacaaaaacatccatttatattacttttacttttgtctataatgaaaaattgatattttccgttcttccatcaagcttttgacctagctaaaaataaaaactaatacttatgaggattcagcaagaatattttagaggcctcctataacataagtatgtgaagtttttatcattttttaataaataaaaccattttaatttgtatcattgtttacaactataaactagatacgagaccatagagaaggttctcttagaagaataagagaaagatcggaaaaggagacaataaggggaagaaacagatgcaatagtcaaagtgtcaagggaataaattgaggaattgaaaaagcttgccaaatcaagctcaaagaaaagcttaccctctgaatttgaaccaatcaacttgagaagccacaagccagaatattctaataagtttggcaagttgtttgagattactccggaaaaaaaatacccttaactttaagatttagatctatttgttagttgtgtggagattaacgagataagtacacaacactaaatatatataaaacatataattttaattatattacagaaatatgttaatgcgtttttgcttatatttttaaggagctctaatgttgccacactacaattcaagggctatagttgtactattggttaatgaaggaaaaggaaaccttgaacttctgggtttaaaaaatgagtaataagagagggaagatagaaaagaaagaaacaatgaggtgtagagatatgaagctagattgtctccgggtgacgttgttatcattccagcaggtcatccggttgccattactgcttcttcaaatttgaatttgcttggatttggtatcaatgctgagaacaatgagagaaactttctttcagatatttagtgaatattagtatgattacttaataagtctcggctaaatgagaattttttgaaattgatattttgattttggtgattgaaaatttgaaagctcggacgacaatgtgataagctaaattgaaaatccagtaaaagagcttacatttcctggatctgtttaagagataaatagactaataaagaactaaaagtaatctcactttgcaaatgctgaacctgaataaaaggagtaaggaagctagggaaaaaggagtcctctgtcttcaattttgggcactttttactaagtaatcagtatgaaaaataatacaacacgtatgtatgatgtaagtgttggataataaactatgaaaaataaggaggaaaatgtatgctgtaagatatagctagctcataatgagctaagaataaataaagggtcatgtaactcttgcttattgagtcccacctttctactatgaagaaataaataatgaataaaatttttgtctttttttaatttaaaagagtgtttgggcgctaaatttcttaac

SEQ ID NO: 47 - DNA, 2746 bp, synthetic construct
  source 1..2746: mol_type = other DNA
tatatggcacaatataaccaaatgtctatccacgttattcatctagctttatgttctatcactataaatatccttcatcttactcttttatttcatcatctaaacttttaactagtgaaatataaatcatggctaccactatcaaatcatgatttccacttttgttgttgctgggaattatattcctggcctctgttgtttgtgtcacttatgccaattacgatgaaggttcagaacctagggtaccggcataaagagagagaggtcgctaagagggtgagaaagaggaaaaacgccatggagaataaagaccttcctacgaaaaggaagaagatgaagaagagggataaagagaaagaggtcgctaagagggtgaaaaagaggaaaaacgccacggagaataaagaccttcgtatgaaaagtaagaagatgaagaagagaagtagaaatatagatattaacgtgaaaaggaagatgaagaagagaagtagaaatattaatattaacgtgaaaagaaggaataaaaggaagtttaacctggacgtgagagataagaaagagaggaagatgaggaataagtagacgaagagtaaagaggaagttaacgtcgtgaagatcccgaagaaagggcaaggctaaggcatagagaggagagaacaaaaagagacagacgccattaacgtgaaggagaggaggaagaaagatcttcagagtcataagaatgaagaaatccctttttatttaagtctaacaagtttctaacactctttgaaaacgaaaacggccacattcgtctcctttaaaggttcgacaaacgttcagacttatttgaaaatctctaaaactatcgtcttgtggaatatagagccaaaccccacaccatcttccttccttaacacatagatgctgacttaatccttgtagtcctcagtgataatttttattttactttataatattattataacaaatctttttgttttatagaaatatgactatttaaaataaaaacattgtaaagttcaatttaacaatatttcttatatttcataattaaattttggtttggttaatatgtattacaaggaaagccatattgacagtgttgagtcccaatgatagaaattcgtataatcttgagcgtggtgataccatcaaacttcctgcaggaacaacctcttatttagttaactaagatgatgaagaagatcttagactggtagatcttgtaatacccgtgaatgggcctggtaaatttgagatactatataaaatacaataaatttttcttcagaagcgttattcttacaaaaacatccatttatattacttttacttttgtctataatgaaaaattgatattttccgttcttccatcaagcttttgacctagctaaaaataaaaactaatacttatgaggattcagcaagaatattttagaggcctcctataacataagtatgtgaagtttttatcattttttaataaataaaaccattttaatttgtatcattgtttacaactataaactagatacgagaccatagagaaggttctcttagaagaataagagaaagatcggaaaaggagataacaaggggaagaaacagatgcaatagtcaaagtgtcaagggaataaattgaggaattgaaaaagcttgccaaatcaagctcaaagaaaagcttaccctctgaatttgaaccaatcaacttgagaagccacaagccagaatattctaataagtttggcaagttgtttgagattactccggaaaaaaaatacccttaactttaagatttagatctatttgttagttgtgtggagattaacgagataagtacacaacactaaatatatataaaacatataattttaattatattacagaaatatgttaatgcgtttttgcttatatttttaaggagctctaatgttgccacactacaattcaagggctatagttgtactattggttaatgaaggaaaaggaaaccttgaacttctgggtttaaaaaatgagtaataagagagggaagatagaaaagaaagaaacaatgaggtgtagagatatgaagctagattgtctccgggtgacgttgttatcattccagcaggtcatccggttgccattactgcttcttcaaatttgaatttgcttggatttggtatcaatgctgagaacaatgagagaaactttctttcagatatttagtgaatattagtatgattacttaataagtctcggctaaatgagaattttttgaaattgatattttgattttggtgattgaaaatttgaaagctcggacgacaatgtgataagctaaattgaaaatccagtaaaagagcttacatttcctggatctgtttaagagataaatagactaataaagaactaaaagtaatctcactttgcaaatgctgaacctgaataaaaggagtaaggaagctagggaaaaaggagtcctctgtcttcaattttgggcactttttactaagtaatcagtatgaaaaataatacaacacgtatgtatgatgtaagtgttggataataaactatgaaaaataaggaggaaaatgtatgctgtaagatatagctagctcataatgagctaagaataaataaagggtcatgtaactcttgcttattgagtcccacctttctactatgaagaaataaataatgaataaaatttttgtctttttttaatttaaaagagtgtttgggcgctaaatttcttaac

SEQ ID NO: 48 - DNA, 2746 bp, synthetic construct
  source 1..2746: mol_type = other DNA
tatatggcacaatataaccaaatgtctatccacgttattcatctagctttatgttctatcactataaatatccttcatcttactcttttatttcatcatctaaacttttaactagtgaaatataaatcatggctaccactatcaaatcatgatttccacttttgttgttgctgggaattatattcctggcctctgttgtttgtgtcacttatgccaattacgatgaaggttcagaacctagggtaccggcataaagagagagaggtcgctaagagggtgagaaagaggaaaaacgccatggagaataaagaccttcctacgaaaaggaagaagatgaagaagagggataaagagaaagaggtcgctaagagggtgaaaaagaggaaaaacgccacggagaataaagaccttcgtatgaaaagtaagaagatgaagaagagaagtagaaatatagatattaacgtgaaaaggaagatgaagaagagaagtagaaatattaatattaacgtgaaaagaaggaataaaaggaagtttaacctggacgtgagagataagaaagagaggaagatgaggaataagtagacgaagagtaaagaggaagttaacgtcgtgaagatcccgaagaaagggcaaggctaaggcatagagaggagagaacaaaaagagacagacgccattaacgtgaaggagaggaggaagaaagatcttcagagtcataagaatgaagaaatccctttttatttaagtctaacaagtttctaacactctttgaaaacgaaaacggccacattcgtctcctttaaaggttcgacaaacgttcagacttatttgaaaatctctaaaactatcgtcttgtggaatatagagccaaaccccacaccatcttccttccttaacacatagatgctgacttaatccttgtagtcctcagtgataatttttattttactttataatattattataacaaatctttttgttttatagaaatatgactatttaaaataaaaacattgtaaagttcaatttaacaatatttcttatatttcataattaaattttggtttggttaatatgtattacaaggaaagccatattgacagtgttgagtcccaatgatagaaattcgtataatcttgagcgtggtgataccatcaaacttcctgcaggaacaacctcttatttagttaactaagatgatgaagaagatcttagactggtagatcttgtaatacccgtgaatgggcctggtaaatttgagatactatataaaatacaataaatttttcttcagaagcgttattcttacaaaaacatccatttatattacttttacttttgtctataatgaaaaattgatattttccgttcttccatcaagcttttgacctagctaaaaataaaaactaatacttatgaggattcagcaagaatattttagaggcctcctataacataagtatgtgaagtttttatcattttttaataaataaaaccattttaatttgtatcattgtttacaactataaactagatacgagaccatagagaaggttctcttagaagaataagagaaagatcggaaaaggagataataaggggaagaaacagatgcaatagtcaaagtgtcaagggaacaaattgaggaattgaaaaagcttgccaaatcaagctcaaagaaaagcttaccctctgaatttgaaccaatcaacttgagaagccacaagccagaatattctaataagtttggcaagttgtttgagattactccggaaaaaaaatacccttaactttaagatttagatctatttgttagttgtgtggagattaacgagataagtacacaacactaaatatatataaaacatataattttaattatattacagaaatatgttaatgcgtttttgcttatatttttaaggagctctaatgttgccacactacaattcaagggctatagttgtactattggttaatgaaggaaaaggaaaccttgaacttctgggtttaaaaaatgagtaataagagagggaagatagaaaagaaagaaacaatgaggtgtagagatatgaagctagattgtctccgggtgacgttgttatcattccagcaggtcatccggttgccattactgcttcttcaaatttgaatttgcttggatttggtatcaatgctgagaacaatgagagaaactttctttcagatatttagtgaatattagtatgattacttaataagtctcggctaaatgagaattttttgaaattgatattttgattttggtgattgaaaatttgaaagctcggacgacaatgtgataagctaaattgaaaatccagtaaaagagcttacatttcctggatctgtttaagagataaatagactaataaagaactaaaagtaatctcactttgcaaatgctgaacctgaataaaaggagtaaggaagctagggaaaaaggagtcctctgtcttcaattttgggcactttttactaagtaatcagtatgaaaaataatacaacacgtatgtatgatgtaagtgttggataataaactatgaaaaataaggaggaaaatgtatgctgtaagatatagctagctcataatgagctaagaataaataaagggtcatgtaactcttgcttattgagtcccacctttctactatgaagaaataaataatgaataaaatttttgtctttttttaatttaaaagagtgtttgggcgctaaatttcttaac

SEQ ID NO: 49 - DNA, 2746 bp, synthetic construct
  source 1..2746: mol_type = other DNA
tatatggcacaatataaccaaatgtctatccacgttattcatctagctttatgttctatcactataaatatccttcatcttactcttttatttcatcatctaaacttttaactagtgaaatataaatcatggctaccactatcaaatcatgatttccacttttgttgttgctgggaattatattcctggcctctgttgtttgtgtcacttatgccaattacgatgaaggttcagaacctagggtaccggcataaagagagagaggtcgctaagagggtgagaaagaggaaaaacgccatggagaataaagaccttcctacgaaaaggaagaagatgaagaagagggataaagagaaagaggtcgctaagagggtgaaaaagaggaaaaacgccacggagaataaagaccttcgtatgaaaagtaagaagatgaagaagagaagtagaaatatagatattaacgtgaaaaggaagatgaagaagagaagtagaaatattaatattaacgtgaaaagaaggaataaaaggaagtttaacctggacgtgagagataagaaagagaggaagatgaggaataagtagacgaagagtaaagaggaagttaacgtcgtgaagatcccgaagaaagggcaaggctaaggcatagagaggagagaacaaaaagagacagacgccattaacgtgaaggagaggaggaagaaagatcttcagagtcataagaatgaagaaatccctttttatttaagtctaacaagtttctaacactctttgaaaacgaaaacggccacattcgtctcctttaaaggttcgacaaacgttcagacttatttgaaaatctctaaaactatcgtcttgtggaatatagagccaaaccccacaccatcttccttccttaacacatagatgctgacttaatccttgtagtcctcagtgataatttttattttactttataatattattataacaaatctttttgttttatagaaatatgactatttaaaataaaaacattgtaaagttcaatttaacaatatttcttatatttcataattaaattttggtttggttaatatgtattacaaggaaagccatattgacagtgttgagtcccaatgatagaaattcgtataatcttgagcgtggtgataccatcaaacttcctgcaggaacaacctcttatttagttaactaagatgatgaagaagatcttagactggtagatcttgtaatacccgtgaatgggcctggtaaatttgagatactatataaaatacaataaatttttcttcagaagcgttattcttacaaaaacatccatttatattacttttacttttgtctataatgaaaaattgatattttccgttcttccatcaagcttttgacctagctaaaaataaaaactaatacttatgaggattcagcaagaatattttagaggcctcctataacataagtatgtgaagtttttatcattttttaataaataaaaccattttaatttgtatcattgtttacaactataaactagatacgagaccatagagaaggttctcttagaagaataagagaaagatcggaaaaggagataataaggggaagaaacagatgcaatagtcaaagtgtcaagggaataaattgaggaattgaaaaagcttgccaaatcaagctcaaagaaaagcttaccctctgaatttgaaccaatcaacttgagaagccacaagccagaatattctaataagtttggcaagttgtttgagattactccggaaaaaaaataccctcaactttaagatttagatctatttgttagttgtgtggagattaacgagataagtacacaacactaaatatatataaaacatataattttaattatattacagaaatatgttaatgcgtttttgcttatatttttaaggagctctaatgttgccacactacaattcaagggctatagttgtactattggttaatgaaggaaaaggaaaccttgaacttctgggtttaaaaaatgagtaataagagagggaagatagaaaagaaagaaacaatgaggtgtagagatatgaagctagattgtctccgggtgacgttgttatcattccagcaggtcatccggttgccattactgcttcttcaaatttgaatttgcttggatttggtatcaatgctgagaacaatgagagaaactttctttcagatatttagtgaatattagtatgattacttaataagtctcggctaaatgagaattttttgaaattgatattttgattttggtgattgaaaatttgaaagctcggacgacaatgtgataagctaaattgaaaatccagtaaaagagcttacatttcctggatctgtttaagagataaatagactaataaagaactaaaagtaatctcactttgcaaatgctgaacctgaataaaaggagtaaggaagctagggaaaaaggagtcctctgtcttcaattttgggcactttttactaagtaatcagtatgaaaaataatacaacacgtatgtatgatgtaagtgttggataataaactatgaaaaataaggaggaaaatgtatgctgtaagatatagctagctcataatgagctaagaataaataaagggtcatgtaactcttgcttattgagtcccacctttctactatgaagaaataaataatgaataaaatttttgtctttttttaatttaaaagagtgtttgggcgctaaatttcttaac

SEQ ID NO: 50 - DNA, 2746 bp, synthetic construct
  source 1..2746: mol_type = other DNA
tatatggcacaatataaccaaatgtctatccacgttattcatctagctttatgttctatcactataaatatccttcatcttactcttttatttcatcatctaaacttttaactagtgaaatataaatcatggctaccactatcaaatcatgatttccacttttgttgttgctgggaattatattcctggcctctgttgtttgtgtcacttatgccaattacgatgaaggttcagaacctagggtaccggcataaagagagagaggtcgctaagagggtgagaaagaggaaaaacgccatggagaataaagaccttcctacgaaaaggaagaagatgaagaagagggataaagagaaagaggtcgctaagagggtgaaaaagaggaaaaacgccacggagaataaagaccttcgtatgaaaagtaagaagatgaagaagagaagtagaaatatagatattaacgtgaaaaggaagatgaagaagagaagtagaaatattaatattaacgtgaaaagaaggaataaaaggaagtttaacctggacgtgagagataagaaagagaggaagatgaggaataagtagacgaagagtaaagaggaagttaacgtcgtgaagatcccgaagaaagggcaaggctaaggcatagagaggagagaacaaaaagagacagacgccattaacgtgaaggagaggaggaagaaagatcttcagagtcataagaatgaagaaatccctttttatttaagtctaacaagtttctaacactctttgaaaacgaaaacggccacattcgtctcctttaaaggttcgacaaacgttcagacttatttgaaaatctctaaaactatcgtcttgtggaatatagagccaaaccccacaccatcttccttccttaacacatagatgctgacttaatccttgtagtcctcagtgataatttttattttactttataatattattataacaaatctttttgttttatagaaatatgactatttaaaataaaaacattgtaaagttcaatttaacaatatttcttatatttcataattaaattttggtttggttaatatgtattacaaggaaagccatattgacagtgttgagtcccaatgatagaaattcgtataatcttgagcgtggtgataccatcaaacttcctgcaggaacaacctcttatttagttaactaagatgatgaagaagatcttagactggtagatcttgtaatacccgtgaatgggcctggtaaatttgagatactatataaaatacaataaatttttcttcagaagcgttattcttacaaaaacatccatttatattacttttacttttgtctataatgaaaaattgatattttccgttcttccatcaagcttttgacctagctaaaaataaaaactaatacttatgaggattcagcaagaatattttagaggcctcctataacataagtatgtgaagtttttatcattttttaataaataaaaccattttaatttgtatcattgtttacaactataaactagatacgagaccatagagaaggttctcttagaagaataagagaaagatcggaaaaggagataataaggggaagaaacagatgcaatagtcaaagtgtcaagggaataaattgaggaattgaaaaagcttgccaaatcaagctcaaagaaaagcttaccctctgaatttgaaccaatcaacttgagaagccacaagccagaatattctaataagtttggcaagttgtttgagattactccggaaaaaaaatacccttaacttcaagatttagatctatttgttagttgtgtggagattaacgagataagtacacaacactaaatatatataaaacatataattttaattatattacagaaatatgttaatgcgtttttgcttatatttttaaggagctctaatgttgccacactacaattcaagggctatagttgtactattggttaatgaaggaaaaggaaaccttgaacttctgggtttaaaaaatgagtaataagagagggaagatagaaaagaaagaaacaatgaggtgtagagatatgaagctagattgtctccgggtgacgttgttatcattccagcaggtcatccggttgccattactgcttcttcaaatttgaatttgcttggatttggtatcaatgctgagaacaatgagagaaactttctttcagatatttagtgaatattagtatgattacttaataagtctcggctaaatgagaattttttgaaattgatattttgattttggtgattgaaaatttgaaagctcggacgacaatgtgataagctaaattgaaaatccagtaaaagagcttacatttcctggatctgtttaagagataaatagactaataaagaactaaaagtaatctcactttgcaaatgctgaacctgaataaaaggagtaaggaagctagggaaaaaggagtcctctgtcttcaattttgggcactttttactaagtaatcagtatgaaaaataatacaacacgtatgtatgatgtaagtgttggataataaactatgaaaaataaggaggaaaatgtatgctgtaagatatagctagctcataatgagctaagaataaataaagggtcatgtaactcttgcttattgagtcccacctttctactatgaagaaataaataatgaataaaatttttgtctttttttaatttaaaagagtgtttgggcgctaaatttcttaac

SEQ ID NO: 51 - DNA, 2746 bp, synthetic construct
  source 1..2746: mol_type = other DNA
tatatggcacaatataaccaaatgtctatccacgttattcatctagctttatgttctatcactataaatatccttcatcttactcttttatttcatcatctaaacttttaactagtgaaatataaatcatggctaccactatcaaatcatgatttccacttttgttgttgctgggaattatattcctggcctctgttgtttgtgtcacttatgccaattacgatgaaggttcagaacctagggtaccggcataaagagagagaggtcgctaagagggtgagaaagaggaaaaacgccatggagaataaagaccttcctacgaaaaggaagaagatgaagaagagggataaagagaaagaggtcgctaagagggtgaaaaagaggaaaaacgccacggagaataaagaccttcgtatgaaaagtaagaagatgaagaagagaagtagaaatatagatattaacgtgaaaaggaagatgaagaagagaagtagaaatattaatattaacgtgaaaagaaggaataaaaggaagtttaacctggacgtgagagataagaaagagaggaagatgaggaataagtagacgaagagtaaagaggaagttaacgtcgtgaagatcccgaagaaagggcaaggctaaggcatagagaggagagaacaaaaagagacagacgccattaacgtgaaggagaggaggaagaaagatcttcagagtcataagaatgaagaaatccctttttatttaagtctaacaagtttctaacactctttgaaaacgaaaacggccacattcgtctcctttaaaggttcgacaaacgttcagacttatttgaaaatctctaaaactatcgtcttgtggaatatagagccaaaccccacaccatcttccttccttaacacatagatgctgacttaatccttgtagtcctcagtgataatttttattttactttataatattattataacaaatctttttgttttatagaaatatgactatttaaaataaaaacattgtaaagttcaatttaacaatatttcttatatttcataattaaattttggtttggttaatatgtattacaaggaaagccatattgacagtgttgagtcccaatgatagaaattcgtataatcttgagcgtggtgataccatcaaacttcctgcaggaacaacctcttatttagttaactaagatgatgaagaagatcttagactggtagatcttgtaatacccgtgaatgggcctggtaaatttgagatactatataaaatacaataaatttttcttcagaagcgttattcttacaaaaacatccatttatattacttttacttttgtctataatgaaaaattgatattttccgttcttccatcaagcttttgacctagctaaaaataaaaactaatacttatgaggattcagcaagaatattttagaggcctcctataacataagtatgtgaagtttttatcattttttaataaataaaaccattttaatttgtatcattgtttacaactataaactagatacgagaccatagagaaggttctcttagaagaataagagaaagatcggaaaaggagataataaggggaagaaacagatgcaatagtcaaagtgtcaagggaataaattgaggaattgaaaaagcttgccaaatcaagctcaaagaaaagcttaccctctgaatttgaaccaatcaacttgagaagccacaagccagaatattctaataagtttggcaagttgtttgagattactccggaaaaaaaatacccttaactttaagatttagatctatttgttagttgtgtggagattaacgaggtaagtacacaacactaaatatatataaaacatataattttaattatattacagaaatatgttaatgcgtttttgcttatatttttaaggagctctaatgttgccacactacaattcaagggctatagttgtactattggttaatgaaggaaaaggaaaccttgaacttctgggtttaaaaaatgagtaataagagagggaagatagaaaagaaagaaacaatgaggtgtagagatatgaagctagattgtctccgggtgacgttgttatcattccagcaggtcatccggttgccattactgcttcttcaaatttgaatttgcttggatttggtatcaatgctgagaacaatgagagaaactttctttcagatatttagtgaatattagtatgattacttaataagtctcggctaaatgagaattttttgaaattgatattttgattttggtgattgaaaatttgaaagctcggacgacaatgtgataagctaaattgaaaatccagtaaaagagcttacatttcctggatctgtttaagagataaatagactaataaagaactaaaagtaatctcactttgcaaatgctgaacctgaataaaaggagtaaggaagctagggaaaaaggagtcctctgtcttcaattttgggcactttttactaagtaatcagtatgaaaaataatacaacacgtatgtatgatgtaagtgttggataataaactatgaaaaataaggaggaaaatgtatgctgtaagatatagctagctcataatgagctaagaataaataaagggtcatgtaactcttgcttattgagtcccacctttctactatgaagaaataaataatgaataaaatttttgtctttttttaatttaaaagagtgtttgggcgctaaatttcttaac

SEQ ID NO: 52 - DNA, 2746 bp, synthetic construct
  source 1..2746: mol_type = other DNA
tatatggcacaatataaccaaatgtctatccacgttattcatctagctttatgttctatcactataaatatccttcatcttactcttttatttcatcatctaaacttttaactagtgaaatataaatcatggctaccactatcaaatcatgatttccacttttgttgttgctgggaattatattcctggcctctgttgtttgtgtcacttatgccaattacgatgaaggttcagaacctagggtaccggcataaagagagagaggtcgctaagagggtgagaaagaggaaaaacgccatggagaataaagaccttcctacgaaaaggaagaagatgaagaagagggataaagagaaagaggtcgctaagagggtgaaaaagaggaaaaacgccacggagaataaagaccttcgtatgaaaagtaagaagatgaagaagagaagtagaaatatagatattaacgtgaaaaggaagatgaagaagagaagtagaaatattaatattaacgtgaaaagaaggaataaaaggaagtttaacctggacgtgagagataagaaagagaggaagatgaggaataagtagacgaagagtaaagaggaagttaacgtcgtgaagatcccgaagaaagggcaaggctaaggcatagagaggagagaacaaaaagagacagacgccattaacgtgaaggagaggaggaagaaagatcttcagagtcataagaatgaagaaatccctttttatttaagtctaacaagtttctaacactctttgaaaacgaaaacggccacattcgtctcctttaaaggttcgacaaacgttcagacttatttgaaaatctctaaaactatcgtcttgtggaatatagagccaaaccccacaccatcttccttccttaacacatagatgctgacttaatccttgtagtcctcagtgataatttttattttactttataatattattataacaaatctttttgttttatagaaatatgactatttaaaataaaaacattgtaaagttcaatttaacaatatttcttatatttcataattaaattttggtttggttaatatgtattacaaggaaagccatattgacagtgttgagtcccaatgatagaaattcgtataatcttgagcgtggtgataccatcaaacttcctgcaggaacaacctcttatttagttaactaagatgatgaagaagatcttagactggtagatcttgtaatacccgtgaatgggcctggtaaatttgagatactatataaaatacaataaatttttcttcagaagcgttattcttacaaaaacatccatttatattacttttacttttgtctataatgaaaaattgatattttccgttcttccatcaagcttttgacctagctaaaaataaaaactaatacttatgaggattcagcaagaatattttagaggcctcctataacataagtatgtgaagtttttatcattttttaataaataaaaccattttaatttgtatcattgtttacaactataaactagatacgagaccatagagaaggttctcttagaagaataagagaaagatcggaaaaggagataataaggggaagaaacagatgcaatagtcaaagtgtcaagggaataaattgaggaattgaaaaagcttgccaaatcaagctcaaagaaaagcttaccctctgaatttgaaccaatcaacttgagaagccacaagccagaatattctaataagtttggcaagttgtttgagattactccggaaaaaaaatacccttaactttaagatttagatctatttgttagttgtgtggagattaacgagataagtacacaacactaaatatatataaaacatataattttaattatattacagaaatatgttaatgcgtttttgcttatatttttagggagctctaatgttgccacactacaattcaagggctatagttgtactattggttaatgaaggaaaaggaaaccttgaacttctgggtttaaaaaatgagtaataagagagggaagatagaaaagaaagaaacaatgaggtgtagagatatgaagctagattgtctccgggtgacgttgttatcattccagcaggtcatccggttgccattactgcttcttcaaatttgaatttgcttggatttggtatcaatgctgagaacaatgagagaaactttctttcagatatttagtgaatattagtatgattacttaataagtctcggctaaatgagaattttttgaaattgatattttgattttggtgattgaaaatttgaaagctcggacgacaatgtgataagctaaattgaaaatccagtaaaagagcttacatttcctggatctgtttaagagataaatagactaataaagaactaaaagtaatctcactttgcaaatgctgaacctgaataaaaggagtaaggaagctagggaaaaaggagtcctctgtcttcaattttgggcactttttactaagtaatcagtatgaaaaataatacaacacgtatgtatgatgtaagtgttggataataaactatgaaaaataaggaggaaaatgtatgctgtaagatatagctagctcataatgagctaagaataaataaagggtcatgtaactcttgcttattgagtcccacctttctactatgaagaaataaataatgaataaaatttttgtctttttttaatttaaaagagtgtttgggcgctaaatttcttaac

SEQ ID NO: 53 - DNA, 2746 bp, synthetic construct
  source 1..2746: mol_type = other DNA
tatatggcacaatataaccaaatgtctatccacgttattcatctagctttatgttctatcactataaatatccttcatcttactcttttatttcatcatctaaacttttaactagtgaaatataaatcatggctaccactatcaaatcatgatttccacttttgttgttgctgggaattatattcctggcctctgttgtttgtgtcacttatgccaattacgatgaaggttcagaacctagggtaccggcataaagagagagaggtcgctaagagggtgagaaagaggaaaaacgccatggagaataaagaccttcctacgaaaaggaagaagatgaagaagagggataaagagaaagaggtcgctaagagggtgaaaaagaggaaaaacgccacggagaataaagaccttcgtatgaaaagtaagaagatgaagaagagaagtagaaatatagatattaacgtgaaaaggaagatgaagaagagaagtagaaatattaatattaacgtgaaaagaaggaataaaaggaagtttaacctggacgtgagagataagaaagagaggaagatgaggaataagtagacgaagagtaaagaggaagttaacgtcgtgaagatcccgaagaaagggcaaggctaaggcatagagaggagagaacaaaaagagacagacgccattaacgtgaaggagaggaggaagaaagatcttcagagtcataagaatgaagaaatccctttttatttaagtctaacaagtttctaacactctttgaaaacgaaaacggccacattcgtctcctttaaaggttcgacaaacgttcagacttatttgaaaatctctaaaactatcgtcttgtggaatatagagccaaaccccacaccatcttccttccttaacacatagatgctgacttaatccttgtagtcctcagtgataatttttattttactttataatattattataacaaatctttttgttttatagaaatatgactatttaaaataaaaacattgtaaagttcaatttaacaatatttcttatatttcataattaaattttggtttggttaatatgtattacaaggaaagccatattgacagtgttgagtcccaatgatagaaattcgtataatcttgagcgtggtgataccatcaaacttcctgcaggaacaacctcttatttagttaactaagatgatgaagaagatcttagactggtagatcttgtaatacccgtgaatgggcctggtaaatttgagatactatataaaatacaataaatttttcttcagaagcgttattcttacaaaaacatccatttatattacttttacttttgtctataatgaaaaattgatattttccgttcttccatcaagcttttgacctagctaaaaataaaaactaatacttatgaggattcagcaagaatattttagaggcctcctataacataagtatgtgaagtttttatcattttttaataaataaaaccattttaatttgtatcattgtttacaactataaactagatacgagaccatagagaaggttctcttagaagaataagagaaagatcggaaaaggagataataaggggaagaaacagatgcaatagtcaaagtgtcaagggaataaattgaggaattgaaaaagcttgccaaatcaagctcaaagaaaagcttaccctctgaatttgaaccaatcaacttgagaagccacaagccagaatattctaataagtttggcaagttgtttgagattactccggaaaaaaaatacccttaactttaagatttagatctatttgttagttgtgtggagattaacgagataagtacacaacactaaatatatataaaacatataattttaattatattacagaaatatgttaatgcgtttttgcttatatttttaaggagctctaatgttgccacactacaattcaagggctatagttgtactattggttaatgaaggaaaaggaaaccttgaacttctgggtttaaaaaatgagcaataagagagggaagatagaaaagaaagaaacaatgaggtgtagagatatgaagctagattgtctccgggtgacgttgttatcattccagcaggtcatccggttgccattactgcttcttcaaatttgaatttgcttggatttggtatcaatgctgagaacaatgagagaaactttctttcagatatttagtgaatattagtatgattacttaataagtctcggctaaatgagaattttttgaaattgatattttgattttggtgattgaaaatttgaaagctcggacgacaatgtgataagctaaattgaaaatccagtaaaagagcttacatttcctggatctgtttaagagataaatagactaataaagaactaaaagtaatctcactttgcaaatgctgaacctgaataaaaggagtaaggaagctagggaaaaaggagtcctctgtcttcaattttgggcactttttactaagtaatcagtatgaaaaataatacaacacgtatgtatgatgtaagtgttggataataaactatgaaaaataaggaggaaaatgtatgctgtaagatatagctagctcataatgagctaagaataaataaagggtcatgtaactcttgcttattgagtcccacctttctactatgaagaaataaataatgaataaaatttttgtctttttttaatttaaaagagtgtttgggcgctaaatttcttaac

SEQ ID NO: 54 - DNA, 2746 bp, synthetic construct
  source 1..2746: mol_type = other DNA
tatatggcacaatataaccaaatgtctatccacgttattcatctagctttatgttctatcactataaatatccttcatcttactcttttatttcatcatctaaacttttaactagtgaaatataaatcatggctaccactatcaaatcatgatttccacttttgttgttgctgggaattatattcctggcctctgttgtttgtgtcacttatgccaattacgatgaaggttcagaacctagggtaccggcataaagagagagaggtcgctaagagggtgagaaagaggaaaaacgccatggagaataaagaccttcctacgaaaaggaagaagatgaagaagagggataaagagaaagaggtcgctaagagggtgaaaaagaggaaaaacgccacggagaataaagaccttcgtatgaaaagtaagaagatgaagaagagaagtagaaatatagatattaacgtgaaaaggaagatgaagaagagaagtagaaatattaatattaacgtgaaaagaaggaataaaaggaagtttaacctggacgtgagagataagaaagagaggaagatgaggaataagtagacgaagagtaaagaggaagttaacgtcgtgaagatcccgaagaaagggcaaggctaaggcatagagaggagagaacaaaaagagacagacgccattaacgtgaaggagaggaggaagaaagatcttcagagtcataagaatgaagaaatccctttttatttaagtctaacaagtttctaacactctttgaaaacgaaaacggccacattcgtctcctttaaaggttcgacaaacgttcagacttatttgaaaatctctaaaactatcgtcttgtggaatatagagccaaaccccacaccatcttccttccttaacacatagatgctgacttaatccttgtagtcctcagtgataatttttattttactttataatattattataacaaatctttttgttttatagaaatatgactatttaaaataaaaacattgtaaagttcaatttaacaatatttcttatatttcataattaaattttggtttggttaatatgtattacaaggaaagccatattgacagtgttgagtcccaatgatagaaattcgtataatcttgagcgtggtgataccatcaaacttcctgcaggaacaacctcttatttagttaactaagatgatgaagaagatcttagactggtagatcttgtaatacccgtgaatgggcctggtaaatttgagatactatataaaatacaataaatttttcttcagaagcgttattcttacaaaaacatccatttatattacttttacttttgtctataatgaaaaattgatattttccgttcttccatcaagcttttgacctagctaaaaataaaaactaatacttatgaggattcagcaagaatattttagaggcctcctataacataagtatgtgaagtttttatcattttttaataaataaaaccattttaatttgtatcattgtttacaactataaactagatacgagaccatagagaaggttctcttagaagaataagagaaagatcggaaaaggagataataaggggaagaaacagatgcaatagtcaaagtgtcaagggaataaattgaggaattgaaaaagcttgccaaatcaagctcaaagaaaagcttaccctctgaatttgaaccaatcaacttgagaagccacaagccagaatattctaataagtttggcaagttgtttgagattactccggaaaaaaaatacccttaactttaagatttagatctatttgttagttgtgtggagattaacgagataagtacacaacactaaatatatataaaacatataattttaattatattacagaaatatgttaatgcgtttttgcttatatttttaaggagctctaatgttgccacactacaattcaagggctatagttgtactattggttaatgaaggaaaaggaaaccttgaacttctgggtttaaaaaatgagtaacaagagagggaagatagaaaagaaagaaacaatgaggtgtagagatatgaagctagattgtctccgggtgacgttgttatcattccagcaggtcatccggttgccattactgcttcttcaaatttgaatttgcttggatttggtatcaatgctgagaacaatgagagaaactttctttcagatatttagtgaatattagtatgattacttaataagtctcggctaaatgagaattttttgaaattgatattttgattttggtgattgaaaatttgaaagctcggacgacaatgtgataagctaaattgaaaatccagtaaaagagcttacatttcctggatctgtttaagagataaatagactaataaagaactaaaagtaatctcactttgcaaatgctgaacctgaataaaaggagtaaggaagctagggaaaaaggagtcctctgtcttcaattttgggcactttttactaagtaatcagtatgaaaaataatacaacacgtatgtatgatgtaagtgttggataataaactatgaaaaataaggaggaaaatgtatgctgtaagatatagctagctcataatgagctaagaataaataaagggtcatgtaactcttgcttattgagtcccacctttctactatgaagaaataaataatgaataaaatttttgtctttttttaatttaaaagagtgtttgggcgctaaatttcttaac

SEQ ID NO: 55 - DNA, 2746 bp, synthetic construct
  source 1..2746: mol_type = other DNA
tatatggcacaatataaccaaatgtctatccacgttattcatctagctttatgttctatcactataaatatccttcatcttactcttttatttcatcatctaaacttttaactagtgaaatataaatcatggctaccactatcaaatcatgatttccacttttgttgttgctgggaattatattcctggcctctgttgtttgtgtcacttatgccaattacgatgaaggttcagaacctagggtaccggcataaagagagagaggtcgctaagagggtgagaaagaggaaaaacgccatggagaataaagaccttcctacgaaaaggaagaagatgaagaagagggataaagagaaagaggtcgctaagagggtgaaaaagaggaaaaacgccacggagaataaagaccttcgtatgaaaagtaagaagatgaagaagagaagtagaaatatagatattaacgtgaaaaggaagatgaagaagagaagtagaaatattaatattaacgtgaaaagaaggaataaaaggaagtttaacctggacgtgagagataagaaagagaggaagatgaggaataagtagacgaagagtaaagaggaagttaacgtcgtgaagatcccgaagaaagggcaaggctaaggcatagagaggagagaacaaaaagagacagacgccattaacgtgaaggagaggaggaagaaagatcttcagagtcataagaatgaagaaatccctttttatttaagtctaacaagtttctaacactctttgaaaacgaaaacggccacattcgtctcctttaaaggttcgacaaacgttcagacttatttgaaaatctctaaaactatcgtcttgtggaatatagagccaaaccccacaccatcttccttccttaacacatagatgctgacttaatccttgtagtcctcagtgataatttttattttactttataatattattataacaaatctttttgttttatagaaatatgactatttaaaataaaaacattgtaaagttcaatttaacaatatttcttatatttcataattaaattttggtttggttaatatgtattacaaggaaagccatattgacagtgttgagtcccaatgatagaaattcgtataatcttgagcgtggtgataccatcaaacttcctgcaggaacaacctcttatttagttaactaagatgatgaagaagatcttagactggtagatcttgtaatacccgtgaatgggcctggtaaatttgagatactatataaaatacaataaatttttcttcagaagcgttattcttacaaaaacatccatttatattacttttacttttgtctataatgaaaaattgatattttccgttcttccatcaagcttttgacctagctaaaaataaaaactaatacttatgaggattcagcaagaatattttagaggcctcctataacataagtatgtgaagtttttatcattttttaataaataaaaccattttaatttgtatcattgtttacaactataaactagatacgagaccatagagaaggttctcttagaagaataagagaaagatcggaaaaggagataataaggggaagaaacagatgcaatagtcaaagtgtcaagggaataaattgaggaattgaaaaagcttgccaaatcaagctcaaagaaaagcttaccctctgaatttgaaccaatcaacttgagaagccacaagccagaatattctaataagtttggcaagttgtttgagattactccggaaaaaaaatacccttaactttaagatttagatctatttgttagttgtgtggagattaacgagataagtacacaacactaaatatatataaaacatataattttaattatattacagaaatatgttaatgcgtttttgcttatatttttaaggagctctaatgttgccacactacaattcaagggctatagttgtactattggttaatgaaggaaaaggaaaccttgaacttctgggtttaaaaaatgagtaataagagagggaagatagaaaagaaagaaacaatgaggtgcagagatatgaagctagattgtctccgggtgacgttgttatcattccagcaggtcatccggttgccattactgcttcttcaaatttgaatttgcttggatttggtatcaatgctgagaacaatgagagaaactttctttcagatatttagtgaatattagtatgattacttaataagtctcggctaaatgagaattttttgaaattgatattttgattttggtgattgaaaatttgaaagctcggacgacaatgtgataagctaaattgaaaatccagtaaaagagcttacatttcctggatctgtttaagagataaatagactaataaagaactaaaagtaatctcactttgcaaatgctgaacctgaataaaaggagtaaggaagctagggaaaaaggagtcctctgtcttcaattttgggcactttttactaagtaatcagtatgaaaaataatacaacacgtatgtatgatgtaagtgttggataataaactatgaaaaataaggaggaaaatgtatgctgtaagatatagctagctcataatgagctaagaataaataaagggtcatgtaactcttgcttattgagtcccacctttctactatgaagaaataaataatgaataaaatttttgtctttttttaatttaaaagagtgtttgggcgctaaatttcttaac

SEQ ID NO: 56 - DNA, 2746 bp, synthetic construct
  source 1..2746: mol_type = other DNA
tatatggcacaatataaccaaatgtctatccacgttattcatctagctttatgttctatcactataaatatccttcatcttactcttttatttcatcatctaaacttttaactagtgaaatataaatcatggctaccactatcaaatcatgatttccacttttgttgttgctgggaattatattcctggcctctgttgtttgtgtcacttatgccaattacgatgaaggttcagaacctagggtaccggcataaagagagagaggtcgctaagagggtgagaaagaggaaaaacgccatggagaataaagaccttcctacgaaaaggaagaagatgaagaagagggataaagagaaagaggtcgctaagagggtgaaaaagaggaaaaacgccacggagaataaagaccttcgtatgaaaagtaagaagatgaagaagagaagtagaaatatagatattaacgtgaaaaggaagatgaagaagagaagtagaaatattaatattaacgtgaaaagaaggaataaaaggaagtttaacctggacgtgagagataagaaagagaggaagatgaggaataagtagacgaagagtaaagaggaagttaacgtcgtgaagatcccgaagaaagggcaaggctaaggcatagagaggagagaacaaaaagagacagacgccattaacgtgaaggagaggaggaagaaagatcttcagagtcataagaatgaagaaatccctttttatttaagtctaacaagtttctaacactctttgaaaacgaaaacggccacattcgtctcctttaaaggttcgacaaacgttcagacttatttgaaaatctctaaaactatcgtcttgtggaatatagagccaaaccccacaccatcttccttccttaacacatagatgctgacttaatccttgtagtcctcagtgataatttttattttactttataatattattataacaaatctttttgttttatagaaatatgactatttaaaataaaaacattgtaaagttcaatttaacaatatttcttatatttcataattaaattttggtttggttaatatgtattacaaggaaagccatattgacagtgttgagtcccaatgatagaaattcgtataatcttgagcgtggtgataccatcaaacttcctgcaggaacaacctcttatttagttaactaagatgatgaagaagatcttagactggtagatcttgtaatacccgtgaatgggcctggtaaatttgagatactatataaaatacaataaatttttcttcagaagcgttattcttacaaaaacatccatttatattacttttacttttgtctataatgaaaaattgatattttccgttcttccatcaagcttttgacctagctaaaaataaaaactaatacttatgaggattcagcaagaatattttagaggcctcctataacataagtatgtgaagtttttatcattttttaataaataaaaccattttaatttgtatcattgtttacaactataaactagatacgagaccatagagaaggttctcttagaagaataagagaaagatcggaaaaggagataataaggggaagaaacagatgcaatagtcaaagtgtcaagggaataaattgaggaattgaaaaagcttgccaaatcaagctcaaagaaaagcttaccctctgaatttgaaccaatcaacttgagaagccacaagccagaatattctaataagtttggcaagttgtttgagattactccggaaaaaaaatacccttaactttaagatttagatctatttgttagttgtgtggagattaacgagataagtacacaacactaaatatatataaaacatataattttaattatattacagaaatatgttaatgcgtttttgcttatatttttaaggagctctaatgttgccacactacaattcaagggctatagttgtactattggttaatgaaggaaaaggaaaccttgaacttctgggtttaaaaaatgagtaataagagagggaagatagaaaagaaagaaacaatgaggtgtagagatatgaagctagattgtctccgggtgacgttgttatcattccagcaggtcatccggttgccattactgcttcttcaaatttgaatttgcttggatttggtatcaatgctgagaacaatgagagaaactttctttcaggtatttagtgaatattagtatgattacttaataagtctcggctaaatgagaattttttgaaattgatattttgattttggtgattgaaaatttgaaagctcggacgacaatgtgataagctaaattgaaaatccagtaaaagagcttacatttcctggatctgtttaagagataaatagactaataaagaactaaaagtaatctcactttgcaaatgctgaacctgaataaaaggagtaaggaagctagggaaaaaggagtcctctgtcttcaattttgggcactttttactaagtaatcagtatgaaaaataatacaacacgtatgtatgatgtaagtgttggataataaactatgaaaaataaggaggaaaatgtatgctgtaagatatagctagctcataatgagctaagaataaataaagggtcatgtaactcttgcttattgagtcccacctttctactatgaagaaataaataatgaataaaatttttgtctttttttaatttaaaagagtgtttgggcgctaaatttcttaac

SEQ ID NO: 57 - DNA, 2746 bp, synthetic construct
  source 1..2746: mol_type = other DNA
tatatggcacaatataaccaaatgtctatccacgttattcatctagctttatgttctatcactataaatatccttcatcttactcttttatttcatcatctaaacttttaactagtgaaatataaatcatggctaccactatcaaatcatgatttccacttttgttgttgctgggaattatattcctggcctctgttgtttgtgtcacttatgccaattacgatgaaggttcagaacctagggtaccggcataaagagagagaggtcgctaagagggtgagaaagaggaaaaacgccatggagaataaagaccttcctacgaaaaggaagaagatgaagaagagggataaagagaaagaggtcgctaagagggtgaaaaagaggaaaaacgccacggagaataaagaccttcgtatgaaaagtaagaagatgaagaagagaagtagaaatatagatattaacgtgaaaaggaagatgaagaagagaagtagaaatattaatattaacgtgaaaagaaggaataaaaggaagtttaacctggacgtgagagataagaaagagaggaagatgaggaataagtagacgaagagtaaagaggaagttaacgtcgtgaagatcccgaagaaagggcaaggctaaggcatagagaggagagaacaaaaagagacagacgccattaacgtgaaggagaggaggaagaaagatcttcagagtcataagaatgaagaaatccctttttatttaagtctaacaagtttctaacactctttgaaaacgaaaacggccacattcgtctcctttaaaggttcgacaaacgttcagacttatttgaaaatctctaaaactatcgtcttgtggaatatagagccaaaccccacaccatcttccttccttaacacatagatgctgacttaatccttgtagtcctcagtgataatttttattttactttataatattattataacaaatctttttgttttatagaaatatgactatttaaaataaaaacattgtaaagttcaatttaacaatatttcttatatttcataattaaattttggtttggttaatatgtattacaaggaaagccatattgacagtgttgagtcccaatgatagaaattcgtataatcttgagcgtggtgataccatcaaacttcctgcaggaacaacctcttatttagttaactaagatgatgaagaagatcttagactggtagatcttgtaatacccgtgaatgggcctggtaaatttgagatactatataaaatacaataaatttttcttcagaagcgttattcttacaaaaacatccatttatattacttttacttttgtctataatgaaaaattgatattttccgttcttccatcaagcttttgacctagctaaaaataaaaactaatacttatgaggattcagcaagaatattttagaggcctcctataacataagtatgtgaagtttttatcattttttaataaataaaaccattttaatttgtatcattgtttacaactataaactagatacgagaccatagagaaggttctcttagaagaataagagaaagatcggaaaaggagataataaggggaagaaacagatgcaatagtcaaagtgtcaagggaataaattgaggaattgaaaaagcttgccaaatcaagctcaaagaaaagcttaccctctgaatttgaaccaatcaacttgagaagccacaagccagaatattctaataagtttggcaagttgtttgagattactccggaaaaaaaatacccttaactttaagatttagatctatttgttagttgtgtggagattaacgagataagtacacaacactaaatatatataaaacatataattttaattatattacagaaatatgttaatgcgtttttgcttatatttttaaggagctctaatgttgccacactacaattcaagggctatagttgtactattggttaatgaaggaaaaggaaaccttgaacttctgggtttaaaaaatgagtaataagagagggaagatagaaaagaaagaaacaatgaggtgtagagatatgaagctagattgtctccgggtgacgttgttatcattccagcaggtcatccggttgccattactgcttcttcaaatttgaatttgcttggatttggtatcaatgctgagaacaatgagagaaactttctttcagatatttagtgaatattagtatgattacttaataagtctcggctaaatgagaattttttgaaattgatattttgattttggtgattgaaaatttgaaggctcggacgacaatgtgataagctaaattgaaaatccagtaaaagagcttacatttcctggatctgtttaagagataaatagactaataaagaactaaaagtaatctcactttgcaaatgctgaacctgaataaaaggagtaaggaagctagggaaaaaggagtcctctgtcttcaattttgggcactttttactaagtaatcagtatgaaaaataatacaacacgtatgtatgatgtaagtgttggataataaactatgaaaaataaggaggaaaatgtatgctgtaagatatagctagctcataatgagctaagaataaataaagggtcatgtaactcttgcttattgagtcccacctttctactatgaagaaataaataatgaataaaatttttgtctttttttaatttaaaagagtgtttgggcgctaaatttcttaac

SEQ ID NO: 58 - DNA, 2746 bp, synthetic construct
  source 1..2746: mol_type = other DNA
tatatggcacaatataaccaaatgtctatccacgttattcatctagctttatgttctatcactataaatatccttcatcttactcttttatttcatcatctaaacttttaactagtgaaatataaatcatggctaccactatcaaatcatgatttccacttttgttgttgctgggaattatattcctggcctctgttgtttgtgtcacttatgccaattacgatgaaggttcagaacctagggtaccggcataaagagagagaggtcgctaagagggtgagaaagaggaaaaacgccatggagaataaagaccttcctacgaaaaggaagaagatgaagaagagggataaagagaaagaggtcgctaagagggtgaaaaagaggaaaaacgccacggagaataaagaccttcgtatgaaaagtaagaagatgaagaagagaagtagaaatatagatattaacgtgaaaaggaagatgaagaagagaagtagaaatattaatattaacgtgaaaagaaggaataaaaggaagtttaacctggacgtgagagataagaaagagaggaagatgaggaataagtagacgaagagtaaagaggaagttaacgtcgtgaagatcccgaagaaagggcaaggctaaggcatagagaggagagaacaaaaagagacagacgccattaacgtgaaggagaggaggaagaaagatcttcagagtcataagaatgaagaaatccctttttatttaagtctaacaagtttctaacactctttgaaaacgaaaacggccacattcgtctcctttaaaggttcgacaaacgttcagacttatttgaaaatctctaaaactatcgtcttgtggaatatagagccaaaccccacaccatcttccttccttaacacatagatgctgacttaatccttgtagtcctcagtgataatttttattttactttataatattattataacaaatctttttgttttatagaaatatgactatttaaaataaaaacattgtaaagttcaatttaacaatatttcttatatttcataattaaattttggtttggttaatatgtattacaaggaaagccatattgacagtgttgagtcccaatgatagaaattcgtataatcttgagcgtggtgataccatcaaacttcctgcaggaacaacctcttatttagttaactaagatgatgaagaagatcttagactggtagatcttgtaatacccgtgaatgggcctggtaaatttgagatactatataaaatacaataaatttttcttcagaagcgttattcttacaaaaacatccatttatattacttttacttttgtctataatgaaaaattgatattttccgttcttccatcaagcttttgacctagctaaaaataaaaactaatacttatgaggattcagcaagaatattttagaggcctcctataacataagtatgtgaagtttttatcattttttaataaataaaaccattttaatttgtatcattgtttacaactataaactagatacgagaccatagagaaggttctcttagaagaataagagaaagatcggaaaaggagataataaggggaagaaacagatgcaatagtcaaagtgtcaagggaataaattgaggaattgaaaaagcttgccaaatcaagctcaaagaaaagcttaccctctgaatttgaaccaatcaacttgagaagccacaagccagaatattctaataagtttggcaagttgtttgagattactccggaaaaaaaatacccttaactttaagatttagatctatttgttagttgtgtggagattaacgagataagtacacaacactaaatatatataaaacatataattttaattatattacagaaatatgttaatgcgtttttgcttatatttttaaggagctctaatgttgccacactacaattcaagggctatagttgtactattggttaatgaaggaaaaggaaaccttgaacttctgggtttaaaaaatgagtaataagagagggaagatagaaaagaaagaaacaatgaggtgtagagatatgaagctagattgtctccgggtgacgttgttatcattccagcaggtcatccggttgccattactgcttcttcaaatttgaatttgcttggatttggtatcaatgctgagaacaatgagagaaactttctttcagatatttagtgaatattagtatgattacttaataagtctcggctaaatgagaattttttgaaattgatattttgattttggtgattgaaaatttgaaagctcggacgacaatgtgataagccaaattgaaaatccagtaaaagagcttacatttcctggatctgtttaagagataaatagactaataaagaactaaaagtaatctcactttgcaaatgctgaacctgaataaaaggagtaaggaagctagggaaaaaggagtcctctgtcttcaattttgggcactttttactaagtaatcagtatgaaaaataatacaacacgtatgtatgatgtaagtgttggataataaactatgaaaaataaggaggaaaatgtatgctgtaagatatagctagctcataatgagctaagaataaataaagggtcatgtaactcttgcttattgagtcccacctttctactatgaagaaataaataatgaataaaatttttgtctttttttaatttaaaagagtgtttgggcgctaaatttcttaac

SEQ ID NO: 59 - DNA, 2746 bp, synthetic construct
  source 1..2746: mol_type = other DNA
tatatggcacaatataaccaaatgtctatccacgttattcatctagctttatgttctatcactataaatatccttcatcttactcttttatttcatcatctaaacttttaactagtgaaatataaatcatggctaccactatcaaatcatgatttccacttttgttgttgctgggaattatattcctggcctctgttgtttgtgtcacttatgccaattacgatgaaggttcagaacctagggtaccggcataaagagagagaggtcgctaagagggtgagaaagaggaaaaacgccatggagaataaagaccttcctacgaaaaggaagaagatgaagaagagggataaagagaaagaggtcgctaagagggtgaaaaagaggaaaaacgccacggagaataaagaccttcgtatgaaaagtaagaagatgaagaagagaagtagaaatatagatattaacgtgaaaaggaagatgaagaagagaagtagaaatattaatattaacgtgaaaagaaggaataaaaggaagtttaacctggacgtgagagataagaaagagaggaagatgaggaataagtagacgaagagtaaagaggaagttaacgtcgtgaagatcccgaagaaagggcaaggctaaggcatagagaggagagaacaaaaagagacagacgccattaacgtgaaggagaggaggaagaaagatcttcagagtcataagaatgaagaaatccctttttatttaagtctaacaagtttctaacactctttgaaaacgaaaacggccacattcgtctcctttaaaggttcgacaaacgttcagacttatttgaaaatctctaaaactatcgtcttgtggaatatagagccaaaccccacaccatcttccttccttaacacatagatgctgacttaatccttgtagtcctcagtgataatttttattttactttataatattattataacaaatctttttgttttatagaaatatgactatttaaaataaaaacattgtaaagttcaatttaacaatatttcttatatttcataattaaattttggtttggttaatatgtattacaaggaaagccatattgacagtgttgagtcccaatgatagaaattcgtataatcttgagcgtggtgataccatcaaacttcctgcaggaacaacctcttatttagttaactaagatgatgaagaagatcttagactggtagatcttgtaatacccgtgaatgggcctggtaaatttgagatactatataaaatacaataaatttttcttcagaagcgttattcttacaaaaacatccatttatattacttttacttttgtctataatgaaaaattgatattttccgttcttccatcaagcttttgacctagctaaaaataaaaactaatacttatgaggattcagcaagaatattttagaggcctcctataacataagtatgtgaagtttttatcattttttaataaataaaaccattttaatttgtatcattgtttacaactataaactagatacgagaccatagagaaggttctcttagaagaataagagaaagatcggaaaaggagataataaggggaagaaacagatgcaatagtcaaagtgtcaagggaataaattgaggaattgaaaaagcttgccaaatcaagctcaaagaaaagcttaccctctgaatttgaaccaatcaacttgagaagccacaagccagaatattctaataagtttggcaagttgtttgagattactccggaaaaaaaatacccttaactttaagatttagatctatttgttagttgtgtggagattaacgagataagtacacaacactaaatatatataaaacatataattttaattatattacagaaatatgttaatgcgtttttgcttatatttttaaggagctctaatgttgccacactacaattcaagggctatagttgtactattggttaatgaaggaaaaggaaaccttgaacttctgggtttaaaaaatgagtaataagagagggaagatagaaaagaaagaaacaatgaggtgtagagatatgaagctagattgtctccgggtgacgttgttatcattccagcaggtcatccggttgccattactgcttcttcaaatttgaatttgcttggatttggtatcaatgctgagaacaatgagagaaactttctttcagatatttagtgaatattagtatgattacttaataagtctcggctaaatgagaattttttgaaattgatattttgattttggtgattgaaaatttgaaagctcggacgacaatgtgataagctaaattgaaaatccagtaaaagagcttacatttcctggatctgttcaagagataaatagactaataaagaactaaaagtaatctcactttgcaaatgctgaacctgaataaaaggagtaaggaagctagggaaaaaggagtcctctgtcttcaattttgggcactttttactaagtaatcagtatgaaaaataatacaacacgtatgtatgatgtaagtgttggataataaactatgaaaaataaggaggaaaatgtatgctgtaagatatagctagctcataatgagctaagaataaataaagggtcatgtaactcttgcttattgagtcccacctttctactatgaagaaataaataatgaataaaatttttgtctttttttaatttaaaagagtgtttgggcgctaaatttcttaac

SEQ ID NO: 60 - DNA, 2746 bp, synthetic construct
  source 1..2746: mol_type = other DNA
tatatggcacaatataaccaaatgtctatccacgttattcatctagctttatgttctatcactataaatatccttcatcttactcttttatttcatcatctaaacttttaactagtgaaatataaatcatggctaccactatcaaatcatgatttccacttttgttgttgctgggaattatattcctggcctctgttgtttgtgtcacttatgccaattacgatgaaggttcagaacctagggtaccggcataaagagagagaggtcgctaagagggtgagaaagaggaaaaacgccatggagaataaagaccttcctacgaaaaggaagaagatgaagaagagggataaagagaaagaggtcgctaagagggtgaaaaagaggaaaaacgccacggagaataaagaccttcgtatgaaaagtaagaagatgaagaagagaagtagaaatatagatattaacgtgaaaaggaagatgaagaagagaagtagaaatattaatattaacgtgaaaagaaggaataaaaggaagtttaacctggacgtgagagataagaaagagaggaagatgaggaataagtagacgaagagtaaagaggaagttaacgtcgtgaagatcccgaagaaagggcaaggctaaggcatagagaggagagaacaaaaagagacagacgccattaacgtgaaggagaggaggaagaaagatcttcagagtcataagaatgaagaaatccctttttatttaagtctaacaagtttctaacactctttgaaaacgaaaacggccacattcgtctcctttaaaggttcgacaaacgttcagacttatttgaaaatctctaaaactatcgtcttgtggaatatagagccaaaccccacaccatcttccttccttaacacatagatgctgacttaatccttgtagtcctcagtgataatttttattttactttataatattattataacaaatctttttgttttatagaaatatgactatttaaaataaaaacattgtaaagttcaatttaacaatatttcttatatttcataattaaattttggtttggttaatatgtattacaaggaaagccatattgacagtgttgagtcccaatgatagaaattcgtataatcttgagcgtggtgataccatcaaacttcctgcaggaacaacctcttatttagttaactaagatgatgaagaagatcttagactggtagatcttgtaatacccgtgaatgggcctggtaaatttgagatactatataaaatacaataaatttttcttcagaagcgttattcttacaaaaacatccatttatattacttttacttttgtctataatgaaaaattgatattttccgttcttccatcaagcttttgacctagctaaaaataaaaactaatacttatgaggattcagcaagaatattttagaggcctcctataacataagtatgtgaagtttttatcattttttaataaataaaaccattttaatttgtatcattgtttacaactataaactagatacgagaccatagagaaggttctcttagaagaataagagaaagatcggaaaaggagataataaggggaagaaacagatgcaatagtcaaagtgtcaagggaataaattgaggaattgaaaaagcttgccaaatcaagctcaaagaaaagcttaccctctgaatttgaaccaatcaacttgagaagccacaagccagaatattctaataagtttggcaagttgtttgagattactccggaaaaaaaatacccttaactttaagatttagatctatttgttagttgtgtggagattaacgagataagtacacaacactaaatatatataaaacatataattttaattatattacagaaatatgttaatgcgtttttgcttatatttttaaggagctctaatgttgccacactacaattcaagggctatagttgtactattggttaatgaaggaaaaggaaaccttgaacttctgggtttaaaaaatgagtaataagagagggaagatagaaaagaaagaaacaatgaggtgtagagatatgaagctagattgtctccgggtgacgttgttatcattccagcaggtcatccggttgccattactgcttcttcaaatttgaatttgcttggatttggtatcaatgctgagaacaatgagagaaactttctttcagatatttagtgaatattagtatgattacttaataagtctcggctaaatgagaattttttgaaattgatattttgattttggtgattgaaaatttgaaagctcggacgacaatgtgataagctaaattgaaaatccagtaaaagagcttacatttcctggatctgtttaagagataaatagactaataaagaaccaaaagtaatctcactttgcaaatgctgaacctgaataaaaggagtaaggaagctagggaaaaaggagtcctctgtcttcaattttgggcactttttactaagtaatcagtatgaaaaataatacaacacgtatgtatgatgtaagtgttggataataaactatgaaaaataaggaggaaaatgtatgctgtaagatatagctagctcataatgagctaagaataaataaagggtcatgtaactcttgcttattgagtcccacctttctactatgaagaaataaataatgaataaaatttttgtctttttttaatttaaaagagtgtttgggcgctaaatttcttaac

SEQ ID NO: 61 - DNA, 2746 bp, synthetic construct
  source 1..2746: mol_type = other DNA
tatatggcacaatataaccaaatgtctatccacgttattcatctagctttatgttctatcactataaatatccttcatcttactcttttatttcatcatctaaacttttaactagtgaaatataaatcatggctaccactatcaaatcatgatttccacttttgttgttgctgggaattatattcctggcctctgttgtttgtgtcacttatgccaattacgatgaaggttcagaacctagggtaccggcataaagagagagaggtcgctaagagggtgagaaagaggaaaaacgccatggagaataaagaccttcctacgaaaaggaagaagatgaagaagagggataaagagaaagaggtcgctaagagggtgaaaaagaggaaaaacgccacggagaataaagaccttcgtatgaaaagtaagaagatgaagaagagaagtagaaatatagatattaacgtgaaaaggaagatgaagaagagaagtagaaatattaatattaacgtgaaaagaaggaataaaaggaagtttaacctggacgtgagagataagaaagagaggaagatgaggaataagtagacgaagagtaaagaggaagttaacgtcgtgaagatcccgaagaaagggcaaggctaaggcatagagaggagagaacaaaaagagacagacgccattaacgtgaaggagaggaggaagaaagatcttcagagtcataagaatgaagaaatccctttttatttaagtctaacaagtttctaacactctttgaaaacgaaaacggccacattcgtctcctttaaaggttcgacaaacgttcagacttatttgaaaatctctaaaactatcgtcttgtggaatatagagccaaaccccacaccatcttccttccttaacacatagatgctgacttaatccttgtagtcctcagtgataatttttattttactttataatattattataacaaatctttttgttttatagaaatatgactatttaaaataaaaacattgtaaagttcaatttaacaatatttcttatatttcataattaaattttggtttggttaatatgtattacaaggaaagccatattgacagtgttgagtcccaatgatagaaattcgtataatcttgagcgtggtgataccatcaaacttcctgcaggaacaacctcttatttagttaactaagatgatgaagaagatcttagactggtagatcttgtaatacccgtgaatgggcctggtaaatttgagatactatataaaatacaataaatttttcttcagaagcgttattcttacaaaaacatccatttatattacttttacttttgtctataatgaaaaattgatattttccgttcttccatcaagcttttgacctagctaaaaataaaaactaatacttatgaggattcagcaagaatattttagaggcctcctataacataagtatgtgaagtttttatcattttttaataaataaaaccattttaatttgtatcattgtttacaactataaactagatacgagaccatagagaaggttctcttagaagaataagagaaagatcggaaaaggagataataaggggaagaaacagatgcaatagtcaaagtgtcaagggaataaattgaggaattgaaaaagcttgccaaatcaagctcaaagaaaagcttaccctctgaatttgaaccaatcaacttgagaagccacaagccagaatattctaataagtttggcaagttgtttgagattactccggaaaaaaaatacccttaactttaagatttagatctatttgttagttgtgtggagattaacgagataagtacacaacactaaatatatataaaacatataattttaattatattacagaaatatgttaatgcgtttttgcttatatttttaaggagctctaatgttgccacactacaattcaagggctatagttgtactattggttaatgaaggaaaaggaaaccttgaacttctgggtttaaaaaatgagtaataagagagggaagatagaaaagaaagaaacaatgaggtgtagagatatgaagctagattgtctccgggtgacgttgttatcattccagcaggtcatccggttgccattactgcttcttcaaatttgaatttgcttggatttggtatcaatgctgagaacaatgagagaaactttctttcagatatttagtgaatattagtatgattacttaataagtctcggctaaatgagaattttttgaaattgatattttgattttggtgattgaaaatttgaaagctcggacgacaatgtgataagctaaattgaaaatccagtaaaagagcttacatttcctggatctgtttaagagataaatagactaataaagaactaaaagcaatctcactttgcaaatgctgaacctgaataaaaggagtaaggaagctagggaaaaaggagtcctctgtcttcaattttgggcactttttactaagtaatcagtatgaaaaataatacaacacgtatgtatgatgtaagtgttggataataaactatgaaaaataaggaggaaaatgtatgctgtaagatatagctagctcataatgagctaagaataaataaagggtcatgtaactcttgcttattgagtcccacctttctactatgaagaaataaataatgaataaaatttttgtctttttttaatttaaaagagtgtttgggcgctaaatttcttaac

SEQ ID NO: 62 - DNA, 2746 bp, synthetic construct
  source 1..2746: mol_type = other DNA
tatatggcacaatataaccaaatgtctatccacgttattcatctagctttatgttctatcactataaatatccttcatcttactcttttatttcatcatctaaacttttaactagtgaaatataaatcatggctaccactatcaaatcatgatttccacttttgttgttgctgggaattatattcctggcctctgttgtttgtgtcacttatgccaattacgatgaaggttcagaacctagggtaccggcataaagagagagaggtcgctaagagggtgagaaagaggaaaaacgccatggagaataaagaccttcctacgaaaaggaagaagatgaagaagagggataaagagaaagaggtcgctaagagggtgaaaaagaggaaaaacgccacggagaataaagaccttcgtatgaaaagtaagaagatgaagaagagaagtagaaatatagatattaacgtgaaaaggaagatgaagaagagaagtagaaatattaatattaacgtgaaaagaaggaataaaaggaagtttaacctggacgtgagagataagaaagagaggaagatgaggaataagtagacgaagagtaaagaggaagttaacgtcgtgaagatcccgaagaaagggcaaggctaaggcatagagaggagagaacaaaaagagacagacgccattaacgtgaaggagaggaggaagaaagatcttcagagtcataagaatgaagaaatccctttttatttaagtctaacaagtttctaacactctttgaaaacgaaaacggccacattcgtctcctttaaaggttcgacaaacgttcagacttatttgaaaatctctaaaactatcgtcttgtggaatatagagccaaaccccacaccatcttccttccttaacacatagatgctgacttaatccttgtagtcctcagtgataatttttattttactttataatattattataacaaatctttttgttttatagaaatatgactatttaaaataaaaacattgtaaagttcaatttaacaatatttcttatatttcataattaaattttggtttggttaatatgtattacaaggaaagccatattgacagtgttgagtcccaatgatagaaattcgtataatcttgagcgtggtgataccatcaaacttcctgcaggaacaacctcttatttagttaactaagatgatgaagaagatcttagactggtagatcttgtaatacccgtgaatgggcctggtaaatttgagatactatataaaatacaataaatttttcttcagaagcgttattcttacaaaaacatccatttatattacttttacttttgtctataatgaaaaattgatattttccgttcttccatcaagcttttgacctagctaaaaataaaaactaatacttatgaggattcagcaagaatattttagaggcctcctataacataagtatgtgaagtttttatcattttttaataaataaaaccattttaatttgtatcattgtttacaactataaactagatacgagaccatagagaaggttctcttagaagaataagagaaagatcggaaaaggagataataaggggaagaaacagatgcaatagtcaaagtgtcaagggaataaattgaggaattgaaaaagcttgccaaatcaagctcaaagaaaagcttaccctctgaatttgaaccaatcaacttgagaagccacaagccagaatattctaataagtttggcaagttgtttgagattactccggaaaaaaaatacccttaactttaagatttagatctatttgttagttgtgtggagattaacgagataagtacacaacactaaatatatataaaacatataattttaattatattacagaaatatgttaatgcgtttttgcttatatttttaaggagctctaatgttgccacactacaattcaagggctatagttgtactattggttaatgaaggaaaaggaaaccttgaacttctgggtttaaaaaatgagtaataagagagggaagatagaaaagaaagaaacaatgaggtgtagagatatgaagctagattgtctccgggtgacgttgttatcattccagcaggtcatccggttgccattactgcttcttcaaatttgaatttgcttggatttggtatcaatgctgagaacaatgagagaaactttctttcagatatttagtgaatattagtatgattacttaataagtctcggctaaatgagaattttttgaaattgatattttgattttggtgattgaaaatttgaaagctcggacgacaatgtgataagctaaattgaaaatccagtaaaagagcttacatttcctggatctgtttaagagataaatagactaataaagaactaaaagtaatctcactttgcaaatgctgaacctgaacaaaaggagtaaggaagctagggaaaaaggagtcctctgtcttcaattttgggcactttttactaagtaatcagtatgaaaaataatacaacacgtatgtatgatgtaagtgttggataataaactatgaaaaataaggaggaaaatgtatgctgtaagatatagctagctcataatgagctaagaataaataaagggtcatgtaactcttgcttattgagtcccacctttctactatgaagaaataaataatgaataaaatttttgtctttttttaatttaaaagagtgtttgggcgctaaatttcttaac

SEQ ID NO: 63 - DNA, 2746 bp, synthetic construct
  source 1..2746: mol_type = other DNA
tatatggcacaatataaccaaatgtctatccacgttattcatctagctttatgttctatcactataaatatccttcatcttactcttttatttcatcatctaaacttttaactagtgaaatataaatcatggctaccactatcaaatcatgatttccacttttgttgttgctgggaattatattcctggcctctgttgtttgtgtcacttatgccaattacgatgaaggttcagaacctagggtaccggcataaagagagagaggtcgctaagagggtgagaaagaggaaaaacgccatggagaataaagaccttcctacgaaaaggaagaagatgaagaagagggataaagagaaagaggtcgctaagagggtgaaaaagaggaaaaacgccacggagaataaagaccttcgtatgaaaagtaagaagatgaagaagagaagtagaaatatagatattaacgtgaaaaggaagatgaagaagagaagtagaaatattaatattaacgtgaaaagaaggaataaaaggaagtttaacctggacgtgagagataagaaagagaggaagatgaggaataagtagacgaagagtaaagaggaagttaacgtcgtgaagatcccgaagaaagggcaaggctaaggcatagagaggagagaacaaaaagagacagacgccattaacgtgaaggagaggaggaagaaagatcttcagagtcataagaatgaagaaatccctttttatttaagtctaacaagtttctaacactctttgaaaacgaaaacggccacattcgtctcctttaaaggttcgacaaacgttcagacttatttgaaaatctctaaaactatcgtcttgtggaatatagagccaaaccccacaccatcttccttccttaacacatagatgctgacttaatccttgtagtcctcagtgataatttttattttactttataatattattataacaaatctttttgttttatagaaatatgactatttaaaataaaaacattgtaaagttcaatttaacaatatttcttatatttcataattaaattttggtttggttaatatgtattacaaggaaagccatattgacagtgttgagtcccaatgatagaaattcgtataatcttgagcgtggtgataccatcaaacttcctgcaggaacaacctcttatttagttaactaagatgatgaagaagatcttagactggtagatcttgtaatacccgtgaatgggcctggtaaatttgagatactatataaaatacaataaatttttcttcagaagcgttattcttacaaaaacatccatttatattacttttacttttgtctataatgaaaaattgatattttccgttcttccatcaagcttttgacctagctaaaaataaaaactaatacttatgaggattcagcaagaatattttagaggcctcctataacataagtatgtgaagtttttatcattttttaataaataaaaccattttaatttgtatcattgtttacaactataaactagatacgagaccatagagaaggttctcttagaagaataagagaaagatcggaaaaggagataataaggggaagaaacagatgcaatagtcaaagtgtcaagggaataaattgaggaattgaaaaagcttgccaaatcaagctcaaagaaaagcttaccctctgaatttgaaccaatcaacttgagaagccacaagccagaatattctaataagtttggcaagttgtttgagattactccggaaaaaaaatacccttaactttaagatttagatctatttgttagttgtgtggagattaacgagataagtacacaacactaaatatatataaaacatataattttaattatattacagaaatatgttaatgcgtttttgcttatatttttaaggagctctaatgttgccacactacaattcaagggctatagttgtactattggttaatgaaggaaaaggaaaccttgaacttctgggtttaaaaaatgagtaataagagagggaagatagaaaagaaagaaacaatgaggtgtagagatatgaagctagattgtctccgggtgacgttgttatcattccagcaggtcatccggttgccattactgcttcttcaaatttgaatttgcttggatttggtatcaatgctgagaacaatgagagaaactttctttcagatatttagtgaatattagtatgattacttaataagtctcggctaaatgagaattttttgaaattgatattttgattttggtgattgaaaatttgaaagctcggacgacaatgtgataagctaaattgaaaatccagtaaaagagcttacatttcctggatctgtttaagagataaatagactaataaagaactaaaagtaatctcactttgcaaatgctgaacctgaataaaaggagcaaggaagctagggaaaaaggagtcctctgtcttcaattttgggcactttttactaagtaatcagtatgaaaaataatacaacacgtatgtatgatgtaagtgttggataataaactatgaaaaataaggaggaaaatgtatgctgtaagatatagctagctcataatgagctaagaataaataaagggtcatgtaactcttgcttattgagtcccacctttctactatgaagaaataaataatgaataaaatttttgtctttttttaatttaaaagagtgtttgggcgctaaatttcttaac

SEQ ID NO: 64 - DNA, 2746 bp, synthetic construct
  source 1..2746: mol_type = other DNA
tatatggcacaatataaccaaatgtctatccacgttattcatctagctttatgttctatcactataaatatccttcatcttactcttttatttcatcatctaaacttttaactagtgaaatataaatcatggctaccactatcaaatcatgatttccacttttgttgttgctgggaattatattcctggcctctgttgtttgtgtcacttatgccaattacgatgaaggttcagaacctagggtaccggcataaagagagagaggtcgctaagagggtgagaaagaggaaaaacgccatggagaataaagaccttcctacgaaaaggaagaagatgaagaagagggataaagagaaagaggtcgctaagagggtgaaaaagaggaaaaacgccacggagaataaagaccttcgtatgaaaagtaagaagatgaagaagagaagtagaaatatagatattaacgtgaaaaggaagatgaagaagagaagtagaaatattaatattaacgtgaaaagaaggaataaaaggaagtttaacctggacgtgagagataagaaagagaggaagatgaggaataagtagacgaagagtaaagaggaagttaacgtcgtgaagatcccgaagaaagggcaaggctaaggcatagagaggagagaacaaaaagagacagacgccattaacgtgaaggagaggaggaagaaagatcttcagagtcataagaatgaagaaatccctttttatttaagtctaacaagtttctaacactctttgaaaacgaaaacggccacattcgtctcctttaaaggttcgacaaacgttcagacttatttgaaaatctctaaaactatcgtcttgtggaatatagagccaaaccccacaccatcttccttccttaacacatagatgctgacttaatccttgtagtcctcagtgataatttttattttactttataatattattataacaaatctttttgttttatagaaatatgactatttaaaataaaaacattgtaaagttcaatttaacaatatttcttatatttcataattaaattttggtttggttaatatgtattacaaggaaagccatattgacagtgttgagtcccaatgatagaaattcgtataatcttgagcgtggtgataccatcaaacttcctgcaggaacaacctcttatttagttaactaagatgatgaagaagatcttagactggtagatcttgtaatacccgtgaatgggcctggtaaatttgagatactatataaaatacaataaatttttcttcagaagcgttattcttacaaaaacatccatttatattacttttacttttgtctataatgaaaaattgatattttccgttcttccatcaagcttttgacctagctaaaaataaaaactaatacttatgaggattcagcaagaatattttagaggcctcctataacataagtatgtgaagtttttatcattttttaataaataaaaccattttaatttgtatcattgtttacaactataaactagatacgagaccatagagaaggttctcttagaagaataagagaaagatcggaaaaggagataataaggggaagaaacagatgcaatagtcaaagtgtcaagggaataaattgaggaattgaaaaagcttgccaaatcaagctcaaagaaaagcttaccctctgaatttgaaccaatcaacttgagaagccacaagccagaatattctaataagtttggcaagttgtttgagattactccggaaaaaaaatacccttaactttaagatttagatctatttgttagttgtgtggagattaacgagataagtacacaacactaaatatatataaaacatataattttaattatattacagaaatatgttaatgcgtttttgcttatatttttaaggagctctaatgttgccacactacaattcaagggctatagttgtactattggttaatgaaggaaaaggaaaccttgaacttctgggtttaaaaaatgagtaataagagagggaagatagaaaagaaagaaacaatgaggtgtagagatatgaagctagattgtctccgggtgacgttgttatcattccagcaggtcatccggttgccattactgcttcttcaaatttgaatttgcttggatttggtatcaatgctgagaacaatgagagaaactttctttcagatatttagtgaatattagtatgattacttaataagtctcggctaaatgagaattttttgaaattgatattttgattttggtgattgaaaatttgaaagctcggacgacaatgtgataagctaaattgaaaatccagtaaaagagcttacatttcctggatctgtttaagagataaatagactaataaagaactaaaagtaatctcactttgcaaatgctgaacctgaataaaaggagtaaggaagccagggaaaaaggagtcctctgtcttcaattttgggcactttttactaagtaatcagtatgaaaaataatacaacacgtatgtatgatgtaagtgttggataataaactatgaaaaataaggaggaaaatgtatgctgtaagatatagctagctcataatgagctaagaataaataaagggtcatgtaactcttgcttattgagtcccacctttctactatgaagaaataaataatgaataaaatttttgtctttttttaatttaaaagagtgtttgggcgctaaatttcttaac

SEQ ID NO: 65 - DNA, 3400 bp, Pisum sativum
  source 1..3400: mol_type = genomic DNA
gacacggtgagagtaacagaagatagtattaatgactaagtagaagaaatatttctgaccattgattggtgacgaaaactacccctataaagtttactcgcagttaaacatcgaaatatccattatttttttgtcatttactttttcattattattatataagtttaaacacttagaatcataaaaattattaaatctatctttaagcacaacaaacaaatctatctatggatagaataatattgtacctgttgactccaaatacacaacaataatatgaaaaatagaataataaattcaaatggttagaatatatttttacttagataccaaagttttaccatctttcttgtctttcttaagaactatctgaatcaattttgacctcaactattagaataagaaactttatccaaatctataaataaaagaaaacatttgaaattgggttaacaatttaggctcaatccttccaagtctcgaagtctcgattattacgcaactcctcttacatttcatcttttcctcatagaacatttacattaaaacaaagagtccaattaatattcagaacttcatattgtaaatctaacattgatataaccgtcatgaaaatatattttctagagagaaaagaaattgcacaacctcgtcttaactcacaaattacaaaacacttccaattttttaatttaaagaaaagatataaaaacataaacaaattaaagcaactaatacaagagtaaggcactgcatgttatgaaccattacaataataacacaaccaataaccattattaaaaacaattttaaaaattccttcattgaatccatagtctttttttaagacttaccccaagaacacaaattaatattatccttgtagttaaagtaaaaaaaaagcacaagttttattaattatttatttattcgtatagaaaagtggggctcaataggtaagagttacaagatccattatttactcttagctcacgaagagctagctagatcttagctcatacatctgcattatttttcatattgattactcagtaaaaactgtccagaactgaagacagaggactcctttttctttggctttcttcctccttttgttcaggttcagcacttgcaaagtgagattgtttttgattcttgattaatctatttacctcttgagaagatccaggaaatgtgagctcctttactggattttctatttggcttatcacattgtcatccgatccttcaaattttcaatccccaaattagaaatataacattcaaatattaactaatgatatttctattcacttaatacctgaaaggaagtttctctgattgttctcggcattgataccaaatccaaccaaattcagatttgatgaagcactaatggcaactgggtgacctgctggaatgataacaacgtcacccggagacaatctagcttcatatctctgcacttcattgtttctttcttttctatcttccctctcttgttgctcattttttaaacccagaagttcaaggtttccttttccttcattaactaatagtacaactattgcccttgaattgtagtgtggcaacattagagctccctaaaaatttaagcaaaaacgcattaacatatttctgtaatataattaaaattatgtgttttatatatatttagtgttgtgtacataccttgttaatctccacacaactaacaagtatatctaaatcttgaagctgagggtattttttctctggagtaatctcaaacaacttgccaaacttattagaatattctggcttgtggcttctcaagttgaaaggttcaaattcagagggtaagcttttctttgagcttgattttgcaagctttctcaattcctcaatttgttcccttgatactttgattattgcgtctctttcttccccttgttgtgttcttttccgatctctcaattgttgtggttttttctcttgctcttctaaaagaaccttctctatggtctcgtatttagtctatatttgcgaaaaaggatacaaaatataatggttatatttattaaacatttgataaaaaaatcacacattaagcttaacatgtgttgtttgcatacttacatttaaggaggcctctaaaatgttcttgctgaatcctcgtaagtattggtttttattttcagatagaccaaaagcctgtagaagaaggataaagatcaatttttcaatccagacaaaaataaaagtaatataaaggaggtgttttaataagaataaaacatgtgaagaaaattattacctcaaatttaccaggcctgttcacgggtattacaaaatccaccactcttagatcttcttcatcatcttggttaactagataagatgttgttcctgcgggaattttgatggtatcaccacgctcaagattatacgagtttctatcattgggactcaacactgtcaatatggctttccctgtagtacatattaaccacaccaaaatttaattatgaaatataagaaatattgctaaattgaactttacaatatttttattttaaatagtcatatttctataaaacaaaagatttgttataataatattataaagaaaaataaaaattaccattgaggactacaaggattaagtcagcatctatgtgttgaggaaggaagatggtgtggggtttggctctatattccacaagacgatagttttggagattttcaaataagtctgaacgtttgtcgaacctttgaaggcgacgaatgtgaccgttttcgttttcaaagagtgtcagaaacttgttagacttgaataaaaaggggtttctttgttcttgtgattctgaagatctttcttcctcctctccttcacgttgatggcgtctgtctctttttgttctctcctctctatgccttagccttgccctttcttcgggatcttcacgacgttgacttcctctccactcttcgtctacttgttcctcatcttcctctctttcccatctctcacgtccaggttgaacttccttttgttccttcttttcacgttgatatcgatatttctgcttctcttcttcatcttcttccttttcatatgaaggtctccattctccatggcgtttttcttctttctcaccctcttggcgacctctttctctttgtcccggtaccctagtttctgaaccttcatcgtaattggcataagtgacgcaaacagaggccaggaatataattcccagaaacaataaaagtggaaatcgtgatttgacagtggtcgccatgatttgtatttcactagttcgaactttagatgatgaaataaaagattaagttgaaggatatttatagtgatagaacgtaaagctagatgaataacgtggatggtcatttgggtaca

SEQ ID NO: 66 - DNA, 3400 bp, Pisum sativum
  source 1..3400: mol_type = other DNA
gacacggtgagagtaacagaagatagtattaatgactaagtagaagaaatatttctgaccattgattggtgacgaaaactacccctataaagtttactcgcagttaaacatcgaaatatccattatttttttgtcatttactttttcattattattatataagtttaaacacttagaatcataaaaattattaaatctatctttaagcacaacaaacaaatctatctatggatagaataatattgtacctgttgactccaaatacacaacaataatatgaaaaatagaataataaattcaaatggttagaatatatttttacttagataccaaagttttaccatctttcttgtctttcttaagaactatctgaatcaattttgacctcaactattagaataagaaactttatccaaatctataaataaaagaaaacatttgaaattgggttaacaatttaggctcaatccttccaagtctcgaagtctcgattattacgcaactcctcttacatttcatcttttcctcatagaacatttacattaaaacaaagagtccaattaatattcagaacttcatattgtaaatctaacattgatataaccgtcatgaaaatatattttctagagagaaaagaaattgcacaacctcgtcttaactcacaaattacaaaacacttccaattttttaatttaaagaaaagatataaaaacataaacaaattaaagcaactaatacaagagtaaggcactgcatgttatgaaccattacaataataacacaaccaataaccattattaaaaacaattttaaaaattccttcattgaatccatagtctttttttaagacttaccccaagaacacaaattaatattatccttgtagttaaagtaaaaaaaaagcacaagttttattaattatttatttattcgtatagaaaagtggggctcaataggtaagagttacaagatccattatttactcttagctcacgaagagctagctagatcttagctcatacatctgcattatttttcatattgattactcagtaaaaactgtccagaactgaagacagaggactcctttttctttagctttcttcctccttttattcaggttcagcacttgcaaagtgagattatttttaattcttgattaatctatttacctcttaagaagatccaggaaatgtgagctcctttactggattttctatttagcttatcacattgtcatccgatctttcaaattttcaatccccaaattagaaatataacattcaaatattaactaatgatatttctattcacttaatatctgaaaggaagtttctctaattgttctcggcattgataccaaatccaaccaaattcagatttgatgaagcactaatggcaactgggtgacctgctggaatgataacaacgtcacccggagacaatctagcttcatatctctacacttcattgtttctttcttttctatcttccctctcttattactcattttttaaacccagaagttcaaggtttccttttccttcattaactaatagtacaactattgcccttgaattgtagtgtggcaacattagagctccttaaaaatttaagcaaaaacgcattaacatatttctgtaatataattaaaattatgtgttttatatatatttagtgttgtgtacatatcttgttaatctccacacaactaacaagtatatctaaatcttaaagctaagggtattttttctctggagtaatctcaaacaacttgccaaacttattagaatattctggcttgtggcttctcaagttgaaaggttcaaattcagagggtaagcttttctttgagcttgattttgcaagctttctcaattcctcaatttattcccttgatactttgattattgcgtctctttcttccccttattatgttcttttccgatctctcaattattatggttttttctcttactcttctaaaagaaccttctctatggtctcgtatttagtttatatttgcgaaaaaggatacaaaatataatggttatatttattaaacatttgataaaaaaatcacacattaagcttaacatgtgttgtttgcatacttatatttaaggaggcctctaaaatgttcttgctgaatcctcataagtattagtttttattttcagatagaccaaaagcttgtagaagaaggataaagatcaatttttcaatccagacaaaaataaaagtaatataaaggaggtgttttaataagaataaaacatgtgaagaaaattattatctcaaatttaccaggcctgttcacgggtattacaaaatccaccactcttagatcttcttcatcatcttagttaactagataagatgttgttcctgcgggaattttgatggtatcaccacgctcaagattatacgagtttctatcattgggactcaacactgtcaatatggctttccttgtagtacatattaaccacaccaaaatttaattatgaaatataagaaatattgctaaattgaactttacaatatttttattttaaatagtcatatttctataaaacaaaagatttgttataataatattataaagaaaaataaaaattatcattgaggactacaaggattaagtcagcatctatgtgttaaggaaggaagatggtgtggggtttggctctatattccacaagacgatagttttagagattttcaaataagtctgaacgtttgtcgaacctttaaaggcgacgaatgtgaccgttttcgttttcaaagagtgtcagaaacttgttagacttgaataaaaaggggtttctttattcttatgattctgaagatctttcttcctcctctccttcacgttaatggcgtctgtctctttttgttctctcctctctatgccttagccttgccctttcttcgggatcttcacgacgttaacttcctctttactcttcgtctacttattcctcatcttcctctctttcttatctctcacgtccaggttaaacttccttttattccttcttttcacgttaatatcaatatttctacttctcttcttcatcttcttccttttcatatgaaggtctttattctccatggcgtttttcttctttctcaccctcttagcgacctctttctctttatcccggtaccctagtttctgaaccttcatcgtaattggcataagtgacgcaaacagaggccaggaatataattcccagaaacaataaaagtggaaatcatgatttgacagtggtcgctatgatttgtatttcactagttcgaactttagatgatgaaataaaagattaagttgaaggatatttatagtgatagaacgtaaagctagatgaataacgtggatggtcatttgggtaca

SEQ ID NO: 67 - DNA, 3400 bp, synthetic construct
  source 1..3400: mol_type = other DNA
gacacggtgagagtaacagaagatagtattaatgactaagtagaagaaatatttctgaccattgattggtgacgaaaactacccctataaagtttactcgcagttaaacatcgaaatatccattatttttttgtcatttactttttcattattattatataagtttaaacacttagaatcataaaaattattaaatctatctttaagcacaacaaacaaatctatctatggatagaataatattgtacctgttgactccaaatacacaacaataatatgaaaaatagaataataaattcaaatggttagaatatatttttacttagataccaaagttttaccatctttcttgtctttcttaagaactatctgaatcaattttgacctcaactattagaataagaaactttatccaaatctataaataaaagaaaacatttgaaattgggttaacaatttaggctcaatccttccaagtctcgaagtctcgattattacgcaactcctcttacatttcatcttttcctcatagaacatttacattaaaacaaagagtccaattaatattcagaacttcatattgtaaatctaacattgatataaccgtcatgaaaatatattttctagagagaaaagaaattgcacaacctcgtcttaactcacaaattacaaaacacttccaattttttaatttaaagaaaagatataaaaacataaacaaattaaagcaactaatacaagagtaaggcactgcatgttatgaaccattacaataataacacaaccaataaccattattaaaaacaattttaaaaattccttcattgaatccatagtctttttttaagacttaccccaagaacacaaattaatattatccttgtagttaaagtaaaaaaaaagcacaagttttattaattatttatttattcgtatagaaaagtggggctcaataggtaagagttacaagatccattatttactcttagctcacgaagagctagctagatcttagctcatacatctgcattatttttcatattgattactcagtaaaaactgtccagaactgaagacagaggactcctttttctttggctttcttcctccttttattcaggttcagcacttgcaaagtgagattatttttaattcttgattaatctatttacctcttaagaagatccaggaaatgtgagctcctttactggattttctatttagcttatcacattgtcatccgatctttcaaattttcaatccccaaattagaaatataacattcaaatattaactaatgatatttctattcacttaatatctgaaaggaagtttctctaattgttctcggcattgataccaaatccaaccaaattcagatttgatgaagcactaatggcaactgggtgacctgctggaatgataacaacgtcacccggagacaatctagcttcatatctctacacttcattgtttctttcttttctatcttccctctcttattactcattttttaaacccagaagttcaaggtttccttttccttcattaactaatagtacaactattgcccttgaattgtagtgtggcaacattagagctccttaaaaatttaagcaaaaacgcattaacatatttctgtaatataattaaaattatgtgttttatatatatttagtgttgtgtacatatcttgttaatctccacacaactaacaagtatatctaaatcttaaagctaagggtattttttctctggagtaatctcaaacaacttgccaaacttattagaatattctggcttgtggcttctcaagttgaaaggttcaaattcagagggtaagcttttctttgagcttgattttgcaagctttctcaattcctcaatttattcccttgatactttgattattgcgtctctttcttccccttattatgttcttttccgatctctcaattattatggttttttctcttactcttctaaaagaaccttctctatggtctcgtatttagtttatatttgcgaaaaaggatacaaaatataatggttatatttattaaacatttgataaaaaaatcacacattaagcttaacatgtgttgtttgcatacttatatttaaggaggcctctaaaatgttcttgctgaatcctcataagtattagtttttattttcagatagaccaaaagcttgtagaagaaggataaagatcaatttttcaatccagacaaaaataaaagtaatataaaggaggtgttttaataagaataaaacatgtgaagaaaattattatctcaaatttaccaggcctgttcacgggtattacaaaatccaccactcttagatcttcttcatcatcttagttaactagataagatgttgttcctgcgggaattttgatggtatcaccacgctcaagattatacgagtttctatcattgggactcaacactgtcaatatggctttccttgtagtacatattaaccacaccaaaatttaattatgaaatataagaaatattgctaaattgaactttacaatatttttattttaaatagtcatatttctataaaacaaaagatttgttataataatattataaagaaaaataaaaattatcattgaggactacaaggattaagtcagcatctatgtgttaaggaaggaagatggtgtggggtttggctctatattccacaagacgatagttttagagattttcaaataagtctgaacgtttgtcgaacctttaaaggcgacgaatgtgaccgttttcgttttcaaagagtgtcagaaacttgttagacttgaataaaaaggggtttctttattcttatgattctgaagatctttcttcctcctctccttcacgttaatggcgtctgtctctttttgttctctcctctctatgccttagccttgccctttcttcgggatcttcacgacgttaacttcctctttactcttcgtctacttattcctcatcttcctctctttcttatctctcacgtccaggttaaacttccttttattccttcttttcacgttaatatcaatatttctacttctcttcttcatcttcttccttttcatatgaaggtctttattctccatggcgtttttcttctttctcaccctcttagcgacctctttctctttatcccggtaccctagtttctgaaccttcatcgtaattggcataagtgacgcaaacagaggccaggaatataattcccagaaacaataaaagtggaaatcatgatttgacagtggtcgctatgatttgtatttcactagttcgaactttagatgatgaaataaaagattaagttgaaggatatttatagtgatagaacgtaaagctagatgaataacgtggatggtcatttgggtaca

SEQ ID NO: 68 - DNA, 3400 bp, synthetic construct
  source 1..3400: mol_type = other DNA
gacacggtgagagtaacagaagatagtattaatgactaagtagaagaaatatttctgaccattgattggtgacgaaaactacccctataaagtttactcgcagttaaacatcgaaatatccattatttttttgtcatttactttttcattattattatataagtttaaacacttagaatcataaaaattattaaatctatctttaagcacaacaaacaaatctatctatggatagaataatattgtacctgttgactccaaatacacaacaataatatgaaaaatagaataataaattcaaatggttagaatatatttttacttagataccaaagttttaccatctttcttgtctttcttaagaactatctgaatcaattttgacctcaactattagaataagaaactttatccaaatctataaataaaagaaaacatttgaaattgggttaacaatttaggctcaatccttccaagtctcgaagtctcgattattacgcaactcctcttacatttcatcttttcctcatagaacatttacattaaaacaaagagtccaattaatattcagaacttcatattgtaaatctaacattgatataaccgtcatgaaaatatattttctagagagaaaagaaattgcacaacctcgtcttaactcacaaattacaaaacacttccaattttttaatttaaagaaaagatataaaaacataaacaaattaaagcaactaatacaagagtaaggcactgcatgttatgaaccattacaataataacacaaccaataaccattattaaaaacaattttaaaaattccttcattgaatccatagtctttttttaagacttaccccaagaacacaaattaatattatccttgtagttaaagtaaaaaaaaagcacaagttttattaattatttatttattcgtatagaaaagtggggctcaataggtaagagttacaagatccattatttactcttagctcacgaagagctagctagatcttagctcatacatctgcattatttttcatattgattactcagtaaaaactgtccagaactgaagacagaggactcctttttctttagctttcttcctccttttgttcaggttcagcacttgcaaagtgagattatttttaattcttgattaatctatttacctcttaagaagatccaggaaatgtgagctcctttactggattttctatttagcttatcacattgtcatccgatctttcaaattttcaatccccaaattagaaatataacattcaaatattaactaatgatatttctattcacttaatatctgaaaggaagtttctctaattgttctcggcattgataccaaatccaaccaaattcagatttgatgaagcactaatggcaactgggtgacctgctggaatgataacaacgtcacccggagacaatctagcttcatatctctacacttcattgtttctttcttttctatcttccctctcttattactcattttttaaacccagaagttcaaggtttccttttccttcattaactaatagtacaactattgcccttgaattgtagtgtggcaacattagagctccttaaaaatttaagcaaaaacgcattaacatatttctgtaatataattaaaattatgtgttttatatatatttagtgttgtgtacatatcttgttaatctccacacaactaacaagtatatctaaatcttaaagctaagggtattttttctctggagtaatctcaaacaacttgccaaacttattagaatattctggcttgtggcttctcaagttgaaaggttcaaattcagagggtaagcttttctttgagcttgattttgcaagctttctcaattcctcaatttattcccttgatactttgattattgcgtctctttcttccccttattatgttcttttccgatctctcaattattatggttttttctcttactcttctaaaagaaccttctctatggtctcgtatttagtttatatttgcgaaaaaggatacaaaatataatggttatatttattaaacatttgataaaaaaatcacacattaagcttaacatgtgttgtttgcatacttatatttaaggaggcctctaaaatgttcttgctgaatcctcataagtattagtttttattttcagatagaccaaaagcttgtagaagaaggataaagatcaatttttcaatccagacaaaaataaaagtaatataaaggaggtgttttaataagaataaaacatgtgaagaaaattattatctcaaatttaccaggcctgttcacgggtattacaaaatccaccactcttagatcttcttcatcatcttagttaactagataagatgttgttcctgcgggaattttgatggtatcaccacgctcaagattatacgagtttctatcattgggactcaacactgtcaatatggctttccttgtagtacatattaaccacaccaaaatttaattatgaaatataagaaatattgctaaattgaactttacaatatttttattttaaatagtcatatttctataaaacaaaagatttgttataataatattataaagaaaaataaaaattatcattgaggactacaaggattaagtcagcatctatgtgttaaggaaggaagatggtgtggggtttggctctatattccacaagacgatagttttagagattttcaaataagtctgaacgtttgtcgaacctttaaaggcgacgaatgtgaccgttttcgttttcaaagagtgtcagaaacttgttagacttgaataaaaaggggtttctttattcttatgattctgaagatctttcttcctcctctccttcacgttaatggcgtctgtctctttttgttctctcctctctatgccttagccttgccctttcttcgggatcttcacgacgttaacttcctctttactcttcgtctacttattcctcatcttcctctctttcttatctctcacgtccaggttaaacttccttttattccttcttttcacgttaatatcaatatttctacttctcttcttcatcttcttccttttcatatgaaggtctttattctccatggcgtttttcttctttctcaccctcttagcgacctctttctctttatcccggtaccctagtttctgaaccttcatcgtaattggcataagtgacgcaaacagaggccaggaatataattcccagaaacaataaaagtggaaatcatgatttgacagtggtcgctatgatttgtatttcactagttcgaactttagatgatgaaataaaagattaagttgaaggatatttatagtgatagaacgtaaagctagatgaataacgtggatggtcatttgggtaca

SEQ ID NO: 69 - DNA, 3400 bp, synthetic construct
  source 1..3400: mol_type = other DNA
gacacggtgagagtaacagaagatagtattaatgactaagtagaagaaatatttctgaccattgattggtgacgaaaactacccctataaagtttactcgcagttaaacatcgaaatatccattatttttttgtcatttactttttcattattattatataagtttaaacacttagaatcataaaaattattaaatctatctttaagcacaacaaacaaatctatctatggatagaataatattgtacctgttgactccaaatacacaacaataatatgaaaaatagaataataaattcaaatggttagaatatatttttacttagataccaaagttttaccatctttcttgtctttcttaagaactatctgaatcaattttgacctcaactattagaataagaaactttatccaaatctataaataaaagaaaacatttgaaattgggttaacaatttaggctcaatccttccaagtctcgaagtctcgattattacgcaactcctcttacatttcatcttttcctcatagaacatttacattaaaacaaagagtccaattaatattcagaacttcatattgtaaatctaacattgatataaccgtcatgaaaatatattttctagagagaaaagaaattgcacaacctcgtcttaactcacaaattacaaaacacttccaattttttaatttaaagaaaagatataaaaacataaacaaattaaagcaactaatacaagagtaaggcactgcatgttatgaaccattacaataataacacaaccaataaccattattaaaaacaattttaaaaattccttcattgaatccatagtctttttttaagacttaccccaagaacacaaattaatattatccttgtagttaaagtaaaaaaaaagcacaagttttattaattatttatttattcgtatagaaaagtggggctcaataggtaagagttacaagatccattatttactcttagctcacgaagagctagctagatcttagctcatacatctgcattatttttcatattgattactcagtaaaaactgtccagaactgaagacagaggactcctttttctttagctttcttcctccttttattcaggttcagcacttgcaaagtgagattgtttttaattcttgattaatctatttacctcttaagaagatccaggaaatgtgagctcctttactggattttctatttagcttatcacattgtcatccgatctttcaaattttcaatccccaaattagaaatataacattcaaatattaactaatgatatttctattcacttaatatctgaaaggaagtttctctaattgttctcggcattgataccaaatccaaccaaattcagatttgatgaagcactaatggcaactgggtgacctgctggaatgataacaacgtcacccggagacaatctagcttcatatctctacacttcattgtttctttcttttctatcttccctctcttattactcattttttaaacccagaagttcaaggtttccttttccttcattaactaatagtacaactattgcccttgaattgtagtgtggcaacattagagctccttaaaaatttaagcaaaaacgcattaacatatttctgtaatataattaaaattatgtgttttatatatatttagtgttgtgtacatatcttgttaatctccacacaactaacaagtatatctaaatcttaaagctaagggtattttttctctggagtaatctcaaacaacttgccaaacttattagaatattctggcttgtggcttctcaagttgaaaggttcaaattcagagggtaagcttttctttgagcttgattttgcaagctttctcaattcctcaatttattcccttgatactttgattattgcgtctctttcttccccttattatgttcttttccgatctctcaattattatggttttttctcttactcttctaaaagaaccttctctatggtctcgtatttagtttatatttgcgaaaaaggatacaaaatataatggttatatttattaaacatttgataaaaaaatcacacattaagcttaacatgtgttgtttgcatacttatatttaaggaggcctctaaaatgttcttgctgaatcctcataagtattagtttttattttcagatagaccaaaagcttgtagaagaaggataaagatcaatttttcaatccagacaaaaataaaagtaatataaaggaggtgttttaataagaataaaacatgtgaagaaaattattatctcaaatttaccaggcctgttcacgggtattacaaaatccaccactcttagatcttcttcatcatcttagttaactagataagatgttgttcctgcgggaattttgatggtatcaccacgctcaagattatacgagtttctatcattgggactcaacactgtcaatatggctttccttgtagtacatattaaccacaccaaaatttaattatgaaatataagaaatattgctaaattgaactttacaatatttttattttaaatagtcatatttctataaaacaaaagatttgttataataatattataaagaaaaataaaaattatcattgaggactacaaggattaagtcagcatctatgtgttaaggaaggaagatggtgtggggtttggctctatattccacaagacgatagttttagagattttcaaataagtctgaacgtttgtcgaacctttaaaggcgacgaatgtgaccgttttcgttttcaaagagtgtcagaaacttgttagacttgaataaaaaggggtttctttattcttatgattctgaagatctttcttcctcctctccttcacgttaatggcgtctgtctctttttgttctctcctctctatgccttagccttgccctttcttcgggatcttcacgacgttaacttcctctttactcttcgtctacttattcctcatcttcctctctttcttatctctcacgtccaggttaaacttccttttattccttcttttcacgttaatatcaatatttctacttctcttcttcatcttcttccttttcatatgaaggtctttattctccatggcgtttttcttctttctcaccctcttagcgacctctttctctttatcccggtaccctagtttctgaaccttcatcgtaattggcataagtgacgcaaacagaggccaggaatataattcccagaaacaataaaagtggaaatcatgatttgacagtggtcgctatgatttgtatttcactagttcgaactttagatgatgaaataaaagattaagttgaaggatatttatagtgatagaacgtaaagctagatgaataacgtggatggtcatttgggtaca

SEQ ID NO: 70 - DNA, 3400 bp, synthetic construct
  source 1..3400: mol_type = other DNA
gacacggtgagagtaacagaagatagtattaatgactaagtagaagaaatatttctgaccattgattggtgacgaaaactacccctataaagtttactcgcagttaaacatcgaaatatccattatttttttgtcatttactttttcattattattatataagtttaaacacttagaatcataaaaattattaaatctatctttaagcacaacaaacaaatctatctatggatagaataatattgtacctgttgactccaaatacacaacaataatatgaaaaatagaataataaattcaaatggttagaatatatttttacttagataccaaagttttaccatctttcttgtctttcttaagaactatctgaatcaattttgacctcaactattagaataagaaactttatccaaatctataaataaaagaaaacatttgaaattgggttaacaatttaggctcaatccttccaagtctcgaagtctcgattattacgcaactcctcttacatttcatcttttcctcatagaacatttacattaaaacaaagagtccaattaatattcagaacttcatattgtaaatctaacattgatataaccgtcatgaaaatatattttctagagagaaaagaaattgcacaacctcgtcttaactcacaaattacaaaacacttccaattttttaatttaaagaaaagatataaaaacataaacaaattaaagcaactaatacaagagtaaggcactgcatgttatgaaccattacaataataacacaaccaataaccattattaaaaacaattttaaaaattccttcattgaatccatagtctttttttaagacttaccccaagaacacaaattaatattatccttgtagttaaagtaaaaaaaaagcacaagttttattaattatttatttattcgtatagaaaagtggggctcaataggtaagagttacaagatccattatttactcttagctcacgaagagctagctagatcttagctcatacatctgcattatttttcatattgattactcagtaaaaactgtccagaactgaagacagaggactcctttttctttagctttcttcctccttttattcaggttcagcacttgcaaagtgagattatttttgattcttgattaatctatttacctcttaagaagatccaggaaatgtgagctcctttactggattttctatttagcttatcacattgtcatccgatctttcaaattttcaatccccaaattagaaatataacattcaaatattaactaatgatatttctattcacttaatatctgaaaggaagtttctctaattgttctcggcattgataccaaatccaaccaaattcagatttgatgaagcactaatggcaactgggtgacctgctggaatgataacaacgtcacccggagacaatctagcttcatatctctacacttcattgtttctttcttttctatcttccctctcttattactcattttttaaacccagaagttcaaggtttccttttccttcattaactaatagtacaactattgcccttgaattgtagtgtggcaacattagagctccttaaaaatttaagcaaaaacgcattaacatatttctgtaatataattaaaattatgtgttttatatatatttagtgttgtgtacatatcttgttaatctccacacaactaacaagtatatctaaatcttaaagctaagggtattttttctctggagtaatctcaaacaacttgccaaacttattagaatattctggcttgtggcttctcaagttgaaaggttcaaattcagagggtaagcttttctttgagcttgattttgcaagctttctcaattcctcaatttattcccttgatactttgattattgcgtctctttcttccccttattatgttcttttccgatctctcaattattatggttttttctcttactcttctaaaagaaccttctctatggtctcgtatttagtttatatttgcgaaaaaggatacaaaatataatggttatatttattaaacatttgataaaaaaatcacacattaagcttaacatgtgttgtttgcatacttatatttaaggaggcctctaaaatgttcttgctgaatcctcataagtattagtttttattttcagatagaccaaaagcttgtagaagaaggataaagatcaatttttcaatccagacaaaaataaaagtaatataaaggaggtgttttaataagaataaaacatgtgaagaaaattattatctcaaatttaccaggcctgttcacgggtattacaaaatccaccactcttagatcttcttcatcatcttagttaactagataagatgttgttcctgcgggaattttgatggtatcaccacgctcaagattatacgagtttctatcattgggactcaacactgtcaatatggctttccttgtagtacatattaaccacaccaaaatttaattatgaaatataagaaatattgctaaattgaactttacaatatttttattttaaatagtcatatttctataaaacaaaagatttgttataataatattataaagaaaaataaaaattatcattgaggactacaaggattaagtcagcatctatgtgttaaggaaggaagatggtgtggggtttggctctatattccacaagacgatagttttagagattttcaaataagtctgaacgtttgtcgaacctttaaaggcgacgaatgtgaccgttttcgttttcaaagagtgtcagaaacttgttagacttgaataaaaaggggtttctttattcttatgattctgaagatctttcttcctcctctccttcacgttaatggcgtctgtctctttttgttctctcctctctatgccttagccttgccctttcttcgggatcttcacgacgttaacttcctctttactcttcgtctacttattcctcatcttcctctctttcttatctctcacgtccaggttaaacttccttttattccttcttttcacgttaatatcaatatttctacttctcttcttcatcttcttccttttcatatgaaggtctttattctccatggcgtttttcttctttctcaccctcttagcgacctctttctctttatcccggtaccctagtttctgaaccttcatcgtaattggcataagtgacgcaaacagaggccaggaatataattcccagaaacaataaaagtggaaatcatgatttgacagtggtcgctatgatttgtatttcactagttcgaactttagatgatgaaataaaagattaagttgaaggatatttatagtgatagaacgtaaagctagatgaataacgtggatggtcatttgggtaca

SEQ ID NO: 71 - DNA, 3400 bp, synthetic construct
  source 1..3400: mol_type = other DNA
gacacggtgagagtaacagaagatagtattaatgactaagtagaagaaatatttctgaccattgattggtgacgaaaactacccctataaagtttactcgcagttaaacatcgaaatatccattatttttttgtcatttactttttcattattattatataagtttaaacacttagaatcataaaaattattaaatctatctttaagcacaacaaacaaatctatctatggatagaataatattgtacctgttgactccaaatacacaacaataatatgaaaaatagaataataaattcaaatggttagaatatatttttacttagataccaaagttttaccatctttcttgtctttcttaagaactatctgaatcaattttgacctcaactattagaataagaaactttatccaaatctataaataaaagaaaacatttgaaattgggttaacaatttaggctcaatccttccaagtctcgaagtctcgattattacgcaactcctcttacatttcatcttttcctcatagaacatttacattaaaacaaagagtccaattaatattcagaacttcatattgtaaatctaacattgatataaccgtcatgaaaatatattttctagagagaaaagaaattgcacaacctcgtcttaactcacaaattacaaaacacttccaattttttaatttaaagaaaagatataaaaacataaacaaattaaagcaactaatacaagagtaaggcactgcatgttatgaaccattacaataataacacaaccaataaccattattaaaaacaattttaaaaattccttcattgaatccatagtctttttttaagacttaccccaagaacacaaattaatattatccttgtagttaaagtaaaaaaaaagcacaagttttattaattatttatttattcgtatagaaaagtggggctcaataggtaagagttacaagatccattatttactcttagctcacgaagagctagctagatcttagctcatacatctgcattatttttcatattgattactcagtaaaaactgtccagaactgaagacagaggactcctttttctttagctttcttcctccttttattcaggttcagcacttgcaaagtgagattatttttaattcttgattaatctatttacctcttgagaagatccaggaaatgtgagctcctttactggattttctatttagcttatcacattgtcatccgatctttcaaattttcaatccccaaattagaaatataacattcaaatattaactaatgatatttctattcacttaatatctgaaaggaagtttctctaattgttctcggcattgataccaaatccaaccaaattcagatttgatgaagcactaatggcaactgggtgacctgctggaatgataacaacgtcacccggagacaatctagcttcatatctctacacttcattgtttctttcttttctatcttccctctcttattactcattttttaaacccagaagttcaaggtttccttttccttcattaactaatagtacaactattgcccttgaattgtagtgtggcaacattagagctccttaaaaatttaagcaaaaacgcattaacatatttctgtaatataattaaaattatgtgttttatatatatttagtgttgtgtacatatcttgttaatctccacacaactaacaagtatatctaaatcttaaagctaagggtattttttctctggagtaatctcaaacaacttgccaaacttattagaatattctggcttgtggcttctcaagttgaaaggttcaaattcagagggtaagcttttctttgagcttgattttgcaagctttctcaattcctcaatttattcccttgatactttgattattgcgtctctttcttccccttattatgttcttttccgatctctcaattattatggttttttctcttactcttctaaaagaaccttctctatggtctcgtatttagtttatatttgcgaaaaaggatacaaaatataatggttatatttattaaacatttgataaaaaaatcacacattaagcttaacatgtgttgtttgcatacttatatttaaggaggcctctaaaatgttcttgctgaatcctcataagtattagtttttattttcagatagaccaaaagcttgtagaagaaggataaagatcaatttttcaatccagacaaaaataaaagtaatataaaggaggtgttttaataagaataaaacatgtgaagaaaattattatctcaaatttaccaggcctgttcacgggtattacaaaatccaccactcttagatcttcttcatcatcttagttaactagataagatgttgttcctgcgggaattttgatggtatcaccacgctcaagattatacgagtttctatcattgggactcaacactgtcaatatggctttccttgtagtacatattaaccacaccaaaatttaattatgaaatataagaaatattgctaaattgaactttacaatatttttattttaaatagtcatatttctataaaacaaaagatttgttataataatattataaagaaaaataaaaattatcattgaggactacaaggattaagtcagcatctatgtgttaaggaaggaagatggtgtggggtttggctctatattccacaagacgatagttttagagattttcaaataagtctgaacgtttgtcgaacctttaaaggcgacgaatgtgaccgttttcgttttcaaagagtgtcagaaacttgttagacttgaataaaaaggggtttctttattcttatgattctgaagatctttcttcctcctctccttcacgttaatggcgtctgtctctttttgttctctcctctctatgccttagccttgccctttcttcgggatcttcacgacgttaacttcctctttactcttcgtctacttattcctcatcttcctctctttcttatctctcacgtccaggttaaacttccttttattccttcttttcacgttaatatcaatatttctacttctcttcttcatcttcttccttttcatatgaaggtctttattctccatggcgtttttcttctttctcaccctcttagcgacctctttctctttatcccggtaccctagtttctgaaccttcatcgtaattggcataagtgacgcaaacagaggccaggaatataattcccagaaacaataaaagtggaaatcatgatttgacagtggtcgctatgatttgtatttcactagttcgaactttagatgatgaaataaaagattaagttgaaggatatttatagtgatagaacgtaaagctagatgaataacgtggatggtcatttgggtaca

SEQ ID NO: 72 - DNA, 3400 bp, synthetic construct
  source 1..3400: mol_type = other DNA
gacacggtgagagtaacagaagatagtattaatgactaagtagaagaaatatttctgaccattgattggtgacgaaaactacccctataaagtttactcgcagttaaacatcgaaatatccattatttttttgtcatttactttttcattattattatataagtttaaacacttagaatcataaaaattattaaatctatctttaagcacaacaaacaaatctatctatggatagaataatattgtacctgttgactccaaatacacaacaataatatgaaaaatagaataataaattcaaatggttagaatatatttttacttagataccaaagttttaccatctttcttgtctttcttaagaactatctgaatcaattttgacctcaactattagaataagaaactttatccaaatctataaataaaagaaaacatttgaaattgggttaacaatttaggctcaatccttccaagtctcgaagtctcgattattacgcaactcctcttacatttcatcttttcctcatagaacatttacattaaaacaaagagtccaattaatattcagaacttcatattgtaaatctaacattgatataaccgtcatgaaaatatattttctagagagaaaagaaattgcacaacctcgtcttaactcacaaattacaaaacacttccaattttttaatttaaagaaaagatataaaaacataaacaaattaaagcaactaatacaagagtaaggcactgcatgttatgaaccattacaataataacacaaccaataaccattattaaaaacaattttaaaaattccttcattgaatccatagtctttttttaagacttaccccaagaacacaaattaatattatccttgtagttaaagtaaaaaaaaagcacaagttttattaattatttatttattcgtatagaaaagtggggctcaataggtaagagttacaagatccattatttactcttagctcacgaagagctagctagatcttagctcatacatctgcattatttttcatattgattactcagtaaaaactgtccagaactgaagacagaggactcctttttctttagctttcttcctccttttattcaggttcagcacttgcaaagtgagattatttttaattcttgattaatctatttacctcttaagaagatccaggaaatgtgagctcctttactggattttctatttggcttatcacattgtcatccgatctttcaaattttcaatccccaaattagaaatataacattcaaatattaactaatgatatttctattcacttaatatctgaaaggaagtttctctaattgttctcggcattgataccaaatccaaccaaattcagatttgatgaagcactaatggcaactgggtgacctgctggaatgataacaacgtcacccggagacaatctagcttcatatctctacacttcattgtttctttcttttctatcttccctctcttattactcattttttaaacccagaagttcaaggtttccttttccttcattaactaatagtacaactattgcccttgaattgtagtgtggcaacattagagctccttaaaaatttaagcaaaaacgcattaacatatttctgtaatataattaaaattatgtgttttatatatatttagtgttgtgtacatatcttgttaatctccacacaactaacaagtatatctaaatcttaaagctaagggtattttttctctggagtaatctcaaacaacttgccaaacttattagaatattctggcttgtggcttctcaagttgaaaggttcaaattcagagggtaagcttttctttgagcttgattttgcaagctttctcaattcctcaatttattcccttgatactttgattattgcgtctctttcttccccttattatgttcttttccgatctctcaattattatggttttttctcttactcttctaaaagaaccttctctatggtctcgtatttagtttatatttgcgaaaaaggatacaaaatataatggttatatttattaaacatttgataaaaaaatcacacattaagcttaacatgtgttgtttgcatacttatatttaaggaggcctctaaaatgttcttgctgaatcctcataagtattagtttttattttcagatagaccaaaagcttgtagaagaaggataaagatcaatttttcaatccagacaaaaataaaagtaatataaaggaggtgttttaataagaataaaacatgtgaagaaaattattatctcaaatttaccaggcctgttcacgggtattacaaaatccaccactcttagatcttcttcatcatcttagttaactagataagatgttgttcctgcgggaattttgatggtatcaccacgctcaagattatacgagtttctatcattgggactcaacactgtcaatatggctttccttgtagtacatattaaccacaccaaaatttaattatgaaatataagaaatattgctaaattgaactttacaatatttttattttaaatagtcatatttctataaaacaaaagatttgttataataatattataaagaaaaataaaaattatcattgaggactacaaggattaagtcagcatctatgtgttaaggaaggaagatggtgtggggtttggctctatattccacaagacgatagttttagagattttcaaataagtctgaacgtttgtcgaacctttaaaggcgacgaatgtgaccgttttcgttttcaaagagtgtcagaaacttgttagacttgaataaaaaggggtttctttattcttatgattctgaagatctttcttcctcctctccttcacgttaatggcgtctgtctctttttgttctctcctctctatgccttagccttgccctttcttcgggatcttcacgacgttaacttcctctttactcttcgtctacttattcctcatcttcctctctttcttatctctcacgtccaggttaaacttccttttattccttcttttcacgttaatatcaatatttctacttctcttcttcatcttcttccttttcatatgaaggtctttattctccatggcgtttttcttctttctcaccctcttagcgacctctttctctttatcccggtaccctagtttctgaaccttcatcgtaattggcataagtgacgcaaacagaggccaggaatataattcccagaaacaataaaagtggaaatcatgatttgacagtggtcgctatgatttgtatttcactagttcgaactttagatgatgaaataaaagattaagttgaaggatatttatagtgatagaacgtaaagctagatgaataacgtggatggtcatttgggtaca

SEQ ID NO: 73 - DNA, 3400 bp, synthetic construct
  source 1..3400: mol_type = other DNA
gacacggtgagagtaacagaagatagtattaatgactaagtagaagaaatatttctgaccattgattggtgacgaaaactacccctataaagtttactcgcagttaaacatcgaaatatccattatttttttgtcatttactttttcattattattatataagtttaaacacttagaatcataaaaattattaaatctatctttaagcacaacaaacaaatctatctatggatagaataatattgtacctgttgactccaaatacacaacaataatatgaaaaatagaataataaattcaaatggttagaatatatttttacttagataccaaagttttaccatctttcttgtctttcttaagaactatctgaatcaattttgacctcaactattagaataagaaactttatccaaatctataaataaaagaaaacatttgaaattgggttaacaatttaggctcaatccttccaagtctcgaagtctcgattattacgcaactcctcttacatttcatcttttcctcatagaacatttacattaaaacaaagagtccaattaatattcagaacttcatattgtaaatctaacattgatataaccgtcatgaaaatatattttctagagagaaaagaaattgcacaacctcgtcttaactcacaaattacaaaacacttccaattttttaatttaaagaaaagatataaaaacataaacaaattaaagcaactaatacaagagtaaggcactgcatgttatgaaccattacaataataacacaaccaataaccattattaaaaacaattttaaaaattccttcattgaatccatagtctttttttaagacttaccccaagaacacaaattaatattatccttgtagttaaagtaaaaaaaaagcacaagttttattaattatttatttattcgtatagaaaagtggggctcaataggtaagagttacaagatccattatttactcttagctcacgaagagctagctagatcttagctcatacatctgcattatttttcatattgattactcagtaaaaactgtccagaactgaagacagaggactcctttttctttagctttcttcctccttttattcaggttcagcacttgcaaagtgagattatttttaattcttgattaatctatttacctcttaagaagatccaggaaatgtgagctcctttactggattttctatttagcttatcacattgtcatccgatccttcaaattttcaatccccaaattagaaatataacattcaaatattaactaatgatatttctattcacttaatatctgaaaggaagtttctctaattgttctcggcattgataccaaatccaaccaaattcagatttgatgaagcactaatggcaactgggtgacctgctggaatgataacaacgtcacccggagacaatctagcttcatatctctacacttcattgtttctttcttttctatcttccctctcttattactcattttttaaacccagaagttcaaggtttccttttccttcattaactaatagtacaactattgcccttgaattgtagtgtggcaacattagagctccttaaaaatttaagcaaaaacgcattaacatatttctgtaatataattaaaattatgtgttttatatatatttagtgttgtgtacatatcttgttaatctccacacaactaacaagtatatctaaatcttaaagctaagggtattttttctctggagtaatctcaaacaacttgccaaacttattagaatattctggcttgtggcttctcaagttgaaaggttcaaattcagagggtaagcttttctttgagcttgattttgcaagctttctcaattcctcaatttattcccttgatactttgattattgcgtctctttcttccccttattatgttcttttccgatctctcaattattatggttttttctcttactcttctaaaagaaccttctctatggtctcgtatttagtttatatttgcgaaaaaggatacaaaatataatggttatatttattaaacatttgataaaaaaatcacacattaagcttaacatgtgttgtttgcatacttatatttaaggaggcctctaaaatgttcttgctgaatcctcataagtattagtttttattttcagatagaccaaaagcttgtagaagaaggataaagatcaatttttcaatccagacaaaaataaaagtaatataaaggaggtgttttaataagaataaaacatgtgaagaaaattattatctcaaatttaccaggcctgttcacgggtattacaaaatccaccactcttagatcttcttcatcatcttagttaactagataagatgttgttcctgcgggaattttgatggtatcaccacgctcaagattatacgagtttctatcattgggactcaacactgtcaatatggctttccttgtagtacatattaaccacaccaaaatttaattatgaaatataagaaatattgctaaattgaactttacaatatttttattttaaatagtcatatttctataaaacaaaagatttgttataataatattataaagaaaaataaaaattatcattgaggactacaaggattaagtcagcatctatgtgttaaggaaggaagatggtgtggggtttggctctatattccacaagacgatagttttagagattttcaaataagtctgaacgtttgtcgaacctttaaaggcgacgaatgtgaccgttttcgttttcaaagagtgtcagaaacttgttagacttgaataaaaaggggtttctttattcttatgattctgaagatctttcttcctcctctccttcacgttaatggcgtctgtctctttttgttctctcctctctatgccttagccttgccctttcttcgggatcttcacgacgttaacttcctctttactcttcgtctacttattcctcatcttcctctctttcttatctctcacgtccaggttaaacttccttttattccttcttttcacgttaatatcaatatttctacttctcttcttcatcttcttccttttcatatgaaggtctttattctccatggcgtttttcttctttctcaccctcttagcgacctctttctctttatcccggtaccctagtttctgaaccttcatcgtaattggcataagtgacgcaaacagaggccaggaatataattcccagaaacaataaaagtggaaatcatgatttgacagtggtcgctatgatttgtatttcactagttcgaactttagatgatgaaataaaagattaagttgaaggatatttatagtgatagaacgtaaagctagatgaataacgtggatggtcatttgggtaca

SEQ ID NO: 74 - DNA, 3400 bp, synthetic construct
  source 1..3400: mol_type = other DNA
gacacggtgagagtaacagaagatagtattaatgactaagtagaagaaatatttctgaccattgattggtgacgaaaactacccctataaagtttactcgcagttaaacatcgaaatatccattatttttttgtcatttactttttcattattattatataagtttaaacacttagaatcataaaaattattaaatctatctttaagcacaacaaacaaatctatctatggatagaataatattgtacctgttgactccaaatacacaacaataatatgaaaaatagaataataaattcaaatggttagaatatatttttacttagataccaaagttttaccatctttcttgtctttcttaagaactatctgaatcaattttgacctcaactattagaataagaaactttatccaaatctataaataaaagaaaacatttgaaattgggttaacaatttaggctcaatccttccaagtctcgaagtctcgattattacgcaactcctcttacatttcatcttttcctcatagaacatttacattaaaacaaagagtccaattaatattcagaacttcatattgtaaatctaacattgatataaccgtcatgaaaatatattttctagagagaaaagaaattgcacaacctcgtcttaactcacaaattacaaaacacttccaattttttaatttaaagaaaagatataaaaacataaacaaattaaagcaactaatacaagagtaaggcactgcatgttatgaaccattacaataataacacaaccaataaccattattaaaaacaattttaaaaattccttcattgaatccatagtctttttttaagacttaccccaagaacacaaattaatattatccttgtagttaaagtaaaaaaaaagcacaagttttattaattatttatttattcgtatagaaaagtggggctcaataggtaagagttacaagatccattatttactcttagctcacgaagagctagctagatcttagctcatacatctgcattatttttcatattgattactcagtaaaaactgtccagaactgaagacagaggactcctttttctttagctttcttcctccttttattcaggttcagcacttgcaaagtgagattatttttaattcttgattaatctatttacctcttaagaagatccaggaaatgtgagctcctttactggattttctatttagcttatcacattgtcatccgatctttcaaattttcaatccccaaattagaaatataacattcaaatattaactaatgatatttctattcacttaatacctgaaaggaagtttctctaattgttctcggcattgataccaaatccaaccaaattcagatttgatgaagcactaatggcaactgggtgacctgctggaatgataacaacgtcacccggagacaatctagcttcatatctctacacttcattgtttctttcttttctatcttccctctcttattactcattttttaaacccagaagttcaaggtttccttttccttcattaactaatagtacaactattgcccttgaattgtagtgtggcaacattagagctccttaaaaatttaagcaaaaacgcattaacatatttctgtaatataattaaaattatgtgttttatatatatttagtgttgtgtacatatcttgttaatctccacacaactaacaagtatatctaaatcttaaagctaagggtattttttctctggagtaatctcaaacaacttgccaaacttattagaatattctggcttgtggcttctcaagttgaaaggttcaaattcagagggtaagcttttctttgagcttgattttgcaagctttctcaattcctcaatttattcccttgatactttgattattgcgtctctttcttccccttattatgttcttttccgatctctcaattattatggttttttctcttactcttctaaaagaaccttctctatggtctcgtatttagtttatatttgcgaaaaaggatacaaaatataatggttatatttattaaacatttgataaaaaaatcacacattaagcttaacatgtgttgtttgcatacttatatttaaggaggcctctaaaatgttcttgctgaatcctcataagtattagtttttattttcagatagaccaaaagcttgtagaagaaggataaagatcaatttttcaatccagacaaaaataaaagtaatataaaggaggtgttttaataagaataaaacatgtgaagaaaattattatctcaaatttaccaggcctgttcacgggtattacaaaatccaccactcttagatcttcttcatcatcttagttaactagataagatgttgttcctgcgggaattttgatggtatcaccacgctcaagattatacgagtttctatcattgggactcaacactgtcaatatggctttccttgtagtacatattaaccacaccaaaatttaattatgaaatataagaaatattgctaaattgaactttacaatatttttattttaaatagtcatatttctataaaacaaaagatttgttataataatattataaagaaaaataaaaattatcattgaggactacaaggattaagtcagcatctatgtgttaaggaaggaagatggtgtggggtttggctctatattccacaagacgatagttttagagattttcaaataagtctgaacgtttgtcgaacctttaaaggcgacgaatgtgaccgttttcgttttcaaagagtgtcagaaacttgttagacttgaataaaaaggggtttctttattcttatgattctgaagatctttcttcctcctctccttcacgttaatggcgtctgtctctttttgttctctcctctctatgccttagccttgccctttcttcgggatcttcacgacgttaacttcctctttactcttcgtctacttattcctcatcttcctctctttcttatctctcacgtccaggttaaacttccttttattccttcttttcacgttaatatcaatatttctacttctcttcttcatcttcttccttttcatatgaaggtctttattctccatggcgtttttcttctttctcaccctcttagcgacctctttctctttatcccggtaccctagtttctgaaccttcatcgtaattggcataagtgacgcaaacagaggccaggaatataattcccagaaacaataaaagtggaaatcatgatttgacagtggtcgctatgatttgtatttcactagttcgaactttagatgatgaaataaaagattaagttgaaggatatttatagtgatagaacgtaaagctagatgaataacgtggatggtcatttgggtaca

SEQ ID NO: 75 - DNA, 3400 bp, synthetic construct
  source 1..3400: mol_type = other DNA
gacacggtgagagtaacagaagatagtattaatgactaagtagaagaaatatttctgaccattgattggtgacgaaaactacccctataaagtttactcgcagttaaacatcgaaatatccattatttttttgtcatttactttttcattattattatataagtttaaacacttagaatcataaaaattattaaatctatctttaagcacaacaaacaaatctatctatggatagaataatattgtacctgttgactccaaatacacaacaataatatgaaaaatagaataataaattcaaatggttagaatatatttttacttagataccaaagttttaccatctttcttgtctttcttaagaactatctgaatcaattttgacctcaactattagaataagaaactttatccaaatctataaataaaagaaaacatttgaaattgggttaacaatttaggctcaatccttccaagtctcgaagtctcgattattacgcaactcctcttacatttcatcttttcctcatagaacatttacattaaaacaaagagtccaattaatattcagaacttcatattgtaaatctaacattgatataaccgtcatgaaaatatattttctagagagaaaagaaattgcacaacctcgtcttaactcacaaattacaaaacacttccaattttttaatttaaagaaaagatataaaaacataaacaaattaaagcaactaatacaagagtaaggcactgcatgttatgaaccattacaataataacacaaccaataaccattattaaaaacaattttaaaaattccttcattgaatccatagtctttttttaagacttaccccaagaacacaaattaatattatccttgtagttaaagtaaaaaaaaagcacaagttttattaattatttatttattcgtatagaaaagtggggctcaataggtaagagttacaagatccattatttactcttagctcacgaagagctagctagatcttagctcatacatctgcattatttttcatattgattactcagtaaaaactgtccagaactgaagacagaggactcctttttctttagctttcttcctccttttattcaggttcagcacttgcaaagtgagattatttttaattcttgattaatctatttacctcttaagaagatccaggaaatgtgagctcctttactggattttctatttagcttatcacattgtcatccgatctttcaaattttcaatccccaaattagaaatataacattcaaatattaactaatgatatttctattcacttaatatctgaaaggaagtttctctgattgttctcggcattgataccaaatccaaccaaattcagatttgatgaagcactaatggcaactgggtgacctgctggaatgataacaacgtcacccggagacaatctagcttcatatctctacacttcattgtttctttcttttctatcttccctctcttattactcattttttaaacccagaagttcaaggtttccttttccttcattaactaatagtacaactattgcccttgaattgtagtgtggcaacattagagctccttaaaaatttaagcaaaaacgcattaacatatttctgtaatataattaaaattatgtgttttatatatatttagtgttgtgtacatatcttgttaatctccacacaactaacaagtatatctaaatcttaaagctaagggtattttttctctggagtaatctcaaacaacttgccaaacttattagaatattctggcttgtggcttctcaagttgaaaggttcaaattcagagggtaagcttttctttgagcttgattttgcaagctttctcaattcctcaatttattcccttgatactttgattattgcgtctctttcttccccttattatgttcttttccgatctctcaattattatggttttttctcttactcttctaaaagaaccttctctatggtctcgtatttagtttatatttgcgaaaaaggatacaaaatataatggttatatttattaaacatttgataaaaaaatcacacattaagcttaacatgtgttgtttgcatacttatatttaaggaggcctctaaaatgttcttgctgaatcctcataagtattagtttttattttcagatagaccaaaagcttgtagaagaaggataaagatcaatttttcaatccagacaaaaataaaagtaatataaaggaggtgttttaataagaataaaacatgtgaagaaaattattatctcaaatttaccaggcctgttcacgggtattacaaaatccaccactcttagatcttcttcatcatcttagttaactagataagatgttgttcctgcgggaattttgatggtatcaccacgctcaagattatacgagtttctatcattgggactcaacactgtcaatatggctttccttgtagtacatattaaccacaccaaaatttaattatgaaatataagaaatattgctaaattgaactttacaatatttttattttaaatagtcatatttctataaaacaaaagatttgttataataatattataaagaaaaataaaaattatcattgaggactacaaggattaagtcagcatctatgtgttaaggaaggaagatggtgtggggtttggctctatattccacaagacgatagttttagagattttcaaataagtctgaacgtttgtcgaacctttaaaggcgacgaatgtgaccgttttcgttttcaaagagtgtcagaaacttgttagacttgaataaaaaggggtttctttattcttatgattctgaagatctttcttcctcctctccttcacgttaatggcgtctgtctctttttgttctctcctctctatgccttagccttgccctttcttcgggatcttcacgacgttaacttcctctttactcttcgtctacttattcctcatcttcctctctttcttatctctcacgtccaggttaaacttccttttattccttcttttcacgttaatatcaatatttctacttctcttcttcatcttcttccttttcatatgaaggtctttattctccatggcgtttttcttctttctcaccctcttagcgacctctttctctttatcccggtaccctagtttctgaaccttcatcgtaattggcataagtgacgcaaacagaggccaggaatataattcccagaaacaataaaagtggaaatcatgatttgacagtggtcgctatgatttgtatttcactagttcgaactttagatgatgaaataaaagattaagttgaaggatatttatagtgatagaacgtaaagctagatgaataacgtggatggtcatttgggtaca

SEQ ID NO: 76 - DNA, 3400 bp, synthetic construct
  source 1..3400: mol_type = other DNA
gacacggtgagagtaacagaagatagtattaatgactaagtagaagaaatatttctgaccattgattggtgacgaaaactacccctataaagtttactcgcagttaaacatcgaaatatccattatttttttgtcatttactttttcattattattatataagtttaaacacttagaatcataaaaattattaaatctatctttaagcacaacaaacaaatctatctatggatagaataatattgtacctgttgactccaaatacacaacaataatatgaaaaatagaataataaattcaaatggttagaatatatttttacttagataccaaagttttaccatctttcttgtctttcttaagaactatctgaatcaattttgacctcaactattagaataagaaactttatccaaatctataaataaaagaaaacatttgaaattgggttaacaatttaggctcaatccttccaagtctcgaagtctcgattattacgcaactcctcttacatttcatcttttcctcatagaacatttacattaaaacaaagagtccaattaatattcagaacttcatattgtaaatctaacattgatataaccgtcatgaaaatatattttctagagagaaaagaaattgcacaacctcgtcttaactcacaaattacaaaacacttccaattttttaatttaaagaaaagatataaaaacataaacaaattaaagcaactaatacaagagtaaggcactgcatgttatgaaccattacaataataacacaaccaataaccattattaaaaacaattttaaaaattccttcattgaatccatagtctttttttaagacttaccccaagaacacaaattaatattatccttgtagttaaagtaaaaaaaaagcacaagttttattaattatttatttattcgtatagaaaagtggggctcaataggtaagagttacaagatccattatttactcttagctcacgaagagctagctagatcttagctcatacatctgcattatttttcatattgattactcagtaaaaactgtccagaactgaagacagaggactcctttttctttagctttcttcctccttttattcaggttcagcacttgcaaagtgagattatttttaattcttgattaatctatttacctcttaagaagatccaggaaatgtgagctcctttactggattttctatttagcttatcacattgtcatccgatctttcaaattttcaatccccaaattagaaatataacattcaaatattaactaatgatatttctattcacttaatatctgaaaggaagtttctctaattgttctcggcattgataccaaatccaaccaaattcagatttgatgaagcactaatggcaactgggtgacctgctggaatgataacaacgtcacccggagacaatctagcttcatatctctgcacttcattgtttctttcttttctatcttccctctcttattactcattttttaaacccagaagttcaaggtttccttttccttcattaactaatagtacaactattgcccttgaattgtagtgtggcaacattagagctccttaaaaatttaagcaaaaacgcattaacatatttctgtaatataattaaaattatgtgttttatatatatttagtgttgtgtacatatcttgttaatctccacacaactaacaagtatatctaaatcttaaagctaagggtattttttctctggagtaatctcaaacaacttgccaaacttattagaatattctggcttgtggcttctcaagttgaaaggttcaaattcagagggtaagcttttctttgagcttgattttgcaagctttctcaattcctcaatttattcccttgatactttgattattgcgtctctttcttccccttattatgttcttttccgatctctcaattattatggttttttctcttactcttctaaaagaaccttctctatggtctcgtatttagtttatatttgcgaaaaaggatacaaaatataatggttatatttattaaacatttgataaaaaaatcacacattaagcttaacatgtgttgtttgcatacttatatttaaggaggcctctaaaatgttcttgctgaatcctcataagtattagtttttattttcagatagaccaaaagcttgtagaagaaggataaagatcaatttttcaatccagacaaaaataaaagtaatataaaggaggtgttttaataagaataaaacatgtgaagaaaattattatctcaaatttaccaggcctgttcacgggtattacaaaatccaccactcttagatcttcttcatcatcttagttaactagataagatgttgttcctgcgggaattttgatggtatcaccacgctcaagattatacgagtttctatcattgggactcaacactgtcaatatggctttccttgtagtacatattaaccacaccaaaatttaattatgaaatataagaaatattgctaaattgaactttacaatatttttattttaaatagtcatatttctataaaacaaaagatttgttataataatattataaagaaaaataaaaattatcattgaggactacaaggattaagtcagcatctatgtgttaaggaaggaagatggtgtggggtttggctctatattccacaagacgatagttttagagattttcaaataagtctgaacgtttgtcgaacctttaaaggcgacgaatgtgaccgttttcgttttcaaagagtgtcagaaacttgttagacttgaataaaaaggggtttctttattcttatgattctgaagatctttcttcctcctctccttcacgttaatggcgtctgtctctttttgttctctcctctctatgccttagccttgccctttcttcgggatcttcacgacgttaacttcctctttactcttcgtctacttattcctcatcttcctctctttcttatctctcacgtccaggttaaacttccttttattccttcttttcacgttaatatcaatatttctacttctcttcttcatcttcttccttttcatatgaaggtctttattctccatggcgtttttcttctttctcaccctcttagcgacctctttctctttatcccggtaccctagtttctgaaccttcatcgtaattggcataagtgacgcaaacagaggccaggaatataattcccagaaacaataaaagtggaaatcatgatttgacagtggtcgctatgatttgtatttcactagttcgaactttagatgatgaaataaaagattaagttgaaggatatttatagtgatagaacgtaaagctagatgaataacgtggatggtcatttgggtaca

SEQ ID NO: 77 - DNA, 3400 bp, synthetic construct
  source 1..3400: mol_type = other DNA
gacacggtgagagtaacagaagatagtattaatgactaagtagaagaaatatttctgaccattgattggtgacgaaaactacccctataaagtttactcgcagttaaacatcgaaatatccattatttttttgtcatttactttttcattattattatataagtttaaacacttagaatcataaaaattattaaatctatctttaagcacaacaaacaaatctatctatggatagaataatattgtacctgttgactccaaatacacaacaataatatgaaaaatagaataataaattcaaatggttagaatatatttttacttagataccaaagttttaccatctttcttgtctttcttaagaactatctgaatcaattttgacctcaactattagaataagaaactttatccaaatctataaataaaagaaaacatttgaaattgggttaacaatttaggctcaatccttccaagtctcgaagtctcgattattacgcaactcctcttacatttcatcttttcctcatagaacatttacattaaaacaaagagtccaattaatattcagaacttcatattgtaaatctaacattgatataaccgtcatgaaaatatattttctagagagaaaagaaattgcacaacctcgtcttaactcacaaattacaaaacacttccaattttttaatttaaagaaaagatataaaaacataaacaaattaaagcaactaatacaagagtaaggcactgcatgttatgaaccattacaataataacacaaccaataaccattattaaaaacaattttaaaaattccttcattgaatccatagtctttttttaagacttaccccaagaacacaaattaatattatccttgtagttaaagtaaaaaaaaagcacaagttttattaattatttatttattcgtatagaaaagtggggctcaataggtaagagttacaagatccattatttactcttagctcacgaagagctagctagatcttagctcatacatctgcattatttttcatattgattactcagtaaaaactgtccagaactgaagacagaggactcctttttctttagctttcttcctccttttattcaggttcagcacttgcaaagtgagattatttttaattcttgattaatctatttacctcttaagaagatccaggaaatgtgagctcctttactggattttctatttagcttatcacattgtcatccgatctttcaaattttcaatccccaaattagaaatataacattcaaatattaactaatgatatttctattcacttaatatctgaaaggaagtttctctaattgttctcggcattgataccaaatccaaccaaattcagatttgatgaagcactaatggcaactgggtgacctgctggaatgataacaacgtcacccggagacaatctagcttcatatctctacacttcattgtttctttcttttctatcttccctctcttgttactcattttttaaacccagaagttcaaggtttccttttccttcattaactaatagtacaactattgcccttgaattgtagtgtggcaacattagagctccttaaaaatttaagcaaaaacgcattaacatatttctgtaatataattaaaattatgtgttttatatatatttagtgttgtgtacatatcttgttaatctccacacaactaacaagtatatctaaatcttaaagctaagggtattttttctctggagtaatctcaaacaacttgccaaacttattagaatattctggcttgtggcttctcaagttgaaaggttcaaattcagagggtaagcttttctttgagcttgattttgcaagctttctcaattcctcaatttattcccttgatactttgattattgcgtctctttcttccccttattatgttcttttccgatctctcaattattatggttttttctcttactcttctaaaagaaccttctctatggtctcgtatttagtttatatttgcgaaaaaggatacaaaatataatggttatatttattaaacatttgataaaaaaatcacacattaagcttaacatgtgttgtttgcatacttatatttaaggaggcctctaaaatgttcttgctgaatcctcataagtattagtttttattttcagatagaccaaaagcttgtagaagaaggataaagatcaatttttcaatccagacaaaaataaaagtaatataaaggaggtgttttaataagaataaaacatgtgaagaaaattattatctcaaatttaccaggcctgttcacgggtattacaaaatccaccactcttagatcttcttcatcatcttagttaactagataagatgttgttcctgcgggaattttgatggtatcaccacgctcaagattatacgagtttctatcattgggactcaacactgtcaatatggctttccttgtagtacatattaaccacaccaaaatttaattatgaaatataagaaatattgctaaattgaactttacaatatttttattttaaatagtcatatttctataaaacaaaagatttgttataataatattataaagaaaaataaaaattatcattgaggactacaaggattaagtcagcatctatgtgttaaggaaggaagatggtgtggggtttggctctatattccacaagacgatagttttagagattttcaaataagtctgaacgtttgtcgaacctttaaaggcgacgaatgtgaccgttttcgttttcaaagagtgtcagaaacttgttagacttgaataaaaaggggtttctttattcttatgattctgaagatctttcttcctcctctccttcacgttaatggcgtctgtctctttttgttctctcctctctatgccttagccttgccctttcttcgggatcttcacgacgttaacttcctctttactcttcgtctacttattcctcatcttcctctctttcttatctctcacgtccaggttaaacttccttttattccttcttttcacgttaatatcaatatttctacttctcttcttcatcttcttccttttcatatgaaggtctttattctccatggcgtttttcttctttctcaccctcttagcgacctctttctctttatcccggtaccctagtttctgaaccttcatcgtaattggcataagtgacgcaaacagaggccaggaatataattcccagaaacaataaaagtggaaatcatgatttgacagtggtcgctatgatttgtatttcactagttcgaactttagatgatgaaataaaagattaagttgaaggatatttatagtgatagaacgtaaagctagatgaataacgtggatggtcatttgggtaca

SEQ ID NO: 78 - DNA, 3400 bp, synthetic construct
  source 1..3400: mol_type = other DNA
gacacggtgagagtaacagaagatagtattaatgactaagtagaagaaatatttctgaccattgattggtgacgaaaactacccctataaagtttactcgcagttaaacatcgaaatatccattatttttttgtcatttactttttcattattattatataagtttaaacacttagaatcataaaaattattaaatctatctttaagcacaacaaacaaatctatctatggatagaataatattgtacctgttgactccaaatacacaacaataatatgaaaaatagaataataaattcaaatggttagaatatatttttacttagataccaaagttttaccatctttcttgtctttcttaagaactatctgaatcaattttgacctcaactattagaataagaaactttatccaaatctataaataaaagaaaacatttgaaattgggttaacaatttaggctcaatccttccaagtctcgaagtctcgattattacgcaactcctcttacatttcatcttttcctcatagaacatttacattaaaacaaagagtccaattaatattcagaacttcatattgtaaatctaacattgatataaccgtcatgaaaatatattttctagagagaaaagaaattgcacaacctcgtcttaactcacaaattacaaaacacttccaattttttaatttaaagaaaagatataaaaacataaacaaattaaagcaactaatacaagagtaaggcactgcatgttatgaaccattacaataataacacaaccaataaccattattaaaaacaattttaaaaattccttcattgaatccatagtctttttttaagacttaccccaagaacacaaattaatattatccttgtagttaaagtaaaaaaaaagcacaagttttattaattatttatttattcgtatagaaaagtggggctcaataggtaagagttacaagatccattatttactcttagctcacgaagagctagctagatcttagctcatacatctgcattatttttcatattgattactcagtaaaaactgtccagaactgaagacagaggactcctttttctttagctttcttcctccttttattcaggttcagcacttgcaaagtgagattatttttaattcttgattaatctatttacctcttaagaagatccaggaaatgtgagctcctttactggattttctatttagcttatcacattgtcatccgatctttcaaattttcaatccccaaattagaaatataacattcaaatattaactaatgatatttctattcacttaatatctgaaaggaagtttctctaattgttctcggcattgataccaaatccaaccaaattcagatttgatgaagcactaatggcaactgggtgacctgctggaatgataacaacgtcacccggagacaatctagcttcatatctctacacttcattgtttctttcttttctatcttccctctcttattgctcattttttaaacccagaagttcaaggtttccttttccttcattaactaatagtacaactattgcccttgaattgtagtgtggcaacattagagctccttaaaaatttaagcaaaaacgcattaacatatttctgtaatataattaaaattatgtgttttatatatatttagtgttgtgtacatatcttgttaatctccacacaactaacaagtatatctaaatcttaaagctaagggtattttttctctggagtaatctcaaacaacttgccaaacttattagaatattctggcttgtggcttctcaagttgaaaggttcaaattcagagggtaagcttttctttgagcttgattttgcaagctttctcaattcctcaatttattcccttgatactttgattattgcgtctctttcttccccttattatgttcttttccgatctctcaattattatggttttttctcttactcttctaaaagaaccttctctatggtctcgtatttagtttatatttgcgaaaaaggatacaaaatataatggttatatttattaaacatttgataaaaaaatcacacattaagcttaacatgtgttgtttgcatacttatatttaaggaggcctctaaaatgttcttgctgaatcctcataagtattagtttttattttcagatagaccaaaagcttgtagaagaaggataaagatcaatttttcaatccagacaaaaataaaagtaatataaaggaggtgttttaataagaataaaacatgtgaagaaaattattatctcaaatttaccaggcctgttcacgggtattacaaaatccaccactcttagatcttcttcatcatcttagttaactagataagatgttgttcctgcgggaattttgatggtatcaccacgctcaagattatacgagtttctatcattgggactcaacactgtcaatatggctttccttgtagtacatattaaccacaccaaaatttaattatgaaatataagaaatattgctaaattgaactttacaatatttttattttaaatagtcatatttctataaaacaaaagatttgttataataatattataaagaaaaataaaaattatcattgaggactacaaggattaagtcagcatctatgtgttaaggaaggaagatggtgtggggtttggctctatattccacaagacgatagttttagagattttcaaataagtctgaacgtttgtcgaacctttaaaggcgacgaatgtgaccgttttcgttttcaaagagtgtcagaaacttgttagacttgaataaaaaggggtttctttattcttatgattctgaagatctttcttcctcctctccttcacgttaatggcgtctgtctctttttgttctctcctctctatgccttagccttgccctttcttcgggatcttcacgacgttaacttcctctttactcttcgtctacttattcctcatcttcctctctttcttatctctcacgtccaggttaaacttccttttattccttcttttcacgttaatatcaatatttctacttctcttcttcatcttcttccttttcatatgaaggtctttattctccatggcgtttttcttctttctcaccctcttagcgacctctttctctttatcccggtaccctagtttctgaaccttcatcgtaattggcataagtgacgcaaacagaggccaggaatataattcccagaaacaataaaagtggaaatcatgatttgacagtggtcgctatgatttgtatttcactagttcgaactttagatgatgaaataaaagattaagttgaaggatatttatagtgatagaacgtaaagctagatgaataacgtggatggtcatttgggtaca

SEQ ID NO: 79 - DNA, 3400 bp, synthetic construct
  source 1..3400: mol_type = other DNA
gacacggtgagagtaacagaagatagtattaatgactaagtagaagaaatatttctgaccattgattggtgacgaaaactacccctataaagtttactcgcagttaaacatcgaaatatccattatttttttgtcatttactttttcattattattatataagtttaaacacttagaatcataaaaattattaaatctatctttaagcacaacaaacaaatctatctatggatagaataatattgtacctgttgactccaaatacacaacaataatatgaaaaatagaataataaattcaaatggttagaatatatttttacttagataccaaagttttaccatctttcttgtctttcttaagaactatctgaatcaattttgacctcaactattagaataagaaactttatccaaatctataaataaaagaaaacatttgaaattgggttaacaatttaggctcaatccttccaagtctcgaagtctcgattattacgcaactcctcttacatttcatcttttcctcatagaacatttacattaaaacaaagagtccaattaatattcagaacttcatattgtaaatctaacattgatataaccgtcatgaaaatatattttctagagagaaaagaaattgcacaacctcgtcttaactcacaaattacaaaacacttccaattttttaatttaaagaaaagatataaaaacataaacaaattaaagcaactaatacaagagtaaggcactgcatgttatgaaccattacaataataacacaaccaataaccattattaaaaacaattttaaaaattccttcattgaatccatagtctttttttaagacttaccccaagaacacaaattaatattatccttgtagttaaagtaaaaaaaaagcacaagttttattaattatttatttattcgtatagaaaagtggggctcaataggtaagagttacaagatccattatttactcttagctcacgaagagctagctagatcttagctcatacatctgcattatttttcatattgattactcagtaaaaactgtccagaactgaagacagaggactcctttttctttagctttcttcctccttttattcaggttcagcacttgcaaagtgagattatttttaattcttgattaatctatttacctcttaagaagatccaggaaatgtgagctcctttactggattttctatttagcttatcacattgtcatccgatctttcaaattttcaatccccaaattagaaatataacattcaaatattaactaatgatatttctattcacttaatatctgaaaggaagtttctctaattgttctcggcattgataccaaatccaaccaaattcagatttgatgaagcactaatggcaactgggtgacctgctggaatgataacaacgtcacccggagacaatctagcttcatatctctacacttcattgtttctttcttttctatcttccctctcttattactcattttttaaacccagaagttcaaggtttccttttccttcattaactaatagtacaactattgcccttgaattgtagtgtggcaacattagagctccctaaaaatttaagcaaaaacgcattaacatatttctgtaatataattaaaattatgtgttttatatatatttagtgttgtgtacatatcttgttaatctccacacaactaacaagtatatctaaatcttaaagctaagggtattttttctctggagtaatctcaaacaacttgccaaacttattagaatattctggcttgtggcttctcaagttgaaaggttcaaattcagagggtaagcttttctttgagcttgattttgcaagctttctcaattcctcaatttattcccttgatactttgattattgcgtctctttcttccccttattatgttcttttccgatctctcaattattatggttttttctcttactcttctaaaagaaccttctctatggtctcgtatttagtttatatttgcgaaaaaggatacaaaatataatggttatatttattaaacatttgataaaaaaatcacacattaagcttaacatgtgttgtttgcatacttatatttaaggaggcctctaaaatgttcttgctgaatcctcataagtattagtttttattttcagatagaccaaaagcttgtagaagaaggataaagatcaatttttcaatccagacaaaaataaaagtaatataaaggaggtgttttaataagaataaaacatgtgaagaaaattattatctcaaatttaccaggcctgttcacgggtattacaaaatccaccactcttagatcttcttcatcatcttagttaactagataagatgttgttcctgcgggaattttgatggtatcaccacgctcaagattatacgagtttctatcattgggactcaacactgtcaatatggctttccttgtagtacatattaaccacaccaaaatttaattatgaaatataagaaatattgctaaattgaactttacaatatttttattttaaatagtcatatttctataaaacaaaagatttgttataataatattataaagaaaaataaaaattatcattgaggactacaaggattaagtcagcatctatgtgttaaggaaggaagatggtgtggggtttggctctatattccacaagacgatagttttagagattttcaaataagtctgaacgtttgtcgaacctttaaaggcgacgaatgtgaccgttttcgttttcaaagagtgtcagaaacttgttagacttgaataaaaaggggtttctttattcttatgattctgaagatctttcttcctcctctccttcacgttaatggcgtctgtctctttttgttctctcctctctatgccttagccttgccctttcttcgggatcttcacgacgttaacttcctctttactcttcgtctacttattcctcatcttcctctctttcttatctctcacgtccaggttaaacttccttttattccttcttttcacgttaatatcaatatttctacttctcttcttcatcttcttccttttcatatgaaggtctttattctccatggcgtttttcttctttctcaccctcttagcgacctctttctctttatcccggtaccctagtttctgaaccttcatcgtaattggcataagtgacgcaaacagaggccaggaatataattcccagaaacaataaaagtggaaatcatgatttgacagtggtcgctatgatttgtatttcactagttcgaactttagatgatgaaataaaagattaagttgaaggatatttatagtgatagaacgtaaagctagatgaataacgtggatggtcatttgggtaca

SEQ ID NO: 80 - DNA, 3400 bp, synthetic construct
  source 1..3400: mol_type = other DNA
gacacggtgagagtaacagaagatagtattaatgactaagtagaagaaatatttctgaccattgattggtgacgaaaactacccctataaagtttactcgcagttaaacatcgaaatatccattatttttttgtcatttactttttcattattattatataagtttaaacacttagaatcataaaaattattaaatctatctttaagcacaacaaacaaatctatctatggatagaataatattgtacctgttgactccaaatacacaacaataatatgaaaaatagaataataaattcaaatggttagaatatatttttacttagataccaaagttttaccatctttcttgtctttcttaagaactatctgaatcaattttgacctcaactattagaataagaaactttatccaaatctataaataaaagaaaacatttgaaattgggttaacaatttaggctcaatccttccaagtctcgaagtctcgattattacgcaactcctcttacatttcatcttttcctcatagaacatttacattaaaacaaagagtccaattaatattcagaacttcatattgtaaatctaacattgatataaccgtcatgaaaatatattttctagagagaaaagaaattgcacaacctcgtcttaactcacaaattacaaaacacttccaattttttaatttaaagaaaagatataaaaacataaacaaattaaagcaactaatacaagagtaaggcactgcatgttatgaaccattacaataataacacaaccaataaccattattaaaaacaattttaaaaattccttcattgaatccatagtctttttttaagacttaccccaagaacacaaattaatattatccttgtagttaaagtaaaaaaaaagcacaagttttattaattatttatttattcgtatagaaaagtggggctcaataggtaagagttacaagatccattatttactcttagctcacgaagagctagctagatcttagctcatacatctgcattatttttcatattgattactcagtaaaaactgtccagaactgaagacagaggactcctttttctttagctttcttcctccttttattcaggttcagcacttgcaaagtgagattatttttaattcttgattaatctatttacctcttaagaagatccaggaaatgtgagctcctttactggattttctatttagcttatcacattgtcatccgatctttcaaattttcaatccccaaattagaaatataacattcaaatattaactaatgatatttctattcacttaatatctgaaaggaagtttctctaattgttctcggcattgataccaaatccaaccaaattcagatttgatgaagcactaatggcaactgggtgacctgctggaatgataacaacgtcacccggagacaatctagcttcatatctctacacttcattgtttctttcttttctatcttccctctcttattactcattttttaaacccagaagttcaaggtttccttttccttcattaactaatagtacaactattgcccttgaattgtagtgtggcaacattagagctccttaaaaatttaagcaaaaacgcattaacatatttctgtaatataattaaaattatgtgttttatatatatttagtgttgtgtacataccttgttaatctccacacaactaacaagtatatctaaatcttaaagctaagggtattttttctctggagtaatctcaaacaacttgccaaacttattagaatattctggcttgtggcttctcaagttgaaaggttcaaattcagagggtaagcttttctttgagcttgattttgcaagctttctcaattcctcaatttattcccttgatactttgattattgcgtctctttcttccccttattatgttcttttccgatctctcaattattatggttttttctcttactcttctaaaagaaccttctctatggtctcgtatttagtttatatttgcgaaaaaggatacaaaatataatggttatatttattaaacatttgataaaaaaatcacacattaagcttaacatgtgttgtttgcatacttatatttaaggaggcctctaaaatgttcttgctgaatcctcataagtattagtttttattttcagatagaccaaaagcttgtagaagaaggataaagatcaatttttcaatccagacaaaaataaaagtaatataaaggaggtgttttaataagaataaaacatgtgaagaaaattattatctcaaatttaccaggcctgttcacgggtattacaaaatccaccactcttagatcttcttcatcatcttagttaactagataagatgttgttcctgcgggaattttgatggtatcaccacgctcaagattatacgagtttctatcattgggactcaacactgtcaatatggctttccttgtagtacatattaaccacaccaaaatttaattatgaaatataagaaatattgctaaattgaactttacaatatttttattttaaatagtcatatttctataaaacaaaagatttgttataataatattataaagaaaaataaaaattatcattgaggactacaaggattaagtcagcatctatgtgttaaggaaggaagatggtgtggggtttggctctatattccacaagacgatagttttagagattttcaaataagtctgaacgtttgtcgaacctttaaaggcgacgaatgtgaccgttttcgttttcaaagagtgtcagaaacttgttagacttgaataaaaaggggtttctttattcttatgattctgaagatctttcttcctcctctccttcacgttaatggcgtctgtctctttttgttctctcctctctatgccttagccttgccctttcttcgggatcttcacgacgttaacttcctctttactcttcgtctacttattcctcatcttcctctctttcttatctctcacgtccaggttaaacttccttttattccttcttttcacgttaatatcaatatttctacttctcttcttcatcttcttccttttcatatgaaggtctttattctccatggcgtttttcttctttctcaccctcttagcgacctctttctctttatcccggtaccctagtttctgaaccttcatcgtaattggcataagtgacgcaaacagaggccaggaatataattcccagaaacaataaaagtggaaatcatgatttgacagtggtcgctatgatttgtatttcactagttcgaactttagatgatgaaataaaagattaagttgaaggatatttatagtgatagaacgtaaagctagatgaataacgtggatggtcatttgggtaca

SEQ ID NO: 81 - DNA, 3400 bp, synthetic construct
  source 1..3400: mol_type = other DNA
gacacggtgagagtaacagaagatagtattaatgactaagtagaagaaatatttctgaccattgattggtgacgaaaactacccctataaagtttactcgcagttaaacatcgaaatatccattatttttttgtcatttactttttcattattattatataagtttaaacacttagaatcataaaaattattaaatctatctttaagcacaacaaacaaatctatctatggatagaataatattgtacctgttgactccaaatacacaacaataatatgaaaaatagaataataaattcaaatggttagaatatatttttacttagataccaaagttttaccatctttcttgtctttcttaagaactatctgaatcaattttgacctcaactattagaataagaaactttatccaaatctataaataaaagaaaacatttgaaattgggttaacaatttaggctcaatccttccaagtctcgaagtctcgattattacgcaactcctcttacatttcatcttttcctcatagaacatttacattaaaacaaagagtccaattaatattcagaacttcatattgtaaatctaacattgatataaccgtcatgaaaatatattttctagagagaaaagaaattgcacaacctcgtcttaactcacaaattacaaaacacttccaattttttaatttaaagaaaagatataaaaacataaacaaattaaagcaactaatacaagagtaaggcactgcatgttatgaaccattacaataataacacaaccaataaccattattaaaaacaattttaaaaattccttcattgaatccatagtctttttttaagacttaccccaagaacacaaattaatattatccttgtagttaaagtaaaaaaaaagcacaagttttattaattatttatttattcgtatagaaaagtggggctcaataggtaagagttacaagatccattatttactcttagctcacgaagagctagctagatcttagctcatacatctgcattatttttcatattgattactcagtaaaaactgtccagaactgaagacagaggactcctttttctttagctttcttcctccttttattcaggttcagcacttgcaaagtgagattatttttaattcttgattaatctatttacctcttaagaagatccaggaaatgtgagctcctttactggattttctatttagcttatcacattgtcatccgatctttcaaattttcaatccccaaattagaaatataacattcaaatattaactaatgatatttctattcacttaatatctgaaaggaagtttctctaattgttctcggcattgataccaaatccaaccaaattcagatttgatgaagcactaatggcaactgggtgacctgctggaatgataacaacgtcacccggagacaatctagcttcatatctctacacttcattgtttctttcttttctatcttccctctcttattactcattttttaaacccagaagttcaaggtttccttttccttcattaactaatagtacaactattgcccttgaattgtagtgtggcaacattagagctccttaaaaatttaagcaaaaacgcattaacatatttctgtaatataattaaaattatgtgttttatatatatttagtgttgtgtacatatcttgttaatctccacacaactaacaagtatatctaaatcttgaagctaagggtattttttctctggagtaatctcaaacaacttgccaaacttattagaatattctggcttgtggcttctcaagttgaaaggttcaaattcagagggtaagcttttctttgagcttgattttgcaagctttctcaattcctcaatttattcccttgatactttgattattgcgtctctttcttccccttattatgttcttttccgatctctcaattattatggttttttctcttactcttctaaaagaaccttctctatggtctcgtatttagtttatatttgcgaaaaaggatacaaaatataatggttatatttattaaacatttgataaaaaaatcacacattaagcttaacatgtgttgtttgcatacttatatttaaggaggcctctaaaatgttcttgctgaatcctcataagtattagtttttattttcagatagaccaaaagcttgtagaagaaggataaagatcaatttttcaatccagacaaaaataaaagtaatataaaggaggtgttttaataagaataaaacatgtgaagaaaattattatctcaaatttaccaggcctgttcacgggtattacaaaatccaccactcttagatcttcttcatcatcttagttaactagataagatgttgttcctgcgggaattttgatggtatcaccacgctcaagattatacgagtttctatcattgggactcaacactgtcaatatggctttccttgtagtacatattaaccacaccaaaatttaattatgaaatataagaaatattgctaaattgaactttacaatatttttattttaaatagtcatatttctataaaacaaaagatttgttataataatattataaagaaaaataaaaattatcattgaggactacaaggattaagtcagcatctatgtgttaaggaaggaagatggtgtggggtttggctctatattccacaagacgatagttttagagattttcaaataagtctgaacgtttgtcgaacctttaaaggcgacgaatgtgaccgttttcgttttcaaagagtgtcagaaacttgttagacttgaataaaaaggggtttctttattcttatgattctgaagatctttcttcctcctctccttcacgttaatggcgtctgtctctttttgttctctcctctctatgccttagccttgccctttcttcgggatcttcacgacgttaacttcctctttactcttcgtctacttattcctcatcttcctctctttcttatctctcacgtccaggttaaacttccttttattccttcttttcacgttaatatcaatatttctacttctcttcttcatcttcttccttttcatatgaaggtctttattctccatggcgtttttcttctttctcaccctcttagcgacctctttctctttatcccggtaccctagtttctgaaccttcatcgtaattggcataagtgacgcaaacagaggccaggaatataattcccagaaacaataaaagtggaaatcatgatttgacagtggtcgctatgatttgtatttcactagttcgaactttagatgatgaaataaaagattaagttgaaggatatttatagtgatagaacgtaaagctagatgaataacgtggatggtcatttgggtaca

SEQ ID NO: 82 - DNA, 3400 bp, synthetic construct
  source 1..3400: mol_type = other DNA
gacacggtgagagtaacagaagatagtattaatgactaagtagaagaaatatttctgaccattgattggtgacgaaaactacccctataaagtttactcgcagttaaacatcgaaatatccattatttttttgtcatttactttttcattattattatataagtttaaacacttagaatcataaaaattattaaatctatctttaagcacaacaaacaaatctatctatggatagaataatattgtacctgttgactccaaatacacaacaataatatgaaaaatagaataataaattcaaatggttagaatatatttttacttagataccaaagttttaccatctttcttgtctttcttaagaactatctgaatcaattttgacctcaactattagaataagaaactttatccaaatctataaataaaagaaaacatttgaaattgggttaacaatttaggctcaatccttccaagtctcgaagtctcgattattacgcaactcctcttacatttcatcttttcctcatagaacatttacattaaaacaaagagtccaattaatattcagaacttcatattgtaaatctaacattgatataaccgtcatgaaaatatattttctagagagaaaagaaattgcacaacctcgtcttaactcacaaattacaaaacacttccaattttttaatttaaagaaaagatataaaaacataaacaaattaaagcaactaatacaagagtaaggcactgcatgttatgaaccattacaataataacacaaccaataaccattattaaaaacaattttaaaaattccttcattgaatccatagtctttttttaagacttaccccaagaacacaaattaatattatccttgtagttaaagtaaaaaaaaagcacaagttttattaattatttatttattcgtatagaaaagtggggctcaataggtaagagttacaagatccattatttactcttagctcacgaagagctagctagatcttagctcatacatctgcattatttttcatattgattactcagtaaaaactgtccagaactgaagacagaggactcctttttctttagctttcttcctccttttattcaggttcagcacttgcaaagtgagattatttttaattcttgattaatctatttacctcttaagaagatccaggaaatgtgagctcctttactggattttctatttagcttatcacattgtcatccgatctttcaaattttcaatccccaaattagaaatataacattcaaatattaactaatgatatttctattcacttaatatctgaaaggaagtttctctaattgttctcggcattgataccaaatccaaccaaattcagatttgatgaagcactaatggcaactgggtgacctgctggaatgataacaacgtcacccggagacaatctagcttcatatctctacacttcattgtttctttcttttctatcttccctctcttattactcattttttaaacccagaagttcaaggtttccttttccttcattaactaatagtacaactattgcccttgaattgtagtgtggcaacattagagctccttaaaaatttaagcaaaaacgcattaacatatttctgtaatataattaaaattatgtgttttatatatatttagtgttgtgtacatatcttgttaatctccacacaactaacaagtatatctaaatcttaaagctgagggtattttttctctggagtaatctcaaacaacttgccaaacttattagaatattctggcttgtggcttctcaagttgaaaggttcaaattcagagggtaagcttttctttgagcttgattttgcaagctttctcaattcctcaatttattcccttgatactttgattattgcgtctctttcttccccttattatgttcttttccgatctctcaattattatggttttttctcttactcttctaaaagaaccttctctatggtctcgtatttagtttatatttgcgaaaaaggatacaaaatataatggttatatttattaaacatttgataaaaaaatcacacattaagcttaacatgtgttgtttgcatacttatatttaaggaggcctctaaaatgttcttgctgaatcctcataagtattagtttttattttcagatagaccaaaagcttgtagaagaaggataaagatcaatttttcaatccagacaaaaataaaagtaatataaaggaggtgttttaataagaataaaacatgtgaagaaaattattatctcaaatttaccaggcctgttcacgggtattacaaaatccaccactcttagatcttcttcatcatcttagttaactagataagatgttgttcctgcgggaattttgatggtatcaccacgctcaagattatacgagtttctatcattgggactcaacactgtcaatatggctttccttgtagtacatattaaccacaccaaaatttaattatgaaatataagaaatattgctaaattgaactttacaatatttttattttaaatagtcatatttctataaaacaaaagatttgttataataatattataaagaaaaataaaaattatcattgaggactacaaggattaagtcagcatctatgtgttaaggaaggaagatggtgtggggtttggctctatattccacaagacgatagttttagagattttcaaataagtctgaacgtttgtcgaacctttaaaggcgacgaatgtgaccgttttcgttttcaaagagtgtcagaaacttgttagacttgaataaaaaggggtttctttattcttatgattctgaagatctttcttcctcctctccttcacgttaatggcgtctgtctctttttgttctctcctctctatgccttagccttgccctttcttcgggatcttcacgacgttaacttcctctttactcttcgtctacttattcctcatcttcctctctttcttatctctcacgtccaggttaaacttccttttattccttcttttcacgttaatatcaatatttctacttctcttcttcatcttcttccttttcatatgaaggtctttattctccatggcgtttttcttctttctcaccctcttagcgacctctttctctttatcccggtaccctagtttctgaaccttcatcgtaattggcataagtgacgcaaacagaggccaggaatataattcccagaaacaataaaagtggaaatcatgatttgacagtggtcgctatgatttgtatttcactagttcgaactttagatgatgaaataaaagattaagttgaaggatatttatagtgatagaacgtaaagctagatgaataacgtggatggtcatttgggtaca

SEQ ID NO: 83 - DNA, 3400 bp, synthetic construct
  source 1..3400: mol_type = other DNA
gacacggtgagagtaacagaagatagtattaatgactaagtagaagaaatatttctgaccattgattggtgacgaaaactacccctataaagtttactcgcagttaaacatcgaaatatccattatttttttgtcatttactttttcattattattatataagtttaaacacttagaatcataaaaattattaaatctatctttaagcacaacaaacaaatctatctatggatagaataatattgtacctgttgactccaaatacacaacaataatatgaaaaatagaataataaattcaaatggttagaatatatttttacttagataccaaagttttaccatctttcttgtctttcttaagaactatctgaatcaattttgacctcaactattagaataagaaactttatccaaatctataaataaaagaaaacatttgaaattgggttaacaatttaggctcaatccttccaagtctcgaagtctcgattattacgcaactcctcttacatttcatcttttcctcatagaacatttacattaaaacaaagagtccaattaatattcagaacttcatattgtaaatctaacattgatataaccgtcatgaaaatatattttctagagagaaaagaaattgcacaacctcgtcttaactcacaaattacaaaacacttccaattttttaatttaaagaaaagatataaaaacataaacaaattaaagcaactaatacaagagtaaggcactgcatgttatgaaccattacaataataacacaaccaataaccattattaaaaacaattttaaaaattccttcattgaatccatagtctttttttaagacttaccccaagaacacaaattaatattatccttgtagttaaagtaaaaaaaaagcacaagttttattaattatttatttattcgtatagaaaagtggggctcaataggtaagagttacaagatccattatttactcttagctcacgaagagctagctagatcttagctcatacatctgcattatttttcatattgattactcagtaaaaactgtccagaactgaagacagaggactcctttttctttagctttcttcctccttttattcaggttcagcacttgcaaagtgagattatttttaattcttgattaatctatttacctcttaagaagatccaggaaatgtgagctcctttactggattttctatttagcttatcacattgtcatccgatctttcaaattttcaatccccaaattagaaatataacattcaaatattaactaatgatatttctattcacttaatatctgaaaggaagtttctctaattgttctcggcattgataccaaatccaaccaaattcagatttgatgaagcactaatggcaactgggtgacctgctggaatgataacaacgtcacccggagacaatctagcttcatatctctacacttcattgtttctttcttttctatcttccctctcttattactcattttttaaacccagaagttcaaggtttccttttccttcattaactaatagtacaactattgcccttgaattgtagtgtggcaacattagagctccttaaaaatttaagcaaaaacgcattaacatatttctgtaatataattaaaattatgtgttttatatatatttagtgttgtgtacatatcttgttaatctccacacaactaacaagtatatctaaatcttaaagctaagggtattttttctctggagtaatctcaaacaacttgccaaacttattagaatattctggcttgtggcttctcaagttgaaaggttcaaattcagagggtaagcttttctttgagcttgattttgcaagctttctcaattcctcaatttgttcccttgatactttgattattgcgtctctttcttccccttattatgttcttttccgatctctcaattattatggttttttctcttactcttctaaaagaaccttctctatggtctcgtatttagtttatatttgcgaaaaaggatacaaaatataatggttatatttattaaacatttgataaaaaaatcacacattaagcttaacatgtgttgtttgcatacttatatttaaggaggcctctaaaatgttcttgctgaatcctcataagtattagtttttattttcagatagaccaaaagcttgtagaagaaggataaagatcaatttttcaatccagacaaaaataaaagtaatataaaggaggtgttttaataagaataaaacatgtgaagaaaattattatctcaaatttaccaggcctgttcacgggtattacaaaatccaccactcttagatcttcttcatcatcttagttaactagataagatgttgttcctgcgggaattttgatggtatcaccacgctcaagattatacgagtttctatcattgggactcaacactgtcaatatggctttccttgtagtacatattaaccacaccaaaatttaattatgaaatataagaaatattgctaaattgaactttacaatatttttattttaaatagtcatatttctataaaacaaaagatttgttataataatattataaagaaaaataaaaattatcattgaggactacaaggattaagtcagcatctatgtgttaaggaaggaagatggtgtggggtttggctctatattccacaagacgatagttttagagattttcaaataagtctgaacgtttgtcgaacctttaaaggcgacgaatgtgaccgttttcgttttcaaagagtgtcagaaacttgttagacttgaataaaaaggggtttctttattcttatgattctgaagatctttcttcctcctctccttcacgttaatggcgtctgtctctttttgttctctcctctctatgccttagccttgccctttcttcgggatcttcacgacgttaacttcctctttactcttcgtctacttattcctcatcttcctctctttcttatctctcacgtccaggttaaacttccttttattccttcttttcacgttaatatcaatatttctacttctcttcttcatcttcttccttttcatatgaaggtctttattctccatggcgtttttcttctttctcaccctcttagcgacctctttctctttatcccggtaccctagtttctgaaccttcatcgtaattggcataagtgacgcaaacagaggccaggaatataattcccagaaacaataaaagtggaaatcatgatttgacagtggtcgctatgatttgtatttcactagttcgaactttagatgatgaaataaaagattaagttgaaggatatttatagtgatagaacgtaaagctagatgaataacgtggatggtcatttgggtaca

SEQ ID NO: 84 - DNA, 3400 bp, synthetic construct
  source 1..3400: mol_type = other DNA
gacacggtgagagtaacagaagatagtattaatgactaagtagaagaaatatttctgaccattgattggtgacgaaaactacccctataaagtttactcgcagttaaacatcgaaatatccattatttttttgtcatttactttttcattattattatataagtttaaacacttagaatcataaaaattattaaatctatctttaagcacaacaaacaaatctatctatggatagaataatattgtacctgttgactccaaatacacaacaataatatgaaaaatagaataataaattcaaatggttagaatatatttttacttagataccaaagttttaccatctttcttgtctttcttaagaactatctgaatcaattttgacctcaactattagaataagaaactttatccaaatctataaataaaagaaaacatttgaaattgggttaacaatttaggctcaatccttccaagtctcgaagtctcgattattacgcaactcctcttacatttcatcttttcctcatagaacatttacattaaaacaaagagtccaattaatattcagaacttcatattgtaaatctaacattgatataaccgtcatgaaaatatattttctagagagaaaagaaattgcacaacctcgtcttaactcacaaattacaaaacacttccaattttttaatttaaagaaaagatataaaaacataaacaaattaaagcaactaatacaagagtaaggcactgcatgttatgaaccattacaataataacacaaccaataaccattattaaaaacaattttaaaaattccttcattgaatccatagtctttttttaagacttaccccaagaacacaaattaatattatccttgtagttaaagtaaaaaaaaagcacaagttttattaattatttatttattcgtatagaaaagtggggctcaataggtaagagttacaagatccattatttactcttagctcacgaagagctagctagatcttagctcatacatctgcattatttttcatattgattactcagtaaaaactgtccagaactgaagacagaggactcctttttctttagctttcttcctccttttattcaggttcagcacttgcaaagtgagattatttttaattcttgattaatctatttacctcttaagaagatccaggaaatgtgagctcctttactggattttctatttagcttatcacattgtcatccgatctttcaaattttcaatccccaaattagaaatataacattcaaatattaactaatgatatttctattcacttaatatctgaaaggaagtttctctaattgttctcggcattgataccaaatccaaccaaattcagatttgatgaagcactaatggcaactgggtgacctgctggaatgataacaacgtcacccggagacaatctagcttcatatctctacacttcattgtttctttcttttctatcttccctctcttattactcattttttaaacccagaagttcaaggtttccttttccttcattaactaatagtacaactattgcccttgaattgtagtgtggcaacattagagctccttaaaaatttaagcaaaaacgcattaacatatttctgtaatataattaaaattatgtgttttatatatatttagtgttgtgtacatatcttgttaatctccacacaactaacaagtatatctaaatcttaaagctaagggtattttttctctggagtaatctcaaacaacttgccaaacttattagaatattctggcttgtggcttctcaagttgaaaggttcaaattcagagggtaagcttttctttgagcttgattttgcaagctttctcaattcctcaatttattcccttgatactttgattattgcgtctctttcttccccttgttatgttcttttccgatctctcaattattatggttttttctcttactcttctaaaagaaccttctctatggtctcgtatttagtttatatttgcgaaaaaggatacaaaatataatggttatatttattaaacatttgataaaaaaatcacacattaagcttaacatgtgttgtttgcatacttatatttaaggaggcctctaaaatgttcttgctgaatcctcataagtattagtttttattttcagatagaccaaaagcttgtagaagaaggataaagatcaatttttcaatccagacaaaaataaaagtaatataaaggaggtgttttaataagaataaaacatgtgaagaaaattattatctcaaatttaccaggcctgttcacgggtattacaaaatccaccactcttagatcttcttcatcatcttagttaactagataagatgttgttcctgcgggaattttgatggtatcaccacgctcaagattatacgagtttctatcattgggactcaacactgtcaatatggctttccttgtagtacatattaaccacaccaaaatttaattatgaaatataagaaatattgctaaattgaactttacaatatttttattttaaatagtcatatttctataaaacaaaagatttgttataataatattataaagaaaaataaaaattatcattgaggactacaaggattaagtcagcatctatgtgttaaggaaggaagatggtgtggggtttggctctatattccacaagacgatagttttagagattttcaaataagtctgaacgtttgtcgaacctttaaaggcgacgaatgtgaccgttttcgttttcaaagagtgtcagaaacttgttagacttgaataaaaaggggtttctttattcttatgattctgaagatctttcttcctcctctccttcacgttaatggcgtctgtctctttttgttctctcctctctatgccttagccttgccctttcttcgggatcttcacgacgttaacttcctctttactcttcgtctacttattcctcatcttcctctctttcttatctctcacgtccaggttaaacttccttttattccttcttttcacgttaatatcaatatttctacttctcttcttcatcttcttccttttcatatgaaggtctttattctccatggcgtttttcttctttctcaccctcttagcgacctctttctctttatcccggtaccctagtttctgaaccttcatcgtaattggcataagtgacgcaaacagaggccaggaatataattcccagaaacaataaaagtggaaatcatgatttgacagtggtcgctatgatttgtatttcactagttcgaactttagatgatgaaataaaagattaagttgaaggatatttatagtgatagaacgtaaagctagatgaataacgtggatggtcatttgggtaca

SEQ ID NO: 85 - DNA, 3400 bp, synthetic construct
  source 1..3400: mol_type = other DNA
gacacggtgagagtaacagaagatagtattaatgactaagtagaagaaatatttctgaccattgattggtgacgaaaactacccctataaagtttactcgcagttaaacatcgaaatatccattatttttttgtcatttactttttcattattattatataagtttaaacacttagaatcataaaaattattaaatctatctttaagcacaacaaacaaatctatctatggatagaataatattgtacctgttgactccaaatacacaacaataatatgaaaaatagaataataaattcaaatggttagaatatatttttacttagataccaaagttttaccatctttcttgtctttcttaagaactatctgaatcaattttgacctcaactattagaataagaaactttatccaaatctataaataaaagaaaacatttgaaattgggttaacaatttaggctcaatccttccaagtctcgaagtctcgattattacgcaactcctcttacatttcatcttttcctcatagaacatttacattaaaacaaagagtccaattaatattcagaacttcatattgtaaatctaacattgatataaccgtcatgaaaatatattttctagagagaaaagaaattgcacaacctcgtcttaactcacaaattacaaaacacttccaattttttaatttaaagaaaagatataaaaacataaacaaattaaagcaactaatacaagagtaaggcactgcatgttatgaaccattacaataataacacaaccaataaccattattaaaaacaattttaaaaattccttcattgaatccatagtctttttttaagacttaccccaagaacacaaattaatattatccttgtagttaaagtaaaaaaaaagcacaagttttattaattatttatttattcgtatagaaaagtggggctcaataggtaagagttacaagatccattatttactcttagctcacgaagagctagctagatcttagctcatacatctgcattatttttcatattgattactcagtaaaaactgtccagaactgaagacagaggactcctttttctttagctttcttcctccttttattcaggttcagcacttgcaaagtgagattatttttaattcttgattaatctatttacctcttaagaagatccaggaaatgtgagctcctttactggattttctatttagcttatcacattgtcatccgatctttcaaattttcaatccccaaattagaaatataacattcaaatattaactaatgatatttctattcacttaatatctgaaaggaagtttctctaattgttctcggcattgataccaaatccaaccaaattcagatttgatgaagcactaatggcaactgggtgacctgctggaatgataacaacgtcacccggagacaatctagcttcatatctctacacttcattgtttctttcttttctatcttccctctcttattactcattttttaaacccagaagttcaaggtttccttttccttcattaactaatagtacaactattgcccttgaattgtagtgtggcaacattagagctccttaaaaatttaagcaaaaacgcattaacatatttctgtaatataattaaaattatgtgttttatatatatttagtgttgtgtacatatcttgttaatctccacacaactaacaagtatatctaaatcttaaagctaagggtattttttctctggagtaatctcaaacaacttgccaaacttattagaatattctggcttgtggcttctcaagttgaaaggttcaaattcagagggtaagcttttctttgagcttgattttgcaagctttctcaattcctcaatttattcccttgatactttgattattgcgtctctttcttccccttattgtgttcttttccgatctctcaattattatggttttttctcttactcttctaaaagaaccttctctatggtctcgtatttagtttatatttgcgaaaaaggatacaaaatataatggttatatttattaaacatttgataaaaaaatcacacattaagcttaacatgtgttgtttgcatacttatatttaaggaggcctctaaaatgttcttgctgaatcctcataagtattagtttttattttcagatagaccaaaagcttgtagaagaaggataaagatcaatttttcaatccagacaaaaataaaagtaatataaaggaggtgttttaataagaataaaacatgtgaagaaaattattatctcaaatttaccaggcctgttcacgggtattacaaaatccaccactcttagatcttcttcatcatcttagttaactagataagatgttgttcctgcgggaattttgatggtatcaccacgctcaagattatacgagtttctatcattgggactcaacactgtcaatatggctttccttgtagtacatattaaccacaccaaaatttaattatgaaatataagaaatattgctaaattgaactttacaatatttttattttaaatagtcatatttctataaaacaaaagatttgttataataatattataaagaaaaataaaaattatcattgaggactacaaggattaagtcagcatctatgtgttaaggaaggaagatggtgtggggtttggctctatattccacaagacgatagttttagagattttcaaataagtctgaacgtttgtcgaacctttaaaggcgacgaatgtgaccgttttcgttttcaaagagtgtcagaaacttgttagacttgaataaaaaggggtttctttattcttatgattctgaagatctttcttcctcctctccttcacgttaatggcgtctgtctctttttgttctctcctctctatgccttagccttgccctttcttcgggatcttcacgacgttaacttcctctttactcttcgtctacttattcctcatcttcctctctttcttatctctcacgtccaggttaaacttccttttattccttcttttcacgttaatatcaatatttctacttctcttcttcatcttcttccttttcatatgaaggtctttattctccatggcgtttttcttctttctcaccctcttagcgacctctttctctttatcccggtaccctagtttctgaaccttcatcgtaattggcataagtgacgcaaacagaggccaggaatataattcccagaaacaataaaagtggaaatcatgatttgacagtggtcgctatgatttgtatttcactagttcgaactttagatgatgaaataaaagattaagttgaaggatatttatagtgatagaacgtaaagctagatgaataacgtggatggtcatttgggtaca

SEQ ID NO: 86 - DNA, 3400 bp, synthetic construct
  source 1..3400: mol_type = other DNA
gacacggtgagagtaacagaagatagtattaatgactaagtagaagaaatatttctgaccattgattggtgacgaaaactacccctataaagtttactcgcagttaaacatcgaaatatccattatttttttgtcatttactttttcattattattatataagtttaaacacttagaatcataaaaattattaaatctatctttaagcacaacaaacaaatctatctatggatagaataatattgtacctgttgactccaaatacacaacaataatatgaaaaatagaataataaattcaaatggttagaatatatttttacttagataccaaagttttaccatctttcttgtctttcttaagaactatctgaatcaattttgacctcaactattagaataagaaactttatccaaatctataaataaaagaaaacatttgaaattgggttaacaatttaggctcaatccttccaagtctcgaagtctcgattattacgcaactcctcttacatttcatcttttcctcatagaacatttacattaaaacaaagagtccaattaatattcagaacttcatattgtaaatctaacattgatataaccgtcatgaaaatatattttctagagagaaaagaaattgcacaacctcgtcttaactcacaaattacaaaacacttccaattttttaatttaaagaaaagatataaaaacataaacaaattaaagcaactaatacaagagtaaggcactgcatgttatgaaccattacaataataacacaaccaataaccattattaaaaacaattttaaaaattccttcattgaatccatagtctttttttaagacttaccccaagaacacaaattaatattatccttgtagttaaagtaaaaaaaaagcacaagttttattaattatttatttattcgtatagaaaagtggggctcaataggtaagagttacaagatccattatttactcttagctcacgaagagctagctagatcttagctcatacatctgcattatttttcatattgattactcagtaaaaactgtccagaactgaagacagaggactcctttttctttagctttcttcctccttttattcaggttcagcacttgcaaagtgagattatttttaattcttgattaatctatttacctcttaagaagatccaggaaatgtgagctcctttactggattttctatttagcttatcacattgtcatccgatctttcaaattttcaatccccaaattagaaatataacattcaaatattaactaatgatatttctattcacttaatatctgaaaggaagtttctctaattgttctcggcattgataccaaatccaaccaaattcagatttgatgaagcactaatggcaactgggtgacctgctggaatgataacaacgtcacccggagacaatctagcttcatatctctacacttcattgtttctttcttttctatcttccctctcttattactcattttttaaacccagaagttcaaggtttccttttccttcattaactaatagtacaactattgcccttgaattgtagtgtggcaacattagagctccttaaaaatttaagcaaaaacgcattaacatatttctgtaatataattaaaattatgtgttttatatatatttagtgttgtgtacatatcttgttaatctccacacaactaacaagtatatctaaatcttaaagctaagggtattttttctctggagtaatctcaaacaacttgccaaacttattagaatattctggcttgtggcttctcaagttgaaaggttcaaattcagagggtaagcttttctttgagcttgattttgcaagctttctcaattcctcaatttattcccttgatactttgattattgcgtctctttcttccccttattatgttcttttccgatctctcaattgttatggttttttctcttactcttctaaaagaaccttctctatggtctcgtatttagtttatatttgcgaaaaaggatacaaaatataatggttatatttattaaacatttgataaaaaaatcacacattaagcttaacatgtgttgtttgcatacttatatttaaggaggcctctaaaatgttcttgctgaatcctcataagtattagtttttattttcagatagaccaaaagcttgtagaagaaggataaagatcaatttttcaatccagacaaaaataaaagtaatataaaggaggtgttttaataagaataaaacatgtgaagaaaattattatctcaaatttaccaggcctgttcacgggtattacaaaatccaccactcttagatcttcttcatcatcttagttaactagataagatgttgttcctgcgggaattttgatggtatcaccacgctcaagattatacgagtttctatcattgggactcaacactgtcaatatggctttccttgtagtacatattaaccacaccaaaatttaattatgaaatataagaaatattgctaaattgaactttacaatatttttattttaaatagtcatatttctataaaacaaaagatttgttataataatattataaagaaaaataaaaattatcattgaggactacaaggattaagtcagcatctatgtgttaaggaaggaagatggtgtggggtttggctctatattccacaagacgatagttttagagattttcaaataagtctgaacgtttgtcgaacctttaaaggcgacgaatgtgaccgttttcgttttcaaagagtgtcagaaacttgttagacttgaataaaaaggggtttctttattcttatgattctgaagatctttcttcctcctctccttcacgttaatggcgtctgtctctttttgttctctcctctctatgccttagccttgccctttcttcgggatcttcacgacgttaacttcctctttactcttcgtctacttattcctcatcttcctctctttcttatctctcacgtccaggttaaacttccttttattccttcttttcacgttaatatcaatatttctacttctcttcttcatcttcttccttttcatatgaaggtctttattctccatggcgtttttcttctttctcaccctcttagcgacctctttctctttatcccggtaccctagtttctgaaccttcatcgtaattggcataagtgacgcaaacagaggccaggaatataattcccagaaacaataaaagtggaaatcatgatttgacagtggtcgctatgatttgtatttcactagttcgaactttagatgatgaaataaaagattaagttgaaggatatttatagtgatagaacgtaaagctagatgaataacgtggatggtcatttgggtaca

SEQ ID NO: 87 - DNA, 3400 bp, synthetic construct
  source 1..3400: mol_type = other DNA
gacacggtgagagtaacagaagatagtattaatgactaagtagaagaaatatttctgaccattgattggtgacgaaaactacccctataaagtttactcgcagttaaacatcgaaatatccattatttttttgtcatttactttttcattattattatataagtttaaacacttagaatcataaaaattattaaatctatctttaagcacaacaaacaaatctatctatggatagaataatattgtacctgttgactccaaatacacaacaataatatgaaaaatagaataataaattcaaatggttagaatatatttttacttagataccaaagttttaccatctttcttgtctttcttaagaactatctgaatcaattttgacctcaactattagaataagaaactttatccaaatctataaataaaagaaaacatttgaaattgggttaacaatttaggctcaatccttccaagtctcgaagtctcgattattacgcaactcctcttacatttcatcttttcctcatagaacatttacattaaaacaaagagtccaattaatattcagaacttcatattgtaaatctaacattgatataaccgtcatgaaaatatattttctagagagaaaagaaattgcacaacctcgtcttaactcacaaattacaaaacacttccaattttttaatttaaagaaaagatataaaaacataaacaaattaaagcaactaatacaagagtaaggcactgcatgttatgaaccattacaataataacacaaccaataaccattattaaaaacaattttaaaaattccttcattgaatccatagtctttttttaagacttaccccaagaacacaaattaatattatccttgtagttaaagtaaaaaaaaagcacaagttttattaattatttatttattcgtatagaaaagtggggctcaataggtaagagttacaagatccattatttactcttagctcacgaagagctagctagatcttagctcatacatctgcattatttttcatattgattactcagtaaaaactgtccagaactgaagacagaggactcctttttctttagctttcttcctccttttattcaggttcagcacttgcaaagtgagattatttttaattcttgattaatctatttacctcttaagaagatccaggaaatgtgagctcctttactggattttctatttagcttatcacattgtcatccgatctttcaaattttcaatccccaaattagaaatataacattcaaatattaactaatgatatttctattcacttaatatctgaaaggaagtttctctaattgttctcggcattgataccaaatccaaccaaattcagatttgatgaagcactaatggcaactgggtgacctgctggaatgataacaacgtcacccggagacaatctagcttcatatctctacacttcattgtttctttcttttctatcttccctctcttattactcattttttaaacccagaagttcaaggtttccttttccttcattaactaatagtacaactattgcccttgaattgtagtgtggcaacattagagctccttaaaaatttaagcaaaaacgcattaacatatttctgtaatataattaaaattatgtgttttatatatatttagtgttgtgtacatatcttgttaatctccacacaactaacaagtatatctaaatcttaaagctaagggtattttttctctggagtaatctcaaacaacttgccaaacttattagaatattctggcttgtggcttctcaagttgaaaggttcaaattcagagggtaagcttttctttgagcttgattttgcaagctttctcaattcctcaatttattcccttgatactttgattattgcgtctctttcttccccttattatgttcttttccgatctctcaattattgtggttttttctcttactcttctaaaagaaccttctctatggtctcgtatttagtttatatttgcgaaaaaggatacaaaatataatggttatatttattaaacatttgataaaaaaatcacacattaagcttaacatgtgttgtttgcatacttatatttaaggaggcctctaaaatgttcttgctgaatcctcataagtattagtttttattttcagatagaccaaaagcttgtagaagaaggataaagatcaatttttcaatccagacaaaaataaaagtaatataaaggaggtgttttaataagaataaaacatgtgaagaaaattattatctcaaatttaccaggcctgttcacgggtattacaaaatccaccactcttagatcttcttcatcatcttagttaactagataagatgttgttcctgcgggaattttgatggtatcaccacgctcaagattatacgagtttctatcattgggactcaacactgtcaatatggctttccttgtagtacatattaaccacaccaaaatttaattatgaaatataagaaatattgctaaattgaactttacaatatttttattttaaatagtcatatttctataaaacaaaagatttgttataataatattataaagaaaaataaaaattatcattgaggactacaaggattaagtcagcatctatgtgttaaggaaggaagatggtgtggggtttggctctatattccacaagacgatagttttagagattttcaaataagtctgaacgtttgtcgaacctttaaaggcgacgaatgtgaccgttttcgttttcaaagagtgtcagaaacttgttagacttgaataaaaaggggtttctttattcttatgattctgaagatctttcttcctcctctccttcacgttaatggcgtctgtctctttttgttctctcctctctatgccttagccttgccctttcttcgggatcttcacgacgttaacttcctctttactcttcgtctacttattcctcatcttcctctctttcttatctctcacgtccaggttaaacttccttttattccttcttttcacgttaatatcaatatttctacttctcttcttcatcttcttccttttcatatgaaggtctttattctccatggcgtttttcttctttctcaccctcttagcgacctctttctctttatcccggtaccctagtttctgaaccttcatcgtaattggcataagtgacgcaaacagaggccaggaatataattcccagaaacaataaaagtggaaatcatgatttgacagtggtcgctatgatttgtatttcactagttcgaactttagatgatgaaataaaagattaagttgaaggatatttatagtgatagaacgtaaagctagatgaataacgtggatggtcatttgggtaca

SEQ ID NO: 88 - DNA, 3400 bp, synthetic construct
  source 1..3400: mol_type = other DNA
gacacggtgagagtaacagaagatagtattaatgactaagtagaagaaatatttctgaccattgattggtgacgaaaactacccctataaagtttactcgcagttaaacatcgaaatatccattatttttttgtcatttactttttcattattattatataagtttaaacacttagaatcataaaaattattaaatctatctttaagcacaacaaacaaatctatctatggatagaataatattgtacctgttgactccaaatacacaacaataatatgaaaaatagaataataaattcaaatggttagaatatatttttacttagataccaaagttttaccatctttcttgtctttcttaagaactatctgaatcaattttgacctcaactattagaataagaaactttatccaaatctataaataaaagaaaacatttgaaattgggttaacaatttaggctcaatccttccaagtctcgaagtctcgattattacgcaactcctcttacatttcatcttttcctcatagaacatttacattaaaacaaagagtccaattaatattcagaacttcatattgtaaatctaacattgatataaccgtcatgaaaatatattttctagagagaaaagaaattgcacaacctcgtcttaactcacaaattacaaaacacttccaattttttaatttaaagaaaagatataaaaacataaacaaattaaagcaactaatacaagagtaaggcactgcatgttatgaaccattacaataataacacaaccaataaccattattaaaaacaattttaaaaattccttcattgaatccatagtctttttttaagacttaccccaagaacacaaattaatattatccttgtagttaaagtaaaaaaaaagcacaagttttattaattatttatttattcgtatagaaaagtggggctcaataggtaagagttacaagatccattatttactcttagctcacgaagagctagctagatcttagctcatacatctgcattatttttcatattgattactcagtaaaaactgtccagaactgaagacagaggactcctttttctttagctttcttcctccttttattcaggttcagcacttgcaaagtgagattatttttaattcttgattaatctatttacctcttaagaagatccaggaaatgtgagctcctttactggattttctatttagcttatcacattgtcatccgatctttcaaattttcaatccccaaattagaaatataacattcaaatattaactaatgatatttctattcacttaatatctgaaaggaagtttctctaattgttctcggcattgataccaaatccaaccaaattcagatttgatgaagcactaatggcaactgggtgacctgctggaatgataacaacgtcacccggagacaatctagcttcatatctctacacttcattgtttctttcttttctatcttccctctcttattactcattttttaaacccagaagttcaaggtttccttttccttcattaactaatagtacaactattgcccttgaattgtagtgtggcaacattagagctccttaaaaatttaagcaaaaacgcattaacatatttctgtaatataattaaaattatgtgttttatatatatttagtgttgtgtacatatcttgttaatctccacacaactaacaagtatatctaaatcttaaagctaagggtattttttctctggagtaatctcaaacaacttgccaaacttattagaatattctggcttgtggcttctcaagttgaaaggttcaaattcagagggtaagcttttctttgagcttgattttgcaagctttctcaattcctcaatttattcccttgatactttgattattgcgtctctttcttccccttattatgttcttttccgatctctcaattattatggttttttctcttgctcttctaaaagaaccttctctatggtctcgtatttagtttatatttgcgaaaaaggatacaaaatataatggttatatttattaaacatttgataaaaaaatcacacattaagcttaacatgtgttgtttgcatacttatatttaaggaggcctctaaaatgttcttgctgaatcctcataagtattagtttttattttcagatagaccaaaagcttgtagaagaaggataaagatcaatttttcaatccagacaaaaataaaagtaatataaaggaggtgttttaataagaataaaacatgtgaagaaaattattatctcaaatttaccaggcctgttcacgggtattacaaaatccaccactcttagatcttcttcatcatcttagttaactagataagatgttgttcctgcgggaattttgatggtatcaccacgctcaagattatacgagtttctatcattgggactcaacactgtcaatatggctttccttgtagtacatattaaccacaccaaaatttaattatgaaatataagaaatattgctaaattgaactttacaatatttttattttaaatagtcatatttctataaaacaaaagatttgttataataatattataaagaaaaataaaaattatcattgaggactacaaggattaagtcagcatctatgtgttaaggaaggaagatggtgtggggtttggctctatattccacaagacgatagttttagagattttcaaataagtctgaacgtttgtcgaacctttaaaggcgacgaatgtgaccgttttcgttttcaaagagtgtcagaaacttgttagacttgaataaaaaggggtttctttattcttatgattctgaagatctttcttcctcctctccttcacgttaatggcgtctgtctctttttgttctctcctctctatgccttagccttgccctttcttcgggatcttcacgacgttaacttcctctttactcttcgtctacttattcctcatcttcctctctttcttatctctcacgtccaggttaaacttccttttattccttcttttcacgttaatatcaatatttctacttctcttcttcatcttcttccttttcatatgaaggtctttattctccatggcgtttttcttctttctcaccctcttagcgacctctttctctttatcccggtaccctagtttctgaaccttcatcgtaattggcataagtgacgcaaacagaggccaggaatataattcccagaaacaataaaagtggaaatcatgatttgacagtggtcgctatgatttgtatttcactagttcgaactttagatgatgaaataaaagattaagttgaaggatatttatagtgatagaacgtaaagctagatgaataacgtggatggtcatttgggtaca

SEQ ID NO: 89 - DNA, 3400 bp, synthetic construct
  source 1..3400: mol_type = other DNA
gacacggtgagagtaacagaagatagtattaatgactaagtagaagaaatatttctgaccattgattggtgacgaaaactacccctataaagtttactcgcagttaaacatcgaaatatccattatttttttgtcatttactttttcattattattatataagtttaaacacttagaatcataaaaattattaaatctatctttaagcacaacaaacaaatctatctatggatagaataatattgtacctgttgactccaaatacacaacaataatatgaaaaatagaataataaattcaaatggttagaatatatttttacttagataccaaagttttaccatctttcttgtctttcttaagaactatctgaatcaattttgacctcaactattagaataagaaactttatccaaatctataaataaaagaaaacatttgaaattgggttaacaatttaggctcaatccttccaagtctcgaagtctcgattattacgcaactcctcttacatttcatcttttcctcatagaacatttacattaaaacaaagagtccaattaatattcagaacttcatattgtaaatctaacattgatataaccgtcatgaaaatatattttctagagagaaaagaaattgcacaacctcgtcttaactcacaaattacaaaacacttccaattttttaatttaaagaaaagatataaaaacataaacaaattaaagcaactaatacaagagtaaggcactgcatgttatgaaccattacaataataacacaaccaataaccattattaaaaacaattttaaaaattccttcattgaatccatagtctttttttaagacttaccccaagaacacaaattaatattatccttgtagttaaagtaaaaaaaaagcacaagttttattaattatttatttattcgtatagaaaagtggggctcaataggtaagagttacaagatccattatttactcttagctcacgaagagctagctagatcttagctcatacatctgcattatttttcatattgattactcagtaaaaactgtccagaactgaagacagaggactcctttttctttagctttcttcctccttttattcaggttcagcacttgcaaagtgagattatttttaattcttgattaatctatttacctcttaagaagatccaggaaatgtgagctcctttactggattttctatttagcttatcacattgtcatccgatctttcaaattttcaatccccaaattagaaatataacattcaaatattaactaatgatatttctattcacttaatatctgaaaggaagtttctctaattgttctcggcattgataccaaatccaaccaaattcagatttgatgaagcactaatggcaactgggtgacctgctggaatgataacaacgtcacccggagacaatctagcttcatatctctacacttcattgtttctttcttttctatcttccctctcttattactcattttttaaacccagaagttcaaggtttccttttccttcattaactaatagtacaactattgcccttgaattgtagtgtggcaacattagagctccttaaaaatttaagcaaaaacgcattaacatatttctgtaatataattaaaattatgtgttttatatatatttagtgttgtgtacatatcttgttaatctccacacaactaacaagtatatctaaatcttaaagctaagggtattttttctctggagtaatctcaaacaacttgccaaacttattagaatattctggcttgtggcttctcaagttgaaaggttcaaattcagagggtaagcttttctttgagcttgattttgcaagctttctcaattcctcaatttattcccttgatactttgattattgcgtctctttcttccccttattatgttcttttccgatctctcaattattatggttttttctcttactcttctaaaagaaccttctctatggtctcgtatttagtctatatttgcgaaaaaggatacaaaatataatggttatatttattaaacatttgataaaaaaatcacacattaagcttaacatgtgttgtttgcatacttatatttaaggaggcctctaaaatgttcttgctgaatcctcataagtattagtttttattttcagatagaccaaaagcttgtagaagaaggataaagatcaatttttcaatccagacaaaaataaaagtaatataaaggaggtgttttaataagaataaaacatgtgaagaaaattattatctcaaatttaccaggcctgttcacgggtattacaaaatccaccactcttagatcttcttcatcatcttagttaactagataagatgttgttcctgcgggaattttgatggtatcaccacgctcaagattatacgagtttctatcattgggactcaacactgtcaatatggctttccttgtagtacatattaaccacaccaaaatttaattatgaaatataagaaatattgctaaattgaactttacaatatttttattttaaatagtcatatttctataaaacaaaagatttgttataataatattataaagaaaaataaaaattatcattgaggactacaaggattaagtcagcatctatgtgttaaggaaggaagatggtgtggggtttggctctatattccacaagacgatagttttagagattttcaaataagtctgaacgtttgtcgaacctttaaaggcgacgaatgtgaccgttttcgttttcaaagagtgtcagaaacttgttagacttgaataaaaaggggtttctttattcttatgattctgaagatctttcttcctcctctccttcacgttaatggcgtctgtctctttttgttctctcctctctatgccttagccttgccctttcttcgggatcttcacgacgttaacttcctctttactcttcgtctacttattcctcatcttcctctctttcttatctctcacgtccaggttaaacttccttttattccttcttttcacgttaatatcaatatttctacttctcttcttcatcttcttccttttcatatgaaggtctttattctccatggcgtttttcttctttctcaccctcttagcgacctctttctctttatcccggtaccctagtttctgaaccttcatcgtaattggcataagtgacgcaaacagaggccaggaatataattcccagaaacaataaaagtggaaatcatgatttgacagtggtcgctatgatttgtatttcactagttcgaactttagatgatgaaataaaagattaagttgaaggatatttatagtgatagaacgtaaagctagatgaataacgtggatggtcatttgggtaca

SEQ ID NO: 90 - DNA, 3400 bp, synthetic construct
  source 1..3400: mol_type = other DNA
gacacggtgagagtaacagaagatagtattaatgactaagtagaagaaatatttctgaccattgattggtgacgaaaactacccctataaagtttactcgcagttaaacatcgaaatatccattatttttttgtcatttactttttcattattattatataagtttaaacacttagaatcataaaaattattaaatctatctttaagcacaacaaacaaatctatctatggatagaataatattgtacctgttgactccaaatacacaacaataatatgaaaaatagaataataaattcaaatggttagaatatatttttacttagataccaaagttttaccatctttcttgtctttcttaagaactatctgaatcaattttgacctcaactattagaataagaaactttatccaaatctataaataaaagaaaacatttgaaattgggttaacaatttaggctcaatccttccaagtctcgaagtctcgattattacgcaactcctcttacatttcatcttttcctcatagaacatttacattaaaacaaagagtccaattaatattcagaacttcatattgtaaatctaacattgatataaccgtcatgaaaatatattttctagagagaaaagaaattgcacaacctcgtcttaactcacaaattacaaaacacttccaattttttaatttaaagaaaagatataaaaacataaacaaattaaagcaactaatacaagagtaaggcactgcatgttatgaaccattacaataataacacaaccaataaccattattaaaaacaattttaaaaattccttcattgaatccatagtctttttttaagacttaccccaagaacacaaattaatattatccttgtagttaaagtaaaaaaaaagcacaagttttattaattatttatttattcgtatagaaaagtggggctcaataggtaagagttacaagatccattatttactcttagctcacgaagagctagctagatcttagctcatacatctgcattatttttcatattgattactcagtaaaaactgtccagaactgaagacagaggactcctttttctttagctttcttcctccttttattcaggttcagcacttgcaaagtgagattatttttaattcttgattaatctatttacctcttaagaagatccaggaaatgtgagctcctttactggattttctatttagcttatcacattgtcatccgatctttcaaattttcaatccccaaattagaaatataacattcaaatattaactaatgatatttctattcacttaatatctgaaaggaagtttctctaattgttctcggcattgataccaaatccaaccaaattcagatttgatgaagcactaatggcaactgggtgacctgctggaatgataacaacgtcacccggagacaatctagcttcatatctctacacttcattgtttctttcttttctatcttccctctcttattactcattttttaaacccagaagttcaaggtttccttttccttcattaactaatagtacaactattgcccttgaattgtagtgtggcaacattagagctccttaaaaatttaagcaaaaacgcattaacatatttctgtaatataattaaaattatgtgttttatatatatttagtgttgtgtacatatcttgttaatctccacacaactaacaagtatatctaaatcttaaagctaagggtattttttctctggagtaatctcaaacaacttgccaaacttattagaatattctggcttgtggcttctcaagttgaaaggttcaaattcagagggtaagcttttctttgagcttgattttgcaagctttctcaattcctcaatttattcccttgatactttgattattgcgtctctttcttccccttattatgttcttttccgatctctcaattattatggttttttctcttactcttctaaaagaaccttctctatggtctcgtatttagtttatatttgcgaaaaaggatacaaaatataatggttatatttattaaacatttgataaaaaaatcacacattaagcttaacatgtgttgtttgcatacttacatttaaggaggcctctaaaatgttcttgctgaatcctcataagtattagtttttattttcagatagaccaaaagcttgtagaagaaggataaagatcaatttttcaatccagacaaaaataaaagtaatataaaggaggtgttttaataagaataaaacatgtgaagaaaattattatctcaaatttaccaggcctgttcacgggtattacaaaatccaccactcttagatcttcttcatcatcttagttaactagataagatgttgttcctgcgggaattttgatggtatcaccacgctcaagattatacgagtttctatcattgggactcaacactgtcaatatggctttccttgtagtacatattaaccacaccaaaatttaattatgaaatataagaaatattgctaaattgaactttacaatatttttattttaaatagtcatatttctataaaacaaaagatttgttataataatattataaagaaaaataaaaattatcattgaggactacaaggattaagtcagcatctatgtgttaaggaaggaagatggtgtggggtttggctctatattccacaagacgatagttttagagattttcaaataagtctgaacgtttgtcgaacctttaaaggcgacgaatgtgaccgttttcgttttcaaagagtgtcagaaacttgttagacttgaataaaaaggggtttctttattcttatgattctgaagatctttcttcctcctctccttcacgttaatggcgtctgtctctttttgttctctcctctctatgccttagccttgccctttcttcgggatcttcacgacgttaacttcctctttactcttcgtctacttattcctcatcttcctctctttcttatctctcacgtccaggttaaacttccttttattccttcttttcacgttaatatcaatatttctacttctcttcttcatcttcttccttttcatatgaaggtctttattctccatggcgtttttcttctttctcaccctcttagcgacctctttctctttatcccggtaccctagtttctgaaccttcatcgtaattggcataagtgacgcaaacagaggccaggaatataattcccagaaacaataaaagtggaaatcatgatttgacagtggtcgctatgatttgtatttcactagttcgaactttagatgatgaaataaaagattaagttgaaggatatttatagtgatagaacgtaaagctagatgaataacgtggatggtcatttgggtaca

SEQ ID NO: 91 - DNA, 3400 bp, synthetic construct
  source 1..3400: mol_type = other DNA
gacacggtgagagtaacagaagatagtattaatgactaagtagaagaaatatttctgaccattgattggtgacgaaaactacccctataaagtttactcgcagttaaacatcgaaatatccattatttttttgtcatttactttttcattattattatataagtttaaacacttagaatcataaaaattattaaatctatctttaagcacaacaaacaaatctatctatggatagaataatattgtacctgttgactccaaatacacaacaataatatgaaaaatagaataataaattcaaatggttagaatatatttttacttagataccaaagttttaccatctttcttgtctttcttaagaactatctgaatcaattttgacctcaactattagaataagaaactttatccaaatctataaataaaagaaaacatttgaaattgggttaacaatttaggctcaatccttccaagtctcgaagtctcgattattacgcaactcctcttacatttcatcttttcctcatagaacatttacattaaaacaaagagtccaattaatattcagaacttcatattgtaaatctaacattgatataaccgtcatgaaaatatattttctagagagaaaagaaattgcacaacctcgtcttaactcacaaattacaaaacacttccaattttttaatttaaagaaaagatataaaaacataaacaaattaaagcaactaatacaagagtaaggcactgcatgttatgaaccattacaataataacacaaccaataaccattattaaaaacaattttaaaaattccttcattgaatccatagtctttttttaagacttaccccaagaacacaaattaatattatccttgtagttaaagtaaaaaaaaagcacaagttttattaattatttatttattcgtatagaaaagtggggctcaataggtaagagttacaagatccattatttactcttagctcacgaagagctagctagatcttagctcatacatctgcattatttttcatattgattactcagtaaaaactgtccagaactgaagacagaggactcctttttctttagctttcttcctccttttattcaggttcagcacttgcaaagtgagattatttttaattcttgattaatctatttacctcttaagaagatccaggaaatgtgagctcctttactggattttctatttagcttatcacattgtcatccgatctttcaaattttcaatccccaaattagaaatataacattcaaatattaactaatgatatttctattcacttaatatctgaaaggaagtttctctaattgttctcggcattgataccaaatccaaccaaattcagatttgatgaagcactaatggcaactgggtgacctgctggaatgataacaacgtcacccggagacaatctagcttcatatctctacacttcattgtttctttcttttctatcttccctctcttattactcattttttaaacccagaagttcaaggtttccttttccttcattaactaatagtacaactattgcccttgaattgtagtgtggcaacattagagctccttaaaaatttaagcaaaaacgcattaacatatttctgtaatataattaaaattatgtgttttatatatatttagtgttgtgtacatatcttgttaatctccacacaactaacaagtatatctaaatcttaaagctaagggtattttttctctggagtaatctcaaacaacttgccaaacttattagaatattctggcttgtggcttctcaagttgaaaggttcaaattcagagggtaagcttttctttgagcttgattttgcaagctttctcaattcctcaatttattcccttgatactttgattattgcgtctctttcttccccttattatgttcttttccgatctctcaattattatggttttttctcttactcttctaaaagaaccttctctatggtctcgtatttagtttatatttgcgaaaaaggatacaaaatataatggttatatttattaaacatttgataaaaaaatcacacattaagcttaacatgtgttgtttgcatacttatatttaaggaggcctctaaaatgttcttgctgaatcctcgtaagtattagtttttattttcagatagaccaaaagcttgtagaagaaggataaagatcaatttttcaatccagacaaaaataaaagtaatataaaggaggtgttttaataagaataaaacatgtgaagaaaattattatctcaaatttaccaggcctgttcacgggtattacaaaatccaccactcttagatcttcttcatcatcttagttaactagataagatgttgttcctgcgggaattttgatggtatcaccacgctcaagattatacgagtttctatcattgggactcaacactgtcaatatggctttccttgtagtacatattaaccacaccaaaatttaattatgaaatataagaaatattgctaaattgaactttacaatatttttattttaaatagtcatatttctataaaacaaaagatttgttataataatattataaagaaaaataaaaattatcattgaggactacaaggattaagtcagcatctatgtgttaaggaaggaagatggtgtggggtttggctctatattccacaagacgatagttttagagattttcaaataagtctgaacgtttgtcgaacctttaaaggcgacgaatgtgaccgttttcgttttcaaagagtgtcagaaacttgttagacttgaataaaaaggggtttctttattcttatgattctgaagatctttcttcctcctctccttcacgttaatggcgtctgtctctttttgttctctcctctctatgccttagccttgccctttcttcgggatcttcacgacgttaacttcctctttactcttcgtctacttattcctcatcttcctctctttcttatctctcacgtccaggttaaacttccttttattccttcttttcacgttaatatcaatatttctacttctcttcttcatcttcttccttttcatatgaaggtctttattctccatggcgtttttcttctttctcaccctcttagcgacctctttctctttatcccggtaccctagtttctgaaccttcatcgtaattggcataagtgacgcaaacagaggccaggaatataattcccagaaacaataaaagtggaaatcatgatttgacagtggtcgctatgatttgtatttcactagttcgaactttagatgatgaaataaaagattaagttgaaggatatttatagtgatagaacgtaaagctagatgaataacgtggatggtcatttgggtaca

SEQ ID NO: 92 - DNA, 3400 bp, synthetic construct
  source 1..3400: mol_type = other DNA
gacacggtgagagtaacagaagatagtattaatgactaagtagaagaaatatttctgaccattgattggtgacgaaaactacccctataaagtttactcgcagttaaacatcgaaatatccattatttttttgtcatttactttttcattattattatataagtttaaacacttagaatcataaaaattattaaatctatctttaagcacaacaaacaaatctatctatggatagaataatattgtacctgttgactccaaatacacaacaataatatgaaaaatagaataataaattcaaatggttagaatatatttttacttagataccaaagttttaccatctttcttgtctttcttaagaactatctgaatcaattttgacctcaactattagaataagaaactttatccaaatctataaataaaagaaaacatttgaaattgggttaacaatttaggctcaatccttccaagtctcgaagtctcgattattacgcaactcctcttacatttcatcttttcctcatagaacatttacattaaaacaaagagtccaattaatattcagaacttcatattgtaaatctaacattgatataaccgtcatgaaaatatattttctagagagaaaagaaattgcacaacctcgtcttaactcacaaattacaaaacacttccaattttttaatttaaagaaaagatataaaaacataaacaaattaaagcaactaatacaagagtaaggcactgcatgttatgaaccattacaataataacacaaccaataaccattattaaaaacaattttaaaaattccttcattgaatccatagtctttttttaagacttaccccaagaacacaaattaatattatccttgtagttaaagtaaaaaaaaagcacaagttttattaattatttatttattcgtatagaaaagtggggctcaataggtaagagttacaagatccattatttactcttagctcacgaagagctagctagatcttagctcatacatctgcattatttttcatattgattactcagtaaaaactgtccagaactgaagacagaggactcctttttctttagctttcttcctccttttattcaggttcagcacttgcaaagtgagattatttttaattcttgattaatctatttacctcttaagaagatccaggaaatgtgagctcctttactggattttctatttagcttatcacattgtcatccgatctttcaaattttcaatccccaaattagaaatataacattcaaatattaactaatgatatttctattcacttaatatctgaaaggaagtttctctaattgttctcggcattgataccaaatccaaccaaattcagatttgatgaagcactaatggcaactgggtgacctgctggaatgataacaacgtcacccggagacaatctagcttcatatctctacacttcattgtttctttcttttctatcttccctctcttattactcattttttaaacccagaagttcaaggtttccttttccttcattaactaatagtacaactattgcccttgaattgtagtgtggcaacattagagctccttaaaaatttaagcaaaaacgcattaacatatttctgtaatataattaaaattatgtgttttatatatatttagtgttgtgtacatatcttgttaatctccacacaactaacaagtatatctaaatcttaaagctaagggtattttttctctggagtaatctcaaacaacttgccaaacttattagaatattctggcttgtggcttctcaagttgaaaggttcaaattcagagggtaagcttttctttgagcttgattttgcaagctttctcaattcctcaatttattcccttgatactttgattattgcgtctctttcttccccttattatgttcttttccgatctctcaattattatggttttttctcttactcttctaaaagaaccttctctatggtctcgtatttagtttatatttgcgaaaaaggatacaaaatataatggttatatttattaaacatttgataaaaaaatcacacattaagcttaacatgtgttgtttgcatacttatatttaaggaggcctctaaaatgttcttgctgaatcctcataagtattggtttttattttcagatagaccaaaagcttgtagaagaaggataaagatcaatttttcaatccagacaaaaataaaagtaatataaaggaggtgttttaataagaataaaacatgtgaagaaaattattatctcaaatttaccaggcctgttcacgggtattacaaaatccaccactcttagatcttcttcatcatcttagttaactagataagatgttgttcctgcgggaattttgatggtatcaccacgctcaagattatacgagtttctatcattgggactcaacactgtcaatatggctttccttgtagtacatattaaccacaccaaaatttaattatgaaatataagaaatattgctaaattgaactttacaatatttttattttaaatagtcatatttctataaaacaaaagatttgttataataatattataaagaaaaataaaaattatcattgaggactacaaggattaagtcagcatctatgtgttaaggaaggaagatggtgtggggtttggctctatattccacaagacgatagttttagagattttcaaataagtctgaacgtttgtcgaacctttaaaggcgacgaatgtgaccgttttcgttttcaaagagtgtcagaaacttgttagacttgaataaaaaggggtttctttattcttatgattctgaagatctttcttcctcctctccttcacgttaatggcgtctgtctctttttgttctctcctctctatgccttagccttgccctttcttcgggatcttcacgacgttaacttcctctttactcttcgtctacttattcctcatcttcctctctttcttatctctcacgtccaggttaaacttccttttattccttcttttcacgttaatatcaatatttctacttctcttcttcatcttcttccttttcatatgaaggtctttattctccatggcgtttttcttctttctcaccctcttagcgacctctttctctttatcccggtaccctagtttctgaaccttcatcgtaattggcataagtgacgcaaacagaggccaggaatataattcccagaaacaataaaagtggaaatcatgatttgacagtggtcgctatgatttgtatttcactagttcgaactttagatgatgaaataaaagattaagttgaaggatatttatagtgatagaacgtaaagctagatgaataacgtggatggtcatttgggtaca

SEQ ID NO: 93 - DNA, 3400 bp, synthetic construct
  source 1..3400: mol_type = other DNA
gacacggtgagagtaacagaagatagtattaatgactaagtagaagaaatatttctgaccattgattggtgacgaaaactacccctataaagtttactcgcagttaaacatcgaaatatccattatttttttgtcatttactttttcattattattatataagtttaaacacttagaatcataaaaattattaaatctatctttaagcacaacaaacaaatctatctatggatagaataatattgtacctgttgactccaaatacacaacaataatatgaaaaatagaataataaattcaaatggttagaatatatttttacttagataccaaagttttaccatctttcttgtctttcttaagaactatctgaatcaattttgacctcaactattagaataagaaactttatccaaatctataaataaaagaaaacatttgaaattgggttaacaatttaggctcaatccttccaagtctcgaagtctcgattattacgcaactcctcttacatttcatcttttcctcatagaacatttacattaaaacaaagagtccaattaatattcagaacttcatattgtaaatctaacattgatataaccgtcatgaaaatatattttctagagagaaaagaaattgcacaacctcgtcttaactcacaaattacaaaacacttccaattttttaatttaaagaaaagatataaaaacataaacaaattaaagcaactaatacaagagtaaggcactgcatgttatgaaccattacaataataacacaaccaataaccattattaaaaacaattttaaaaattccttcattgaatccatagtctttttttaagacttaccccaagaacacaaattaatattatccttgtagttaaagtaaaaaaaaagcacaagttttattaattatttatttattcgtatagaaaagtggggctcaataggtaagagttacaagatccattatttactcttagctcacgaagagctagctagatcttagctcatacatctgcattatttttcatattgattactcagtaaaaactgtccagaactgaagacagaggactcctttttctttagctttcttcctccttttattcaggttcagcacttgcaaagtgagattatttttaattcttgattaatctatttacctcttaagaagatccaggaaatgtgagctcctttactggattttctatttagcttatcacattgtcatccgatctttcaaattttcaatccccaaattagaaatataacattcaaatattaactaatgatatttctattcacttaatatctgaaaggaagtttctctaattgttctcggcattgataccaaatccaaccaaattcagatttgatgaagcactaatggcaactgggtgacctgctggaatgataacaacgtcacccggagacaatctagcttcatatctctacacttcattgtttctttcttttctatcttccctctcttattactcattttttaaacccagaagttcaaggtttccttttccttcattaactaatagtacaactattgcccttgaattgtagtgtggcaacattagagctccttaaaaatttaagcaaaaacgcattaacatatttctgtaatataattaaaattatgtgttttatatatatttagtgttgtgtacatatcttgttaatctccacacaactaacaagtatatctaaatcttaaagctaagggtattttttctctggagtaatctcaaacaacttgccaaacttattagaatattctggcttgtggcttctcaagttgaaaggttcaaattcagagggtaagcttttctttgagcttgattttgcaagctttctcaattcctcaatttattcccttgatactttgattattgcgtctctttcttccccttattatgttcttttccgatctctcaattattatggttttttctcttactcttctaaaagaaccttctctatggtctcgtatttagtttatatttgcgaaaaaggatacaaaatataatggttatatttattaaacatttgataaaaaaatcacacattaagcttaacatgtgttgtttgcatacttatatttaaggaggcctctaaaatgttcttgctgaatcctcataagtattagtttttattttcagatagaccaaaagcctgtagaagaaggataaagatcaatttttcaatccagacaaaaataaaagtaatataaaggaggtgttttaataagaataaaacatgtgaagaaaattattatctcaaatttaccaggcctgttcacgggtattacaaaatccaccactcttagatcttcttcatcatcttagttaactagataagatgttgttcctgcgggaattttgatggtatcaccacgctcaagattatacgagtttctatcattgggactcaacactgtcaatatggctttccttgtagtacatattaaccacaccaaaatttaattatgaaatataagaaatattgctaaattgaactttacaatatttttattttaaatagtcatatttctataaaacaaaagatttgttataataatattataaagaaaaataaaaattatcattgaggactacaaggattaagtcagcatctatgtgttaaggaaggaagatggtgtggggtttggctctatattccacaagacgatagttttagagattttcaaataagtctgaacgtttgtcgaacctttaaaggcgacgaatgtgaccgttttcgttttcaaagagtgtcagaaacttgttagacttgaataaaaaggggtttctttattcttatgattctgaagatctttcttcctcctctccttcacgttaatggcgtctgtctctttttgttctctcctctctatgccttagccttgccctttcttcgggatcttcacgacgttaacttcctctttactcttcgtctacttattcctcatcttcctctctttcttatctctcacgtccaggttaaacttccttttattccttcttttcacgttaatatcaatatttctacttctcttcttcatcttcttccttttcatatgaaggtctttattctccatggcgtttttcttctttctcaccctcttagcgacctctttctctttatcccggtaccctagtttctgaaccttcatcgtaattggcataagtgacgcaaacagaggccaggaatataattcccagaaacaataaaagtggaaatcatgatttgacagtggtcgctatgatttgtatttcactagttcgaactttagatgatgaaataaaagattaagttgaaggatatttatagtgatagaacgtaaagctagatgaataacgtggatggtcatttgggtaca

SEQ ID NO: 94 - DNA, 3400 bp, synthetic construct
  source 1..3400: mol_type = other DNA
gacacggtgagagtaacagaagatagtattaatgactaagtagaagaaatatttctgaccattgattggtgacgaaaactacccctataaagtttactcgcagttaaacatcgaaatatccattatttttttgtcatttactttttcattattattatataagtttaaacacttagaatcataaaaattattaaatctatctttaagcacaacaaacaaatctatctatggatagaataatattgtacctgttgactccaaatacacaacaataatatgaaaaatagaataataaattcaaatggttagaatatatttttacttagataccaaagttttaccatctttcttgtctttcttaagaactatctgaatcaattttgacctcaactattagaataagaaactttatccaaatctataaataaaagaaaacatttgaaattgggttaacaatttaggctcaatccttccaagtctcgaagtctcgattattacgcaactcctcttacatttcatcttttcctcatagaacatttacattaaaacaaagagtccaattaatattcagaacttcatattgtaaatctaacattgatataaccgtcatgaaaatatattttctagagagaaaagaaattgcacaacctcgtcttaactcacaaattacaaaacacttccaattttttaatttaaagaaaagatataaaaacataaacaaattaaagcaactaatacaagagtaaggcactgcatgttatgaaccattacaataataacacaaccaataaccattattaaaaacaattttaaaaattccttcattgaatccatagtctttttttaagacttaccccaagaacacaaattaatattatccttgtagttaaagtaaaaaaaaagcacaagttttattaattatttatttattcgtatagaaaagtggggctcaataggtaagagttacaagatccattatttactcttagctcacgaagagctagctagatcttagctcatacatctgcattatttttcatattgattactcagtaaaaactgtccagaactgaagacagaggactcctttttctttagctttcttcctccttttattcaggttcagcacttgcaaagtgagattatttttaattcttgattaatctatttacctcttaagaagatccaggaaatgtgagctcctttactggattttctatttagcttatcacattgtcatccgatctttcaaattttcaatccccaaattagaaatataacattcaaatattaactaatgatatttctattcacttaatatctgaaaggaagtttctctaattgttctcggcattgataccaaatccaaccaaattcagatttgatgaagcactaatggcaactgggtgacctgctggaatgataacaacgtcacccggagacaatctagcttcatatctctacacttcattgtttctttcttttctatcttccctctcttattactcattttttaaacccagaagttcaaggtttccttttccttcattaactaatagtacaactattgcccttgaattgtagtgtggcaacattagagctccttaaaaatttaagcaaaaacgcattaacatatttctgtaatataattaaaattatgtgttttatatatatttagtgttgtgtacatatcttgttaatctccacacaactaacaagtatatctaaatcttaaagctaagggtattttttctctggagtaatctcaaacaacttgccaaacttattagaatattctggcttgtggcttctcaagttgaaaggttcaaattcagagggtaagcttttctttgagcttgattttgcaagctttctcaattcctcaatttattcccttgatactttgattattgcgtctctttcttccccttattatgttcttttccgatctctcaattattatggttttttctcttactcttctaaaagaaccttctctatggtctcgtatttagtttatatttgcgaaaaaggatacaaaatataatggttatatttattaaacatttgataaaaaaatcacacattaagcttaacatgtgttgtttgcatacttatatttaaggaggcctctaaaatgttcttgctgaatcctcataagtattagtttttattttcagatagaccaaaagcttgtagaagaaggataaagatcaatttttcaatccagacaaaaataaaagtaatataaaggaggtgttttaataagaataaaacatgtgaagaaaattattacctcaaatttaccaggcctgttcacgggtattacaaaatccaccactcttagatcttcttcatcatcttagttaactagataagatgttgttcctgcgggaattttgatggtatcaccacgctcaagattatacgagtttctatcattgggactcaacactgtcaatatggctttccttgtagtacatattaaccacaccaaaatttaattatgaaatataagaaatattgctaaattgaactttacaatatttttattttaaatagtcatatttctataaaacaaaagatttgttataataatattataaagaaaaataaaaattatcattgaggactacaaggattaagtcagcatctatgtgttaaggaaggaagatggtgtggggtttggctctatattccacaagacgatagttttagagattttcaaataagtctgaacgtttgtcgaacctttaaaggcgacgaatgtgaccgttttcgttttcaaagagtgtcagaaacttgttagacttgaataaaaaggggtttctttattcttatgattctgaagatctttcttcctcctctccttcacgttaatggcgtctgtctctttttgttctctcctctctatgccttagccttgccctttcttcgggatcttcacgacgttaacttcctctttactcttcgtctacttattcctcatcttcctctctttcttatctctcacgtccaggttaaacttccttttattccttcttttcacgttaatatcaatatttctacttctcttcttcatcttcttccttttcatatgaaggtctttattctccatggcgtttttcttctttctcaccctcttagcgacctctttctctttatcccggtaccctagtttctgaaccttcatcgtaattggcataagtgacgcaaacagaggccaggaatataattcccagaaacaataaaagtggaaatcatgatttgacagtggtcgctatgatttgtatttcactagttcgaactttagatgatgaaataaaagattaagttgaaggatatttatagtgatagaacgtaaagctagatgaataacgtggatggtcatttgggtaca

SEQ ID NO: 95 - DNA, 3400 bp, synthetic construct
  source 1..3400: mol_type = other DNA
gacacggtgagagtaacagaagatagtattaatgactaagtagaagaaatatttctgaccattgattggtgacgaaaactacccctataaagtttactcgcagttaaacatcgaaatatccattatttttttgtcatttactttttcattattattatataagtttaaacacttagaatcataaaaattattaaatctatctttaagcacaacaaacaaatctatctatggatagaataatattgtacctgttgactccaaatacacaacaataatatgaaaaatagaataataaattcaaatggttagaatatatttttacttagataccaaagttttaccatctttcttgtctttcttaagaactatctgaatcaattttgacctcaactattagaataagaaactttatccaaatctataaataaaagaaaacatttgaaattgggttaacaatttaggctcaatccttccaagtctcgaagtctcgattattacgcaactcctcttacatttcatcttttcctcatagaacatttacattaaaacaaagagtccaattaatattcagaacttcatattgtaaatctaacattgatataaccgtcatgaaaatatattttctagagagaaaagaaattgcacaacctcgtcttaactcacaaattacaaaacacttccaattttttaatttaaagaaaagatataaaaacataaacaaattaaagcaactaatacaagagtaaggcactgcatgttatgaaccattacaataataacacaaccaataaccattattaaaaacaattttaaaaattccttcattgaatccatagtctttttttaagacttaccccaagaacacaaattaatattatccttgtagttaaagtaaaaaaaaagcacaagttttattaattatttatttattcgtatagaaaagtggggctcaataggtaagagttacaagatccattatttactcttagctcacgaagagctagctagatcttagctcatacatctgcattatttttcatattgattactcagtaaaaactgtccagaactgaagacagaggactcctttttctttagctttcttcctccttttattcaggttcagcacttgcaaagtgagattatttttaattcttgattaatctatttacctcttaagaagatccaggaaatgtgagctcctttactggattttctatttagcttatcacattgtcatccgatctttcaaattttcaatccccaaattagaaatataacattcaaatattaactaatgatatttctattcacttaatatctgaaaggaagtttctctaattgttctcggcattgataccaaatccaaccaaattcagatttgatgaagcactaatggcaactgggtgacctgctggaatgataacaacgtcacccggagacaatctagcttcatatctctacacttcattgtttctttcttttctatcttccctctcttattactcattttttaaacccagaagttcaaggtttccttttccttcattaactaatagtacaactattgcccttgaattgtagtgtggcaacattagagctccttaaaaatttaagcaaaaacgcattaacatatttctgtaatataattaaaattatgtgttttatatatatttagtgttgtgtacatatcttgttaatctccacacaactaacaagtatatctaaatcttaaagctaagggtattttttctctggagtaatctcaaacaacttgccaaacttattagaatattctggcttgtggcttctcaagttgaaaggttcaaattcagagggtaagcttttctttgagcttgattttgcaagctttctcaattcctcaatttattcccttgatactttgattattgcgtctctttcttccccttattatgttcttttccgatctctcaattattatggttttttctcttactcttctaaaagaaccttctctatggtctcgtatttagtttatatttgcgaaaaaggatacaaaatataatggttatatttattaaacatttgataaaaaaatcacacattaagcttaacatgtgttgtttgcatacttatatttaaggaggcctctaaaatgttcttgctgaatcctcataagtattagtttttattttcagatagaccaaaagcttgtagaagaaggataaagatcaatttttcaatccagacaaaaataaaagtaatataaaggaggtgttttaataagaataaaacatgtgaagaaaattattatctcaaatttaccaggcctgttcacgggtattacaaaatccaccactcttagatcttcttcatcatcttggttaactagataagatgttgttcctgcgggaattttgatggtatcaccacgctcaagattatacgagtttctatcattgggactcaacactgtcaatatggctttccttgtagtacatattaaccacaccaaaatttaattatgaaatataagaaatattgctaaattgaactttacaatatttttattttaaatagtcatatttctataaaacaaaagatttgttataataatattataaagaaaaataaaaattatcattgaggactacaaggattaagtcagcatctatgtgttaaggaaggaagatggtgtggggtttggctctatattccacaagacgatagttttagagattttcaaataagtctgaacgtttgtcgaacctttaaaggcgacgaatgtgaccgttttcgttttcaaagagtgtcagaaacttgttagacttgaataaaaaggggtttctttattcttatgattctgaagatctttcttcctcctctccttcacgttaatggcgtctgtctctttttgttctctcctctctatgccttagccttgccctttcttcgggatcttcacgacgttaacttcctctttactcttcgtctacttattcctcatcttcctctctttcttatctctcacgtccaggttaaacttccttttattccttcttttcacgttaatatcaatatttctacttctcttcttcatcttcttccttttcatatgaaggtctttattctccatggcgtttttcttctttctcaccctcttagcgacctctttctctttatcccggtaccctagtttctgaaccttcatcgtaattggcataagtgacgcaaacagaggccaggaatataattcccagaaacaataaaagtggaaatcatgatttgacagtggtcgctatgatttgtatttcactagttcgaactttagatgatgaaataaaagattaagttgaaggatatttatagtgatagaacgtaaagctagatgaataacgtggatggtcatttgggtaca

SEQ ID NO: 96 - DNA, 3400 bp, synthetic construct
  source 1..3400: mol_type = other DNA
gacacggtgagagtaacagaagatagtattaatgactaagtagaagaaatatttctgaccattgattggtgacgaaaactacccctataaagtttactcgcagttaaacatcgaaatatccattatttttttgtcatttactttttcattattattatataagtttaaacacttagaatcataaaaattattaaatctatctttaagcacaacaaacaaatctatctatggatagaataatattgtacctgttgactccaaatacacaacaataatatgaaaaatagaataataaattcaaatggttagaatatatttttacttagataccaaagttttaccatctttcttgtctttcttaagaactatctgaatcaattttgacctcaactattagaataagaaactttatccaaatctataaataaaagaaaacatttgaaattgggttaacaatttaggctcaatccttccaagtctcgaagtctcgattattacgcaactcctcttacatttcatcttttcctcatagaacatttacattaaaacaaagagtccaattaatattcagaacttcatattgtaaatctaacattgatataaccgtcatgaaaatatattttctagagagaaaagaaattgcacaacctcgtcttaactcacaaattacaaaacacttccaattttttaatttaaagaaaagatataaaaacataaacaaattaaagcaactaatacaagagtaaggcactgcatgttatgaaccattacaataataacacaaccaataaccattattaaaaacaattttaaaaattccttcattgaatccatagtctttttttaagacttaccccaagaacacaaattaatattatccttgtagttaaagtaaaaaaaaagcacaagttttattaattatttatttattcgtatagaaaagtggggctcaataggtaagagttacaagatccattatttactcttagctcacgaagagctagctagatcttagctcatacatctgcattatttttcatattgattactcagtaaaaactgtccagaactgaagacagaggactcctttttctttagctttcttcctccttttattcaggttcagcacttgcaaagtgagattatttttaattcttgattaatctatttacctcttaagaagatccaggaaatgtgagctcctttactggattttctatttagcttatcacattgtcatccgatctttcaaattttcaatccccaaattagaaatataacattcaaatattaactaatgatatttctattcacttaatatctgaaaggaagtttctctaattgttctcggcattgataccaaatccaaccaaattcagatttgatgaagcactaatggcaactgggtgacctgctggaatgataacaacgtcacccggagacaatctagcttcatatctctacacttcattgtttctttcttttctatcttccctctcttattactcattttttaaacccagaagttcaaggtttccttttccttcattaactaatagtacaactattgcccttgaattgtagtgtggcaacattagagctccttaaaaatttaagcaaaaacgcattaacatatttctgtaatataattaaaattatgtgttttatatatatttagtgttgtgtacatatcttgttaatctccacacaactaacaagtatatctaaatcttaaagctaagggtattttttctctggagtaatctcaaacaacttgccaaacttattagaatattctggcttgtggcttctcaagttgaaaggttcaaattcagagggtaagcttttctttgagcttgattttgcaagctttctcaattcctcaatttattcccttgatactttgattattgcgtctctttcttccccttattatgttcttttccgatctctcaattattatggttttttctcttactcttctaaaagaaccttctctatggtctcgtatttagtttatatttgcgaaaaaggatacaaaatataatggttatatttattaaacatttgataaaaaaatcacacattaagcttaacatgtgttgtttgcatacttatatttaaggaggcctctaaaatgttcttgctgaatcctcataagtattagtttttattttcagatagaccaaaagcttgtagaagaaggataaagatcaatttttcaatccagacaaaaataaaagtaatataaaggaggtgttttaataagaataaaacatgtgaagaaaattattatctcaaatttaccaggcctgttcacgggtattacaaaatccaccactcttagatcttcttcatcatcttagttaactagataagatgttgttcctgcgggaattttgatggtatcaccacgctcaagattatacgagtttctatcattgggactcaacactgtcaatatggctttccctgtagtacatattaaccacaccaaaatttaattatgaaatataagaaatattgctaaattgaactttacaatatttttattttaaatagtcatatttctataaaacaaaagatttgttataataatattataaagaaaaataaaaattatcattgaggactacaaggattaagtcagcatctatgtgttaaggaaggaagatggtgtggggtttggctctatattccacaagacgatagttttagagattttcaaataagtctgaacgtttgtcgaacctttaaaggcgacgaatgtgaccgttttcgttttcaaagagtgtcagaaacttgttagacttgaataaaaaggggtttctttattcttatgattctgaagatctttcttcctcctctccttcacgttaatggcgtctgtctctttttgttctctcctctctatgccttagccttgccctttcttcgggatcttcacgacgttaacttcctctttactcttcgtctacttattcctcatcttcctctctttcttatctctcacgtccaggttaaacttccttttattccttcttttcacgttaatatcaatatttctacttctcttcttcatcttcttccttttcatatgaaggtctttattctccatggcgtttttcttctttctcaccctcttagcgacctctttctctttatcccggtaccctagtttctgaaccttcatcgtaattggcataagtgacgcaaacagaggccaggaatataattcccagaaacaataaaagtggaaatcatgatttgacagtggtcgctatgatttgtatttcactagttcgaactttagatgatgaaataaaagattaagttgaaggatatttatagtgatagaacgtaaagctagatgaataacgtggatggtcatttgggtaca

SEQ ID NO: 97 - DNA, 3400 bp, synthetic construct
  source 1..3400: mol_type = other DNA
gacacggtgagagtaacagaagatagtattaatgactaagtagaagaaatatttctgaccattgattggtgacgaaaactacccctataaagtttactcgcagttaaacatcgaaatatccattatttttttgtcatttactttttcattattattatataagtttaaacacttagaatcataaaaattattaaatctatctttaagcacaacaaacaaatctatctatggatagaataatattgtacctgttgactccaaatacacaacaataatatgaaaaatagaataataaattcaaatggttagaatatatttttacttagataccaaagttttaccatctttcttgtctttcttaagaactatctgaatcaattttgacctcaactattagaataagaaactttatccaaatctataaataaaagaaaacatttgaaattgggttaacaatttaggctcaatccttccaagtctcgaagtctcgattattacgcaactcctcttacatttcatcttttcctcatagaacatttacattaaaacaaagagtccaattaatattcagaacttcatattgtaaatctaacattgatataaccgtcatgaaaatatattttctagagagaaaagaaattgcacaacctcgtcttaactcacaaattacaaaacacttccaattttttaatttaaagaaaagatataaaaacataaacaaattaaagcaactaatacaagagtaaggcactgcatgttatgaaccattacaataataacacaaccaataaccattattaaaaacaattttaaaaattccttcattgaatccatagtctttttttaagacttaccccaagaacacaaattaatattatccttgtagttaaagtaaaaaaaaagcacaagttttattaattatttatttattcgtatagaaaagtggggctcaataggtaagagttacaagatccattatttactcttagctcacgaagagctagctagatcttagctcatacatctgcattatttttcatattgattactcagtaaaaactgtccagaactgaagacagaggactcctttttctttagctttcttcctccttttattcaggttcagcacttgcaaagtgagattatttttaattcttgattaatctatttacctcttaagaagatccaggaaatgtgagctcctttactggattttctatttagcttatcacattgtcatccgatctttcaaattttcaatccccaaattagaaatataacattcaaatattaactaatgatatttctattcacttaatatctgaaaggaagtttctctaattgttctcggcattgataccaaatccaaccaaattcagatttgatgaagcactaatggcaactgggtgacctgctggaatgataacaacgtcacccggagacaatctagcttcatatctctacacttcattgtttctttcttttctatcttccctctcttattactcattttttaaacccagaagttcaaggtttccttttccttcattaactaatagtacaactattgcccttgaattgtagtgtggcaacattagagctccttaaaaatttaagcaaaaacgcattaacatatttctgtaatataattaaaattatgtgttttatatatatttagtgttgtgtacatatcttgttaatctccacacaactaacaagtatatctaaatcttaaagctaagggtattttttctctggagtaatctcaaacaacttgccaaacttattagaatattctggcttgtggcttctcaagttgaaaggttcaaattcagagggtaagcttttctttgagcttgattttgcaagctttctcaattcctcaatttattcccttgatactttgattattgcgtctctttcttccccttattatgttcttttccgatctctcaattattatggttttttctcttactcttctaaaagaaccttctctatggtctcgtatttagtttatatttgcgaaaaaggatacaaaatataatggttatatttattaaacatttgataaaaaaatcacacattaagcttaacatgtgttgtttgcatacttatatttaaggaggcctctaaaatgttcttgctgaatcctcataagtattagtttttattttcagatagaccaaaagcttgtagaagaaggataaagatcaatttttcaatccagacaaaaataaaagtaatataaaggaggtgttttaataagaataaaacatgtgaagaaaattattatctcaaatttaccaggcctgttcacgggtattacaaaatccaccactcttagatcttcttcatcatcttagttaactagataagatgttgttcctgcgggaattttgatggtatcaccacgctcaagattatacgagtttctatcattgggactcaacactgtcaatatggctttccttgtagtacatattaaccacaccaaaatttaattatgaaatataagaaatattgctaaattgaactttacaatatttttattttaaatagtcatatttctataaaacaaaagatttgttataataatattataaagaaaaataaaaattaccattgaggactacaaggattaagtcagcatctatgtgttaaggaaggaagatggtgtggggtttggctctatattccacaagacgatagttttagagattttcaaataagtctgaacgtttgtcgaacctttaaaggcgacgaatgtgaccgttttcgttttcaaagagtgtcagaaacttgttagacttgaataaaaaggggtttctttattcttatgattctgaagatctttcttcctcctctccttcacgttaatggcgtctgtctctttttgttctctcctctctatgccttagccttgccctttcttcgggatcttcacgacgttaacttcctctttactcttcgtctacttattcctcatcttcctctctttcttatctctcacgtccaggttaaacttccttttattccttcttttcacgttaatatcaatatttctacttctcttcttcatcttcttccttttcatatgaaggtctttattctccatggcgtttttcttctttctcaccctcttagcgacctctttctctttatcccggtaccctagtttctgaaccttcatcgtaattggcataagtgacgcaaacagaggccaggaatataattcccagaaacaataaaagtggaaatcatgatttgacagtggtcgctatgatttgtatttcactagttcgaactttagatgatgaaataaaagattaagttgaaggatatttatagtgatagaacgtaaagctagatgaataacgtggatggtcatttgggtaca

SEQ ID NO: 98 - DNA, 3400 bp, synthetic construct
  source 1..3400: mol_type = other DNA
gacacggtgagagtaacagaagatagtattaatgactaagtagaagaaatatttctgaccattgattggtgacgaaaactacccctataaagtttactcgcagttaaacatcgaaatatccattatttttttgtcatttactttttcattattattatataagtttaaacacttagaatcataaaaattattaaatctatctttaagcacaacaaacaaatctatctatggatagaataatattgtacctgttgactccaaatacacaacaataatatgaaaaatagaataataaattcaaatggttagaatatatttttacttagataccaaagttttaccatctttcttgtctttcttaagaactatctgaatcaattttgacctcaactattagaataagaaactttatccaaatctataaataaaagaaaacatttgaaattgggttaacaatttaggctcaatccttccaagtctcgaagtctcgattattacgcaactcctcttacatttcatcttttcctcatagaacatttacattaaaacaaagagtccaattaatattcagaacttcatattgtaaatctaacattgatataaccgtcatgaaaatatattttctagagagaaaagaaattgcacaacctcgtcttaactcacaaattacaaaacacttccaattttttaatttaaagaaaagatataaaaacataaacaaattaaagcaactaatacaagagtaaggcactgcatgttatgaaccattacaataataacacaaccaataaccattattaaaaacaattttaaaaattccttcattgaatccatagtctttttttaagacttaccccaagaacacaaattaatattatccttgtagttaaagtaaaaaaaaagcacaagttttattaattatttatttattcgtatagaaaagtggggctcaataggtaagagttacaagatccattatttactcttagctcacgaagagctagctagatcttagctcatacatctgcattatttttcatattgattactcagtaaaaactgtccagaactgaagacagaggactcctttttctttagctttcttcctccttttattcaggttcagcacttgcaaagtgagattatttttaattcttgattaatctatttacctcttaagaagatccaggaaatgtgagctcctttactggattttctatttagcttatcacattgtcatccgatctttcaaattttcaatccccaaattagaaatataacattcaaatattaactaatgatatttctattcacttaatatctgaaaggaagtttctctaattgttctcggcattgataccaaatccaaccaaattcagatttgatgaagcactaatggcaactgggtgacctgctggaatgataacaacgtcacccggagacaatctagcttcatatctctacacttcattgtttctttcttttctatcttccctctcttattactcattttttaaacccagaagttcaaggtttccttttccttcattaactaatagtacaactattgcccttgaattgtagtgtggcaacattagagctccttaaaaatttaagcaaaaacgcattaacatatttctgtaatataattaaaattatgtgttttatatatatttagtgttgtgtacatatcttgttaatctccacacaactaacaagtatatctaaatcttaaagctaagggtattttttctctggagtaatctcaaacaacttgccaaacttattagaatattctggcttgtggcttctcaagttgaaaggttcaaattcagagggtaagcttttctttgagcttgattttgcaagctttctcaattcctcaatttattcccttgatactttgattattgcgtctctttcttccccttattatgttcttttccgatctctcaattattatggttttttctcttactcttctaaaagaaccttctctatggtctcgtatttagtttatatttgcgaaaaaggatacaaaatataatggttatatttattaaacatttgataaaaaaatcacacattaagcttaacatgtgttgtttgcatacttatatttaaggaggcctctaaaatgttcttgctgaatcctcataagtattagtttttattttcagatagaccaaaagcttgtagaagaaggataaagatcaatttttcaatccagacaaaaataaaagtaatataaaggaggtgttttaataagaataaaacatgtgaagaaaattattatctcaaatttaccaggcctgttcacgggtattacaaaatccaccactcttagatcttcttcatcatcttagttaactagataagatgttgttcctgcgggaattttgatggtatcaccacgctcaagattatacgagtttctatcattgggactcaacactgtcaatatggctttccttgtagtacatattaaccacaccaaaatttaattatgaaatataagaaatattgctaaattgaactttacaatatttttattttaaatagtcatatttctataaaacaaaagatttgttataataatattataaagaaaaataaaaattatcattgaggactacaaggattaagtcagcatctatgtgtttaggaaggaagatggtgtggggtttggctctatattccacaagacgatagttttagagattttcaaataagtctgaacgtttgtcgaacctttaaaggcgacgaatgtgaccgttttcgttttcaaagagtgtcagaaacttgttagacttgaataaaaaggggtttctttattcttatgattctgaagatctttcttcctcctctccttcacgttaatggcgtctgtctctttttgttctctcctctctatgccttagccttgccctttcttcgggatcttcacgacgttaacttcctctttactcttcgtctacttattcctcatcttcctctctttcttatctctcacgtccaggttaaacttccttttattccttcttttcacgttaatatcaatatttctacttctcttcttcatcttcttccttttcatatgaaggtctttattctccatggcgtttttcttctttctcaccctcttagcgacctctttctctttatcccggtaccctagtttctgaaccttcatcgtaattggcataagtgacgcaaacagaggccaggaatataattcccagaaacaataaaagtggaaatcatgatttgacagtggtcgctatgatttgtatttcactagttcgaactttagatgatgaaataaaagattaagttgaaggatatttatagtgatagaacgtaaagctagatgaataacgtggatggtcatttgggtaca

SEQ ID NO: 99 - DNA, 3400 bp, synthetic construct
  source 1..3400: mol_type = other DNA
gacacggtgagagtaacagaagatagtattaatgactaagtagaagaaatatttctgaccattgattggtgacgaaaactacccctataaagtttactcgcagttaaacatcgaaatatccattatttttttgtcatttactttttcattattattatataagtttaaacacttagaatcataaaaattattaaatctatctttaagcacaacaaacaaatctatctatggatagaataatattgtacctgttgactccaaatacacaacaataatatgaaaaatagaataataaattcaaatggttagaatatatttttacttagataccaaagttttaccatctttcttgtctttcttaagaactatctgaatcaattttgacctcaactattagaataagaaactttatccaaatctataaataaaagaaaacatttgaaattgggttaacaatttaggctcaatccttccaagtctcgaagtctcgattattacgcaactcctcttacatttcatcttttcctcatagaacatttacattaaaacaaagagtccaattaatattcagaacttcatattgtaaatctaacattgatataaccgtcatgaaaatatattttctagagagaaaagaaattgcacaacctcgtcttaactcacaaattacaaaacacttccaattttttaatttaaagaaaagatataaaaacataaacaaattaaagcaactaatacaagagtaaggcactgcatgttatgaaccattacaataataacacaaccaataaccattattaaaaacaattttaaaaattccttcattgaatccatagtctttttttaagacttaccccaagaacacaaattaatattatccttgtagttaaagtaaaaaaaaagcacaagttttattaattatttatttattcgtatagaaaagtggggctcaataggtaagagttacaagatccattatttactcttagctcacgaagagctagctagatcttagctcatacatctgcattatttttcatattgattactcagtaaaaactgtccagaactgaagacagaggactcctttttctttagctttcttcctccttttattcaggttcagcacttgcaaagtgagattatttttaattcttgattaatctatttacctcttaagaagatccaggaaatgtgagctcctttactggattttctatttagcttatcacattgtcatccgatctttcaaattttcaatccccaaattagaaatataacattcaaatattaactaatgatatttctattcacttaatatctgaaaggaagtttctctaattgttctcggcattgataccaaatccaaccaaattcagatttgatgaagcactaatggcaactgggtgacctgctggaatgataacaacgtcacccggagacaatctagcttcatatctctacacttcattgtttctttcttttctatcttccctctcttattactcattttttaaacccagaagttcaaggtttccttttccttcattaactaatagtacaactattgcccttgaattgtagtgtggcaacattagagctccttaaaaatttaagcaaaaacgcattaacatatttctgtaatataattaaaattatgtgttttatatatatttagtgttgtgtacatatcttgttaatctccacacaactaacaagtatatctaaatcttaaagctaagggtattttttctctggagtaatctcaaacaacttgccaaacttattagaatattctggcttgtggcttctcaagttgaaaggttcaaattcagagggtaagcttttctttgagcttgattttgcaagctttctcaattcctcaatttattcccttgatactttgattattgcgtctctttcttccccttattatgttcttttccgatctctcaattattatggttttttctcttactcttctaaaagaaccttctctatggtctcgtatttagtttatatttgcgaaaaaggatacaaaatataatggttatatttattaaacatttgataaaaaaatcacacattaagcttaacatgtgttgtttgcatacttatatttaaggaggcctctaaaatgttcttgctgaatcctcataagtattagtttttattttcagatagaccaaaagcttgtagaagaaggataaagatcaatttttcaatccagacaaaaataaaagtaatataaaggaggtgttttaataagaataaaacatgtgaagaaaattattatctcaaatttaccaggcctgttcacgggtattacaaaatccaccactcttagatcttcttcatcatcttagttaactagataagatgttgttcctgcgggaattttgatggtatcaccacgctcaagattatacgagtttctatcattgggactcaacactgtcaatatggctttccttgtagtacatattaaccacaccaaaatttaattatgaaatataagaaatattgctaaattgaactttacaatatttttattttaaatagtcatatttctataaaacaaaagatttgttataataatattataaagaaaaataaaaattatcattgaggactacaaggattaagtcagcatctatgtgttaaggaaggaagatggtgtggggtttggctctatattccacaagacgatagttttggagattttcaaataagtctgaacgtttgtcgaacctttaaaggcgacgaatgtgaccgttttcgttttcaaagagtgtcagaaacttgttagacttgaataaaaaggggtttctttattcttatgattctgaagatctttcttcctcctctccttcacgttaatggcgtctgtctctttttgttctctcctctctatgccttagccttgccctttcttcgggatcttcacgacgttaacttcctctttactcttcgtctacttattcctcatcttcctctctttcttatctctcacgtccaggttaaacttccttttattccttcttttcacgttaatatcaatatttctacttctcttcttcatcttcttccttttcatatgaaggtctttattctccatggcgtttttcttctttctcaccctcttagcgacctctttctctttatcccggtaccctagtttctgaaccttcatcgtaattggcataagtgacgcaaacagaggccaggaatataattcccagaaacaataaaagtggaaatcatgatttgacagtggtcgctatgatttgtatttcactagttcgaactttagatgatgaaataaaagattaagttgaaggatatttatagtgatagaacgtaaagctagatgaataacgtggatggtcatttgggtaca

SEQ ID NO: 100 - DNA, 3400 bp, synthetic construct
  source 1..3400: mol_type = other DNA
gacacggtgagagtaacagaagatagtattaatgactaagtagaagaaatatttctgaccattgattggtgacgaaaactacccctataaagtttactcgcagttaaacatcgaaatatccattatttttttgtcatttactttttcattattattatataagtttaaacacttagaatcataaaaattattaaatctatctttaagcacaacaaacaaatctatctatggatagaataatattgtacctgttgactccaaatacacaacaataatatgaaaaatagaataataaattcaaatggttagaatatatttttacttagataccaaagttttaccatctttcttgtctttcttaagaactatctgaatcaattttgacctcaactattagaataagaaactttatccaaatctataaataaaagaaaacatttgaaattgggttaacaatttaggctcaatccttccaagtctcgaagtctcgattattacgcaactcctcttacatttcatcttttcctcatagaacatttacattaaaacaaagagtccaattaatattcagaacttcatattgtaaatctaacattgatataaccgtcatgaaaatatattttctagagagaaaagaaattgcacaacctcgtcttaactcacaaattacaaaacacttccaattttttaatttaaagaaaagatataaaaacataaacaaattaaagcaactaatacaagagtaaggcactgcatgttatgaaccattacaataataacacaaccaataaccattattaaaaacaattttaaaaattccttcattgaatccatagtctttttttaagacttaccccaagaacacaaattaatattatccttgtagttaaagtaaaaaaaaagcacaagttttattaattatttatttattcgtatagaaaagtggggctcaataggtaagagttacaagatccattatttactcttagctcacgaagagctagctagatcttagctcatacatctgcattatttttcatattgattactcagtaaaaactgtccagaactgaagacagaggactcctttttctttagctttcttcctccttttattcaggttcagcacttgcaaagtgagattatttttaattcttgattaatctatttacctcttaagaagatccaggaaatgtgagctcctttactggattttctatttagcttatcacattgtcatccgatctttcaaattttcaatccccaaattagaaatataacattcaaatattaactaatgatatttctattcacttaatatctgaaaggaagtttctctaattgttctcggcattgataccaaatccaaccaaattcagatttgatgaagcactaatggcaactgggtgacctgctggaatgataacaacgtcacccggagacaatctagcttcatatctctacacttcattgtttctttcttttctatcttccctctcttattactcattttttaaacccagaagttcaaggtttccttttccttcattaactaatagtacaactattgcccttgaattgtagtgtggcaacattagagctccttaaaaatttaagcaaaaacgcattaacatatttctgtaatataattaaaattatgtgttttatatatatttagtgttgtgtacatatcttgttaatctccacacaactaacaagtatatctaaatcttaaagctaagggtattttttctctggagtaatctcaaacaacttgccaaacttattagaatattctggcttgtggcttctcaagttgaaaggttcaaattcagagggtaagcttttctttgagcttgattttgcaagctttctcaattcctcaatttattcccttgatactttgattattgcgtctctttcttccccttattatgttcttttccgatctctcaattattatggttttttctcttactcttctaaaagaaccttctctatggtctcgtatttagtttatatttgcgaaaaaggatacaaaatataatggttatatttattaaacatttgataaaaaaatcacacattaagcttaacatgtgttgtttgcatacttatatttaaggaggcctctaaaatgttcttgctgaatcctcataagtattagtttttattttcagatagaccaaaagcttgtagaagaaggataaagatcaatttttcaatccagacaaaaataaaagtaatataaaggaggtgttttaataagaataaaacatgtgaagaaaattattatctcaaatttaccaggcctgttcacgggtattacaaaatccaccactcttagatcttcttcatcatcttagttaactagataagatgttgttcctgcgggaattttgatggtatcaccacgctcaagattatacgagtttctatcattgggactcaacactgtcaatatggctttccttgtagtacatattaaccacaccaaaatttaattatgaaatataagaaatattgctaaattgaactttacaatatttttattttaaatagtcatatttctataaaacaaaagatttgttataataatattataaagaaaaataaaaattatcattgaggactacaaggattaagtcagcatctatgtgttaaggaaggaagatggtgtggggtttggctctatattccacaagacgatagttttagagattttcaaataagtctgaacgtttgtcgaacctttgaaggcgacgaatgtgaccgttttcgttttcaaagagtgtcagaaacttgttagacttgaataaaaaggggtttctttattcttatgattctgaagatctttcttcctcctctccttcacgttaatggcgtctgtctctttttgttctctcctctctatgccttagccttgccctttcttcgggatcttcacgacgttaacttcctctttactcttcgtctacttattcctcatcttcctctctttcttatctctcacgtccaggttaaacttccttttattccttcttttcacgttaatatcaatatttctacttctcttcttcatcttcttccttttcatatgaaggtctttattctccatggcgtttttcttctttctcaccctcttagcgacctctttctctttatcccggtaccctagtttctgaaccttcatcgtaattggcataagtgacgcaaacagaggccaggaatataattcccagaaacaataaaagtggaaatcatgatttgacagtggtcgctatgatttgtatttcactagttcgaactttagatgatgaaataaaagattaagttgaaggatatttatagtgatagaacgtaaagctagatgaataacgtggatggtcatttgggtaca

SEQ ID NO: 101 - DNA, 3400 bp, synthetic construct
  source 1..3400: mol_type = other DNA
gacacggtgagagtaacagaagatagtattaatgactaagtagaagaaatatttctgaccattgattggtgacgaaaactacccctataaagtttactcgcagttaaacatcgaaatatccattatttttttgtcatttactttttcattattattatataagtttaaacacttagaatcataaaaattattaaatctatctttaagcacaacaaacaaatctatctatggatagaataatattgtacctgttgactccaaatacacaacaataatatgaaaaatagaataataaattcaaatggttagaatatatttttacttagataccaaagttttaccatctttcttgtctttcttaagaactatctgaatcaattttgacctcaactattagaataagaaactttatccaaatctataaataaaagaaaacatttgaaattgggttaacaatttaggctcaatccttccaagtctcgaagtctcgattattacgcaactcctcttacatttcatcttttcctcatagaacatttacattaaaacaaagagtccaattaatattcagaacttcatattgtaaatctaacattgatataaccgtcatgaaaatatattttctagagagaaaagaaattgcacaacctcgtcttaactcacaaattacaaaacacttccaattttttaatttaaagaaaagatataaaaacataaacaaattaaagcaactaatacaagagtaaggcactgcatgttatgaaccattacaataataacacaaccaataaccattattaaaaacaattttaaaaattccttcattgaatccatagtctttttttaagacttaccccaagaacacaaattaatattatccttgtagttaaagtaaaaaaaaagcacaagttttattaattatttatttattcgtatagaaaagtggggctcaataggtaagagttacaagatccattatttactcttagctcacgaagagctagctagatcttagctcatacatctgcattatttttcatattgattactcagtaaaaactgtccagaactgaagacagaggactcctttttctttagctttcttcctccttttattcaggttcagcacttgcaaagtgagattatttttaattcttgattaatctatttacctcttaagaagatccaggaaatgtgagctcctttactggattttctatttagcttatcacattgtcatccgatctttcaaattttcaatccccaaattagaaatataacattcaaatattaactaatgatatttctattcacttaatatctgaaaggaagtttctctaattgttctcggcattgataccaaatccaaccaaattcagatttgatgaagcactaatggcaactgggtgacctgctggaatgataacaacgtcacccggagacaatctagcttcatatctctacacttcattgtttctttcttttctatcttccctctcttattactcattttttaaacccagaagttcaaggtttccttttccttcattaactaatagtacaactattgcccttgaattgtagtgtggcaacattagagctccttaaaaatttaagcaaaaacgcattaacatatttctgtaatataattaaaattatgtgttttatatatatttagtgttgtgtacatatcttgttaatctccacacaactaacaagtatatctaaatcttaaagctaagggtattttttctctggagtaatctcaaacaacttgccaaacttattagaatattctggcttgtggcttctcaagttgaaaggttcaaattcagagggtaagcttttctttgagcttgattttgcaagctttctcaattcctcaatttattcccttgatactttgattattgcgtctctttcttccccttattatgttcttttccgatctctcaattattatggttttttctcttactcttctaaaagaaccttctctatggtctcgtatttagtttatatttgcgaaaaaggatacaaaatataatggttatatttattaaacatttgataaaaaaatcacacattaagcttaacatgtgttgtttgcatacttatatttaaggaggcctctaaaatgttcttgctgaatcctcataagtattagtttttattttcagatagaccaaaagcttgtagaagaaggataaagatcaatttttcaatccagacaaaaataaaagtaatataaaggaggtgttttaataagaataaaacatgtgaagaaaattattatctcaaatttaccaggcctgttcacgggtattacaaaatccaccactcttagatcttcttcatcatcttagttaactagataagatgttgttcctgcgggaattttgatggtatcaccacgctcaagattatacgagtttctatcattgggactcaacactgtcaatatggctttccttgtagtacatattaaccacaccaaaatttaattatgaaatataagaaatattgctaaattgaactttacaatatttttattttaaatagtcatatttctataaaacaaaagatttgttataataatattataaagaaaaataaaaattatcattgaggactacaaggattaagtcagcatctatgtgttaaggaaggaagatggtgtggggtttggctctatattccacaagacgatagttttagagattttcaaataagtctgaacgtttgtcgaacctttaaaggcgacgaatgtgaccgttttcgttttcaaagagtgtcagaaacttgttagacttgaataaaaaggggtttctttgttcttatgattctgaagatctttcttcctcctctccttcacgttaatggcgtctgtctctttttgttctctcctctctatgccttagccttgccctttcttcgggatcttcacgacgttaacttcctctttactcttcgtctacttattcctcatcttcctctctttcttatctctcacgtccaggttaaacttccttttattccttcttttcacgttaatatcaatatttctacttctcttcttcatcttcttccttttcatatgaaggtctttattctccatggcgtttttcttctttctcaccctcttagcgacctctttctctttatcccggtaccctagtttctgaaccttcatcgtaattggcataagtgacgcaaacagaggccaggaatataattcccagaaacaataaaagtggaaatcatgatttgacagtggtcgctatgatttgtatttcactagttcgaactttagatgatgaaataaaagattaagttgaaggatatttatagtgatagaacgtaaagctagatgaataacgtggatggtcatttgggtaca

SEQ ID NO: 102 - DNA, 3400 bp, synthetic construct
  source 1..3400: mol_type = other DNA
gacacggtgagagtaacagaagatagtattaatgactaagtagaagaaatatttctgaccattgattggtgacgaaaactacccctataaagtttactcgcagttaaacatcgaaatatccattatttttttgtcatttactttttcattattattatataagtttaaacacttagaatcataaaaattattaaatctatctttaagcacaacaaacaaatctatctatggatagaataatattgtacctgttgactccaaatacacaacaataatatgaaaaatagaataataaattcaaatggttagaatatatttttacttagataccaaagttttaccatctttcttgtctttcttaagaactatctgaatcaattttgacctcaactattagaataagaaactttatccaaatctataaataaaagaaaacatttgaaattgggttaacaatttaggctcaatccttccaagtctcgaagtctcgattattacgcaactcctcttacatttcatcttttcctcatagaacatttacattaaaacaaagagtccaattaatattcagaacttcatattgtaaatctaacattgatataaccgtcatgaaaatatattttctagagagaaaagaaattgcacaacctcgtcttaactcacaaattacaaaacacttccaattttttaatttaaagaaaagatataaaaacataaacaaattaaagcaactaatacaagagtaaggcactgcatgttatgaaccattacaataataacacaaccaataaccattattaaaaacaattttaaaaattccttcattgaatccatagtctttttttaagacttaccccaagaacacaaattaatattatccttgtagttaaagtaaaaaaaaagcacaagttttattaattatttatttattcgtatagaaaagtggggctcaataggtaagagttacaagatccattatttactcttagctcacgaagagctagctagatcttagctcatacatctgcattatttttcatattgattactcagtaaaaactgtccagaactgaagacagaggactcctttttctttagctttcttcctccttttattcaggttcagcacttgcaaagtgagattatttttaattcttgattaatctatttacctcttaagaagatccaggaaatgtgagctcctttactggattttctatttagcttatcacattgtcatccgatctttcaaattttcaatccccaaattagaaatataacattcaaatattaactaatgatatttctattcacttaatatctgaaaggaagtttctctaattgttctcggcattgataccaaatccaaccaaattcagatttgatgaagcactaatggcaactgggtgacctgctggaatgataacaacgtcacccggagacaatctagcttcatatctctacacttcattgtttctttcttttctatcttccctctcttattactcattttttaaacccagaagttcaaggtttccttttccttcattaactaatagtacaactattgcccttgaattgtagtgtggcaacattagagctccttaaaaatttaagcaaaaacgcattaacatatttctgtaatataattaaaattatgtgttttatatatatttagtgttgtgtacatatcttgttaatctccacacaactaacaagtatatctaaatcttaaagctaagggtattttttctctggagtaatctcaaacaacttgccaaacttattagaatattctggcttgtggcttctcaagttgaaaggttcaaattcagagggtaagcttttctttgagcttgattttgcaagctttctcaattcctcaatttattcccttgatactttgattattgcgtctctttcttccccttattatgttcttttccgatctctcaattattatggttttttctcttactcttctaaaagaaccttctctatggtctcgtatttagtttatatttgcgaaaaaggatacaaaatataatggttatatttattaaacatttgataaaaaaatcacacattaagcttaacatgtgttgtttgcatacttatatttaaggaggcctctaaaatgttcttgctgaatcctcataagtattagtttttattttcagatagaccaaaagcttgtagaagaaggataaagatcaatttttcaatccagacaaaaataaaagtaatataaaggaggtgttttaataagaataaaacatgtgaagaaaattattatctcaaatttaccaggcctgttcacgggtattacaaaatccaccactcttagatcttcttcatcatcttagttaactagataagatgttgttcctgcgggaattttgatggtatcaccacgctcaagattatacgagtttctatcattgggactcaacactgtcaatatggctttccttgtagtacatattaaccacaccaaaatttaattatgaaatataagaaatattgctaaattgaactttacaatatttttattttaaatagtcatatttctataaaacaaaagatttgttataataatattataaagaaaaataaaaattatcattgaggactacaaggattaagtcagcatctatgtgttaaggaaggaagatggtgtggggtttggctctatattccacaagacgatagttttagagattttcaaataagtctgaacgtttgtcgaacctttaaaggcgacgaatgtgaccgttttcgttttcaaagagtgtcagaaacttgttagacttgaataaaaaggggtttctttattcttgtgattctgaagatctttcttcctcctctccttcacgttaatggcgtctgtctctttttgttctctcctctctatgccttagccttgccctttcttcgggatcttcacgacgttaacttcctctttactcttcgtctacttattcctcatcttcctctctttcttatctctcacgtccaggttaaacttccttttattccttcttttcacgttaatatcaatatttctacttctcttcttcatcttcttccttttcatatgaaggtctttattctccatggcgtttttcttctttctcaccctcttagcgacctctttctctttatcccggtaccctagtttctgaaccttcatcgtaattggcataagtgacgcaaacagaggccaggaatataattcccagaaacaataaaagtggaaatcatgatttgacagtggtcgctatgatttgtatttcactagttcgaactttagatgatgaaataaaagattaagttgaaggatatttatagtgatagaacgtaaagctagatgaataacgtggatggtcatttgggtaca

SEQ ID NO: 103 - DNA, 3400 bp, synthetic construct
  source 1..3400: mol_type = other DNA
gacacggtgagagtaacagaagatagtattaatgactaagtagaagaaatatttctgaccattgattggtgacgaaaactacccctataaagtttactcgcagttaaacatcgaaatatccattatttttttgtcatttactttttcattattattatataagtttaaacacttagaatcataaaaattattaaatctatctttaagcacaacaaacaaatctatctatggatagaataatattgtacctgttgactccaaatacacaacaataatatgaaaaatagaataataaattcaaatggttagaatatatttttacttagataccaaagttttaccatctttcttgtctttcttaagaactatctgaatcaattttgacctcaactattagaataagaaactttatccaaatctataaataaaagaaaacatttgaaattgggttaacaatttaggctcaatccttccaagtctcgaagtctcgattattacgcaactcctcttacatttcatcttttcctcatagaacatttacattaaaacaaagagtccaattaatattcagaacttcatattgtaaatctaacattgatataaccgtcatgaaaatatattttctagagagaaaagaaattgcacaacctcgtcttaactcacaaattacaaaacacttccaattttttaatttaaagaaaagatataaaaacataaacaaattaaagcaactaatacaagagtaaggcactgcatgttatgaaccattacaataataacacaaccaataaccattattaaaaacaattttaaaaattccttcattgaatccatagtctttttttaagacttaccccaagaacacaaattaatattatccttgtagttaaagtaaaaaaaaagcacaagttttattaattatttatttattcgtatagaaaagtggggctcaataggtaagagttacaagatccattatttactcttagctcacgaagagctagctagatcttagctcatacatctgcattatttttcatattgattactcagtaaaaactgtccagaactgaagacagaggactcctttttctttagctttcttcctccttttattcaggttcagcacttgcaaagtgagattatttttaattcttgattaatctatttacctcttaagaagatccaggaaatgtgagctcctttactggattttctatttagcttatcacattgtcatccgatctttcaaattttcaatccccaaattagaaatataacattcaaatattaactaatgatatttctattcacttaatatctgaaaggaagtttctctaattgttctcggcattgataccaaatccaaccaaattcagatttgatgaagcactaatggcaactgggtgacctgctggaatgataacaacgtcacccggagacaatctagcttcatatctctacacttcattgtttctttcttttctatcttccctctcttattactcattttttaaacccagaagttcaaggtttccttttccttcattaactaatagtacaactattgcccttgaattgtagtgtggcaacattagagctccttaaaaatttaagcaaaaacgcattaacatatttctgtaatataattaaaattatgtgttttatatatatttagtgttgtgtacatatcttgttaatctccacacaactaacaagtatatctaaatcttaaagctaagggtattttttctctggagtaatctcaaacaacttgccaaacttattagaatattctggcttgtggcttctcaagttgaaaggttcaaattcagagggtaagcttttctttgagcttgattttgcaagctttctcaattcctcaatttattcccttgatactttgattattgcgtctctttcttccccttattatgttcttttccgatctctcaattattatggttttttctcttactcttctaaaagaaccttctctatggtctcgtatttagtttatatttgcgaaaaaggatacaaaatataatggttatatttattaaacatttgataaaaaaatcacacattaagcttaacatgtgttgtttgcatacttatatttaaggaggcctctaaaatgttcttgctgaatcctcataagtattagtttttattttcagatagaccaaaagcttgtagaagaaggataaagatcaatttttcaatccagacaaaaataaaagtaatataaaggaggtgttttaataagaataaaacatgtgaagaaaattattatctcaaatttaccaggcctgttcacgggtattacaaaatccaccactcttagatcttcttcatcatcttagttaactagataagatgttgttcctgcgggaattttgatggtatcaccacgctcaagattatacgagtttctatcattgggactcaacactgtcaatatggctttccttgtagtacatattaaccacaccaaaatttaattatgaaatataagaaatattgctaaattgaactttacaatatttttattttaaatagtcatatttctataaaacaaaagatttgttataataatattataaagaaaaataaaaattatcattgaggactacaaggattaagtcagcatctatgtgttaaggaaggaagatggtgtggggtttggctctatattccacaagacgatagttttagagattttcaaataagtctgaacgtttgtcgaacctttaaaggcgacgaatgtgaccgttttcgttttcaaagagtgtcagaaacttgttagacttgaataaaaaggggtttctttattcttatgattctgaagatctttcttcctcctctccttcacgttgatggcgtctgtctctttttgttctctcctctctatgccttagccttgccctttcttcgggatcttcacgacgttaacttcctctttactcttcgtctacttattcctcatcttcctctctttcttatctctcacgtccaggttaaacttccttttattccttcttttcacgttaatatcaatatttctacttctcttcttcatcttcttccttttcatatgaaggtctttattctccatggcgtttttcttctttctcaccctcttagcgacctctttctctttatcccggtaccctagtttctgaaccttcatcgtaattggcataagtgacgcaaacagaggccaggaatataattcccagaaacaataaaagtggaaatcatgatttgacagtggtcgctatgatttgtatttcactagttcgaactttagatgatgaaataaaagattaagttgaaggatatttatagtgatagaacgtaaagctagatgaataacgtggatggtcatttgggtaca

SEQ ID NO: 104 - DNA, 3400 bp, synthetic construct
  source 1..3400: mol_type = other DNA
gacacggtgagagtaacagaagatagtattaatgactaagtagaagaaatatttctgaccattgattggtgacgaaaactacccctataaagtttactcgcagttaaacatcgaaatatccattatttttttgtcatttactttttcattattattatataagtttaaacacttagaatcataaaaattattaaatctatctttaagcacaacaaacaaatctatctatggatagaataatattgtacctgttgactccaaatacacaacaataatatgaaaaatagaataataaattcaaatggttagaatatatttttacttagataccaaagttttaccatctttcttgtctttcttaagaactatctgaatcaattttgacctcaactattagaataagaaactttatccaaatctataaataaaagaaaacatttgaaattgggttaacaatttaggctcaatccttccaagtctcgaagtctcgattattacgcaactcctcttacatttcatcttttcctcatagaacatttacattaaaacaaagagtccaattaatattcagaacttcatattgtaaatctaacattgatataaccgtcatgaaaatatattttctagagagaaaagaaattgcacaacctcgtcttaactcacaaattacaaaacacttccaattttttaatttaaagaaaagatataaaaacataaacaaattaaagcaactaatacaagagtaaggcactgcatgttatgaaccattacaataataacacaaccaataaccattattaaaaacaattttaaaaattccttcattgaatccatagtctttttttaagacttaccccaagaacacaaattaatattatccttgtagttaaagtaaaaaaaaagcacaagttttattaattatttatttattcgtatagaaaagtggggctcaataggtaagagttacaagatccattatttactcttagctcacgaagagctagctagatcttagctcatacatctgcattatttttcatattgattactcagtaaaaactgtccagaactgaagacagaggactcctttttctttagctttcttcctccttttattcaggttcagcacttgcaaagtgagattatttttaattcttgattaatctatttacctcttaagaagatccaggaaatgtgagctcctttactggattttctatttagcttatcacattgtcatccgatctttcaaattttcaatccccaaattagaaatataacattcaaatattaactaatgatatttctattcacttaatatctgaaaggaagtttctctaattgttctcggcattgataccaaatccaaccaaattcagatttgatgaagcactaatggcaactgggtgacctgctggaatgataacaacgtcacccggagacaatctagcttcatatctctacacttcattgtttctttcttttctatcttccctctcttattactcattttttaaacccagaagttcaaggtttccttttccttcattaactaatagtacaactattgcccttgaattgtagtgtggcaacattagagctccttaaaaatttaagcaaaaacgcattaacatatttctgtaatataattaaaattatgtgttttatatatatttagtgttgtgtacatatcttgttaatctccacacaactaacaagtatatctaaatcttaaagctaagggtattttttctctggagtaatctcaaacaacttgccaaacttattagaatattctggcttgtggcttctcaagttgaaaggttcaaattcagagggtaagcttttctttgagcttgattttgcaagctttctcaattcctcaatttattcccttgatactttgattattgcgtctctttcttccccttattatgttcttttccgatctctcaattattatggttttttctcttactcttctaaaagaaccttctctatggtctcgtatttagtttatatttgcgaaaaaggatacaaaatataatggttatatttattaaacatttgataaaaaaatcacacattaagcttaacatgtgttgtttgcatacttatatttaaggaggcctctaaaatgttcttgctgaatcctcataagtattagtttttattttcagatagaccaaaagcttgtagaagaaggataaagatcaatttttcaatccagacaaaaataaaagtaatataaaggaggtgttttaataagaataaaacatgtgaagaaaattattatctcaaatttaccaggcctgttcacgggtattacaaaatccaccactcttagatcttcttcatcatcttagttaactagataagatgttgttcctgcgggaattttgatggtatcaccacgctcaagattatacgagtttctatcattgggactcaacactgtcaatatggctttccttgtagtacatattaaccacaccaaaatttaattatgaaatataagaaatattgctaaattgaactttacaatatttttattttaaatagtcatatttctataaaacaaaagatttgttataataatattataaagaaaaataaaaattatcattgaggactacaaggattaagtcagcatctatgtgttaaggaaggaagatggtgtggggtttggctctatattccacaagacgatagttttagagattttcaaataagtctgaacgtttgtcgaacctttaaaggcgacgaatgtgaccgttttcgttttcaaagagtgtcagaaacttgttagacttgaataaaaaggggtttctttattcttatgattctgaagatctttcttcctcctctccttcacgttaatggcgtctgtctctttttgttctctcctctctatgccttagccttgccctttcttcgggatcttcacgacgttgacttcctctttactcttcgtctacttattcctcatcttcctctctttcttatctctcacgtccaggttaaacttccttttattccttcttttcacgttaatatcaatatttctacttctcttcttcatcttcttccttttcatatgaaggtctttattctccatggcgtttttcttctttctcaccctcttagcgacctctttctctttatcccggtaccctagtttctgaaccttcatcgtaattggcataagtgacgcaaacagaggccaggaatataattcccagaaacaataaaagtggaaatcatgatttgacagtggtcgctatgatttgtatttcactagttcgaactttagatgatgaaataaaagattaagttgaaggatatttatagtgatagaacgtaaagctagatgaataacgtggatggtcatttgggtaca

SEQ ID NO: 105 - DNA, 3400 bp, synthetic construct
  source 1..3400: mol_type = other DNA
gacacggtgagagtaacagaagatagtattaatgactaagtagaagaaatatttctgaccattgattggtgacgaaaactacccctataaagtttactcgcagttaaacatcgaaatatccattatttttttgtcatttactttttcattattattatataagtttaaacacttagaatcataaaaattattaaatctatctttaagcacaacaaacaaatctatctatggatagaataatattgtacctgttgactccaaatacacaacaataatatgaaaaatagaataataaattcaaatggttagaatatatttttacttagataccaaagttttaccatctttcttgtctttcttaagaactatctgaatcaattttgacctcaactattagaataagaaactttatccaaatctataaataaaagaaaacatttgaaattgggttaacaatttaggctcaatccttccaagtctcgaagtctcgattattacgcaactcctcttacatttcatcttttcctcatagaacatttacattaaaacaaagagtccaattaatattcagaacttcatattgtaaatctaacattgatataaccgtcatgaaaatatattttctagagagaaaagaaattgcacaacctcgtcttaactcacaaattacaaaacacttccaattttttaatttaaagaaaagatataaaaacataaacaaattaaagcaactaatacaagagtaaggcactgcatgttatgaaccattacaataataacacaaccaataaccattattaaaaacaattttaaaaattccttcattgaatccatagtctttttttaagacttaccccaagaacacaaattaatattatccttgtagttaaagtaaaaaaaaagcacaagttttattaattatttatttattcgtatagaaaagtggggctcaataggtaagagttacaagatccattatttactcttagctcacgaagagctagctagatcttagctcatacatctgcattatttttcatattgattactcagtaaaaactgtccagaactgaagacagaggactcctttttctttagctttcttcctccttttattcaggttcagcacttgcaaagtgagattatttttaattcttgattaatctatttacctcttaagaagatccaggaaatgtgagctcctttactggattttctatttagcttatcacattgtcatccgatctttcaaattttcaatccccaaattagaaatataacattcaaatattaactaatgatatttctattcacttaatatctgaaaggaagtttctctaattgttctcggcattgataccaaatccaaccaaattcagatttgatgaagcactaatggcaactgggtgacctgctggaatgataacaacgtcacccggagacaatctagcttcatatctctacacttcattgtttctttcttttctatcttccctctcttattactcattttttaaacccagaagttcaaggtttccttttccttcattaactaatagtacaactattgcccttgaattgtagtgtggcaacattagagctccttaaaaatttaagcaaaaacgcattaacatatttctgtaatataattaaaattatgtgttttatatatatttagtgttgtgtacatatcttgttaatctccacacaactaacaagtatatctaaatcttaaagctaagggtattttttctctggagtaatctcaaacaacttgccaaacttattagaatattctggcttgtggcttctcaagttgaaaggttcaaattcagagggtaagcttttctttgagcttgattttgcaagctttctcaattcctcaatttattcccttgatactttgattattgcgtctctttcttccccttattatgttcttttccgatctctcaattattatggttttttctcttactcttctaaaagaaccttctctatggtctcgtatttagtttatatttgcgaaaaaggatacaaaatataatggttatatttattaaacatttgataaaaaaatcacacattaagcttaacatgtgttgtttgcatacttatatttaaggaggcctctaaaatgttcttgctgaatcctcataagtattagtttttattttcagatagaccaaaagcttgtagaagaaggataaagatcaatttttcaatccagacaaaaataaaagtaatataaaggaggtgttttaataagaataaaacatgtgaagaaaattattatctcaaatttaccaggcctgttcacgggtattacaaaatccaccactcttagatcttcttcatcatcttagttaactagataagatgttgttcctgcgggaattttgatggtatcaccacgctcaagattatacgagtttctatcattgggactcaacactgtcaatatggctttccttgtagtacatattaaccacaccaaaatttaattatgaaatataagaaatattgctaaattgaactttacaatatttttattttaaatagtcatatttctataaaacaaaagatttgttataataatattataaagaaaaataaaaattatcattgaggactacaaggattaagtcagcatctatgtgttaaggaaggaagatggtgtggggtttggctctatattccacaagacgatagttttagagattttcaaataagtctgaacgtttgtcgaacctttaaaggcgacgaatgtgaccgttttcgttttcaaagagtgtcagaaacttgttagacttgaataaaaaggggtttctttattcttatgattctgaagatctttcttcctcctctccttcacgttaatggcgtctgtctctttttgttctctcctctctatgccttagccttgccctttcttcgggatcttcacgacgttaacttcctctctactcttcgtctacttattcctcatcttcctctctttcttatctctcacgtccaggttaaacttccttttattccttcttttcacgttaatatcaatatttctacttctcttcttcatcttcttccttttcatatgaaggtctttattctccatggcgtttttcttctttctcaccctcttagcgacctctttctctttatcccggtaccctagtttctgaaccttcatcgtaattggcataagtgacgcaaacagaggccaggaatataattcccagaaacaataaaagtggaaatcatgatttgacagtggtcgctatgatttgtatttcactagttcgaactttagatgatgaaataaaagattaagttgaaggatatttatagtgatagaacgtaaagctagatgaataacgtggatggtcatttgggtaca

SEQ ID NO: 106 - DNA, 3400 bp, synthetic construct
  source 1..3400: mol_type = other DNA
gacacggtgagagtaacagaagatagtattaatgactaagtagaagaaatatttctgaccattgattggtgacgaaaactacccctataaagtttactcgcagttaaacatcgaaatatccattatttttttgtcatttactttttcattattattatataagtttaaacacttagaatcataaaaattattaaatctatctttaagcacaacaaacaaatctatctatggatagaataatattgtacctgttgactccaaatacacaacaataatatgaaaaatagaataataaattcaaatggttagaatatatttttacttagataccaaagttttaccatctttcttgtctttcttaagaactatctgaatcaattttgacctcaactattagaataagaaactttatccaaatctataaataaaagaaaacatttgaaattgggttaacaatttaggctcaatccttccaagtctcgaagtctcgattattacgcaactcctcttacatttcatcttttcctcatagaacatttacattaaaacaaagagtccaattaatattcagaacttcatattgtaaatctaacattgatataaccgtcatgaaaatatattttctagagagaaaagaaattgcacaacctcgtcttaactcacaaattacaaaacacttccaattttttaatttaaagaaaagatataaaaacataaacaaattaaagcaactaatacaagagtaaggcactgcatgttatgaaccattacaataataacacaaccaataaccattattaaaaacaattttaaaaattccttcattgaatccatagtctttttttaagacttaccccaagaacacaaattaatattatccttgtagttaaagtaaaaaaaaagcacaagttttattaattatttatttattcgtatagaaaagtggggctcaataggtaagagttacaagatccattatttactcttagctcacgaagagctagctagatcttagctcatacatctgcattatttttcatattgattactcagtaaaaactgtccagaactgaagacagaggactcctttttctttagctttcttcctccttttattcaggttcagcacttgcaaagtgagattatttttaattcttgattaatctatttacctcttaagaagatccaggaaatgtgagctcctttactggattttctatttagcttatcacattgtcatccgatctttcaaattttcaatccccaaattagaaatataacattcaaatattaactaatgatatttctattcacttaatatctgaaaggaagtttctctaattgttctcggcattgataccaaatccaaccaaattcagatttgatgaagcactaatggcaactgggtgacctgctggaatgataacaacgtcacccggagacaatctagcttcatatctctacacttcattgtttctttcttttctatcttccctctcttattactcattttttaaacccagaagttcaaggtttccttttccttcattaactaatagtacaactattgcccttgaattgtagtgtggcaacattagagctccttaaaaatttaagcaaaaacgcattaacatatttctgtaatataattaaaattatgtgttttatatatatttagtgttgtgtacatatcttgttaatctccacacaactaacaagtatatctaaatcttaaagctaagggtattttttctctggagtaatctcaaacaacttgccaaacttattagaatattctggcttgtggcttctcaagttgaaaggttcaaattcagagggtaagcttttctttgagcttgattttgcaagctttctcaattcctcaatttattcccttgatactttgattattgcgtctctttcttccccttattatgttcttttccgatctctcaattattatggttttttctcttactcttctaaaagaaccttctctatggtctcgtatttagtttatatttgcgaaaaaggatacaaaatataatggttatatttattaaacatttgataaaaaaatcacacattaagcttaacatgtgttgtttgcatacttatatttaaggaggcctctaaaatgttcttgctgaatcctcataagtattagtttttattttcagatagaccaaaagcttgtagaagaaggataaagatcaatttttcaatccagacaaaaataaaagtaatataaaggaggtgttttaataagaataaaacatgtgaagaaaattattatctcaaatttaccaggcctgttcacgggtattacaaaatccaccactcttagatcttcttcatcatcttagttaactagataagatgttgttcctgcgggaattttgatggtatcaccacgctcaagattatacgagtttctatcattgggactcaacactgtcaatatggctttccttgtagtacatattaaccacaccaaaatttaattatgaaatataagaaatattgctaaattgaactttacaatatttttattttaaatagtcatatttctataaaacaaaagatttgttataataatattataaagaaaaataaaaattatcattgaggactacaaggattaagtcagcatctatgtgttaaggaaggaagatggtgtggggtttggctctatattccacaagacgatagttttagagattttcaaataagtctgaacgtttgtcgaacctttaaaggcgacgaatgtgaccgttttcgttttcaaagagtgtcagaaacttgttagacttgaataaaaaggggtttctttattcttatgattctgaagatctttcttcctcctctccttcacgttaatggcgtctgtctctttttgttctctcctctctatgccttagccttgccctttcttcgggatcttcacgacgttaacttcctcttcactcttcgtctacttattcctcatcttcctctctttcttatctctcacgtccaggttaaacttccttttattccttcttttcacgttaatatcaatatttctacttctcttcttcatcttcttccttttcatatgaaggtctttattctccatggcgtttttcttctttctcaccctcttagcgacctctttctctttatcccggtaccctagtttctgaaccttcatcgtaattggcataagtgacgcaaacagaggccaggaatataattcccagaaacaataaaagtggaaatcatgatttgacagtggtcgctatgatttgtatttcactagttcgaactttagatgatgaaataaaagattaagttgaaggatatttatagtgatagaacgtaaagctagatgaataacgtggatggtcatttgggtaca

SEQ ID NO: 107 - DNA, 3400 bp, synthetic construct
  source 1..3400: mol_type = other DNA
gacacggtgagagtaacagaagatagtattaatgactaagtagaagaaatatttctgaccattgattggtgacgaaaactacccctataaagtttactcgcagttaaacatcgaaatatccattatttttttgtcatttactttttcattattattatataagtttaaacacttagaatcataaaaattattaaatctatctttaagcacaacaaacaaatctatctatggatagaataatattgtacctgttgactccaaatacacaacaataatatgaaaaatagaataataaattcaaatggttagaatatatttttacttagataccaaagttttaccatctttcttgtctttcttaagaactatctgaatcaattttgacctcaactattagaataagaaactttatccaaatctataaataaaagaaaacatttgaaattgggttaacaatttaggctcaatccttccaagtctcgaagtctcgattattacgcaactcctcttacatttcatcttttcctcatagaacatttacattaaaacaaagagtccaattaatattcagaacttcatattgtaaatctaacattgatataaccgtcatgaaaatatattttctagagagaaaagaaattgcacaacctcgtcttaactcacaaattacaaaacacttccaattttttaatttaaagaaaagatataaaaacataaacaaattaaagcaactaatacaagagtaaggcactgcatgttatgaaccattacaataataacacaaccaataaccattattaaaaacaattttaaaaattccttcattgaatccatagtctttttttaagacttaccccaagaacacaaattaatattatccttgtagttaaagtaaaaaaaaagcacaagttttattaattatttatttattcgtatagaaaagtggggctcaataggtaagagttacaagatccattatttactcttagctcacgaagagctagctagatcttagctcatacatctgcattatttttcatattgattactcagtaaaaactgtccagaactgaagacagaggactcctttttctttagctttcttcctccttttattcaggttcagcacttgcaaagtgagattatttttaattcttgattaatctatttacctcttaagaagatccaggaaatgtgagctcctttactggattttctatttagcttatcacattgtcatccgatctttcaaattttcaatccccaaattagaaatataacattcaaatattaactaatgatatttctattcacttaatatctgaaaggaagtttctctaattgttctcggcattgataccaaatccaaccaaattcagatttgatgaagcactaatggcaactgggtgacctgctggaatgataacaacgtcacccggagacaatctagcttcatatctctacacttcattgtttctttcttttctatcttccctctcttattactcattttttaaacccagaagttcaaggtttccttttccttcattaactaatagtacaactattgcccttgaattgtagtgtggcaacattagagctccttaaaaatttaagcaaaaacgcattaacatatttctgtaatataattaaaattatgtgttttatatatatttagtgttgtgtacatatcttgttaatctccacacaactaacaagtatatctaaatcttaaagctaagggtattttttctctggagtaatctcaaacaacttgccaaacttattagaatattctggcttgtggcttctcaagttgaaaggttcaaattcagagggtaagcttttctttgagcttgattttgcaagctttctcaattcctcaatttattcccttgatactttgattattgcgtctctttcttccccttattatgttcttttccgatctctcaattattatggttttttctcttactcttctaaaagaaccttctctatggtctcgtatttagtttatatttgcgaaaaaggatacaaaatataatggttatatttattaaacatttgataaaaaaatcacacattaagcttaacatgtgttgtttgcatacttatatttaaggaggcctctaaaatgttcttgctgaatcctcataagtattagtttttattttcagatagaccaaaagcttgtagaagaaggataaagatcaatttttcaatccagacaaaaataaaagtaatataaaggaggtgttttaataagaataaaacatgtgaagaaaattattatctcaaatttaccaggcctgttcacgggtattacaaaatccaccactcttagatcttcttcatcatcttagttaactagataagatgttgttcctgcgggaattttgatggtatcaccacgctcaagattatacgagtttctatcattgggactcaacactgtcaatatggctttccttgtagtacatattaaccacaccaaaatttaattatgaaatataagaaatattgctaaattgaactttacaatatttttattttaaatagtcatatttctataaaacaaaagatttgttataataatattataaagaaaaataaaaattatcattgaggactacaaggattaagtcagcatctatgtgttaaggaaggaagatggtgtggggtttggctctatattccacaagacgatagttttagagattttcaaataagtctgaacgtttgtcgaacctttaaaggcgacgaatgtgaccgttttcgttttcaaagagtgtcagaaacttgttagacttgaataaaaaggggtttctttattcttatgattctgaagatctttcttcctcctctccttcacgttaatggcgtctgtctctttttgttctctcctctctatgccttagccttgccctttcttcgggatcttcacgacgttaacttcctctttactcttcgtctacttgttcctcatcttcctctctttcttatctctcacgtccaggttaaacttccttttattccttcttttcacgttaatatcaatatttctacttctcttcttcatcttcttccttttcatatgaaggtctttattctccatggcgtttttcttctttctcaccctcttagcgacctctttctctttatcccggtaccctagtttctgaaccttcatcgtaattggcataagtgacgcaaacagaggccaggaatataattcccagaaacaataaaagtggaaatcatgatttgacagtggtcgctatgatttgtatttcactagttcgaactttagatgatgaaataaaagattaagttgaaggatatttatagtgatagaacgtaaagctagatgaataacgtggatggtcatttgggtaca

SEQ ID NO: 108 - DNA, 3400 bp, synthetic construct
  source 1..3400: mol_type = other DNA
gacacggtgagagtaacagaagatagtattaatgactaagtagaagaaatatttctgaccattgattggtgacgaaaactacccctataaagtttactcgcagttaaacatcgaaatatccattatttttttgtcatttactttttcattattattatataagtttaaacacttagaatcataaaaattattaaatctatctttaagcacaacaaacaaatctatctatggatagaataatattgtacctgttgactccaaatacacaacaataatatgaaaaatagaataataaattcaaatggttagaatatatttttacttagataccaaagttttaccatctttcttgtctttcttaagaactatctgaatcaattttgacctcaactattagaataagaaactttatccaaatctataaataaaagaaaacatttgaaattgggttaacaatttaggctcaatccttccaagtctcgaagtctcgattattacgcaactcctcttacatttcatcttttcctcatagaacatttacattaaaacaaagagtccaattaatattcagaacttcatattgtaaatctaacattgatataaccgtcatgaaaatatattttctagagagaaaagaaattgcacaacctcgtcttaactcacaaattacaaaacacttccaattttttaatttaaagaaaagatataaaaacataaacaaattaaagcaactaatacaagagtaaggcactgcatgttatgaaccattacaataataacacaaccaataaccattattaaaaacaattttaaaaattccttcattgaatccatagtctttttttaagacttaccccaagaacacaaattaatattatccttgtagttaaagtaaaaaaaaagcacaagttttattaattatttatttattcgtatagaaaagtggggctcaataggtaagagttacaagatccattatttactcttagctcacgaagagctagctagatcttagctcatacatctgcattatttttcatattgattactcagtaaaaactgtccagaactgaagacagaggactcctttttctttagctttcttcctccttttattcaggttcagcacttgcaaagtgagattatttttaattcttgattaatctatttacctcttaagaagatccaggaaatgtgagctcctttactggattttctatttagcttatcacattgtcatccgatctttcaaattttcaatccccaaattagaaatataacattcaaatattaactaatgatatttctattcacttaatatctgaaaggaagtttctctaattgttctcggcattgataccaaatccaaccaaattcagatttgatgaagcactaatggcaactgggtgacctgctggaatgataacaacgtcacccggagacaatctagcttcatatctctacacttcattgtttctttcttttctatcttccctctcttattactcattttttaaacccagaagttcaaggtttccttttccttcattaactaatagtacaactattgcccttgaattgtagtgtggcaacattagagctccttaaaaatttaagcaaaaacgcattaacatatttctgtaatataattaaaattatgtgttttatatatatttagtgttgtgtacatatcttgttaatctccacacaactaacaagtatatctaaatcttaaagctaagggtattttttctctggagtaatctcaaacaacttgccaaacttattagaatattctggcttgtggcttctcaagttgaaaggttcaaattcagagggtaagcttttctttgagcttgattttgcaagctttctcaattcctcaatttattcccttgatactttgattattgcgtctctttcttccccttattatgttcttttccgatctctcaattattatggttttttctcttactcttctaaaagaaccttctctatggtctcgtatttagtttatatttgcgaaaaaggatacaaaatataatggttatatttattaaacatttgataaaaaaatcacacattaagcttaacatgtgttgtttgcatacttatatttaaggaggcctctaaaatgttcttgctgaatcctcataagtattagtttttattttcagatagaccaaaagcttgtagaagaaggataaagatcaatttttcaatccagacaaaaataaaagtaatataaaggaggtgttttaataagaataaaacatgtgaagaaaattattatctcaaatttaccaggcctgttcacgggtattacaaaatccaccactcttagatcttcttcatcatcttagttaactagataagatgttgttcctgcgggaattttgatggtatcaccacgctcaagattatacgagtttctatcattgggactcaacactgtcaatatggctttccttgtagtacatattaaccacaccaaaatttaattatgaaatataagaaatattgctaaattgaactttacaatatttttattttaaatagtcatatttctataaaacaaaagatttgttataataatattataaagaaaaataaaaattatcattgaggactacaaggattaagtcagcatctatgtgttaaggaaggaagatggtgtggggtttggctctatattccacaagacgatagttttagagattttcaaataagtctgaacgtttgtcgaacctttaaaggcgacgaatgtgaccgttttcgttttcaaagagtgtcagaaacttgttagacttgaataaaaaggggtttctttattcttatgattctgaagatctttcttcctcctctccttcacgttaatggcgtctgtctctttttgttctctcctctctatgccttagccttgccctttcttcgggatcttcacgacgttaacttcctctttactcttcgtctacttattcctcatcttcctctctttcctatctctcacgtccaggttaaacttccttttattccttcttttcacgttaatatcaatatttctacttctcttcttcatcttcttccttttcatatgaaggtctttattctccatggcgtttttcttctttctcaccctcttagcgacctctttctctttatcccggtaccctagtttctgaaccttcatcgtaattggcataagtgacgcaaacagaggccaggaatataattcccagaaacaataaaagtggaaatcatgatttgacagtggtcgctatgatttgtatttcactagttcgaactttagatgatgaaataaaagattaagttgaaggatatttatagtgatagaacgtaaagctagatgaataacgtggatggtcatttgggtaca

SEQ ID NO: 109 - DNA, 3400 bp, synthetic construct
  source 1..3400: mol_type = other DNA
gacacggtgagagtaacagaagatagtattaatgactaagtagaagaaatatttctgaccattgattggtgacgaaaactacccctataaagtttactcgcagttaaacatcgaaatatccattatttttttgtcatttactttttcattattattatataagtttaaacacttagaatcataaaaattattaaatctatctttaagcacaacaaacaaatctatctatggatagaataatattgtacctgttgactccaaatacacaacaataatatgaaaaatagaataataaattcaaatggttagaatatatttttacttagataccaaagttttaccatctttcttgtctttcttaagaactatctgaatcaattttgacctcaactattagaataagaaactttatccaaatctataaataaaagaaaacatttgaaattgggttaacaatttaggctcaatccttccaagtctcgaagtctcgattattacgcaactcctcttacatttcatcttttcctcatagaacatttacattaaaacaaagagtccaattaatattcagaacttcatattgtaaatctaacattgatataaccgtcatgaaaatatattttctagagagaaaagaaattgcacaacctcgtcttaactcacaaattacaaaacacttccaattttttaatttaaagaaaagatataaaaacataaacaaattaaagcaactaatacaagagtaaggcactgcatgttatgaaccattacaataataacacaaccaataaccattattaaaaacaattttaaaaattccttcattgaatccatagtctttttttaagacttaccccaagaacacaaattaatattatccttgtagttaaagtaaaaaaaaagcacaagttttattaattatttatttattcgtatagaaaagtggggctcaataggtaagagttacaagatccattatttactcttagctcacgaagagctagctagatcttagctcatacatctgcattatttttcatattgattactcagtaaaaactgtccagaactgaagacagaggactcctttttctttagctttcttcctccttttattcaggttcagcacttgcaaagtgagattatttttaattcttgattaatctatttacctcttaagaagatccaggaaatgtgagctcctttactggattttctatttagcttatcacattgtcatccgatctttcaaattttcaatccccaaattagaaatataacattcaaatattaactaatgatatttctattcacttaatatctgaaaggaagtttctctaattgttctcggcattgataccaaatccaaccaaattcagatttgatgaagcactaatggcaactgggtgacctgctggaatgataacaacgtcacccggagacaatctagcttcatatctctacacttcattgtttctttcttttctatcttccctctcttattactcattttttaaacccagaagttcaaggtttccttttccttcattaactaatagtacaactattgcccttgaattgtagtgtggcaacattagagctccttaaaaatttaagcaaaaacgcattaacatatttctgtaatataattaaaattatgtgttttatatatatttagtgttgtgtacatatcttgttaatctccacacaactaacaagtatatctaaatcttaaagctaagggtattttttctctggagtaatctcaaacaacttgccaaacttattagaatattctggcttgtggcttctcaagttgaaaggttcaaattcagagggtaagcttttctttgagcttgattttgcaagctttctcaattcctcaatttattcccttgatactttgattattgcgtctctttcttccccttattatgttcttttccgatctctcaattattatggttttttctcttactcttctaaaagaaccttctctatggtctcgtatttagtttatatttgcgaaaaaggatacaaaatataatggttatatttattaaacatttgataaaaaaatcacacattaagcttaacatgtgttgtttgcatacttatatttaaggaggcctctaaaatgttcttgctgaatcctcataagtattagtttttattttcagatagaccaaaagcttgtagaagaaggataaagatcaatttttcaatccagacaaaaataaaagtaatataaaggaggtgttttaataagaataaaacatgtgaagaaaattattatctcaaatttaccaggcctgttcacgggtattacaaaatccaccactcttagatcttcttcatcatcttagttaactagataagatgttgttcctgcgggaattttgatggtatcaccacgctcaagattatacgagtttctatcattgggactcaacactgtcaatatggctttccttgtagtacatattaaccacaccaaaatttaattatgaaatataagaaatattgctaaattgaactttacaatatttttattttaaatagtcatatttctataaaacaaaagatttgttataataatattataaagaaaaataaaaattatcattgaggactacaaggattaagtcagcatctatgtgttaaggaaggaagatggtgtggggtttggctctatattccacaagacgatagttttagagattttcaaataagtctgaacgtttgtcgaacctttaaaggcgacgaatgtgaccgttttcgttttcaaagagtgtcagaaacttgttagacttgaataaaaaggggtttctttattcttatgattctgaagatctttcttcctcctctccttcacgttaatggcgtctgtctctttttgttctctcctctctatgccttagccttgccctttcttcgggatcttcacgacgttaacttcctctttactcttcgtctacttattcctcatcttcctctctttctcatctctcacgtccaggttaaacttccttttattccttcttttcacgttaatatcaatatttctacttctcttcttcatcttcttccttttcatatgaaggtctttattctccatggcgtttttcttctttctcaccctcttagcgacctctttctctttatcccggtaccctagtttctgaaccttcatcgtaattggcataagtgacgcaaacagaggccaggaatataattcccagaaacaataaaagtggaaatcatgatttgacagtggtcgctatgatttgtatttcactagttcgaactttagatgatgaaataaaagattaagttgaaggatatttatagtgatagaacgtaaagctagatgaataacgtggatggtcatttgggtaca

SEQ ID NO: 110 - DNA, 3400 bp, synthetic construct
  source 1..3400: mol_type = other DNA
gacacggtgagagtaacagaagatagtattaatgactaagtagaagaaatatttctgaccattgattggtgacgaaaactacccctataaagtttactcgcagttaaacatcgaaatatccattatttttttgtcatttactttttcattattattatataagtttaaacacttagaatcataaaaattattaaatctatctttaagcacaacaaacaaatctatctatggatagaataatattgtacctgttgactccaaatacacaacaataatatgaaaaatagaataataaattcaaatggttagaatatatttttacttagataccaaagttttaccatctttcttgtctttcttaagaactatctgaatcaattttgacctcaactattagaataagaaactttatccaaatctataaataaaagaaaacatttgaaattgggttaacaatttaggctcaatccttccaagtctcgaagtctcgattattacgcaactcctcttacatttcatcttttcctcatagaacatttacattaaaacaaagagtccaattaatattcagaacttcatattgtaaatctaacattgatataaccgtcatgaaaatatattttctagagagaaaagaaattgcacaacctcgtcttaactcacaaattacaaaacacttccaattttttaatttaaagaaaagatataaaaacataaacaaattaaagcaactaatacaagagtaaggcactgcatgttatgaaccattacaataataacacaaccaataaccattattaaaaacaattttaaaaattccttcattgaatccatagtctttttttaagacttaccccaagaacacaaattaatattatccttgtagttaaagtaaaaaaaaagcacaagttttattaattatttatttattcgtatagaaaagtggggctcaataggtaagagttacaagatccattatttactcttagctcacgaagagctagctagatcttagctcatacatctgcattatttttcatattgattactcagtaaaaactgtccagaactgaagacagaggactcctttttctttagctttcttcctccttttattcaggttcagcacttgcaaagtgagattatttttaattcttgattaatctatttacctcttaagaagatccaggaaatgtgagctcctttactggattttctatttagcttatcacattgtcatccgatctttcaaattttcaatccccaaattagaaatataacattcaaatattaactaatgatatttctattcacttaatatctgaaaggaagtttctctaattgttctcggcattgataccaaatccaaccaaattcagatttgatgaagcactaatggcaactgggtgacctgctggaatgataacaacgtcacccggagacaatctagcttcatatctctacacttcattgtttctttcttttctatcttccctctcttattactcattttttaaacccagaagttcaaggtttccttttccttcattaactaatagtacaactattgcccttgaattgtagtgtggcaacattagagctccttaaaaatttaagcaaaaacgcattaacatatttctgtaatataattaaaattatgtgttttatatatatttagtgttgtgtacatatcttgttaatctccacacaactaacaagtatatctaaatcttaaagctaagggtattttttctctggagtaatctcaaacaacttgccaaacttattagaatattctggcttgtggcttctcaagttgaaaggttcaaattcagagggtaagcttttctttgagcttgattttgcaagctttctcaattcctcaatttattcccttgatactttgattattgcgtctctttcttccccttattatgttcttttccgatctctcaattattatggttttttctcttactcttctaaaagaaccttctctatggtctcgtatttagtttatatttgcgaaaaaggatacaaaatataatggttatatttattaaacatttgataaaaaaatcacacattaagcttaacatgtgttgtttgcatacttatatttaaggaggcctctaaaatgttcttgctgaatcctcataagtattagtttttattttcagatagaccaaaagcttgtagaagaaggataaagatcaatttttcaatccagacaaaaataaaagtaatataaaggaggtgttttaataagaataaaacatgtgaagaaaattattatctcaaatttaccaggcctgttcacgggtattacaaaatccaccactcttagatcttcttcatcatcttagttaactagataagatgttgttcctgcgggaattttgatggtatcaccacgctcaagattatacgagtttctatcattgggactcaacactgtcaatatggctttccttgtagtacatattaaccacaccaaaatttaattatgaaatataagaaatattgctaaattgaactttacaatatttttattttaaatagtcatatttctataaaacaaaagatttgttataataatattataaagaaaaataaaaattatcattgaggactacaaggattaagtcagcatctatgtgttaaggaaggaagatggtgtggggtttggctctatattccacaagacgatagttttagagattttcaaataagtctgaacgtttgtcgaacctttaaaggcgacgaatgtgaccgttttcgttttcaaagagtgtcagaaacttgttagacttgaataaaaaggggtttctttattcttatgattctgaagatctttcttcctcctctccttcacgttaatggcgtctgtctctttttgttctctcctctctatgccttagccttgccctttcttcgggatcttcacgacgttaacttcctctttactcttcgtctacttattcctcatcttcctctctttcttatctctcacgtccaggttgaacttccttttattccttcttttcacgttaatatcaatatttctacttctcttcttcatcttcttccttttcatatgaaggtctttattctccatggcgtttttcttctttctcaccctcttagcgacctctttctctttatcccggtaccctagtttctgaaccttcatcgtaattggcataagtgacgcaaacagaggccaggaatataattcccagaaacaataaaagtggaaatcatgatttgacagtggtcgctatgatttgtatttcactagttcgaactttagatgatgaaataaaagattaagttgaaggatatttatagtgatagaacgtaaagctagatgaataacgtggatggtcatttgggtaca

SEQ ID NO: 111 - DNA, 3400 bp, synthetic construct
  source 1..3400: mol_type = other DNA
gacacggtgagagtaacagaagatagtattaatgactaagtagaagaaatatttctgaccattgattggtgacgaaaactacccctataaagtttactcgcagttaaacatcgaaatatccattatttttttgtcatttactttttcattattattatataagtttaaacacttagaatcataaaaattattaaatctatctttaagcacaacaaacaaatctatctatggatagaataatattgtacctgttgactccaaatacacaacaataatatgaaaaatagaataataaattcaaatggttagaatatatttttacttagataccaaagttttaccatctttcttgtctttcttaagaactatctgaatcaattttgacctcaactattagaataagaaactttatccaaatctataaataaaagaaaacatttgaaattgggttaacaatttaggctcaatccttccaagtctcgaagtctcgattattacgcaactcctcttacatttcatcttttcctcatagaacatttacattaaaacaaagagtccaattaatattcagaacttcatattgtaaatctaacattgatataaccgtcatgaaaatatattttctagagagaaaagaaattgcacaacctcgtcttaactcacaaattacaaaacacttccaattttttaatttaaagaaaagatataaaaacataaacaaattaaagcaactaatacaagagtaaggcactgcatgttatgaaccattacaataataacacaaccaataaccattattaaaaacaattttaaaaattccttcattgaatccatagtctttttttaagacttaccccaagaacacaaattaatattatccttgtagttaaagtaaaaaaaaagcacaagttttattaattatttatttattcgtatagaaaagtggggctcaataggtaagagttacaagatccattatttactcttagctcacgaagagctagctagatcttagctcatacatctgcattatttttcatattgattactcagtaaaaactgtccagaactgaagacagaggactcctttttctttagctttcttcctccttttattcaggttcagcacttgcaaagtgagattatttttaattcttgattaatctatttacctcttaagaagatccaggaaatgtgagctcctttactggattttctatttagcttatcacattgtcatccgatctttcaaattttcaatccccaaattagaaatataacattcaaatattaactaatgatatttctattcacttaatatctgaaaggaagtttctctaattgttctcggcattgataccaaatccaaccaaattcagatttgatgaagcactaatggcaactgggtgacctgctggaatgataacaacgtcacccggagacaatctagcttcatatctctacacttcattgtttctttcttttctatcttccctctcttattactcattttttaaacccagaagttcaaggtttccttttccttcattaactaatagtacaactattgcccttgaattgtagtgtggcaacattagagctccttaaaaatttaagcaaaaacgcattaacatatttctgtaatataattaaaattatgtgttttatatatatttagtgttgtgtacatatcttgttaatctccacacaactaacaagtatatctaaatcttaaagctaagggtattttttctctggagtaatctcaaacaacttgccaaacttattagaatattctggcttgtggcttctcaagttgaaaggttcaaattcagagggtaagcttttctttgagcttgattttgcaagctttctcaattcctcaatttattcccttgatactttgattattgcgtctctttcttccccttattatgttcttttccgatctctcaattattatggttttttctcttactcttctaaaagaaccttctctatggtctcgtatttagtttatatttgcgaaaaaggatacaaaatataatggttatatttattaaacatttgataaaaaaatcacacattaagcttaacatgtgttgtttgcatacttatatttaaggaggcctctaaaatgttcttgctgaatcctcataagtattagtttttattttcagatagaccaaaagcttgtagaagaaggataaagatcaatttttcaatccagacaaaaataaaagtaatataaaggaggtgttttaataagaataaaacatgtgaagaaaattattatctcaaatttaccaggcctgttcacgggtattacaaaatccaccactcttagatcttcttcatcatcttagttaactagataagatgttgttcctgcgggaattttgatggtatcaccacgctcaagattatacgagtttctatcattgggactcaacactgtcaatatggctttccttgtagtacatattaaccacaccaaaatttaattatgaaatataagaaatattgctaaattgaactttacaatatttttattttaaatagtcatatttctataaaacaaaagatttgttataataatattataaagaaaaataaaaattatcattgaggactacaaggattaagtcagcatctatgtgttaaggaaggaagatggtgtggggtttggctctatattccacaagacgatagttttagagattttcaaataagtctgaacgtttgtcgaacctttaaaggcgacgaatgtgaccgttttcgttttcaaagagtgtcagaaacttgttagacttgaataaaaaggggtttctttattcttatgattctgaagatctttcttcctcctctccttcacgttaatggcgtctgtctctttttgttctctcctctctatgccttagccttgccctttcttcgggatcttcacgacgttaacttcctctttactcttcgtctacttattcctcatcttcctctctttcttatctctcacgtccaggttaaacttccttttgttccttcttttcacgttaatatcaatatttctacttctcttcttcatcttcttccttttcatatgaaggtctttattctccatggcgtttttcttctttctcaccctcttagcgacctctttctctttatcccggtaccctagtttctgaaccttcatcgtaattggcataagtgacgcaaacagaggccaggaatataattcccagaaacaataaaagtggaaatcatgatttgacagtggtcgctatgatttgtatttcactagttcgaactttagatgatgaaataaaagattaagttgaaggatatttatagtgatagaacgtaaagctagatgaataacgtggatggtcatttgggtaca

SEQ ID NO: 112 - DNA, 3400 bp, synthetic construct
  source 1..3400: mol_type = other DNA
gacacggtgagagtaacagaagatagtattaatgactaagtagaagaaatatttctgaccattgattggtgacgaaaactacccctataaagtttactcgcagttaaacatcgaaatatccattatttttttgtcatttactttttcattattattatataagtttaaacacttagaatcataaaaattattaaatctatctttaagcacaacaaacaaatctatctatggatagaataatattgtacctgttgactccaaatacacaacaataatatgaaaaatagaataataaattcaaatggttagaatatatttttacttagataccaaagttttaccatctttcttgtctttcttaagaactatctgaatcaattttgacctcaactattagaataagaaactttatccaaatctataaataaaagaaaacatttgaaattgggttaacaatttaggctcaatccttccaagtctcgaagtctcgattattacgcaactcctcttacatttcatcttttcctcatagaacatttacattaaaacaaagagtccaattaatattcagaacttcatattgtaaatctaacattgatataaccgtcatgaaaatatattttctagagagaaaagaaattgcacaacctcgtcttaactcacaaattacaaaacacttccaattttttaatttaaagaaaagatataaaaacataaacaaattaaagcaactaatacaagagtaaggcactgcatgttatgaaccattacaataataacacaaccaataaccattattaaaaacaattttaaaaattccttcattgaatccatagtctttttttaagacttaccccaagaacacaaattaatattatccttgtagttaaagtaaaaaaaaagcacaagttttattaattatttatttattcgtatagaaaagtggggctcaataggtaagagttacaagatccattatttactcttagctcacgaagagctagctagatcttagctcatacatctgcattatttttcatattgattactcagtaaaaactgtccagaactgaagacagaggactcctttttctttagctttcttcctccttttattcaggttcagcacttgcaaagtgagattatttttaattcttgattaatctatttacctcttaagaagatccaggaaatgtgagctcctttactggattttctatttagcttatcacattgtcatccgatctttcaaattttcaatccccaaattagaaatataacattcaaatattaactaatgatatttctattcacttaatatctgaaaggaagtttctctaattgttctcggcattgataccaaatccaaccaaattcagatttgatgaagcactaatggcaactgggtgacctgctggaatgataacaacgtcacccggagacaatctagcttcatatctctacacttcattgtttctttcttttctatcttccctctcttattactcattttttaaacccagaagttcaaggtttccttttccttcattaactaatagtacaactattgcccttgaattgtagtgtggcaacattagagctccttaaaaatttaagcaaaaacgcattaacatatttctgtaatataattaaaattatgtgttttatatatatttagtgttgtgtacatatcttgttaatctccacacaactaacaagtatatctaaatcttaaagctaagggtattttttctctggagtaatctcaaacaacttgccaaacttattagaatattctggcttgtggcttctcaagttgaaaggttcaaattcagagggtaagcttttctttgagcttgattttgcaagctttctcaattcctcaatttattcccttgatactttgattattgcgtctctttcttccccttattatgttcttttccgatctctcaattattatggttttttctcttactcttctaaaagaaccttctctatggtctcgtatttagtttatatttgcgaaaaaggatacaaaatataatggttatatttattaaacatttgataaaaaaatcacacattaagcttaacatgtgttgtttgcatacttatatttaaggaggcctctaaaatgttcttgctgaatcctcataagtattagtttttattttcagatagaccaaaagcttgtagaagaaggataaagatcaatttttcaatccagacaaaaataaaagtaatataaaggaggtgttttaataagaataaaacatgtgaagaaaattattatctcaaatttaccaggcctgttcacgggtattacaaaatccaccactcttagatcttcttcatcatcttagttaactagataagatgttgttcctgcgggaattttgatggtatcaccacgctcaagattatacgagtttctatcattgggactcaacactgtcaatatggctttccttgtagtacatattaaccacaccaaaatttaattatgaaatataagaaatattgctaaattgaactttacaatatttttattttaaatagtcatatttctataaaacaaaagatttgttataataatattataaagaaaaataaaaattatcattgaggactacaaggattaagtcagcatctatgtgttaaggaaggaagatggtgtggggtttggctctatattccacaagacgatagttttagagattttcaaataagtctgaacgtttgtcgaacctttaaaggcgacgaatgtgaccgttttcgttttcaaagagtgtcagaaacttgttagacttgaataaaaaggggtttctttattcttatgattctgaagatctttcttcctcctctccttcacgttaatggcgtctgtctctttttgttctctcctctctatgccttagccttgccctttcttcgggatcttcacgacgttaacttcctctttactcttcgtctacttattcctcatcttcctctctttcttatctctcacgtccaggttaaacttccttttattccttcttttcacgttgatatcaatatttctacttctcttcttcatcttcttccttttcatatgaaggtctttattctccatggcgtttttcttctttctcaccctcttagcgacctctttctctttatcccggtaccctagtttctgaaccttcatcgtaattggcataagtgacgcaaacagaggccaggaatataattcccagaaacaataaaagtggaaatcatgatttgacagtggtcgctatgatttgtatttcactagttcgaactttagatgatgaaataaaagattaagttgaaggatatttatagtgatagaacgtaaagctagatgaataacgtggatggtcatttgggtaca

SEQ ID NO: 113 - DNA, 3400 bp, synthetic construct
  source 1..3400: mol_type = other DNA
gacacggtgagagtaacagaagatagtattaatgactaagtagaagaaatatttctgaccattgattggtgacgaaaactacccctataaagtttactcgcagttaaacatcgaaatatccattatttttttgtcatttactttttcattattattatataagtttaaacacttagaatcataaaaattattaaatctatctttaagcacaacaaacaaatctatctatggatagaataatattgtacctgttgactccaaatacacaacaataatatgaaaaatagaataataaattcaaatggttagaatatatttttacttagataccaaagttttaccatctttcttgtctttcttaagaactatctgaatcaattttgacctcaactattagaataagaaactttatccaaatctataaataaaagaaaacatttgaaattgggttaacaatttaggctcaatccttccaagtctcgaagtctcgattattacgcaactcctcttacatttcatcttttcctcatagaacatttacattaaaacaaagagtccaattaatattcagaacttcatattgtaaatctaacattgatataaccgtcatgaaaatatattttctagagagaaaagaaattgcacaacctcgtcttaactcacaaattacaaaacacttccaattttttaatttaaagaaaagatataaaaacataaacaaattaaagcaactaatacaagagtaaggcactgcatgttatgaaccattacaataataacacaaccaataaccattattaaaaacaattttaaaaattccttcattgaatccatagtctttttttaagacttaccccaagaacacaaattaatattatccttgtagttaaagtaaaaaaaaagcacaagttttattaattatttatttattcgtatagaaaagtggggctcaataggtaagagttacaagatccattatttactcttagctcacgaagagctagctagatcttagctcatacatctgcattatttttcatattgattactcagtaaaaactgtccagaactgaagacagaggactcctttttctttagctttcttcctccttttattcaggttcagcacttgcaaagtgagattatttttaattcttgattaatctatttacctcttaagaagatccaggaaatgtgagctcctttactggattttctatttagcttatcacattgtcatccgatctttcaaattttcaatccccaaattagaaatataacattcaaatattaactaatgatatttctattcacttaatatctgaaaggaagtttctctaattgttctcggcattgataccaaatccaaccaaattcagatttgatgaagcactaatggcaactgggtgacctgctggaatgataacaacgtcacccggagacaatctagcttcatatctctacacttcattgtttctttcttttctatcttccctctcttattactcattttttaaacccagaagttcaaggtttccttttccttcattaactaatagtacaactattgcccttgaattgtagtgtggcaacattagagctccttaaaaatttaagcaaaaacgcattaacatatttctgtaatataattaaaattatgtgttttatatatatttagtgttgtgtacatatcttgttaatctccacacaactaacaagtatatctaaatcttaaagctaagggtattttttctctggagtaatctcaaacaacttgccaaacttattagaatattctggcttgtggcttctcaagttgaaaggttcaaattcagagggtaagcttttctttgagcttgattttgcaagctttctcaattcctcaatttattcccttgatactttgattattgcgtctctttcttccccttattatgttcttttccgatctctcaattattatggttttttctcttactcttctaaaagaaccttctctatggtctcgtatttagtttatatttgcgaaaaaggatacaaaatataatggttatatttattaaacatttgataaaaaaatcacacattaagcttaacatgtgttgtttgcatacttatatttaaggaggcctctaaaatgttcttgctgaatcctcataagtattagtttttattttcagatagaccaaaagcttgtagaagaaggataaagatcaatttttcaatccagacaaaaataaaagtaatataaaggaggtgttttaataagaataaaacatgtgaagaaaattattatctcaaatttaccaggcctgttcacgggtattacaaaatccaccactcttagatcttcttcatcatcttagttaactagataagatgttgttcctgcgggaattttgatggtatcaccacgctcaagattatacgagtttctatcattgggactcaacactgtcaatatggctttccttgtagtacatattaaccacaccaaaatttaattatgaaatataagaaatattgctaaattgaactttacaatatttttattttaaatagtcatatttctataaaacaaaagatttgttataataatattataaagaaaaataaaaattatcattgaggactacaaggattaagtcagcatctatgtgttaaggaaggaagatggtgtggggtttggctctatattccacaagacgatagttttagagattttcaaataagtctgaacgtttgtcgaacctttaaaggcgacgaatgtgaccgttttcgttttcaaagagtgtcagaaacttgttagacttgaataaaaaggggtttctttattcttatgattctgaagatctttcttcctcctctccttcacgttaatggcgtctgtctctttttgttctctcctctctatgccttagccttgccctttcttcgggatcttcacgacgttaacttcctctttactcttcgtctacttattcctcatcttcctctctttcttatctctcacgtccaggttaaacttccttttattccttcttttcacgttaatatcgatatttctacttctcttcttcatcttcttccttttcatatgaaggtctttattctccatggcgtttttcttctttctcaccctcttagcgacctctttctctttatcccggtaccctagtttctgaaccttcatcgtaattggcataagtgacgcaaacagaggccaggaatataattcccagaaacaataaaagtggaaatcatgatttgacagtggtcgctatgatttgtatttcactagttcgaactttagatgatgaaataaaagattaagttgaaggatatttatagtgatagaacgtaaagctagatgaataacgtggatggtcatttgggtaca

SEQ ID NO: 114 - DNA, 3400 bp, synthetic construct
  source 1..3400: mol_type = other DNA
gacacggtgagagtaacagaagatagtattaatgactaagtagaagaaatatttctgaccattgattggtgacgaaaactacccctataaagtttactcgcagttaaacatcgaaatatccattatttttttgtcatttactttttcattattattatataagtttaaacacttagaatcataaaaattattaaatctatctttaagcacaacaaacaaatctatctatggatagaataatattgtacctgttgactccaaatacacaacaataatatgaaaaatagaataataaattcaaatggttagaatatatttttacttagataccaaagttttaccatctttcttgtctttcttaagaactatctgaatcaattttgacctcaactattagaataagaaactttatccaaatctataaataaaagaaaacatttgaaattgggttaacaatttaggctcaatccttccaagtctcgaagtctcgattattacgcaactcctcttacatttcatcttttcctcatagaacatttacattaaaacaaagagtccaattaatattcagaacttcatattgtaaatctaacattgatataaccgtcatgaaaatatattttctagagagaaaagaaattgcacaacctcgtcttaactcacaaattacaaaacacttccaattttttaatttaaagaaaagatataaaaacataaacaaattaaagcaactaatacaagagtaaggcactgcatgttatgaaccattacaataataacacaaccaataaccattattaaaaacaattttaaaaattccttcattgaatccatagtctttttttaagacttaccccaagaacacaaattaatattatccttgtagttaaagtaaaaaaaaagcacaagttttattaattatttatttattcgtatagaaaagtggggctcaataggtaagagttacaagatccattatttactcttagctcacgaagagctagctagatcttagctcatacatctgcattatttttcatattgattactcagtaaaaactgtccagaactgaagacagaggactcctttttctttagctttcttcctccttttattcaggttcagcacttgcaaagtgagattatttttaattcttgattaatctatttacctcttaagaagatccaggaaatgtgagctcctttactggattttctatttagcttatcacattgtcatccgatctttcaaattttcaatccccaaattagaaatataacattcaaatattaactaatgatatttctattcacttaatatctgaaaggaagtttctctaattgttctcggcattgataccaaatccaaccaaattcagatttgatgaagcactaatggcaactgggtgacctgctggaatgataacaacgtcacccggagacaatctagcttcatatctctacacttcattgtttctttcttttctatcttccctctcttattactcattttttaaacccagaagttcaaggtttccttttccttcattaactaatagtacaactattgcccttgaattgtagtgtggcaacattagagctccttaaaaatttaagcaaaaacgcattaacatatttctgtaatataattaaaattatgtgttttatatatatttagtgttgtgtacatatcttgttaatctccacacaactaacaagtatatctaaatcttaaagctaagggtattttttctctggagtaatctcaaacaacttgccaaacttattagaatattctggcttgtggcttctcaagttgaaaggttcaaattcagagggtaagcttttctttgagcttgattttgcaagctttctcaattcctcaatttattcccttgatactttgattattgcgtctctttcttccccttattatgttcttttccgatctctcaattattatggttttttctcttactcttctaaaagaaccttctctatggtctcgtatttagtttatatttgcgaaaaaggatacaaaatataatggttatatttattaaacatttgataaaaaaatcacacattaagcttaacatgtgttgtttgcatacttatatttaaggaggcctctaaaatgttcttgctgaatcctcataagtattagtttttattttcagatagaccaaaagcttgtagaagaaggataaagatcaatttttcaatccagacaaaaataaaagtaatataaaggaggtgttttaataagaataaaacatgtgaagaaaattattatctcaaatttaccaggcctgttcacgggtattacaaaatccaccactcttagatcttcttcatcatcttagttaactagataagatgttgttcctgcgggaattttgatggtatcaccacgctcaagattatacgagtttctatcattgggactcaacactgtcaatatggctttccttgtagtacatattaaccacaccaaaatttaattatgaaatataagaaatattgctaaattgaactttacaatatttttattttaaatagtcatatttctataaaacaaaagatttgttataataatattataaagaaaaataaaaattatcattgaggactacaaggattaagtcagcatctatgtgttaaggaaggaagatggtgtggggtttggctctatattccacaagacgatagttttagagattttcaaataagtctgaacgtttgtcgaacctttaaaggcgacgaatgtgaccgttttcgttttcaaagagtgtcagaaacttgttagacttgaataaaaaggggtttctttattcttatgattctgaagatctttcttcctcctctccttcacgttaatggcgtctgtctctttttgttctctcctctctatgccttagccttgccctttcttcgggatcttcacgacgttaacttcctctttactcttcgtctacttattcctcatcttcctctctttcttatctctcacgtccaggttaaacttccttttattccttcttttcacgttaatatcaatatttctgcttctcttcttcatcttcttccttttcatatgaaggtctttattctccatggcgtttttcttctttctcaccctcttagcgacctctttctctttatcccggtaccctagtttctgaaccttcatcgtaattggcataagtgacgcaaacagaggccaggaatataattcccagaaacaataaaagtggaaatcatgatttgacagtggtcgctatgatttgtatttcactagttcgaactttagatgatgaaataaaagattaagttgaaggatatttatagtgatagaacgtaaagctagatgaataacgtggatggtcatttgggtaca

SEQ ID NO: 115 - DNA, 3400 bp, synthetic construct
  source 1..3400: mol_type = other DNA
gacacggtgagagtaacagaagatagtattaatgactaagtagaagaaatatttctgaccattgattggtgacgaaaactacccctataaagtttactcgcagttaaacatcgaaatatccattatttttttgtcatttactttttcattattattatataagtttaaacacttagaatcataaaaattattaaatctatctttaagcacaacaaacaaatctatctatggatagaataatattgtacctgttgactccaaatacacaacaataatatgaaaaatagaataataaattcaaatggttagaatatatttttacttagataccaaagttttaccatctttcttgtctttcttaagaactatctgaatcaattttgacctcaactattagaataagaaactttatccaaatctataaataaaagaaaacatttgaaattgggttaacaatttaggctcaatccttccaagtctcgaagtctcgattattacgcaactcctcttacatttcatcttttcctcatagaacatttacattaaaacaaagagtccaattaatattcagaacttcatattgtaaatctaacattgatataaccgtcatgaaaatatattttctagagagaaaagaaattgcacaacctcgtcttaactcacaaattacaaaacacttccaattttttaatttaaagaaaagatataaaaacataaacaaattaaagcaactaatacaagagtaaggcactgcatgttatgaaccattacaataataacacaaccaataaccattattaaaaacaattttaaaaattccttcattgaatccatagtctttttttaagacttaccccaagaacacaaattaatattatccttgtagttaaagtaaaaaaaaagcacaagttttattaattatttatttattcgtatagaaaagtggggctcaataggtaagagttacaagatccattatttactcttagctcacgaagagctagctagatcttagctcatacatctgcattatttttcatattgattactcagtaaaaactgtccagaactgaagacagaggactcctttttctttagctttcttcctccttttattcaggttcagcacttgcaaagtgagattatttttaattcttgattaatctatttacctcttaagaagatccaggaaatgtgagctcctttactggattttctatttagcttatcacattgtcatccgatctttcaaattttcaatccccaaattagaaatataacattcaaatattaactaatgatatttctattcacttaatatctgaaaggaagtttctctaattgttctcggcattgataccaaatccaaccaaattcagatttgatgaagcactaatggcaactgggtgacctgctggaatgataacaacgtcacccggagacaatctagcttcatatctctacacttcattgtttctttcttttctatcttccctctcttattactcattttttaaacccagaagttcaaggtttccttttccttcattaactaatagtacaactattgcccttgaattgtagtgtggcaacattagagctccttaaaaatttaagcaaaaacgcattaacatatttctgtaatataattaaaattatgtgttttatatatatttagtgttgtgtacatatcttgttaatctccacacaactaacaagtatatctaaatcttaaagctaagggtattttttctctggagtaatctcaaacaacttgccaaacttattagaatattctggcttgtggcttctcaagttgaaaggttcaaattcagagggtaagcttttctttgagcttgattttgcaagctttctcaattcctcaatttattcccttgatactttgattattgcgtctctttcttccccttattatgttcttttccgatctctcaattattatggttttttctcttactcttctaaaagaaccttctctatggtctcgtatttagtttatatttgcgaaaaaggatacaaaatataatggttatatttattaaacatttgataaaaaaatcacacattaagcttaacatgtgttgtttgcatacttatatttaaggaggcctctaaaatgttcttgctgaatcctcataagtattagtttttattttcagatagaccaaaagcttgtagaagaaggataaagatcaatttttcaatccagacaaaaataaaagtaatataaaggaggtgttttaataagaataaaacatgtgaagaaaattattatctcaaatttaccaggcctgttcacgggtattacaaaatccaccactcttagatcttcttcatcatcttagttaactagataagatgttgttcctgcgggaattttgatggtatcaccacgctcaagattatacgagtttctatcattgggactcaacactgtcaatatggctttccttgtagtacatattaaccacaccaaaatttaattatgaaatataagaaatattgctaaattgaactttacaatatttttattttaaatagtcatatttctataaaacaaaagatttgttataataatattataaagaaaaataaaaattatcattgaggactacaaggattaagtcagcatctatgtgttaaggaaggaagatggtgtggggtttggctctatattccacaagacgatagttttagagattttcaaataagtctgaacgtttgtcgaacctttaaaggcgacgaatgtgaccgttttcgttttcaaagagtgtcagaaacttgttagacttgaataaaaaggggtttctttattcttatgattctgaagatctttcttcctcctctccttcacgttaatggcgtctgtctctttttgttctctcctctctatgccttagccttgccctttcttcgggatcttcacgacgttaacttcctctttactcttcgtctacttattcctcatcttcctctctttcttatctctcacgtccaggttaaacttccttttattccttcttttcacgttaatatcaatatttctacttctcttcttcatcttcttccttttcatatgaaggtctctattctccatggcgtttttcttctttctcaccctcttagcgacctctttctctttatcccggtaccctagtttctgaaccttcatcgtaattggcataagtgacgcaaacagaggccaggaatataattcccagaaacaataaaagtggaaatcatgatttgacagtggtcgctatgatttgtatttcactagttcgaactttagatgatgaaataaaagattaagttgaaggatatttatagtgatagaacgtaaagctagatgaataacgtggatggtcatttgggtaca

SEQ ID NO: 116 - DNA, 3400 bp, synthetic construct
  source 1..3400: mol_type = other DNA
gacacggtgagagtaacagaagatagtattaatgactaagtagaagaaatatttctgaccattgattggtgacgaaaactacccctataaagtttactcgcagttaaacatcgaaatatccattatttttttgtcatttactttttcattattattatataagtttaaacacttagaatcataaaaattattaaatctatctttaagcacaacaaacaaatctatctatggatagaataatattgtacctgttgactccaaatacacaacaataatatgaaaaatagaataataaattcaaatggttagaatatatttttacttagataccaaagttttaccatctttcttgtctttcttaagaactatctgaatcaattttgacctcaactattagaataagaaactttatccaaatctataaataaaagaaaacatttgaaattgggttaacaatttaggctcaatccttccaagtctcgaagtctcgattattacgcaactcctcttacatttcatcttttcctcatagaacatttacattaaaacaaagagtccaattaatattcagaacttcatattgtaaatctaacattgatataaccgtcatgaaaatatattttctagagagaaaagaaattgcacaacctcgtcttaactcacaaattacaaaacacttccaattttttaatttaaagaaaagatataaaaacataaacaaattaaagcaactaatacaagagtaaggcactgcatgttatgaaccattacaataataacacaaccaataaccattattaaaaacaattttaaaaattccttcattgaatccatagtctttttttaagacttaccccaagaacacaaattaatattatccttgtagttaaagtaaaaaaaaagcacaagttttattaattatttatttattcgtatagaaaagtggggctcaataggtaagagttacaagatccattatttactcttagctcacgaagagctagctagatcttagctcatacatctgcattatttttcatattgattactcagtaaaaactgtccagaactgaagacagaggactcctttttctttagctttcttcctccttttattcaggttcagcacttgcaaagtgagattatttttaattcttgattaatctatttacctcttaagaagatccaggaaatgtgagctcctttactggattttctatttagcttatcacattgtcatccgatctttcaaattttcaatccccaaattagaaatataacattcaaatattaactaatgatatttctattcacttaatatctgaaaggaagtttctctaattgttctcggcattgataccaaatccaaccaaattcagatttgatgaagcactaatggcaactgggtgacctgctggaatgataacaacgtcacccggagacaatctagcttcatatctctacacttcattgtttctttcttttctatcttccctctcttattactcattttttaaacccagaagttcaaggtttccttttccttcattaactaatagtacaactattgcccttgaattgtagtgtggcaacattagagctccttaaaaatttaagcaaaaacgcattaacatatttctgtaatataattaaaattatgtgttttatatatatttagtgttgtgtacatatcttgttaatctccacacaactaacaagtatatctaaatcttaaagctaagggtattttttctctggagtaatctcaaacaacttgccaaacttattagaatattctggcttgtggcttctcaagttgaaaggttcaaattcagagggtaagcttttctttgagcttgattttgcaagctttctcaattcctcaatttattcccttgatactttgattattgcgtctctttcttccccttattatgttcttttccgatctctcaattattatggttttttctcttactcttctaaaagaaccttctctatggtctcgtatttagtttatatttgcgaaaaaggatacaaaatataatggttatatttattaaacatttgataaaaaaatcacacattaagcttaacatgtgttgtttgcatacttatatttaaggaggcctctaaaatgttcttgctgaatcctcataagtattagtttttattttcagatagaccaaaagcttgtagaagaaggataaagatcaatttttcaatccagacaaaaataaaagtaatataaaggaggtgttttaataagaataaaacatgtgaagaaaattattatctcaaatttaccaggcctgttcacgggtattacaaaatccaccactcttagatcttcttcatcatcttagttaactagataagatgttgttcctgcgggaattttgatggtatcaccacgctcaagattatacgagtttctatcattgggactcaacactgtcaatatggctttccttgtagtacatattaaccacaccaaaatttaattatgaaatataagaaatattgctaaattgaactttacaatatttttattttaaatagtcatatttctataaaacaaaagatttgttataataatattataaagaaaaataaaaattatcattgaggactacaaggattaagtcagcatctatgtgttaaggaaggaagatggtgtggggtttggctctatattccacaagacgatagttttagagattttcaaataagtctgaacgtttgtcgaacctttaaaggcgacgaatgtgaccgttttcgttttcaaagagtgtcagaaacttgttagacttgaataaaaaggggtttctttattcttatgattctgaagatctttcttcctcctctccttcacgttaatggcgtctgtctctttttgttctctcctctctatgccttagccttgccctttcttcgggatcttcacgacgttaacttcctctttactcttcgtctacttattcctcatcttcctctctttcttatctctcacgtccaggttaaacttccttttattccttcttttcacgttaatatcaatatttctacttctcttcttcatcttcttccttttcatatgaaggtcttcattctccatggcgtttttcttctttctcaccctcttagcgacctctttctctttatcccggtaccctagtttctgaaccttcatcgtaattggcataagtgacgcaaacagaggccaggaatataattcccagaaacaataaaagtggaaatcatgatttgacagtggtcgctatgatttgtatttcactagttcgaactttagatgatgaaataaaagattaagttgaaggatatttatagtgatagaacgtaaagctagatgaataacgtggatggtcatttgggtaca

SEQ ID NO: 117 - DNA, 3400 bp, synthetic construct
  source 1..3400: mol_type = other DNA
gacacggtgagagtaacagaagatagtattaatgactaagtagaagaaatatttctgaccattgattggtgacgaaaactacccctataaagtttactcgcagttaaacatcgaaatatccattatttttttgtcatttactttttcattattattatataagtttaaacacttagaatcataaaaattattaaatctatctttaagcacaacaaacaaatctatctatggatagaataatattgtacctgttgactccaaatacacaacaataatatgaaaaatagaataataaattcaaatggttagaatatatttttacttagataccaaagttttaccatctttcttgtctttcttaagaactatctgaatcaattttgacctcaactattagaataagaaactttatccaaatctataaataaaagaaaacatttgaaattgggttaacaatttaggctcaatccttccaagtctcgaagtctcgattattacgcaactcctcttacatttcatcttttcctcatagaacatttacattaaaacaaagagtccaattaatattcagaacttcatattgtaaatctaacattgatataaccgtcatgaaaatatattttctagagagaaaagaaattgcacaacctcgtcttaactcacaaattacaaaacacttccaattttttaatttaaagaaaagatataaaaacataaacaaattaaagcaactaatacaagagtaaggcactgcatgttatgaaccattacaataataacacaaccaataaccattattaaaaacaattttaaaaattccttcattgaatccatagtctttttttaagacttaccccaagaacacaaattaatattatccttgtagttaaagtaaaaaaaaagcacaagttttattaattatttatttattcgtatagaaaagtggggctcaataggtaagagttacaagatccattatttactcttagctcacgaagagctagctagatcttagctcatacatctgcattatttttcatattgattactcagtaaaaactgtccagaactgaagacagaggactcctttttctttagctttcttcctccttttattcaggttcagcacttgcaaagtgagattatttttaattcttgattaatctatttacctcttaagaagatccaggaaatgtgagctcctttactggattttctatttagcttatcacattgtcatccgatctttcaaattttcaatccccaaattagaaatataacattcaaatattaactaatgatatttctattcacttaatatctgaaaggaagtttctctaattgttctcggcattgataccaaatccaaccaaattcagatttgatgaagcactaatggcaactgggtgacctgctggaatgataacaacgtcacccggagacaatctagcttcatatctctacacttcattgtttctttcttttctatcttccctctcttattactcattttttaaacccagaagttcaaggtttccttttccttcattaactaatagtacaactattgcccttgaattgtagtgtggcaacattagagctccttaaaaatttaagcaaaaacgcattaacatatttctgtaatataattaaaattatgtgttttatatatatttagtgttgtgtacatatcttgttaatctccacacaactaacaagtatatctaaatcttaaagctaagggtattttttctctggagtaatctcaaacaacttgccaaacttattagaatattctggcttgtggcttctcaagttgaaaggttcaaattcagagggtaagcttttctttgagcttgattttgcaagctttctcaattcctcaatttattcccttgatactttgattattgcgtctctttcttccccttattatgttcttttccgatctctcaattattatggttttttctcttactcttctaaaagaaccttctctatggtctcgtatttagtttatatttgcgaaaaaggatacaaaatataatggttatatttattaaacatttgataaaaaaatcacacattaagcttaacatgtgttgtttgcatacttatatttaaggaggcctctaaaatgttcttgctgaatcctcataagtattagtttttattttcagatagaccaaaagcttgtagaagaaggataaagatcaatttttcaatccagacaaaaataaaagtaatataaaggaggtgttttaataagaataaaacatgtgaagaaaattattatctcaaatttaccaggcctgttcacgggtattacaaaatccaccactcttagatcttcttcatcatcttagttaactagataagatgttgttcctgcgggaattttgatggtatcaccacgctcaagattatacgagtttctatcattgggactcaacactgtcaatatggctttccttgtagtacatattaaccacaccaaaatttaattatgaaatataagaaatattgctaaattgaactttacaatatttttattttaaatagtcatatttctataaaacaaaagatttgttataataatattataaagaaaaataaaaattatcattgaggactacaaggattaagtcagcatctatgtgttaaggaaggaagatggtgtggggtttggctctatattccacaagacgatagttttagagattttcaaataagtctgaacgtttgtcgaacctttaaaggcgacgaatgtgaccgttttcgttttcaaagagtgtcagaaacttgttagacttgaataaaaaggggtttctttattcttatgattctgaagatctttcttcctcctctccttcacgttaatggcgtctgtctctttttgttctctcctctctatgccttagccttgccctttcttcgggatcttcacgacgttaacttcctctttactcttcgtctacttattcctcatcttcctctctttcttatctctcacgtccaggttaaacttccttttattccttcttttcacgttaatatcaatatttctacttctcttcttcatcttcttccttttcatatgaaggtctttattctccatggcgtttttcttctttctcaccctcttggcgacctctttctctttatcccggtaccctagtttctgaaccttcatcgtaattggcataagtgacgcaaacagaggccaggaatataattcccagaaacaataaaagtggaaatcatgatttgacagtggtcgctatgatttgtatttcactagttcgaactttagatgatgaaataaaagattaagttgaaggatatttatagtgatagaacgtaaagctagatgaataacgtggatggtcatttgggtaca

SEQ ID NO: 118 - DNA, 3400 bp, synthetic construct
  source 1..3400: mol_type = other DNA
gacacggtgagagtaacagaagatagtattaatgactaagtagaagaaatatttctgaccattgattggtgacgaaaactacccctataaagtttactcgcagttaaacatcgaaatatccattatttttttgtcatttactttttcattattattatataagtttaaacacttagaatcataaaaattattaaatctatctttaagcacaacaaacaaatctatctatggatagaataatattgtacctgttgactccaaatacacaacaataatatgaaaaatagaataataaattcaaatggttagaatatatttttacttagataccaaagttttaccatctttcttgtctttcttaagaactatctgaatcaattttgacctcaactattagaataagaaactttatccaaatctataaataaaagaaaacatttgaaattgggttaacaatttaggctcaatccttccaagtctcgaagtctcgattattacgcaactcctcttacatttcatcttttcctcatagaacatttacattaaaacaaagagtccaattaatattcagaacttcatattgtaaatctaacattgatataaccgtcatgaaaatatattttctagagagaaaagaaattgcacaacctcgtcttaactcacaaattacaaaacacttccaattttttaatttaaagaaaagatataaaaacataaacaaattaaagcaactaatacaagagtaaggcactgcatgttatgaaccattacaataataacacaaccaataaccattattaaaaacaattttaaaaattccttcattgaatccatagtctttttttaagacttaccccaagaacacaaattaatattatccttgtagttaaagtaaaaaaaaagcacaagttttattaattatttatttattcgtatagaaaagtggggctcaataggtaagagttacaagatccattatttactcttagctcacgaagagctagctagatcttagctcatacatctgcattatttttcatattgattactcagtaaaaactgtccagaactgaagacagaggactcctttttctttagctttcttcctccttttattcaggttcagcacttgcaaagtgagattatttttaattcttgattaatctatttacctcttaagaagatccaggaaatgtgagctcctttactggattttctatttagcttatcacattgtcatccgatctttcaaattttcaatccccaaattagaaatataacattcaaatattaactaatgatatttctattcacttaatatctgaaaggaagtttctctaattgttctcggcattgataccaaatccaaccaaattcagatttgatgaagcactaatggcaactgggtgacctgctggaatgataacaacgtcacccggagacaatctagcttcatatctctacacttcattgtttctttcttttctatcttccctctcttattactcattttttaaacccagaagttcaaggtttccttttccttcattaactaatagtacaactattgcccttgaattgtagtgtggcaacattagagctccttaaaaatttaagcaaaaacgcattaacatatttctgtaatataattaaaattatgtgttttatatatatttagtgttgtgtacatatcttgttaatctccacacaactaacaagtatatctaaatcttaaagctaagggtattttttctctggagtaatctcaaacaacttgccaaacttattagaatattctggcttgtggcttctcaagttgaaaggttcaaattcagagggtaagcttttctttgagcttgattttgcaagctttctcaattcctcaatttattcccttgatactttgattattgcgtctctttcttccccttattatgttcttttccgatctctcaattattatggttttttctcttactcttctaaaagaaccttctctatggtctcgtatttagtttatatttgcgaaaaaggatacaaaatataatggttatatttattaaacatttgataaaaaaatcacacattaagcttaacatgtgttgtttgcatacttatatttaaggaggcctctaaaatgttcttgctgaatcctcataagtattagtttttattttcagatagaccaaaagcttgtagaagaaggataaagatcaatttttcaatccagacaaaaataaaagtaatataaaggaggtgttttaataagaataaaacatgtgaagaaaattattatctcaaatttaccaggcctgttcacgggtattacaaaatccaccactcttagatcttcttcatcatcttagttaactagataagatgttgttcctgcgggaattttgatggtatcaccacgctcaagattatacgagtttctatcattgggactcaacactgtcaatatggctttccttgtagtacatattaaccacaccaaaatttaattatgaaatataagaaatattgctaaattgaactttacaatatttttattttaaatagtcatatttctataaaacaaaagatttgttataataatattataaagaaaaataaaaattatcattgaggactacaaggattaagtcagcatctatgtgttaaggaaggaagatggtgtggggtttggctctatattccacaagacgatagttttagagattttcaaataagtctgaacgtttgtcgaacctttaaaggcgacgaatgtgaccgttttcgttttcaaagagtgtcagaaacttgttagacttgaataaaaaggggtttctttattcttatgattctgaagatctttcttcctcctctccttcacgttaatggcgtctgtctctttttgttctctcctctctatgccttagccttgccctttcttcgggatcttcacgacgttaacttcctctttactcttcgtctacttattcctcatcttcctctctttcttatctctcacgtccaggttaaacttccttttattccttcttttcacgttaatatcaatatttctacttctcttcttcatcttcttccttttcatatgaaggtctttattctccatggcgtttttcttctttctcaccctcttagcgacctctttctctttgtcccggtaccctagtttctgaaccttcatcgtaattggcataagtgacgcaaacagaggccaggaatataattcccagaaacaataaaagtggaaatcatgatttgacagtggtcgctatgatttgtatttcactagttcgaactttagatgatgaaataaaagattaagttgaaggatatttatagtgatagaacgtaaagctagatgaataacgtggatggtcatttgggtaca

SEQ ID NO: 119 - DNA, 3400 bp, synthetic construct
  source 1..3400: mol_type = other DNA
gacacggtgagagtaacagaagatagtattaatgactaagtagaagaaatatttctgaccattgattggtgacgaaaactacccctataaagtttactcgcagttaaacatcgaaatatccattatttttttgtcatttactttttcattattattatataagtttaaacacttagaatcataaaaattattaaatctatctttaagcacaacaaacaaatctatctatggatagaataatattgtacctgttgactccaaatacacaacaataatatgaaaaatagaataataaattcaaatggttagaatatatttttacttagataccaaagttttaccatctttcttgtctttcttaagaactatctgaatcaattttgacctcaactattagaataagaaactttatccaaatctataaataaaagaaaacatttgaaattgggttaacaatttaggctcaatccttccaagtctcgaagtctcgattattacgcaactcctcttacatttcatcttttcctcatagaacatttacattaaaacaaagagtccaattaatattcagaacttcatattgtaaatctaacattgatataaccgtcatgaaaatatattttctagagagaaaagaaattgcacaacctcgtcttaactcacaaattacaaaacacttccaattttttaatttaaagaaaagatataaaaacataaacaaattaaagcaactaatacaagagtaaggcactgcatgttatgaaccattacaataataacacaaccaataaccattattaaaaacaattttaaaaattccttcattgaatccatagtctttttttaagacttaccccaagaacacaaattaatattatccttgtagttaaagtaaaaaaaaagcacaagttttattaattatttatttattcgtatagaaaagtggggctcaataggtaagagttacaagatccattatttactcttagctcacgaagagctagctagatcttagctcatacatctgcattatttttcatattgattactcagtaaaaactgtccagaactgaagacagaggactcctttttctttagctttcttcctccttttattcaggttcagcacttgcaaagtgagattatttttaattcttgattaatctatttacctcttaagaagatccaggaaatgtgagctcctttactggattttctatttagcttatcacattgtcatccgatctttcaaattttcaatccccaaattagaaatataacattcaaatattaactaatgatatttctattcacttaatatctgaaaggaagtttctctaattgttctcggcattgataccaaatccaaccaaattcagatttgatgaagcactaatggcaactgggtgacctgctggaatgataacaacgtcacccggagacaatctagcttcatatctctacacttcattgtttctttcttttctatcttccctctcttattactcattttttaaacccagaagttcaaggtttccttttccttcattaactaatagtacaactattgcccttgaattgtagtgtggcaacattagagctccttaaaaatttaagcaaaaacgcattaacatatttctgtaatataattaaaattatgtgttttatatatatttagtgttgtgtacatatcttgttaatctccacacaactaacaagtatatctaaatcttaaagctaagggtattttttctctggagtaatctcaaacaacttgccaaacttattagaatattctggcttgtggcttctcaagttgaaaggttcaaattcagagggtaagcttttctttgagcttgattttgcaagctttctcaattcctcaatttattcccttgatactttgattattgcgtctctttcttccccttattatgttcttttccgatctctcaattattatggttttttctcttactcttctaaaagaaccttctctatggtctcgtatttagtttatatttgcgaaaaaggatacaaaatataatggttatatttattaaacatttgataaaaaaatcacacattaagcttaacatgtgttgtttgcatacttatatttaaggaggcctctaaaatgttcttgctgaatcctcataagtattagtttttattttcagatagaccaaaagcttgtagaagaaggataaagatcaatttttcaatccagacaaaaataaaagtaatataaaggaggtgttttaataagaataaaacatgtgaagaaaattattatctcaaatttaccaggcctgttcacgggtattacaaaatccaccactcttagatcttcttcatcatcttagttaactagataagatgttgttcctgcgggaattttgatggtatcaccacgctcaagattatacgagtttctatcattgggactcaacactgtcaatatggctttccttgtagtacatattaaccacaccaaaatttaattatgaaatataagaaatattgctaaattgaactttacaatatttttattttaaatagtcatatttctataaaacaaaagatttgttataataatattataaagaaaaataaaaattatcattgaggactacaaggattaagtcagcatctatgtgttaaggaaggaagatggtgtggggtttggctctatattccacaagacgatagttttagagattttcaaataagtctgaacgtttgtcgaacctttaaaggcgacgaatgtgaccgttttcgttttcaaagagtgtcagaaacttgttagacttgaataaaaaggggtttctttattcttatgattctgaagatctttcttcctcctctccttcacgttaatggcgtctgtctctttttgttctctcctctctatgccttagccttgccctttcttcgggatcttcacgacgttaacttcctctttactcttcgtctacttattcctcatcttcctctctttcttatctctcacgtccaggttaaacttccttttattccttcttttcacgttaatatcaatatttctacttctcttcttcatcttcttccttttcatatgaaggtctttattctccatggcgtttttcttctttctcaccctcttagcgacctctttctctttatcccggtaccctagtttctgaaccttcatcgtaattggcataagtgacgcaaacagaggccaggaatataattcccagaaacaataaaagtggaaatcgtgatttgacagtggtcgctatgatttgtatttcactagttcgaactttagatgatgaaataaaagattaagttgaaggatatttatagtgatagaacgtaaagctagatgaataacgtggatggtcatttgggtaca

SEQ ID NO: 120 - DNA, 3400 bp, synthetic construct
  source 1..3400: mol_type = other DNA
gacacggtgagagtaacagaagatagtattaatgactaagtagaagaaatatttctgaccattgattggtgacgaaaactacccctataaagtttactcgcagttaaacatcgaaatatccattatttttttgtcatttactttttcattattattatataagtttaaacacttagaatcataaaaattattaaatctatctttaagcacaacaaacaaatctatctatggatagaataatattgtacctgttgactccaaatacacaacaataatatgaaaaatagaataataaattcaaatggttagaatatatttttacttagataccaaagttttaccatctttcttgtctttcttaagaactatctgaatcaattttgacctcaactattagaataagaaactttatccaaatctataaataaaagaaaacatttgaaattgggttaacaatttaggctcaatccttccaagtctcgaagtctcgattattacgcaactcctcttacatttcatcttttcctcatagaacatttacattaaaacaaagagtccaattaatattcagaacttcatattgtaaatctaacattgatataaccgtcatgaaaatatattttctagagagaaaagaaattgcacaacctcgtcttaactcacaaattacaaaacacttccaattttttaatttaaagaaaagatataaaaacataaacaaattaaagcaactaatacaagagtaaggcactgcatgttatgaaccattacaataataacacaaccaataaccattattaaaaacaattttaaaaattccttcattgaatccatagtctttttttaagacttaccccaagaacacaaattaatattatccttgtagttaaagtaaaaaaaaagcacaagttttattaattatttatttattcgtatagaaaagtggggctcaataggtaagagttacaagatccattatttactcttagctcacgaagagctagctagatcttagctcatacatctgcattatttttcatattgattactcagtaaaaactgtccagaactgaagacagaggactcctttttctttagctttcttcctccttttattcaggttcagcacttgcaaagtgagattatttttaattcttgattaatctatttacctcttaagaagatccaggaaatgtgagctcctttactggattttctatttagcttatcacattgtcatccgatctttcaaattttcaatccccaaattagaaatataacattcaaatattaactaatgatatttctattcacttaatatctgaaaggaagtttctctaattgttctcggcattgataccaaatccaaccaaattcagatttgatgaagcactaatggcaactgggtgacctgctggaatgataacaacgtcacccggagacaatctagcttcatatctctacacttcattgtttctttcttttctatcttccctctcttattactcattttttaaacccagaagttcaaggtttccttttccttcattaactaatagtacaactattgcccttgaattgtagtgtggcaacattagagctccttaaaaatttaagcaaaaacgcattaacatatttctgtaatataattaaaattatgtgttttatatatatttagtgttgtgtacatatcttgttaatctccacacaactaacaagtatatctaaatcttaaagctaagggtattttttctctggagtaatctcaaacaacttgccaaacttattagaatattctggcttgtggcttctcaagttgaaaggttcaaattcagagggtaagcttttctttgagcttgattttgcaagctttctcaattcctcaatttattcccttgatactttgattattgcgtctctttcttccccttattatgttcttttccgatctctcaattattatggttttttctcttactcttctaaaagaaccttctctatggtctcgtatttagtttatatttgcgaaaaaggatacaaaatataatggttatatttattaaacatttgataaaaaaatcacacattaagcttaacatgtgttgtttgcatacttatatttaaggaggcctctaaaatgttcttgctgaatcctcataagtattagtttttattttcagatagaccaaaagcttgtagaagaaggataaagatcaatttttcaatccagacaaaaataaaagtaatataaaggaggtgttttaataagaataaaacatgtgaagaaaattattatctcaaatttaccaggcctgttcacgggtattacaaaatccaccactcttagatcttcttcatcatcttagttaactagataagatgttgttcctgcgggaattttgatggtatcaccacgctcaagattatacgagtttctatcattgggactcaacactgtcaatatggctttccttgtagtacatattaaccacaccaaaatttaattatgaaatataagaaatattgctaaattgaactttacaatatttttattttaaatagtcatatttctataaaacaaaagatttgttataataatattataaagaaaaataaaaattatcattgaggactacaaggattaagtcagcatctatgtgttaaggaaggaagatggtgtggggtttggctctatattccacaagacgatagttttagagattttcaaataagtctgaacgtttgtcgaacctttaaaggcgacgaatgtgaccgttttcgttttcaaagagtgtcagaaacttgttagacttgaataaaaaggggtttctttattcttatgattctgaagatctttcttcctcctctccttcacgttaatggcgtctgtctctttttgttctctcctctctatgccttagccttgccctttcttcgggatcttcacgacgttaacttcctctttactcttcgtctacttattcctcatcttcctctctttcttatctctcacgtccaggttaaacttccttttattccttcttttcacgttaatatcaatatttctacttctcttcttcatcttcttccttttcatatgaaggtctttattctccatggcgtttttcttctttctcaccctcttagcgacctctttctctttatcccggtaccctagtttctgaaccttcatcgtaattggcataagtgacgcaaacagaggccaggaatataattcccagaaacaataaaagtggaaatcatgatttgacagtggtcgccatgatttgtatttcactagttcgaactttagatgatgaaataaaagattaagttgaaggatatttatagtgatagaacgtaaagctagatgaataacgtggatggtcatttgggtaca

SEQ ID NO: 121 - protein, 613 aa, Pisum sativum
MATTIKSRFPLLLLLGIIFLASVVCVTYANYDEGSEPRVPAQRERGRQEGEKEEKRHGEWRPSYEKEEDEEEGQRERGRQEGEKEEKRHGEWRPSYEKQEDEEEKQKYRYQREKEDEEEKQKYQYQREKKEQKEVQPGRERWEREEDEEQVDEEWRGSQRREDPEERARLRHREERTKRDRRHQREGEEEERSSESQERRNPFLFKSNKFLTLFENENGHIRLLQRFDKRSDLFENLQNYRLVEYRAKPHTIFLPQHIDADLILVVLSGKAILTVLSPNDRNSYNLERGDTIKLPAGTTSYLVNQDDEEDLRLVDLVIPVNGPGKFEAFDLAKNKNQYLRGFSKNILEASYNTRYETIEKVLLEEQEKDRKRRQQGEETDAIVKVSREQIEELKKLAKSSSKKSLPSEFEPINLRSHKPEYSNKFGKLFEITPEKKYPQLQDLDLFVSCVEINEGALMLPHYNSRAIVVLLVNEGKGNLELLGLKNEQQEREDRKERNNEVQRYEARLSPGDVVIIPAGHPVAITASSNLNLLGFGINAENNERNFLSGSDDNVISQIENPVKELTFPGSVQEINRLIKNQKQSHFANAEPEQKEQGSQGKRSPLSSILGTFY

SEQ ID NO: 122 - protein, 571 aa, Pisum sativum
MATTVKSRFPLLLFLGIIFLASVCVTYANYDEGSETRVPGQRERGRQEGEKEEKRHGEWRPSYEKEEDEEEKQKYRYQREKKEQKEVQPGRERWEREEDEEQVDEEWRGSQRREDPEERARLRHREERTKRDRRHQREGEEEERSSESQEQRNPFLFKSNKFLTLFENENGHIRRLQRFDKRSDLFENLQNYRLVEYRAKPHTIFLPQHIDADLILVVLNGKAILTVLSPNDRNSYNLERGDTIKIPAGTTSYLVNQDDEEDLRVVDFVIPVNRPGKFEAFGLSENKNQYLRGFSKNILEASLNTKYETIEKVLLEEQEKKPQQLRDRKRTQQGEERDAIIKVSREQIEELRKLAKSSSKKSLPSEFEPFNLRSHKPEYSNKFGKLFEITPEKKYPQLQDLDILVSCVEINKGALMLPHYNSRAIVVLLVNEGKGNLELLGLKNEQQEREDRKERNNEVQRYEARLSPGDVVIIPAGHPVAISASSNLNLVGFGINAENNQRNFLSGSDDNVISQIENPVKELTFPGSSQEVNRLIKNQKQSHFASAEPEQKEEESQRKRSPLSSVLDSFY

SEQ ID NO: 123 - protein, 459 aa, Pisum sativum
MAATTMKASFPLLMLMGISFLASVCVSSRSDPQNPFIFKSNKFQTLFENENGHIRLLQKFDQRSKIFENLQNYRLLEYKSKPHTIFLPQHTDADYILVVLSGKAILTVLKPDDRNSFNLERGDTIKLPAGTIAYLVNRDDNEELRVLDLAIPVNRPGQLQSFLLSGNQNQQNYLSGFSKNILEASFNTDYEEIEKVLLEEHEKETQHRRSLKDKRQQSQEENVIVKLSRGQIEELSKNAKSTSKKSVSSESEPFNLRSRGPIYSNEFGKFFEITPEKNPQLQDLDIFVNSVEIKEGSLLLPHYNSRAIVIVTVNEGKGDFELVGQRNENQQEQRKEDDEEEEQGEEEINKQVQNYKAKLSSGDVFVIPAGHPVAVKASSNLDLLGFGINAENNQRNFLAGDEDNVISQIQRPVKELAFPGSAQEVDRILENQKQSHFADAQPQQRERGSRETRDRLSSV